European Patent Specification EP 3 690 063 B1, published August 20, 2025. Title: Diagnosis of lung cancer. Applicant: AIT Austrian Institute of Technology GmbH. The sequence listing filed with the application follows.

SEQUENCE LISTING (321 sequences)

SEQ ID NO: 1 - DNA, 105 bp, Artificial Sequence
  subsequence of PAX9
cagcgggtcgctgactacctcgccctagcactcggtccgcgccccgggaaggcttcagcatcaccctcttctgctgggatcccgctgaccctgtctgcagcttcg

SEQ ID NO: 2 - DNA, 98 bp, Artificial Sequence
  subsequence of HOXD10
cctggagaggcggacaggagggcggcggagagcgctgggccggttgtctccagcgcgcactatcgcgggcgcgtagtagatgtcgctgttgtccgtgc

SEQ ID NO: 3 - DNA, 104 bp, Artificial Sequence
  subsequence of TBX20
gcgacgcgtagtgggagagtgcgaaccttatggtagcgcccggactaagcggacacagacccctctggttttacaaaggcggctgtgacgaggacttcccacgg

SEQ ID NO: 4 - DNA, 105 bp, Artificial Sequence
  subsequence of CACNA1B
ggccagcgggtcctctacaagcaatcgatcgcgcagcgcgcgcggaccatggcgctgtacaaccccatcccggtcaagcagaactgcttcaccgtcaaccgctcg

SEQ ID NO: 5 - DNA, 83 bp, Artificial Sequence
  subsequence of ZIC1
tctcttggctctcggcttggggtcgggcggcgagtggcagacaggcggtggcgggagccagaggaagcgggaaggcaaaggtt

SEQ ID NO: 6 - DNA, 91 bp, Artificial Sequence
  subsequence of SIM1
tggccaatagggctgagtgacacgagtcggccccgagccgccctccgcgcgcccaggctccgggctctgaatcttactacccgcgggaccg

SEQ ID NO: 7 - DNA, 89 bp, Artificial Sequence
  subsequence of DLX1
gaggaaacgcgggctcctatatccccagctacacatcgtggtacccttcagcgcaccaagaagctatgcagcaaccccaacttatgtga

SEQ ID NO: 8 - DNA, 112 bp, Artificial Sequence
  subsequence of LMX1A
gcttccctatcgcggaccaggtcccagagagcggggctccagagctcagcgccaagcggaaagagagtgcgcccaggacgcacggcctgaacactcacccagcagcgaggag

SEQ ID NO: 9 - DNA, 102 bp, Artificial Sequence
  subsequence of DLX6AS1
gccacgtctacctgctggtattgaggacattacaaacagtctcggcgcgcagcccgcgtgtaccgagagcgcactagggttgggagtgggaaggtggggtgg

SEQ ID NO: 10 - DNA, 88 bp, Artificial Sequence
  subsequence of MIR196A1
ccgcctacacggaaaatccacagagccccgcgcagaccctatgatcggctcggcccgccgggcttgggatgaggctccctgcttctcg

SEQ ID NO: 11 - DNA, 107 bp, Artificial Sequence
  subsequence of FEZF2
aagcgtcacggagagcaaggccgctcgccggcatctcgggggcctcggcgccgcgcaggtgcgcctccagctttatggccagctctgggtctgaggctgggggagac

SEQ ID NO: 12 - DNA, 97 bp, Artificial Sequence
  subsequence of STAG3
agggcaggacgcctgagagcttgaggccacacgaggctgtggagcggcgtgactcaaacgtggcgcgcatcagctcgcacacttccaaacctcgcga

SEQ ID NO: 13 - DNA, 89 bp, Artificial Sequence
  subsequence of PTPRN2
gaagcccgacccacaacaaagctagtgacagttcatttccttcctgcttacgggggccggcgagaggaaaggatggcggatgtgagagg

SEQ ID NO: 14 - DNA, 92 bp, Artificial Sequence
  subsequence of BARHL1
tggaggatggcaggtgcagcctgctccagccggcagggcgtgcgagccgggagcgggtcctctccggttgccatttcaggcctgctcgcttc

SEQ ID NO: 15 - DNA, 96 bp, Artificial Sequence
  subsequence of CCDC140
gagtcttgggcctcccctttatttctttctgaagtctctccggagcccaagccaccccacacccaaaccccgcagctggatgggagtccaggccac

SEQ ID NO: 16 - DNA, 90 bp, Artificial Sequence
  subsequence
gaagcgagctgggctgtgagcaagggacacccacagcctggagaaacagccccgctctcttgcgcgctgtctgctccagccgctactggg

SEQ ID NO: 17 - DNA, 106 bp, Artificial Sequence
  subsequence of GATA2
cgtccagccagggcaaacccgggctgtgcaacaagtgtgggcggcacatctggcctccggtcaggcgggctgcgggcaaagagagagaggatcagggtgggcagaa

SEQ ID NO: 18 - DNA, 100 bp, Artificial Sequence
  subsequence of ADCYAP1
gggctctccggttactttctctgtatgtcgcgggtgagaggaacagcgaggacaatttagcgcaaacacacgaagggtcggatctcaagggggcagcgct

SEQ ID NO: 19 - DNA, 107 bp, Artificial Sequence
  subsequence of TBX5
aatgtgcagggaggcagtcggccggcagagctgcggcgggagccaaggtcaggcccgcggggagagcgggcagcttccagcgccggccacaagctcccaggccagct

SEQ ID NO: 20 - DNA, 93 bp, Artificial Sequence
  subsequence
acagcagatggcacgagcacgtgcggcgctcagcttaggctctcggaggcagctgagttggaaatcccgacggaaagcacccacaagctccca

SEQ ID NO: 21 - DNA, 81 bp, Artificial Sequence
  subsequence of NECAB1
aacaatccttgccccatagcaaacgtttcgaagcctactctaggcagagttcatagcaccgcctttgtcagcagcactgcc

SEQ ID NO: 22 - DNA, 93 bp, Artificial Sequence
  subsequence of ADRB1
cgtcaccaaccgggcctacgccatcgcctcgtccgtagtctccttctacgtgcccctgtgcatcatggccttcgtgtacctgcgggtgttccg

SEQ ID NO: 23 - DNA, 90 bp, Artificial Sequence
  subsequence of OTX2
ccgcctacagaactccacgttcgcagaggggcatcggtcggtctattggaggtactggggtgatggccgacagacacggggacacgtaga

SEQ ID NO: 24 - DNA, 93 bp, Artificial Sequence
  subsequence of NKX2-6
agaagggggtggaggtgacggggctcagcagcatcccgaaggcggatggggcggggccgaggaggtccgggtgaggagcggcaccctgaactt

SEQ ID NO: 25 - DNA, 103 bp, Artificial Sequence
  subsequence of SIM1
accccaaatcccatgtatcctgccgggcctgcacatcctcgctaaatgtgtactgtgcaagtcttccccgggctgaggcgtcgagtggccttcgtgttcagcc

SEQ ID NO: 26 - DNA, 103 bp, Artificial Sequence
  subsequence of DRD4
gaccagcagcacgggacacgcgtgacctgtgctcctttcgagccgcagacgtcacagtgacgacgtttaagctcctaatctccccaaatcggcgggaaggatt

SEQ ID NO: 27 - DNA, 90 bp, Artificial Sequence
  subsequence of TBX15
tggctgttcagcaggagcaccttccagcatggttttagaagtccgggctggaaagcttctgaaaccgctaaaccaagttgcgagcgttgt

SEQ ID NO: 28 - DNA, 80 bp, Artificial Sequence
  subsequence of TRH
actcctgacctgccgactgcggatcccgagtccccggatcccggacccatcctgtggagcccactcctggcaggtaaccg

SEQ ID NO: 29 - DNA, 94 bp, Artificial Sequence
  subsequence of FBP1
accgccgaagagatggctttgactgctgtgcagagcgagttgagcagctgggtcaactcgcccgtgccgcgggccttcctgccctcctccatga

SEQ ID NO: 30 - DNA, 91 bp, Artificial Sequence
  subsequence
gtgtgatgcccggtgtcctaccctaggccacgcggagctctctcccggcgtgtcgggccctgcgcccctgcccagtggctcacctcggctc

SEQ ID NO: 31 - protein, 120 aa, Artificial Sequence
  subsequence of BCAN
GCGTTCCGGATCAGTCCTTGCCTCCGTGCCCCCACGCACAGGCAGCTCCAGGAGCAGCGGCCAGCAACCCTTCTGGGGACACCTTACTGTAGTCCGGCAGGACAGCCGATCAGAGCCGCT

SEQ ID NO: 32 - DNA, 113 bp, Artificial Sequence
  subsequence of TP73
cgccacaccatcaccatccccaaccgcggcggcccaggcggcggccctgacgagtgggcggacttcggcttcgacctgcccgactgcaaggcccgcaagcagcccatcaagga

SEQ ID NO: 33 - DNA, 87 bp, Artificial Sequence
  subsequence of MIIP
cagcctccctagtagctgggattacaggcgccggccacctcgcccggctaatttttgtatttttaggtttactggcgtgagcaaccg

SEQ ID NO: 34 - DNA, 90 bp, Artificial Sequence
  subsequence of HOXC4
agaaaagcgcttggctctccccaaatgggcccagcccgccgcctgctcaggctgccgcgcgctctcccgccgctcaggcacggcccagtg

SEQ ID NO: 35 - DNA, 84 bp, Artificial Sequence
  subsequence of HOXA7
cctccgccaatctcagcagtcctcacaggtggtctcgctccgcagggcccgcagccgcctagaatggaagggcaagaggctcaa

SEQ ID NO: 36 - DNA, 109 bp, Artificial Sequence
  subsequence of BST1
gaacgggaaacggcaaacagcgagatatccgagcgagagtcccgccctgcatcagtttgcggaaccgccttggtagaaggagagaaggggagtggaggaagcacgggac

SEQ ID NO: 37 - DNA, 91 bp, Artificial Sequence
  subsequence of C1orf114
gtgcctctgcgtcctccatccgggcctctctaactacgagagcgacaaaaatctgcgcaggcgcatgcaatatcctcagaccaccgacccc

SEQ ID NO: 38 - DNA, 90 bp, Artificial Sequence
  subsequence of FOXG1
acaagcagggctggcagaactccatccgccacaatctgtccctcaacaagtgcttcgtgaaggtgccgcgccactacgacgacccgggca

SEQ ID NO: 39 - DNA, 113 bp, Artificial Sequence
  subsequence of ATP4A
gcgcacctggaacttgttggtggagttgaagggtatctcgcagacttttgggaagcggtcccggtagcccatggcgttgcccagcgtcagctccgagaacttgagcagcgccg

SEQ ID NO: 40 - DNA, 86 bp, Artificial Sequence
  subsequence of NOTCH1
ggaactgggctgcggtcacgggtgggaccagcgaggatggcagcgacgtgggcagggcggggctctcctggggcagaatagtgtgc

SEQ ID NO: 41 - DNA, 109 bp, Artificial Sequence
  subsequence
acggctcggccatctacacctacctgcagcccgcgcagcgctacaaccaggcacggggcaagttcgtatcgctcttctacaccgtggtcacacctgctctcaacccgct

SEQ ID NO: 42 - DNA, 96 bp, Artificial Sequence
  subsequence
agcgggcacagacacaagcggttggacatgaagaggaacacaccggcgggagaacacagaacacccaccctctctttagtcaccctggaggcctcg

SEQ ID NO: 43 - DNA, 84 bp, Artificial Sequence; identical to SEQ ID NO: 35
  subsequence of HOXA7

SEQ ID NO: 44 - DNA, 107 bp, Artificial Sequence
  subsequence of ZNF529
gtgctgaggaggccaaggagggcactgggagctccgttccgggagagctgtctaaggacgcggaaccgggtggggaggccagggaggtaaccaagagtccgagccgg

SEQ ID NO: 45 - DNA, 92 bp, Artificial Sequence
  subsequence of PRLHR
acacgagccccctgcttggctgcagcgcgctcagcgggcagcgggtccggccaagccaaaggcaggagtcagcaccacggacagcttccgct

SEQ ID NO: 46 - DNA, 93 bp, Artificial Sequence
  subsequence of ARL5C
cgggacggtggaaaagacagctgagcccccacctcccttcacattccagaaaagtgtctgaaaggcccggggcgcttcggggcttgccaagag

SEQ ID NO: 47 - DNA, 1006 bp, Artificial Sequence
  subsequence of PAX9
cggagtccggtcgatccgatgctggggtctaaagcttccccagccacacgcctgggccgagtcgcccccagagtccccggcccctgctccccttgggcgggtgtacacaaggatccggccagcgccgagtgtactggttcctcccacccagtgtagccccctccttcacactctcggcccggcttccagtctcccactgagtaaatatttatccagagagcgagtcgcccctcggaggaggcctcgacgcggctagggaaaggctttttggcttctccctggcctgagccagctgcaggccttactggtgttttggttttggtcttaaatttctccttttagtcgaaattcttccgatctctttgagatcttctgagtccagagtgagcagtgtaaccaggcggcagactccagctgacccttgttcttgttctaggtcctgcatccttacattcatcgggactgaccagaccttagtgttctctcttttccttccttcatcctctttctctgcctcagatccgtcgtctctcggtcggtctcagcgggtcgctgactacctcgccctagcactcggtccgcgccccgggaaggcttcagcatcaccctcttctgctgggatcccgctgaccctgtctgcagcttcggcttctcttgctcccagagcggggtcttcggcttgccgcggatacttagtggcccaaaacacctaaaattgactcttcctgcgctcttgagaatgccaagagcacccagtacctgcaaccgccggcatgagtggggcctgcggggagccgccagagctgcggacaggccccctgcccactgagttgctacccctggcacgcccaggggatccgcagcagctgaggccacatggtcacagccaagttcagcaggtggaaagggagagatggcattgaacctatgtgagaactgggaagatgtgtggcagctgaaggagttggtaggaacaagagggagttgtatgttacctccatataac

SEQ ID NO: 48 - DNA, 1001 bp, Artificial Sequence
  subsequence of HOXD10
tggttcctctgagagccgaagcctcgtgtagccctccggggcgcataggaacccggagccaggcaggaggaccgagcgggaggacaacgcagggaccaacccatccatggggatccgggcccggccagctgcttggcctcccggccctcgcggccctttttgcctccgccctcctagagacaccttggccgcttcttagccccaagggatctttcctttggacccctggggtgggatgtctcagggcccgcggaatccgactcaccttcccgctgggctgcccgggactaaattaaccagcctgcgcccccacccgcttgtcctggacccggccctcttaagcgcgttctgcctggttgtgtgtggggggaatgcttctgtgcgctggcgccagggcactctggcttccctccccgtccgtgcgtgtccacttggaggcccctagagctgagactttccttccgccggttgggcccaggggccgaagcgggggacgcgagtggggcgggctggccgagcgagccctggagaggcggacaggagggcggcggagagcgctgggccggttgtctccagcgcgcactatcgcgggcgcgtagtagatgtcgctgttgtccgtgcttacccggccggccggccaggctctggagcacgtgacccgagaggaggctgcggctcaaggccattttcaaatctcattggcttggttgtcatgtggtcggcagaggcatccacaattacacggggaatgttttcctagagatgtcagcctacaaaggacacaatctctcttcttcaaattcttccccaaaatgtcctttcccaacagctctcctgctgctaatacttttttagtagattccttgatcagtgcctgcaggagtgacagtttttattccagcagcgccagcatgtacatgccaccacctagcgcagacatggggacctatggaatgcaaacctgtggactgctcccgtctctggccaaaagagaagtgaac

SEQ ID NO: 49 - DNA, 468 bp, Artificial Sequence
  subsequence of TBX20
gtggcttctgctcctcaccagtgcgtctctagcctggggctcctattttccctagagggaccctggaaaatgggacggctgccgaagagaaggcgaaggtcagggcgcggagctctacggtaaccacgcgacgcgtagtgggagagtgcgaaccttatggtagcgcccggactaagcggacacagacccctctggttttacaaaggcggctgtgacgaggacttcccacggccttgttggagggcgtcctgttagccctgctcagcctgaataactcaaattctccgaattcgcagggtaatccgcttcgcttggagccgtgtaaactcaggctgacatacacactcaagctgtatatgtaaatatttgttctcttttccagccagtcggtctggctattagaagcctcttcgtgggtcttaaaattaaaataataataataatttttaaaactccaacttttcactg

SEQ ID NO: 50 - DNA, 1003 bp, Artificial Sequence
  subsequence of CACNA1B
ccgagggcacccaggggcggtgcggccggcagagtgggctccggggacggcccgggctggcgctgagcggccgtcgaggacccacaggctcgtccgctcctgggcccggcccagccccggggtgggaggcgcggggcgagggaggcgcagccggaggggccggggcggggcgggggcggccgcggggcggggccggcgcggcagggtgggcggggccggcgcggattggccgggccccgccacgtgaccggccccttatagggcgtggcgcggggccgcggagtcgggtgaggcggcggcggctgcggcggtggggccgggcgaggtccgctgcggtcccggcggctccgtggctgctccgctctgagcgcctggcgcgccccgcgccctccctgccggggccgctgggccggggatgcacgcggggcccgggagccatggtccgcttcggggacgagctgggcggccgctatgggggccccggcggcggagagcgggcccggggcggcggggccggcggggcggggggcccgggtcccggggggctgcagcccggccagcgggtcctctacaagcaatcgatcgcgcagcgcgcgcggaccatggcgctgtacaaccccatcccggtcaagcagaactgcttcaccgtcaaccgctcgctcttcgtcttcagcgaggacaacgtcgtccgcaaatacgcgaagcgcatcaccgagtggccatatcctgccgggcggggccgggcggggccgggcggggaccggggtgggggccggggccggggccatcttcccggtggccgggagggcgcgacctggggaggcgtcgggagacgggcgaggggggtacggagcgccccagggcccctcggagcggcgggtgcgggagcatttccgtgagtgcggcgggcgcggggcggagcccctctgctccggactcgtccctccgcacgccgggtcctggggatcctggtcggtgcacagtgcgcggctagcctggaggg

SEQ ID NO: 51 - DNA, 1058 bp, Artificial Sequence
  subsequence of ZIC1
aagcaatagggcaggagaataagccgcaaacgtgaaaactagaaaccaggagccaggtggaagcaatccgaaatcgtgtgtagctctgggtaatacgagtttccagatctgatgctaaaaaccgactcctcctactattaatttttttaaacataaaaataaaatgtagatccaattgtattagggattacaatagagttaagatatttataattccactgcagatgtaagaatttattgacgttccgggtttttaagcttgcaaagtgctaatcctgggctgctggctttttgttttattttttttctatttgtttagtttttgaaaaacggccgcggtatttttttctaattagacccctctcattctactttggcaccaggggagaagcccttcaagtgcgagtttgagggctgtgaccggcgcttcgctaacagcagcgaccgcaagaagcacatgcacgtgcacacgagcgacaagccctatctttgcaagatgtgcgacaagtcctacacgcatcccagttcgctgcgcaaacacatgaaggtaatcgccgcactctcgtcgccccctttgaggcaggagctctcttggctctcggcttggggtcgggcggcgagtggcagacaggcggtggcgggagccagaggaagcgggaaggcaaaggttccactcagtggaactgggcagagaaggtagggcgggacctggaaaaggggatgggagtgtccaaggccgttttaaatttttggtttaataataaaagttaaaagaggcgagtatgagcaaaggccgccactgaatttggcccagagctagggcttttgcagggggttgacgctgcggaaactgctgcccttgcagctgccagtgagacgcaagaattggactcctgcgcccaggcctgagctctggctcacctaaacatggacaagcaaagttcagggaaagaaagtgcagtctctggcctcatatccagtctccctcttcccagacctatttttcttttgtgagtcttggggaccctgactttcccaggagcacggtttctgcaggc

SEQ ID NO: 52 - DNA, 851 bp, Artificial Sequence
  subsequence of SIM1
cttctgcttcacctaccttcagtccccacaagcggcagaggtttcgggggcgcccatctcttaactgttctcatgcctaccgtccaacccagcgacaccgccggcctctccgcttcccaccggcagagaggagcagagcattcccggctcccttttctggatcatgaattggaggaggggtgcgtggcagaaagaggaggatgcaagctttgggacgagtgaggtgattttagaatcctggtcctccgtagttgctacgaagccagttcactattattcctaattggaagccgaaaactgccccccgtaacttctttatagcttaagggtttagcttcaacttcactccggggccgcctctctcccgccctccctcaatgccactcacaagccccctcgcctcccattggcctggcgcggccaggggcgaggcgctcattggccaatagggctgagtgacacgagtcggccccgagccgccctccgcgcgcccaggctccgggctctgaatcttactacccgcgggaccgctggactcctaatgagctcagggtgccgggtcggcgctgtccggttgccgccgctgctcgcggcctcctgggccttcccgacgtcgtgcgcgacccgcgctcctcgagctccctggggtcgggtggttgagcgctcagtccagcgcggcggcccagcagaaccgggaacgtccggaggcagcggaggtcgggcctgcgggttaggtctaccggcggaggaggcagggttcgcccaaaggcccatcccgctggcagtcgctggccgacggcgtgcgcgaggccggtttggggagttattttctctttctcgtttctctgaaa

SEQ ID NO: 53 - DNA, 1068 bp, Artificial Sequence
  subsequence of DLX1
tccgcaggcggtagccacggtcggactgagcccctggcaggctaaggcctggatcccggttctcccctcatcacaactcctccctggctctctgagagctgcccccgtgggctgacggcggcgggaggttcggccttcgagcctttggctcttatgggggaagggaggaaggagggatgtctctgcttctctggcagggagctgccagctggcgcagggttgggaggtcctatctctgctgttctgcggtcccttttttcctccctgtgacctaggtaggctcagtggtcccagcctgagtcacgttgttgtccgctcttgcaggtcaagatctggttccaaaacaagcgatccaagttcaagaagctgatgaagcagggtggggcggctctggagggtagtgcgttggccaacggtcgggccctgtctgctggctccccacccgtgccgcccggctggaaccctaactcttcatccgggaagggctcaggaggaaacgcgggctcctatatccccagctacacatcgtggtacccttcagcgcaccaagaagctatgcagcaaccccaacttatgtgaggttgcccgcccgtctccttcttgtctccccggcccaggtccctcccgcctccaggtccatccatcccgtccggaaaagaaggacccagagggaagaaggaacagtggaggcgggacgccctccatctcctcggagccccgcgaggtccggcccagcaacttcccggcatccgcgctctagcctgaaccctggcctgggccgagcagtggcagcagagagtggcctcggagggaagccactgccacctgagacagcccaagcagcaagataaacccgctccacccgacccgccgaccttcagctttgtgggactatcaggaaaaaacaaaacaaaaacaaaatgtagaaaaagcaaaagctcttttctgtcctgtcagtctcctgtctccttttgctctgtctgtgcgctggtaaagtccaggtcctcatccgtccgctgtcctcattctgcggcctcagcaaaaagccacaaggtctgagcggcccgg

SEQ ID NO: 54 - DNA, 1008 bp, Artificial Sequence
  subsequence of LMX1A
ctaggccgcgagaagagggcggcatttatgagacgtcgatcagctccgagattaaaaatccagccctgggtatttttaatcacttgccactcagacgcctacgaacaagctcgcccgcccctcgcggctttggggaattcggtgcccagtgcgtgaggcctggggcggcttgttggatttatttgggtagggacgacccacaagcactgacggacagatagtgatggggctcaatttagtgtatgaagaggggcgctagcttccctatcgcggaccaggtcccagagagcggggctccagagctcagcgccaagcggaaagagagtgcgcccaggacgcacggcctgaacactcacccagcagcgaggagaaggaggccgaggtgtcgatcgcgctttggaagttctcctccatctttaggccgtccagcatgttcgggccgggccgggaggacctgtagaggagaagaaacgatgcgtctgacgtccgtgcccgctgggactcggcgccagcagccaccgcactcctgggaaagaactgagggagtgtccagggcgaccagaatcagccaggaggatagggtccagccaagagaatgtagggtgggaggagagatcagtcacagcgaactgctctggctgatctgatttcacttgaagtcaacacgttatgtacttaggcctccgccccccaactgcgtttctccttctcctgcccccctcacccccacctacatcccttgccccaggttttccatcccgaatccgactccgccccaacctatacgaaggtgggccctcgggacgtctctgcaggaacgcagctactggggtatattgggtatataaagagtgggtaccctccctcgagcgaccgggtccaggcacgcgggacgatggggtttgcaatcccgcgtcccagccgccccgttgcggccctcacctgccccaggtcgagaaggggcactgtaagggacccggagggcgtcccgcccgcttctggactcct

SEQ ID NO: 55 - DNA, 1007 bp, Artificial Sequence
  subsequence of DLX6AS1
tcgtggcgcgccaccttggcatgttgtgtgcgggtcacactatctccagttttccattctcgatactggcaggaaagtctgatagtcaggcctgaagtttagattccatcccgcaagcgcagagatatcacaccaagtgggacctctcgctcgttccacttcccagcccctgactgtctctgagctcagactgggtcgcccagcaggtttcagcaggacctttaccatgcaccacaactaccacctcagtgcagctgcttcactggaacagagtgcaaggattttagccactaactattaggggaaggttgagagccctgaagctacaacccggacaatcccagccttcccggcttcctcagcaatcaaacaaatgagaaaaaaaaatccccttgcaagtagaggcagctgcactctggatacagtgctcaattgcagggaccttccgaggccctgccacgacatactctaattggggtgcagccagagttgcaggaagctggcgaggaaagcggtgcacctgtgagcataaagcgaaaaacatagacaagcacagggtgagggtgtagggggtgaaacgccttcacggtgttaacaacaagctgcagggtataaagcaataaaactgccacgtctacctgctggtattgaggacattacaaacagtctcggcgcgcagcccgcgtgtaccgagagcgcactagggttgggagtgggaaggtggggtgggaaatcttctcttttcctgacattcccttctgtcccccaccccccacatctcccccttacttagcccacctttctttttccatgaagcttttctgttgttgttttaattcattgccgatttgtaaacgtgtagatcgtgttactggttcgcgtgttaaagtgcacctcttgttaaaaggtggggaacagggcacgccacttaaaaatgaattcagagttactgaaccggctccccagactcaagaacttaagcgcaacgggctgggaaaaggaggggg

SEQ ID NO: 56 - DNA, 973 bp, Artificial Sequence
  subsequence of MIR196A1
tcacacccgcacccatcgcaaaaacgcagctgtgcaggccgagggcggcggcggacttacctgggcggcggcggtgccggcagtgcgcggccgtcggaaggtgcggagccagcggccgcggcccagtccaggctccctcccgccctcgcccagaagcgagggtccgagtggccacgtgtccggcagggaagtccgaggtagcgagggagtccacctggccgcccgctccccctcccgggtataaatcttggggaccggaaatacaataaaacttcaccgtgttgatgaacttcaaacggtttacatcccctcctgtcctgaaaagaaagacgtccgggggcggattaaaaggaaggggaaacaaatttacgagcggcagaagcacccgcctcggcccctttctttgcccgcacactttgtccgcgtggagagaagcagccccagcccccgggacttggcctccgccgaaccggccgccaggcgcgctcttctctcggaggagtcggcgctgacccagcccgcgcccggcagagactggaagccgccgcctacacggaaaatccacagagccccgcgcagaccctatgatcggctcggcccgccgggcttgggatgaggctccctgcttctcgctagagcagaactgggctccctggcgcttccttgcgaaagcccaggctctcccaaccacgcccggtggcctccattttttgcatctttccgctgaaagcgggttttttcttttttctttttttttgacagagtcctgctgtgtcacccaggctggagtgcagtggcgcgatctcggctcactgcaacctccgcctcccggttcaagcgattctcctgcctcagcctcccgagtagctggaactacaggcgcccgccaccacgcccggctaatttttgtatttttagtagagacggggtttcacaatattggccaagctgatcttgaactcctgacctcgtg

SEQ ID NO: 57 - DNA, 1050 bp, Artificial Sequence
  subsequence of FEZF2
ctttaaaaggaggcaactggcgcccgcgctcctctcgggaaagtgcgagcggtttgcgaatagggaaagagggaagagacgggagggggagggggaggaatcgtgatggttttgccggtggaaggaaagggggggggggacccaaacccaaacctaggcagagttccgtgcgtgattcacaactttggaggcctgcaggtttgggggacgcggggagggcggagggtcccggacgcggcgcccccaaagggcccctgggtatcagtctagtagccgaagtatcccttagccctccgcagccgagctgggcatcgtgctaataaactgccatttacccacggaaccggcgccagccccgaacacgcgcaaatgataattacctcattaggatgtggcgcatggacgcgggcgccgcgtttggaggggggaacttgttaatggggaaatattaatttatgcaaaagcaatgagctcgccttggctggcgtcggaggtcgggagaaagctcccactgactaaggacgaccccgaagcgtcacggagagcaaggccgctcgccggcatctcgggggcctcggcgccgcgcaggtgcgcctccagctttatggccagctctgggtctgaggctgggggagactaaaccgagagctggaagactttcggagatcctaatagatcagaattgttgatttatgatcgggtttctgaggcaaagccgagttctgcttctggtttagggctgcgtgcggggaggattcggagggcagctctcccagctgatgggtacttactgtttgtataattgagaaggtcccatctccacctgtttaaggagcagattgaaacagcagaacctccccctggatcctattaaaacgtttttcctcctaaggccattcagtcgaaccaattttccgaagtgattcatagagctgaattctgccaaggcagctctttcacttttagccactaaagcaccgcgtggaaccgggttttgtgtttttctaaaataaagagaaggattatcagagaggagagggagggggcctg

SEQ ID NO: 58 - DNA, 974 bp, Artificial Sequence
  subsequence of STAG3
cggacagggggcggggcccgaggcggggccccgccaataatggctcggagccggcttcaggggcgggggcaaggaagaaattaagccaatgtagcgcggaagctcggcaggggggcgggacccggctggcactcaggaggttggtgaaataggggcgtggtctccctcgggggcgtggcgatccggctcaaaaggcggggcctgggtggaacctagcctatggcaattgagaagccagattaaaggggttactagcagtctggtccaaaacccgcccaatggagtaggagattgagggtagcgggggtgggacctgggtgggggcggggctaaagcgggccgcccgcgtgcccaagcccacgtgagagggcaggacgcctgagagcttgaggccacacgaggctgtggagcggcgtgactcaaacgtggcgcgcatcagctcgcacacttccaaacctcgcgatagctactggccctgggcgagccgttgggattgcgcttgcgcacagcgtgtcttgtacgttcccgcgcttttctggaatctttcgcccccggaagggcagcggcgggcgcctgtgtggaaggtggggtggccagagacacccgagggacctgaggtggggaccttccctgaaccctgctcggccagaagtcactcttccaggctctgacaggtttctccttgacccaagaataggccctctcgcgaccctcccggccctgacactaggagccttcccgggccgtgccccaatggcctccgccacagagctggagaatcctctccccaggcctccatagactgagagtccattctcttaagcgcttggaaggctctttatcctggagccgcttaccccaggggcagtcgtagatatttttaccttctggaaaaataggaaacgcgcacctgcctttcctccttttgcgtttccagccctattctcatggcgcctccacccccaaatccttaa

SEQ ID NO: 59 - DNA, 981 bp, Artificial Sequence
  subsequence of PTPRN2
caacaacactgaaggacccgagggtggcttctccgtggctctgaggttaacgctgcagcgtatgcagcaaacacctgtcaaggacccactgtgtgctcggcacaccaaggcaggtaacaaaggacccagtgcatgctcggcacgcagaggcaggtaacaaaggacccactgcaggctcggcacgcagaggcaggtaacaaacgaccagcctcagaagcagatgtgcttgctgcaaaccaccttcctacggcccagcagaggcacaacaagcagcgaattttttccagggcctcccgtgaacacggcaccctacgttgccatagcgacgccatcccagctctgagccgcaacaaagcggcagtgtctgtgtctcacctttggccatcttgttgagaaccatgtcgatcaggacgtaggtgccgctccggcctgcaccgtcactgccaacagaaggagagaaatgaaagtgctgccgtccacacggaagcccgacccacaacaaagctagtgacagttcatttccttcctgcttacgggggccggcgagaggaaaggatggcggatgtgagagggggaggaaggacgcgggctgggagaatccaagtgaggggagaagggaggcccctgggggcttcgagcctctgagcagcttgtagcttgtgggatgagctgctgtgctcagatgtgactccctcttgcttgttcccccctctttggccaaagatgtggtaaattttgccagaacaaaatgaactaagcgtttgactgtgtcagagttgatggcatttgtattgaaaatatctgcaaggtgccttctctagtgttgccgggcaacctcccgagcggagaggggagggcgctgggcggctgggccccgctggctcatgcacgcagggacacttcaggcacatccccctaggctgcctgccaccccttctaaacgcaggtcctccgtctcagaaggagaaattgacataacag

SEQ ID NO: 60 - DNA, 1004 bp, Artificial Sequence
  subsequence of BARHL1
ggggcaccggacttgaactcgtttcctaatttccctcccgaacacactcaccagacgtagatgcaaatgtacaaacacagaggcatccacacactcaacccaaatagccacacaccgacacacacatcaatacaacttgcagtcacacacgcacgcacgctcagccccacagtcactcgcacgctcttagcagaggcaggaatggtgcttttcataaacaagcctcagaacacatcgccccattaataataaatactgattactgctccgggcatcaataattaaggcctgttacagtaattacacaattatgatgatgatgaataattcagggagggaaacagggctggtgtggctgagcccaccttagtgggaccctggctggtccgcctagcctcacctgcaggtgagcctagggtccaggcctgacttctccaaaccccaggccgttggctggccaaggcctctggactttggggccagacagtgcgcagggctcgcagtgcgagccctggaggatggcaggtgcagcctgctccagccggcagggcgtgcgagccgggagcgggtcctctccggttgccatttcaggcctgctcgcttctgctagcttgcagcccggccagcctgcagaggaatcaatcgcattcccttccctgaagagcacccccccatcccctcaggcctctccagggtgatcctaccttcataaagaggcacgcgcagggaggagcaccccctacccagctccaagggttcgttctgcgatctcctgggcagggtaaggcgcagttagagccgggctttggggtcagacagcagggcttaaaacccaggctcctttttgaaaaccggcccagacctcagttttcctctctgtaaagtggggtaagagccacggaaggccggtggaagataaaaggagaggatgcacgtaaggcgtgcgatggtgcctggcactcggttatttattaacaaatgagtacgatccctcttggcctccc

SEQ ID NO: 61 - DNA, 1064 bp, Artificial Sequence
  subsequence of CCDC140
tgcccatgggttcataaactagctgtcacttgctataaacatgtacaaatggaggccacaaggatgtgggggtgctggggacctaaagctccggaatcaggaggcgactcattttctctcctttccggcctctttcttttctgccgagcgctctgagattcatatgtacccagatgatcagcccggcccttctcaccggccagtggccagaggtccctggacacccggagaggggtgggagggcacccttaggctctggacagctgggccacatccaaagacttaatgaatctaaatttcttgtggcctgtgtccccgaagtccgacctgggatggccaggacagcaaagttggctgaggctgcctggcctagggcgcccgcacgccgccaaacctaacccggctcagagccgtgactccgcagaacagggcgcaacaggtctcaggaatgccgggtgattccagccactctttctctgtctccgagtcttgggcctcccctttatttctttctgaagtctctccggagcccaagccaccccacacccaaaccccgcagctggatgggagtccaggccacttccctatccgcagccggtgggccaaggagtcctggtgccaaatttggccgcggtacaggcgctaattggtaaagggatgacccagcggtggggcttggaaggcgagggcccgcgccctgcatccttgaaccctggtttgggaggcagtgacttttacctgggctaacaaattacccagaaagcatcagtgggactctccacaacggtgttgtgaacgagtgtagggtccactcacgctctgtgcacgttcgaaatgaaacgggagccttgaagacgatatttggataatttgacaaaaaaaaaaaaaaggtgggcgggggagatagcttctattgtcccctctgcgcctctgcccccagtttcagagacactacaggtgaaaataacagcgggctggctgtccaggcctgagtggagcgtgcccttgttagcttgaaagttctccctcgcagcccgtttggatgcgtgcgtctacagcccagt

SEQ ID NO: 62 - DNA, 1780 bp, Artificial Sequence
  subsequence
cgtttcgctggggctccctccgctctgcaaagggagcggggagctgggggagccttgcacaccagtcttcctggagctgcagacgaggagccccgcgccttcgggagcctctcggcggcttcccctctaacgcgcgactgtgcagcctctccccgccgcccccacccgcggctcgccctcgctccctccctccagccccgccagccggagcgcgcacaccgggactccggcacgtgggcgcgcgggaggtggcggccgctgctgccgctgctgccgctgccggagcccgaacccaagccccagctggagccggagtcggagccggcgagatcgccctccatgctgcgggagctgcggccgccttccgctcagcctctggtcccaggcgagcctggcgagccggcgaagcaccggcggggaggaggactagaacaggaggaggggcacggcggattgaagcgagctgggctgtgagcaagggacacccacagcctggagaaacagccccgctctcttgcgcgctgtctgctccagccgctactgggggctctaagcagcgcgatgctgcttcgcttcttctaggcggcggccggcggaggctttccgcagccgcttggccggcgccggcccctattccgttggcaagtcccttgtctatcccggagggcgcacccggacgctcgagccggagcgagcgcgaagtccgaagtccgcccccagagccgccaacttccctgtgagcccctctccccgccgcagcctgcgccagacctgggagcgatgcgcccccacccgggcggcgcgccctctgccaactcgccacccatgggatcgactgccctcagctgcccggcttggagtgcgtagccttcgccgcgtggcccaggagaggagcgagacaccaaggcgtttcgcggactccgcgcgcaccagtcggcttggtggccctgcgggatagcgtttatacccaggggtgagtaggccgctaatggaggccccctttacccccagctagcggcttgcatggacggcaaagagacgggagaaagttgggtctccttgcgcttaatctggcattggcagaggaatgcaacactgtttcctccaactcgattgccgcgggggtttccccagttccctccatctctaagccaaggagggagtccccttccgcttcctaaggagaaaaggggctccctagagcagatcgctgacttcctcaccaacgtgccatttggggcttttcagccgcccgcgcgttaagctagctcccagcataagcgcttagagatccgcagccgcctgggcgcgctaagagatcgtgggcagacctagcccttagggcagcctaagcgcgcttcactaaagaaaaaagactgttggtatattaaagaagtgtgtgtgtgagagagaaagagacagagaaagagacagagagacatgggtgggggcaccaggaaaggtagcccgagtaggaggtgctagtgaaatttatcttttgctgacggatccagcctccggaatgcccgattgtcttgatccgcggtgcggtgcgggttttaggggcgcacaatacagggtgtccagacagagtccaacaggtggcctgcgcgggcatcctgtggctaggcgcgggggaggggaacggctccctccccgagccccgggctgcctctgctgcttctaggggtgcatctgaacatggataaggaaatgcgctccctgctctcaggccctatttggggtgagtgtgtgaggcatccaaatgcctcctgtcgga

SEQ ID NO: 63 - DNA, 1038 bp, Artificial Sequence
  subsequence of GATA2
gccggcacataggaggggtaggtggggatggggtggtgtgtagcaggctgggtgcccatagtagctaggcctgggcgcaggggactgccactttccatcttcatgctctccgtcagtgacacctggtacttgacgccgtccttgtcctctcctcgggctgcactaccccccgcggaagatgaggctggagacgcagcccccgtggtgctagggtcaggagacacttctttgggtggcgtgggtgggaagccgaaaaggtgggagccagagtgggctgctgtaggggtgagggaggccactgagctcccgctgcctcccccgctcccacccccagcccctgggtacacagagagtgggcctccagggcctccagcagctgaggggtgcagtggcgtcttggagaaggggctcacggtccaggggttgtggtggtgggccgcagcggcagagagggctgctttgcccccgtccagccagggcaaacccgggctgtgcaacaagtgtgggcggcacatctggcctccggtcaggcgggctgcgggcaaagagagagaggatcagggtgggcagaaagatcagggtaggcagagctagggacgcccctgacagacattgagatcacgactcccagaaccagcagtcatcccctccccaaagaaagccagaaacataataccccaccggtaataatcaggaatgtcagtccaagctgaaggacaagtggcatagaaggaaccccaccggacagaccctacagggaaccctcacaggccagctggaagtgggcagaaaccctgtgggtcccagaccctccccaatcggccgctgctcccacctctcccgccccaatttttcagcagctcgattcctgcggatcctacatccgggaagcaagcagacgggccctcctcccctccctcgcctggcgcgcggcgcctgggttctcatcaccacgggcccagtgctcaccgtgcgcggggctgtaggagacgcgcgcccgcgcgtgagcggggttggcatagtaggggttgccctgcg

SEQ ID NO: 64 - DNA, 1100 bp, Artificial Sequence
  subsequence of ADCYAP1
gaggcaaaaagggaacgcgagccagggagtttgatccgttttgaatgaaaagaaagagaaaccaaaccaaacctctcagtcatccaaaaccttcaggcttccagggaggttttgctataattttctctaagcatgactgtttctgggggaggggaaaggggtggttgtatttactgaaaattcaaatcgaaataataaatggccaaatgtggacacttatggacccaaacagttttgctcacgccagagaaactgagagcacagggcttgtgtgaagcctatctcggcagaaggcaacattctaataaagcccgtgggaaaacagattacattttcgccatgaataagtcatgcagtgaaaaatattgcctacagcctgtcgacttatattattatcacgtttttcaactcggcgtgaggagggagaggagtgttcatatttgactaggaattgcaggatcgatgcaaactccagggcagcagccagactggcatatgtagggctctccggttactttctctgtatgtcgcgggtgagaggaacagcgaggacaatttagcgcaaacacacgaagggtcggatctcaagggggcagcgctgggagaaaggttaggcttgaagcgcgcgtcgcctgcccggatcttatcccgggccccctccgcagggtttggtgccaggagatcctgcgtggggaggggggcatcgaggggctgccgtctcggccctccccacggctgcttccaggcagaggcgggcgacgcggtgggcagtgcgagccccgggccctccccgaaggctcccgcgtggggtggggcccgcctgctccccgcggcgattgaacctgtgtctcccgccccgccaccctcttcccgacccctttgcttgcagtgggagcctcggcggcggcgcgggggacgacgcggagccgctctccaagcgccactcggacgggatcttcacggacagctacagccgctaccggaaacaaatggctgtcaagaaatacttggcggccgtcctagggaagaggtataaacaaagggttaaaaacaaaggacgccgaatagcttatttgtagcgatgggttaccagctaccct

SEQ ID NO: 65 - DNA, 963 bp, Artificial Sequence
  subsequence of TBX5
gtagagaataattattgtaccagggcccgccgaggcacgaggcactctattttgttttgtaatcacgacgactattatttttagtctgatcaatgggcacaatttctaagcagcgcagtggtggatgctcgcaaacttttgcgcaccgctggaaacccactaggttgagttgcaaaacgtaccgcgtagacgcccctggtggcgccgagagaagagctaggcctgcccagcacagagccggagagcgtcgggccttccggaagggtaagttctccgccaaggggtcccgagggagctggacgtctgaatctggacttgcccccagcttcggggttcgattctgggttttgcgcgtccccaacccccagggctttccgaagcatggcctggctccaggcccggtcctgtaaggactggaacggcagcaaaatgtgcagggaggcagtcggccggcagagctgcggcgggagccaaggtcaggcccgcggggagagcgggcagcttccagcgccggccacaagctcccaggccagctgggccgcagacccctttgcttccagagagcacaacccgcgtcctttctctcagccaggctgcagtggctgccccgagcttcgctttcgtttcccaagctgttaataacgatatgtccccaaatccgaggctcgtgtttgctcccagatgccaagaacgcaacccgaaatccttctcccaaaccctaggtcgacgagatgagttcctacttgacctctgagccgaggtgggccggaaaccgaggcctaggccccgccggggctgcaaggaaaaggggaaactccgagcgtagcgtcttttccttgtggttcctttctccggcatcccggactgcgggccctgcagccacctggaccggcattcaaaggattctgcaagtccagcttcacagactggctttcccagacgctccgaagcccgcaccacgaa

SEQ ID NO: 66 - DNA, 837 bp, Artificial Sequence
  subsequence
ccagcccttacccacacctttgtcacgacgggcaattgggtatgtgtaggggaaaaacagcaacgttaaaacgcaactgtgtaaatgaggatagagagtgcgaaaggagggagaggcgaggagctgctctatttctagggaggttttggggagactgatcagctccaaggacagaccgctgggaagggaaaaacggcccacatcgaactggatgccggatggaaacctctctgcgctattagactgcgtccagtacagcagatggcacgagcacgtgcggcgctcagcttaggctctcggaggcagctgagttggaaatcccgacggaaagcacccacaagctcccactctgcgctggcccacccgcgtgcacgcccaccccccacgcgcgtccctggctcagaagcgcacagatgtttactgcttagagccggtaccgctggggagatcgagcgacttgcgcggcgcacagtgcggcgctggcagggctctgggctcccggtcgggggttcgagcggccaagggatgggggtgggggcggggagagtggggggagggcgaaagaccgccgagaggaggggggagtgggtggactaatgatgaaaaagtctcctccatcccagttccttaattaaatgcatggaaagaaccgaggcgagcacatctggtttcaatctacagccctttgatggcatcaaatgttcttttcccagatcagggctggaagttctgggctaactatggccgtttggagcccagaaaccatttacacacactcgtacccttctttctctccagtcgagcctcttgactataggacgaaaaaaaaaaaaagtc

SEQ ID NO: 67 - DNA, 1012 bp, Artificial Sequence
  subsequence of NECAB1
cttgtgactttgggaaacttcatatttgaacattacctaacaatccttgccccatagcaaacgtttcgaagcctactctaggcagagttcatagcaccgcctttgtcagcagcactgccataggtaagcctcagaaccctctggggtgagaccggtgtaaccattttactgatgaggaaaagtgaggcttacaggttaagtccttcgagcgcaagataacaccgaatggcttaatccctacaccaaaccagctgctcctcgattgctggtattcgtgaaccctgcccccgcctttggggaaggtcgggcagacaggccactgggaccaaaagcagagtaggtagaacctctctgagttcctccctatttatggcatccactcaggtgaggctgggggcgtccttaccttgcgctttggctgctcaggacaaacgccctgccattcgtcccttctctctgtccggacgccctcctccatccctgcacttggggccgtcgtggggctggtaggggtccccaggctatctccagccgtggccgatggccgtgccgggggcagagcccgctcccctccgcgcgttgctacgtgcggggatgacatggatccagacgccgtcaactacgggaaggaggaggcgagagttggagcgcgtgggagcgcagaggccggaggagggagggggggacaccgagcgcggagagcgcggagagcgcggagggaggcgcgcgcgggagcgaacaccctcccggatccagagcccggcggcggcgaagcagcagctgcggccgcgcccttgccagagccggtgcgtccgcctagccccgctccgcctgaggccgtcagggctcccgaggatggaagattcccaggagacatcgccgtcctccaacaactcctcggaggagctcagctctgctctgcacctgtccaagggcatgtcgatcttcctcgacgtaagtacagatggtgggagctgggcggttgcttcccagcacctttcttttccccgaa

SEQ ID NO: 68 - DNA, 1017 bp, Artificial Sequence
  subsequence of ADRB1
cccgagccgctgtctcagcagtggacagcgggcatgggtctgctgatggcgctcatcgtgctgctcatcgtggcgggcaatgtgctggtgatcgtggccatcgccaagacgccgcggctgcagacgctcaccaacctcttcatcatgtccctggccagcgccgacctggtcatggggctgctggtggtgccgttcggggccaccatcgtggtgtggggccgctgggagtacggctccttcttctgcgagctgtggacctcagtggacgtgctgtgcgtgacggccagcatcgagaccctgtgtgtcattgccctggaccgctacctcgccatcacctcgcccttccgctaccagagcctgctgacgcgcgcgcgggcgcggggcctcgtgtgcaccgtgtgggccatctcggccctggtgtccttcctgcccatcctcatgcactggtggcgggcggagagcgacgaggcgcgccgctgctacaacgaccccaagtgctgcgacttcgtcaccaaccgggcctacgccatcgcctcgtccgtagtctccttctacgtgcccctgtgcatcatggccttcgtgtacctgcgggtgttccgcgaggcccagaagcaggtgaagaagatcgacagctgcgagcgccgtttcctcggcggcccagcgcggccgccctcgccctcgccctcgcccgtccccgcgcccgcgccgccgcccggacccccgcgccccgccgccgccgccgccaccgccccgctggccaacgggcgtgcgggtaagcggcggccctcgcgcctcgtggccctgcgcgagcagaaggcgctcaagacgctgggcatcatcatgggcgtcttcacgctctgctggctgcccttcttcctggccaacgtggtgaaggccttccaccgcgagctggtgcccgaccgcctcttcgtcttcttcaactggctgggctacgccaactcggccttcaaccccatcatctactgccgcagccccgacttccgcaaggccttccag

SEQ ID NO: 69 - DNA, 1030 bp, Artificial Sequence
  subsequence of OTX2
ggcggcccccggcccaggccgacccgcaagcgaaccgagcttccggcgcgcgggcccaaggaggcgcctggctttttattattgttgtttcaatccatccatctagttacatctgcatctttttgtctcggactctaaaaaggtccctgggatccatccaaacgaccccaaccaaatctgggggccaaaacgcaaagatcgcgggagaagcccagaacggcgttgacataaaaacaaaaccacaaacaaaaccttccaaaacaccccagattacattcgcagcgtttcgacgacgttttgcagaagcgacgacccccaggagcacgctctctgcctctctcccactaccgctctcatctctagatcacatttttctttttgcaacgatcgttattacacctcaaaatttgtaagagaaaaaatacatccgcctacagaactccacgttcgcagaggggcatcggtcggtctattggaggtactggggtgatggccgacagacacggggacacgtagatatggatatagacaagacagacggacacttaccttacagcctcatgggaggttagaaaaagtcaaatatcctttaaattccaaatagccagctatcctaaaagaaatcaagagtattgagttagaaaccttgcagtcttcacccttccatgaaaagtcaaacacaaccaaaaaaaattttttttaaagaacgaaaatgaggaaggcggctagagttctaaacacgcgtgggcccctctgcaatacatacaaagtagatgtggcgagtgagggctgctctagcaatttttatttttaatcacagtggaggctgtgttggagctgaggccggtcccgctctcagggagatttgctgagaaagcgcctctctggcaactttttgacgcaaactctccaaccaatggcagggagagaatgattgacacatctaagccagagggaaaataataaaaacacacaacagggggaggaaaacaggccgctgctgcacggggggacgagcaggcaacaaatc

SEQ ID NO: 70 - DNA, 1076 bp, Artificial Sequence
  subsequence of NKX2-6
aagtgaatccttgagattcagggccttactttcgttaggggtgtgtgaagcacactgggtgtcaggagaggatgggaatgggattcgagaggcctttttttggactcctcgagagaaaatggagagagtctcgaacccaggagataggaggcgtattttccccatgcacccatggatcacgcccccgcccccacattccccccgtaggaggcaagacctgagcgcttactcacgtggctcccccatccgttccgcgtccatctccaagactgcctcacagggacccccaggaggctccgaaccatccagctttctgtcaccgccgccgccaccagcgttgtgaacctctgaccctcgcggctctgcgtccattctcaggtactgaaagttttccgggctcttccgcacccgcggatgtggcgaagccgcggggcagctccgctcgcgctccagtcgcaggatgtccttgaccgagaagggggtggaggtgacggggctcagcagcatcccgaaggcggatggggcggggccgaggaggtccgggtgaggagcggcaccctgaacttcccgtcttgtcgctgcaggccccgcagacagacccaagctctgggacagacgcccagcgtcccagacagcgccttcctctgggccatgctggtaggcccgggtccagggccgggtgacgagaccgtagccccccattggttctcgcagaaaccacgtgctagctctgcaccttcctcccccagcgctttcttcccgcgcccgtcgaatcctctccagtccccagtcgccttcctgggaggtttggttcgtattgacggttctcaaagcaaagaaaacgtggagagacagtgctgcgcgcggcttggatctccgtcaatacggtactagcgggagcttccgaggtcaacctagggtccacggggaccctcctagtggacatgcggggattggaggtggagtccttgctgtgcaacccgatccggtccatccagcctggtcttagctcaactctgcattcttatggcggaggaaagctaagatagagacagctgggacccgcggaatttgag

SEQ ID NO: 71 - DNA, 927 bp, Artificial Sequence
  subsequence of SIM1
ttgatagagcttttccttcggaatgaatttaatacccttgacaaaatatatattacagacccgacatcatcaccgccctcactctgacaggaagaggaggaagataagcgtgtgttctgttcttttaaaatttttctttattttaataaataaacgctacatctcaatagaaatgtatcctccttgcagtccttcccgggaaccttcacctccccaactaattgaggtgccttgtaggcaatgggggagggtggcggaggccctgttccatgacctgactacgacttggtgactgaggaggggaaagccctcctaggccgaggccactgcggttcctgaacagcttgtctcaaccaactgtgtatcccttgagagagtgtaggagagtctggcccagggggtaatcctgaaaaccccaaatcccatgtatcctgccgggcctgcacatcctcgctaaatgtgtactgtgcaagtcttccccgggctgaggcgtcgagtggccttcgtgttcagcctccgggcgcctccgcagccgagctctttagagaaaaaaagagagggaaattggtgcaaccagcccgaatcaagctcctagagcagtcactggtaggaggtcccttcacgcaccaaggcgcacccgaccccacctctggcactgctgcccgccctgcctgcggccctctccggctaaggagcctgtgtggttgacctgagggcatcggcgagcgcgccgggccaggtcttgttccacgcagcagcctggaccccacagtgtgtgcctgcactcggcagtgccctgatctctcctgcctgctgatcccgggccagagacaccgcggccgcacccagggaatccactaatgttactgtaaatgtggggtggaggccgaaggtcacaccgctgtctgtctctctctttctctctct

SEQ ID NO: 72 - DNA, 927 bp, Artificial Sequence
  subsequence of DRD4
acaggcagatgcaggctcagccccctggctgccgtgggacacacacacacacacactgccacagccactgcccaccacacacacctagtgcagatgctggcacacccccagaaggaggctcacagctcgcaggggagacctgggctggacaaaacccaggggaggggagggtgtgtggggaccaggcccctgctgagaaccctggggggaagcctgagggggaattgggggatggagcccacactccacaccaggtctggccctcgagtgggtcggccttggtgccagcccctctgcggccagagaaaagcagcttagggctgagctggagacgcggtgtccccgactgtgggggagggggactcgaggtttccccttgatggacacagtgaatccaggcggctggggcagagaccagcagcacgggacacgcgtgacctgtgctcctttcgagccgcagacgtcacagtgacgacgtttaagctcctaatctccccaaatcggcgggaaggattagaggggctgcctgctcctttgcccttggagagagtcactccacgtggagtcctacgctgggcactgggcacggtcttcatatttttaattataatttatcttcaagacaattatgatgtggatactatcatcacccttgtcttacagatgaagaaacagaaatgaattaacgtgcccgagtctcccacagagaacttagccaacagagcagccagcttcgcttctaggcccagcggggaccctgcctaccccaggctggggaggggctccctttgagcccgatgatatcaggcccgcccccagggaattccccaggccgttctcatgtttgtaacaaaagggagaccaaggccagaagccgtgattcacgcctgtaatcccaggactttgggaggcaaaggcaggaggata

SEQ ID NO: 73 - DNA, 810 bp, Artificial Sequence
  subsequence of TBX15
gaaaaggcttggacggtcgaaataaatctccttttaattttcttttcatcgactaataaaaataattccccagcactaaactcaaataccgtaacgggccacaaaaacacggagaattcataaaactctatctctgcaggtcacccgctaatcgcattattattagcctcgggagcatggaaattgaactgtcactgcctaaagagaaaatgtaagcgacagctgtccctcctctgagttggacagctttgtggctgagatccccaagctcctgagccccagaccgtctctatcccagtgcaggccgctgccccctccccgggcttgtcagcgtgtgaagcggggtctactccccagctctggctgttcagcaggagcaccttccagcatggttttagaagtccgggctggaaagcttctgaaaccgctaaaccaagttgcgagcgttgtatgtgcgcgcgcgcacactcaagattcttccgacaacagctgttcccccgggctgtttttgcacagttgaaatcttggcacttaacacaaaacgttaaagttggcttctcccctcctagggttctgttaaaatacagacatgacatcccccctgctttttacatgttccgtgcacataatatacatgggttactgtaggatctgagacacaaatcaatcgtacccacaccctaaatacacagagatgtgggccctgaagagtgacccaaggagtaaggggtctaacatccattcttgtttccgtaaacgccaaaggagtagaaatataattatgttccaccatcgaaaagttggtgggag

SEQ ID NO: 74 - DNA, 1080 bp, Artificial Sequence
  subsequence of TRH
tttctctctctctctctcttgctctactctcgcccgtctgcgttctacattggttctgcggccgtgtccctttcgtgtgtgtctgccctgtgtttctccgtcgtctccgtgtggatctcggtctttgtctcgccctctagctctctcgtgcgcctgtgtttaatcgtgcgcttctctcaatctctctgtccctccctttgccccctacacgcgtgttctcgtcaacagatctccagaggtggtgcagaaacgaccccgcgccggcgccccatcctgcggccagtgcctccgcgccccggctccggtccccaccgtccccgccccagatttccggaggagcaggcgggcggggtcccgcggggccggctgccgtcagcgccccttcccggcggccgcgacccctccccgctgacctcactcgagccgccgcctggcgcagatataagcggcggcccatctgaagagggctcggcaggcgcccggggtcctcagcgctgcagactcctgacctgccgactgcggatcccgagtccccggatcccggacccatcctgtggagcccactcctggcaggtaaccgccccaacccctctccttccgcagacggtgtccgggagcactggaaagggagccctctcggcccgccctcaccttcggttctctgagagcttcctggagaacagggccggtgcacaggcgggcgctgtgctcgcacccccgggtcctccccgagcgcaggccggggacccgacgggaggcacggcgcgggcacatcggaggctctcgctgctgggcactcaggtcgccagagtccgcagcgcggggtgggagctccgcggcaccccctgcctgggtgccgccggacagagctgggtattcagggcgtcggcctgagaacctgggagttcgaatcccaatctcaacgctagaaatagaattttagcgttgaagttaggattttagcgttagaatcagattcctggcttagtcatgaaagcttagcattagaaatagaatcttagctttgcaaatagactttgagctttagaacctgaatcttagcgatagaaatgggatctt

SEQ ID NO: 75 - DNA, 1050 bp, Artificial Sequence
  subsequence of FBP1
gcaagaggattgcttgagcccaggagtttgaggctgcagtgagctagtgagaaacctgacttgggtccctaattgcagaaagagtgaaggaggacaaagaagaaatggggaaggaaggcacctgagctagcactttcctgtctgaggctagggcgggtatgacgggcaggccaggtgcccacacttggccggctgagaggggtacgaggcaggctgctcagggcagagaagaggaatgcaagatggaatcaggtgtacacctgtgagacggacccccaggtgggcccctccaaggtcaagggaggagatgaggacttgagtgaggctgagccagcttctggagagaggggctaccagacagagagcgagagaggcgctcagacatcagacggacagacagaggctgacggcaggaggctcagagggcccaacgtcagcccgccgggcaggctccccaggcagacagacaggacggggcccaccgcccaaggcccgactcacaggtgcgcgatgcccgccttgcgcaccgccgaagagatggctttgactgctgtgcagagcgagttgagcagctgggtcaactcgcccgtgccgcgggccttcctgccctcctccatgacgaagcgggtcagggtgttgacgtccgtgtcgaagggcgcctggtcagccatgcttgaaccgggtagagcgcggggctgcaggtgcaagcggcaggtgcggggctgcaggtgcgggcggcaagagagggcagtaggcactggccgcaggtgcggagctgcaggtgcgggcggcaggtgcgggccgcgggacctggcgggaggactgacagaccgactgccgccccgagtgtccgcagcgctcgtggtgcaactgggccaggccaggcgccggcgggtgaatcgcggaaacctttagacgcgggtcggccccccgcccccgggaacactcttgcgccccgcctaccccgcggaccagaccgcggctccgcctgcttggatcttcagacaaggtcggggatcctccctgcggtctcccaacccccgcccccac

SEQ ID NO: 76 - DNA, 968 bp, Artificial Sequence
  subsequence
caccccgtggtgccttccctccccgccctacagccaagcccagaggaacagggcatcgcctcgcgcggtcccggagccacatccggacttgggaaccccgtgtcgggcttagaggacttcactgggcgggttggggtttattttcaataaattcagctgttcacatacacccccaccaccatttccacgcgcgcgcgcgcacacacacacacacacacacagagggacttgtcaactattgagacagcgacccagaaaggtgtaaattcacctggtgcccacccaattgcaaagctcccagacccacacaaaacactagcgagccctggaggtctgagacgccccgcgcccgactcacggcgcgaacaccagcgctccggccgggtcgcaggggccggtgcccagcgggccggggtctggcgagccaggcagcgggccggctgagctcctgcgccccgcggtcgcgtggcctactcgcctactcccttattattggctgggacctgttcctttccaaagtgtgatgcccggtgtcctaccctaggccacgcggagctctctcccggcgtgtcgggccctgcgcccctgcccagtggctcacctcggctcgctgcgcccgccttcgccccaagtgcccaggacggagcgaggggctgtgggtcggcgcagggacgctggctgctcacctccaggagccgacagaaggtgccttcggcgtcacgcgtccaaccctggggctgatttaaataactaataagctcagagaaattttacgaggggaacttttccttttagtatcaataaagcctagtaattgggtttgttggttacctaagctcgagttcgactttctcagtctctctctctctctctctttctcattcagaggcaacgttttcaaaaaccggcaattgcgtgtgcgtttggggtgtgcaagtgtgagtgtagatgtgtgaaagttatttgtt

SEQ ID NO: 77 - DNA, 1080 bp, Artificial Sequence
  subsequence of BCAN
cagcctctcctcacgctcgcgcagtctccgccgcagtctcagctgcagctgcaggactgagccgtgcacccggaggagacccccggaggaggcgacaaacttcgcagtgccgcgacccaaccccagccctgggtaggtgagtgcctccgcagccccgccgcccgccgtggggtcggggacagggagaagggagtgcctgcctggtctgcgccccccgcctgtcagcccttgcctcgaggctctggggcacccaactcgtcgactcctgacaccgcagcggggtaggctgctggacagccccgagcgcctgcagctgctgctgccatctctgatctacatgcttccagctctgccagtggcagcccccctgctgctcgcagtctgatcagcaacccctcgggtcctcgcatcttccctgctgcgcgctcctgtcccagcgcggccgccgagatttccgaccttgtcccaggcagggcggtagcgttccggatcagtccttgcctccgtgcccccacgcacaggcagctccaggagcagcggccagcaacccttctggggacaccttactgtagtccggcaggacagccgatcagagccgctctagggggtggtcggagtgcccatttcggctggaatcccaactcggctccttgctctgtgaccttggggtagttagttgacttctctgaacctcgggttcctcatcggtgtaatgagcaaaacataaacaatctttttctcacagttgaggttatccacaggaagcatttaggagaactggctcaggtagacatcagtaactattagctggaattcggttaccactattgcattccttcctagcactgccaggggcctgggaattccctctcccaggtatttccatatcctgtcaggtattcccccacctattggaatagctctgcctacatggttctaataggaccaagagattggcgtcaagtccaaggggcaccattattatctgcattacttagattgcagatgatgacagtaagatcagggaacagtgttacccttagacccacccacagtattaccagtgcctatgttgctatg

SEQ ID NO: 78 - DNA, 1017 bp, Artificial Sequence
  subsequence of TP73
ctcccaggtcagggcccaggccccgcacaggccaggagtgactctggtgggctctccccctcccccgtctcctgcctactctggttgggggtgtaggggccagggtgtggtgtggccagacctccaggcccagggcgaccccccctgctctccctgctccactgccccctgcccctaatgcgccggcctctcgcaggacctgggggccctgaagatccccgagcagtaccgcatgaccatctggcggggcctgcaggacctgaagcagggccacgactacagcaccgcgcagcagctgctccgctctagcaacgcggccaccatctccatcggcggctcaggggaactgcagcgccagcgggtcatggaggccgtgcacttccgcgtgcgccacaccatcaccatccccaaccgcggcggcccaggcggcggccctgacgagtgggcggacttcggcttcgacctgcccgactgcaaggcccgcaagcagcccatcaaggaggagttcacggaggccgagatccactgagggcctcgcctggctgcagcctgcgccaccgcccagagacccaagctgcctcccctctccttcctgtgtgtccaaaactgcctcaggaggcaggaccttcgggctgtgcccggggaaaggcaaggtccggcccatccccaggcacctcacaggccccaggaaaggcccagccaccgaagccgcctgtggacagcctgagtcacctgcagaaccttctggagctgccctagtgctgggcttgtggggcgggggctggcccactctcagccctgccactgccccggcgtgctccatggcaggcgtgggtggggaccgcagcgtcggctccgacttccaggcttcatcctagagactgtcatctcccaaccaggcgaggtccttccaaaggaaaggatcctctttgctgatggactgccaaaaagtattttgcgacatcttttggttctggatagtagtgagcagccaagtgactgtgtctgaaacaccag

SEQ ID NO: 79 - DNA, 1058 bp, Artificial Sequence
  subsequence of MIIP
gcctcccgagtagctggactacaggtacgtgcctggctcattttttgtagagacggggttttgccatgttgcccaggctgggtatcttttttttttttttcttttttgagatggagtcttgcgtcttgctctgtcatccaggctggagtgcagtggcgcgatctcggttcactgcaatctctgcctccctagtagctgggttcaagcgattctcctgcctcagcctccctagtagctgggattacaggcgccggccacctcgcccggctaatttttgtatttttaggtttactggcgtgagcaaccgcggccggccccaatactacactttcttgtttactgtgtagtccttatcttctggcgcaaagcgggcactcgctaaaaacctgaatgaaagtataaagcaggccgggcgcagtggctcatgcctgtaatcccagcattttgggaggccggggcgggcggatcacgaggtcaggagttcgagaccagcctggccaacatagtgaaaccctgtctctactaaaaatacaaaaaaaaaaaaaaaaaaaaaaaaaaaaaaaaaaaaagccgggcatggtggcgctcgcctgtagtcccagctactcgggaggctgaggcaggagaatcaatcgcttgaactcgggaggcagagattgtggtgagccgagatcgcgccactgcactccagcctgggcaacagagtgagactccgtctccaaaaaaaaaaaaaaaaagaaaagtatgaaacgatgagtacaatgagtagccagccgcctgccccacctaccccgccgttccggactgccgcctgcgccgagcctaggccgcccagcctgactgaaactgccgctgctgaactcagcgtatccagtcccgcagctgaccaatcggagctcgcccttccggggcccgccccattccaggaatcgacctccgcaccggcctcgaaaattgaccaatcggttgtgtagctccgctcttagtcccgcccccacgctgaaactgacacttcggatcgccgagtaacgctcaccagacgtcccggccctgcccct

SEQ ID NO: 80 - DNA, 1166 bp, Artificial Sequence
  subsequence of HOXC4
cccggcctgggtccgaggctccgaggcggccccataagtgtgaatttctgtttataaacggcgacgcacacgcaaacgcctacacacccaggcagacacacccggaggcgtgggggaacatattccagacgaggtccgagagaacctgggggccagacttaccttaatctaagccaagacaccccctctacccccaccctctcccagaggcgcgactgggattctgcgccaagtcccagtgggggaggggatcgctccacgatttcctgtttaaaccctgacccgtcgcctgtgggggggcggggatgggggaagaaacctgtttttatcaaatttttaaaaatacagtttgcattcagatcaaaccgtttgggccagagctgacggtgaattttatctcccctccccccacaacccccttcccttccttttctgcccccgctaaattcccctttcgcagccatcataaaggcctctgaggtattctcccgcgggaagaaatggcattttctctccccctcccccacccccccacccccagtaggacttgtgtgtcggcagaggcgtctgacgaggggctaatttcgctttccttgtttacgatcgagaaaagcgcttggctctccccaaatgggcccagcccgccgcctgctcaggctgccgcgcgctctcccgccgctcaggcacggcccagtggctgatgccccgcggatccagcctgcggcaggccggaacccggagtctgtgggacctgaaaagggcaaagggagtgcggtgggacacaagaggggcccgagaggcccgaaaaagggagcctttctcctggagtaatgtgggaatcgccgaccggtgaggcctctatttctctctttcgcctgcattttgtccgcccccgcccctgtggatggccgctgatgggggggaacacaagtgtcctttgtccgtccccgaaagaaaaccttttccagagaaggccattcaggccagtggagattcacctagaatattagaagggccccctcccacccgaggggcgggcctgggcgaggctgaggtatttctcttaatcctagaacgacctcactgagtgtacccacagcgagatttggaggtgctagagttcgaggttggccgcttaacagcaccatcctgaggtgtctttatat

SEQ ID NO: 81 - DNA, 1334 bp, Artificial Sequence
  subsequence of HOXA7
ccggccccgcgccccgcgctccgcgctccccagcgctgcgctccccgctcccggtcccgctccgccagcctggcccgcctagcgactgcgcctacctgaagaccgcatccaggggtagatgcggaaattggcctcagccgcgccatgcagcgcgccctcgtccgtcttgtcgcaggcgcctttggcgaggtcactgcagagcccggggatgttttggtcgtaggaggcgcagggcaggttgccgtaggcgtcggcgcccaggccgtagccggacgcaaaggggctctgataaagggggctgttgacattgtataagcccggaacggtcgaggcgaaggcgccggcgcccgccccgtagccgcttctctgtgagttgggagcaaaggagcaagaagtcggctcggcattttggaacagagaagcccccgccgtatatttgctaaaaagcgcgttcacataatacgaagaactcataattttgacctgtgatttgttgtccggcagctttcagtgtcggttttacgaggtagagtgatatatgataacattacacccccagatttacaccaaaccccattttcttttggacggagctcgccgcagcacgtgaccgcccacatgaccgcctccgccaatctcagcagtcctcacaggtggtctcgctccgcagggcccgcagccgcctagaatggaagggcaagaggctcaaatatgcggccaaagaatccgcccgcgcccggcgggcctggcgcgtcccgcggaaaaagacctggaggctccgcgggagcgcccagctggcggccaacctccgcactggggtctgcggacgccaggcggcccggccccacgcagcaccccccaccccgcccccccgccgactcctgctagtgagccctggaccaagcttgggatcctccccatccctctcctgtccgcctgcccagaccctggaagggtctctgtcccccgcaacagcctgccccgcggtggccttgtgggcaggactcagctatgagcagatcgactctgcccaagtcttctctcacccaggtccagtgggcgacaggccggacttagactcggatccagacggggaaggcgcagcatctcttgcagctgcagagagattgccaccgcaaactggagccatgtggttcgaataaagtcaacgtctcccagcttcctttccttaatcggaggcacactgtttatccgccctaaaggaagcagtgaaatatttatctattaatgagactcatttgccaacagatttattaacgtggggttcccctccctcctcccggacgctgtagtgctgcaggctctgtgccttc

SEQ ID NO: 82 - DNA, 1181 bp, Artificial Sequence
  subsequence of BST1
aaagagggcatctgtcaaagttgtcgtcctttggagccagaaaagtatttcttctgatgatgactgacctctcctcacctctccttcaaccttgcggcttctttggggctccctccccgtggacagcggtcaagattagcctgggccacagtgcactggtcctgtcctgggtgatgttccaagctcactcttttttaattttatttatttattaattttttttttagacagagtctcactctgtcgcccagggctggagtgcagtggtgcaatcactgctcgctgcagcctcgatcccctggggtcaagcctcctcacatctcacctcgcaggtagctgagactacagatgcgcaccaccaggaccagctaagttttgtatttttttgtagagaggaggtttctcacctgtatgttactcaggtttgtctcgaactcctatactcaagcgatccgcccgtctaggcctctcaaagtgctgggattacaggcatgagccgccgcgccccgccccacgctcagtcttgaaattgtctggaacgggaaacggcaaacagcgagatatccgagcgagagtcccgccctgcatcagtttgcggaaccgccttggtagaaggagagaaggggagtggaggaagcacgggactggagggaccaaagttccccgatggcggcccaggggtgcgcggcatcgcggctgctccagctgctgctgcagcttctgcttctactgttgctgctggcggcgggcggggcgcgcgcgcggtggcgcggggagggcaccagcgcacacttgcgggacatcttcctgggccgctgcgccgagtaccgcgcactgctgagtcccgagcagcggtgaggcagtcggccgggtggaaggggagccggaaagaggcaacggtggggagggcctggggaggggaaaactggcgctaaagttcggggtgagggggcaatgagagaggccttgaggggagaggtgagtgtggagacagcgatggtcctgaacgatgggggcgagtgaggagggggctgtgaagtgtgtctgcaggtgaggggtgcgctgtgcggggtctagagatgagtgtgtgtgtgtgcgcgcacacacacactgtagaggtgaggggtgtgtgcgtgtgttctagaggtgaggggggtgtgtgtgtgcgcgcgctctagagg

SEQ ID NO: 83 - DNA, 1039 bp, Artificial Sequence
  subsequence of C1orf114
aggtaccaccaacgaaatgaataccattgcctcctcatggaagctacaatttcgggagtgactttttctcccagggacaaaattattactttccacgttcaagaactttgagaggggaaagaatatgacaaaaatttagtctaagctactctcagacgagtatccttcatacatagtgaagaaaggtgttaccagacttccccaccagtgccagactcggtggacctcggactccagaggataaggcgccaccagaaagcttcttccctcactacctaccctccctcccagctataccagacgtttatacctttaccctctatcccaccattaacatctccgcatcgtccttcccttctctccctctatatccctcttgcctgtgtaaaatgcggcggctgggatcacagagatggccgggggagttctcctctcctcctctttctaagctcttcacattgaggcaaaggagaccccggcacctgcctccgcggcagccaggaccacactgccatggcaacagcgtgcctctgcgtcctccatccgggcctctctaactacgagagcgacaaaaatctgcgcaggcgcatgcaatatcctcagaccaccgacccctcccggcacccatcccggtgcttgcgaagggccagtgaagctgaggtttctaaggggacgactaaggaatccacgcatcactaacgttatagagactcgcgaagtgccgctgtgttggttgtgaaatttccctcttgtagctgtctctcgtcagatttagaatttcttaggacaacttctaaaactatatttctatatgttatgtgcttcacagttaacgtagaaaagtagtttttagttttcattagtagataagcaaattgctaatgagttaccatatttttgaccctcagcttctttttttcctaatcaaaaccaaaactttacccaagagagttgccaaagaaaataggatttttgctctagctttgaggcatgtcaaaatggtcaactagaattttctcaaattctgcttatctttatg

SEQ ID NO: 84 - DNA, 1027 bp, Artificial Sequence
  subsequence of FOXG1
ctgctcccgccgccgccaccgccaccaccggccgccgccctggacggggctaaagcggacgggctgggcggcaagggcgagccgggcggcgggccgggggagctggcgcccgtcgggccggacgagaaggagaagggcgccggcgccgggggggaggagaagaagggggcgggcgagggcggcaaggacggggaggggggcaaggagggcgagaagaagaacggcaagtacgagaagccgccgttcagctacaacgcgctcatcatgatggccatccggcagagccccgagaagcggctcacgctcaacggcatctacgagttcatcatgaagaacttcccttactaccgcgagaacaagcagggctggcagaactccatccgccacaatctgtccctcaacaagtgcttcgtgaaggtgccgcgccactacgacgacccgggcaagggcaactactggatgctggacccgtcgagcgacgacgtgttcatcggcggcaccacgggcaagctgcggcgccgctccaccacctcgcgggccaagctggccttcaagcgcggtgcgcgcctcacctccaccggcctcaccttcatggaccgcgccggctccctctactggcccatgtcgcccttcctgtccctgcaccacccccgcgccagcagcactttgagttacaacggcaccacgtcggcctaccccagccaccccatgccctacagctccgtgttgactcagaactcgctgggcaacaaccactccttctccaccgccaacggcctgagcgtggaccggctggtcaacggggagatcccgtacgccacgcaccacctcacggccgccgcgctagccgcctcggtgccctgcggcctgtcggtgccctgctctgggacctactccctcaacccctgctccgtcaacctgctcgcgggccagaccagttactttttcccccacgtcccgcacccgtcaatgacttcgcagagcagcacgtccatgagcgccagggccgcgtcctcctccacgtcgc

SEQ ID NO: 85 - DNA, 1017 bp, Artificial Sequence
  subsequence of ATP4A
acgagggaacggggcggggctgaggagaggggcggggccgagagctcggtgcgggctctgagagctgcggggaagggtgaaggtggaagatggaggccttgtgtggaggggtccttggtagaaggtaagcgttaaggcggggctaggtgcagatttggagtcctggacgcagggaatgaacagaattagggtgcggagttgggctgggggcggatttggagagcgaggtgctccccatggacagtcccgccgaggagaagctgtgggcggggctgggtggtgggcggggccttgcctctggtggacggggccataggcggagcgggagatggggtggggtttggctgcggagagaaggggcaaggagcgaagcccctcgtggcccgctgatgtgggtgtggcctggggcggggcccgaggtgggcgggcccaggccgtgggcggggccggctgcgcacctggaacttgttggtggagttgaagggtatctcgcagacttttgggaagcggtcccggtagcccatggcgttgcccagcgtcagctccgagaacttgagcagcgccgtctccgatgcgtctccaatcacgatgcgctgggagcggggaccggtgtcaggggcgaagccggctacaccagcctcccgggattccctggaggccccctggctctcaccttgggcacaggcactgcatcctggccggacttgaaggcggcgcggttgcacagggtgagcacccggcacagcgcccgccacgtctccgaggactggtcaaacgtctgccctgcagaccaggcgtccaggctgggtcccgcacggcggctctcccggaccagaaccgagccccctcctcctaggctcatatcgcgggccccctccccagacctgggtggaattgggttccacccaaccctgagggacccagcccccggatgacccttccctctagacccggtagcgagtctcctttgagacctggagccgagccgccccgccttcgtacaaagccctccctacc

SEQ ID NO: 86 - DNA, 1161 bp, Artificial Sequence
  subsequence of NOTCH1
tttataaacacagaagaatcttttcatcctacgtaggaaaaccctggctctcagaacttgcttgttttctcagaatagataaaagtttctacctggggccagataaaacagtacatataaataaaaaggcagtgtttctgtgtaaaataaaagtacataaataaatactaaaaaaaattaaaatcctcgttcttattttgtataaaaacatgtgttttaaaaaggctcctctggtcggccctggcatccacagagcgcacacagacgcccgaaggcttgggaaaggaagccggggtctcgtggggcgcgccgtttacttgaaggcctccggaatgcgggcgatctgggactgcatgctggtgggagggctggagacgccctcggaccagtcggagacgttggaatgcggggacgagctggaccactggtcaggggactcaggggacggggtgaggaaggggtgctcaggcacctgtagctggtggctgggggtgttgtccacaggcgaggagtagctgtgctgcgaggggggcgtcaggaactgggctgcggtcacgggtgggaccagcgaggatggcagcgacgtgggcagggcggggctctcctggggcagaatagtgtgcaccgccaggctgctggggcccagtggctgcacgtctgcctggctcggctctccactcaggaagctccggcccaggtggccgctggctgctgagctcacgccaaggtgcggctgtggtggtggtggtggcggctgcaggctttgctgctgctggatgtttgctggctgcaggttctgctgctgcatctgtaagttttgtggctgcacctgctgggtctgcaccaggtgaggctgggtggccagccgggtgctgggcaggccctggtagctcatcatctgggacagggcgctggcagcaaggctactgtgcagcgggcctaccatgccatgctgcagggagggggcctgtgtgctcagggggcctggtgccacactcccccgcagagggttgtattggttcggcaccatgccgctctgcagccgggacagccactcgcattgaccattcaaactggtggacccgcccacagtgaaattcagggcccctccgctgctggagcccaggacggtgctggtgccagaggccacaggcaggtggg

SEQ ID NO: 87 - DNA, 981 bp, Artificial Sequence
  subsequence
ggttccgccgaatgcgtcctcctggcggtgatggctctggaccgcgcggccgcagtgtgccgcccgctgcgctatgcggggctcgtctccccgcgcctatgtcgcacgctggccagcgcctcctggctaagcggcctcaccaactcggttgcgcaaaccgcgctcctggctgagcggccgctgtgcgcgccccgcctgctggaccacttcatctgtgagctgccggcgttgctcaagctggcctgcggaggcgacggagacactaccgagaaccagatgttcgccgcccgcgtggtcatcctgctgctgccgtttgccgtcatcctggcctcctacggtgccgtggcccgagctgtctgttgcatgcggttcagcggaggccggaggagggcggtgggcacgtgtgggtcccacctgacagccgtctgcctgttctacggctcggccatctacacctacctgcagcccgcgcagcgctacaaccaggcacggggcaagttcgtatcgctcttctacaccgtggtcacacctgctctcaacccgctcatctacaccctcaggaataagaaagtgaagggggcagcgaggaggctgctgcggagtctggggagaggccaggctgggcagtgagtagttggggaggggagaaagtattaagccagaacccaaggatggaaataccccttagtgagtcagtttagacttcaggctgttcatttttgtatgataatctgcaagatttgtcctaaggagtccaatgggggatatgttttcctcccgtgaggaaatgtttagttcttgagggaaaatccctaaatcctctatatactcaggtttagggaaggaaaacctacccctcacaactccacgcgcagggaaaatgatggacgtgatgctcgcctttagcttcctccctatctgatggaagaccatggaagacctcttggtctctgcaatcagaagtctcaagttgacaagaaa

SEQ ID NO: 88 - DNA, 864 bp, Artificial Sequence
  subsequence
aatgcccttctttgaggcagctggaggcctcctcctcctgagagcttaattgtggacacagccttgagtagaggcgaaaaggaaagaaggctgggagacaatcggggaaaaacacacacctttggtctggtttgaaagctggcgcccgaaaaggaacaagaaaaaaaacacgcttcggaagtgtctgagattgctgcggccataaagcagagcactaaccctggtactgatacgggaggggagcaagactccacccccgggcctgtgcccatgaacctaggtgaggaggggcacttcttcctccgcgcccaaatgttgcatttcccaagaccaccctggcccgccacgcccccatcctgtgcctataaaaacccccgagaccctagcgggcacagacacaagcggttggacatgaagaggaacacaccggcgggagaacacagaacacccaccctctctttagtcaccctggaggcctcggagaaggcggtttcagtgatccgtgaagagaccctgagtcttttacatcccggagaatgacaagagagtacctgggcgacgtaactttctgggttttccggagatgcggttttctacacgccaggggccaagcctgagaaataggtggacggcaaggacaggagctctctccgcgccacaaacgcccctgctcacacctgggttccttgattttcctgcctatataaccgagccacccatggccgggctccgagctctcattctgcggactgggacaaaggggttaactgtgatgtgctttgtataaccccaggattctgcacttgcccaagggcgaggtgcaaatccaaaatcacgcacgactgaacgccgagatcagctgag

SEQ ID NO: 89 - DNA, 1004 bp, Artificial Sequence
  subsequence of HOXA7
catccaggggtagatgcggaaattggcctcagccgcgccatgcagcgcgccctcgtccgtcttgtcgcaggcgcctttggcgaggtcactgcagagcccggggatgttttggtcgtaggaggcgcagggcaggttgccgtaggcgtcggcgcccaggccgtagccggacgcaaaggggctctgataaagggggctgttgacattgtataagcccggaacggtcgaggcgaaggcgccggcgcccgccccgtagccgcttctctgtgagttgggagcaaaggagcaagaagtcggctcggcattttggaacagagaagcccccgccgtatatttgctaaaaagcgcgttcacataatacgaagaactcataattttgacctgtgatttgttgtccggcagctttcagtgtcggttttacgaggtagagtgatatatgataacattacacccccagatttacaccaaaccccattttcttttggacggagctcgccgcagcacgtgaccgcccacatgaccgcctccgccaatctcagcagtcctcacaggtggtctcgctccgcagggcccgcagccgcctagaatggaagggcaagaggctcaaatatgcggccaaagaatccgcccgcgcccggcgggcctggcgcgtcccgcggaaaaagacctggaggctccgcgggagcgcccagctggcggccaacctccgcactggggtctgcggacgccaggcggcccggccccacgcagcaccccccaccccgcccccccgccgactcctgctagtgagccctggaccaagcttgggatcctccccatccctctcctgtccgcctgcccagaccctggaagggtctctgtcccccgcaacagcctgccccgcggtggccttgtgggcaggactcagctatgagcagatcgactctgcccaagtcttctctcacccaggtccagtgggcgacaggccggacttagactcggatccagacggggaaggcgcagcatct

SEQ ID NO: 90 - DNA, 963 bp, Artificial Sequence
  subsequence of ZNF529
cactcacaccaccacacacggacgcagccacagaacggcacacacaaacacaatcacacagtctccctccccagcaggtgacttgcacacaggcctggggcttctgcctccacaaaccctctccgcgtcccatgaacccaggtcccctgccgtgagctcttctcgcatccagacccgggtcacctcaactcaccacatggaaaacgaacaccaggtcaacggaaaagggagccggggtcctggcagaagcgtagtgccagccgcaatagggcggccgtgggtgcaaacggaggggagcgccggcagctagcaccgcgcggcgactaacgggccgccccggagactcctgggagctcaggcccacgcgcgagtgcgcaggcgcagacgactcaccctgggccgggggtgaggcttggtgggtgccaggggtgctgaggaggccaaggagggcactgggagctccgttccgggagagctgtctaaggacgcggaaccgggtggggaggccagggaggtaaccaagagtccgagccgggcctggaaattctgaggaggaaaccgggaccgcggtatccagacgctccgatctgtacgagccgggcctcgggcgtggtccatgggcgtgaccttgagggtgacccggagcgagctccgcgaagggggattttgcccgttctgatcccgcggaagcgccatcgctggcggcgggtccccgcgcggagcgggcgctgtgtgttcgcgcgcgcgggcgcgcgctgaataggggtggcctcctgcgcccaacctgctgcattttaggtgcttgcctctctttgggatgttgtggccgattgtgtgtgaaaagtgaacggagtagtgttgctgcgcgaggtttcctctgcgtgtgtctatttttagattaggtgtgagtcgcatttgagactgcctttgagtgtggagaattgcaagtgatttgtaggtgtg

SEQ ID NO: 91 - DNA, 956 bp, Artificial Sequence
  subsequence of PRLHR
ctccgcgggagctgaacggatccaaatgtttcccagtgggctagcagcttcttagagggactgggagcgcctcccctcagctccgccccccactccagctcccatgtatggaaaataggggtggagcgcgctctgccatgctcggtgcttagagaactagtgaagaggacagtgtggggaggatggaatccgaaacgggaggaggggccggcaaacctggccagagcagcgaagaggacgaatctctactgcaggagcttgcacggcccctggagggtcagggtccggaggagcgcacagtggaggagggcggaggagaggcgcgaagcgtcaggctatcgggaggagccggtgcagtcttaggagggaaggagcggggaaggaagtagcggtgggagattgcaatgcagctgggggcttgagagaggcacgactgacccgttcttaaaggctggatcctgcctagcggccaggttgcggagggcagagacgctagagggctcgggctgggatttaacagcagagcctggagctggtcgcggacctgaggaccctcaccctcccgtggccccgccacacgagccccctgcttggctgcagcgcgctcagcgggcagcgggtccggccaagccaaaggcaggagtcagcaccacggacagcttccgctggatctgccgcccctcgggcggatgatgtggggaggagcaggggaaaatgactagggaattcctgcccctctctggatccgggtgtttggggaaggaacctggtccggttcaaagacctgcctcgctgcctgctttctgggctggggctgagaagagtagggtggagtggaggcagctgagccgggggcctgggggtcggagactcatgacttttgctcctcttggtggtcaccgcactcagtgccaaggacggcgtcgtcttttacctcccggggtcagaaaatgcag

SEQ ID NO: 92 - DNA, 1037 bp, Artificial Sequence
  subsequence of ARL5C
gagggagcgaagagcagggaggcagtttgggacacttggcaggcctggagctgggtttggcagggcccccgggaagatggaggaaagcagtgggagctagggttgcctgtacggtgcaggatttgaatgccagaccgaggagccgcagtactaggaaggtccaagcagcgtgcccaatcgctcctccggactacagaggagcccgggaacccagggaagagctccagtgattggtccccctgcctgtcagtctggtgggaggcccagctctctaccctccccgcccgagagtcacttacaaccggtagagaatggtggtctttccttcattgtccagtcccacgatgatgaccgtgtgctctggaagcgtcggaggaagggcagcgtcagggccaaacccgaagaccaagggactgtgtgcccccaccagacctcccaggaaggagatagcgctccccgcaggctggggacctctgcccaccgtaccgcgtctgcttcccacccagctccgacacctgccccactccgggacggtggaaaagacagctgagcccccacctcccttcacattccagaaaagtgtctgaaaggcccggggcgcttcggggcttgccaagagacggtgtttagagaaagagcataacgcgaagtcacaatcgcaggaaactcgcagcagccccccatccccgccgctggctccgtttagcggggagaaaggagggtcgcccagctttgcgtcctggggcgcaccgaagcgccgggacccaagaggagcaggcagggacgggggcaggggaggccgcggggcagtcgaggagcgcccatatacgaccctcggagcccgaggtccccccgtgcgtccgaccacagatcagaggagtcccagaagagggcgagatcaaagcgctcgcttggatgccctgtgcgccccttaccctggttcccgaagatgctcattaacttggcgatcagctgtcccatggcacttcccgggccggacaggtgcaggagggctcagcggcctcaggagcggagtc

SEQ ID NO: 93 - DNA, 7709 bp, Artificial Sequence
  subsequence of PAX9
ctccgcttcctgttttcgagggattagctaggactgtgcaacaccagtctccgctctcggagtcggcacgggggctggtgggtggcgggatgaactcggggaaggcgacaggctggaaacgcagctcctcgactttgcagcgcaccaaccccctatcgccccgtccgctgctcaggtgcgaggattcgccagacgccacaggactgggggcgactcgcaagggcatcatgccacctagaggaaacgcgcagtgagtgagccctgggtcactgaaaatgggagaacgttcgagtcggtcaagatgactccggcctgcgagttgattcagactcctcggaagccagaaattgggtctagagtgggttggtccctccgtcagcagttcgggcccagccgaagcttggggcctagagggcagacgtccggctctgatcagagtacagcgggctgggcctggcagcctgcaggcaacctggaccttgcaataaagctgcattcaacataactcagaccacagtgggagcccccgaagggcttcatgtgagtcccgaaaccagagtttagaggcgcggcctggttctcgtttatcttttccagacagcatttaggccaataaggtctttgaaaggaggcagccccaaagccctcaggccgacacctgagggcagggtctcaaacagctgtgcttgaagaaccggcaatcttgcttttcccacacgcagctgcacctctcctgagcgctgcagctgatggctgtatagtgaccacggactgcgtcctcctcacgaagctgcgcaacttctgctaatgctgcaaccctggcaagacgaaatccccctccctctggctagatcagcccagcctcccctcagggaccttcctgcccctccctacccctccctacccctaggccgctccccccttcctctgttgggatccgatccttgttcgctcttgcaatcccgcagcccggagttttgccccgtgcattaaaacatgttctctttcatttgcagatttaataaacaaacgtaaccatatcacatggagctccacactgtccttctgaaagcaattccgctgttgaaaactgaaaaatgggtgtaatttgctttcagaaagtaatgttagggtcacggcaatttctcgggccgttatttatttttactttaaagtctttaggaaagatttgcttatatgctcggaaaacttccaaatgcgcgaataccagcaatcccgctcgccttcaacgcgtggggtaagggggggtggggaacaattactgagtgacgctaatatggggaaactgaaaagaaatgtcgattgtttttattgtaatagaaggagtgagcaaacagaaaaaccaaccccgggtgatcggaaacaggcaggcggagaattaaaagcgggtttcagacagcaacaggcccctcccctgctctcgcaaggagaaagcgggcgacgagcgctcgcagcccgtggggctgatcccacctcccgcagggctccggtcgtgtcgctgtcggaccgcagaacgccgggacgcatttccgagctcgggcccgacccaacccgctgccattctagctacctagtggagccgcggagagactcttgaaccgtgaggctccttgatgagaaggtggagaggctgccgggctattctccgagcatcttccggccgagctctgctcctctccgtgcgcttgcggcttctccttgggctagcgcgtccgcagtccctccaagtccaggccgcaggtcagtgtgcgggcgcctcctgtcctcctctcccaccagaggacccctgagggctgtctccatccccaatccccgcgactgctccttttagccgccatcccctcccgcagcgcagatcctgcaggggccagcggtccagggcggaccctccctcgccctgggcgcggggcgagcttctggctgtcacttgccgctgcagtttcagggaaactcagctggccgcttaccctgcaagacggggacatagcagagggccgagttctggagaagctgggcttgtttttctctctgcaccgcgcgcaatgccccaactgaccctgaagggtcttgcctttactgcatttgcccccagacggctagaagtcaatgcactatgaaaatcccagtcccggacctcggactctggctgtcttacaatccctgcaactcctccgagtggacaagaggcgggcaccgtcgcctgggcctcgcttggggggggggggtcctgtccccagcagggggcaagttggaggaatcagctccttaatattttctgctagctctgcttgtcataactgcaactcggaatagaacaacctctctcccgtgcatacgcacccccaactctcgccctatcctcccatccacagtcatcactgacctgtagacccggaggagcaggcttccgggggtcggtccaggttggggatacagggaggggtcctcgcgttccgcacaacctgtagtgcttgggtctgacttcggcagccctcgggtacagtctgccgggctagattcccgttgcttctccgcgtctctccgcgggccgctctagcgccgggaagggggcgccgcaggtgactgcccgcggcactgggacggctgacagatttatggagacttcacagcatctggctggggtccgcgagggcagggcggagtccggtcgatccgatgctggggtctaaagcttccccagccacacgcctgggccgagtcgcccccagagtccccggcccctgctccccttgggcgggtgtacacaaggatccggccagcgccgagtgtactggttcctcccacccagtgtagccccctccttcacactctcggcccggcttccagtctcccactgagtaaatatttatccagagagcgagtcgcccctcggaggaggcctcgacgcggctagggaaaggctttttggcttctccctggcctgagccagctgcaggccttactggtgttttggttttggtcttaaatttctccttttagtcgaaattcttccgatctctttgagatcttctgagtccagagtgagcagtgtaaccaggcggcagactccagctgacccttgttcttgttctaggtcctgcatccttacattcatcgggactgaccagaccttagtgttctctcttttccttccttcatcctctttctctgcctcagatccgtcgtctctcggtcggtctcagcgggtcgctgactacctcgccctagcactcggtccgcgccccgggaaggcttcagcatcaccctcttctgctgggatcccgctgaccctgtctgcagcttcggcttctcttgctcccagagcggggtcttcggcttgccgcggatacttagtggcccaaaacacctaaaattgactcttcctgcgctcttgagaatgccaagagcacccagtacctgcaaccgccggcatgagtggggcctgcggggagccgccagagctgcggacaggccccctgcccactgagttgctacccctggcacgcccaggggatccgcagcagctgaggccacatggtcacagccaagttcagcaggtggaaagggagagatggcattgaacctatgtgagaactgggaagatgtgtggcagctgaaggagttggtaggaacaagagggagttgtatgttacctccatataaccagagctctaaaccatatcagtttctgaaccagtctaggctggtgctgcagaactgctaaagctctcgcagagtccccagaccccccgcgggacatgaggtcttgcctgttcgtatgcgaacatccttgtacccgcctagcagccctgcagactgcaaattttccctgggtgcacggaagtagagcagatttggcgcagaggtcgatactcactgcctgtctgtgaggggggaggaggattccttcctggtcaagttgccgggcatgttcattccctcccgcaagcctaaggcagagtcataagctcccctacgatgcggcaaagtctcaactaatttatctaccagccttaagaaggagctgctgcttctaaaatctttagatttccgaaggctctccttgtgtaaaaatgccaggcggtgccacacgatgtcacccaacaggtattggaggtcagaccaggctgaaattgctatcaagtcaaacttcaagaagattttaaacatttgaaaccaaccaacaaaaagggacaagttcaagtatgtctagttgtgggatttcccccaagattccgattctaaagagtggtgttttagttcatctttacctttcacatcctccattctgttaggtaattttgaatttagagtgcatcctaaccatagaagtgggaatctggagatctgttcctttgcagaagcatggctgatcatagttttttcctgggttcttgcaacttactgacctgagatctgggaccagtcagcttctctgggtgtagaccgcagccacacacatccctggggactgttggggaagcagcctgaatcctgtgtgcacaaggagccttctggattgtcaagtagcagtaacagagttcacgaccccaagcagtacaaactcccaaattcacgaaaatatttctcttcttgtttattattttgattcacattctccacaaccctaactgcaaatattaataactttggctgcaaaaaagcatacggtacactttagattagacttacagtgaataaaagtgaaaattcagaagtaggcagaacgacagggcctctggagcttaatggaagacgagggaattacatccatgtgcagcgtcggtgtccactgtcttgggactaagtctctttcatatttaaacaaaactctttcgagagggctcgctggtttggagaaccctcacaaacgctgccaccgagggccaggggcccaggacagtggctgaatgtggcagagccttgggctccgtagtgagtgccccacgcactggcaattggtcgacttggggctgtgcgctagcgttagccgcctgtggttcagttccccgcacacggcgtggcccgtgcctcgagcctgtgtggctagtggttggccggtccacctggactggggggtcgccgcaggaagctggcggtaggaggaacctccctggccttaacagtggcccccacctgtggctcgggctccccgcaacctcctggtttctttggccggcctatcttctcacacctgcgctctcgccacctggcatggactgaagtgaggtagaatcggcaggtgacacagatcctctcctgacagtccccagaggcccgcatgacagattttgctaagacaactccctcacccctgtgcacggtggcgcccgcctcccacctatagccttaacttcaattctgagatgtccatcgttccccggaggaggtctcctcgggccccttctcccttcgagtcattcacattcagaccaaacgctttcatttgtttattcagcattttaccagcctgattttgctgtctttttgtgccgcttctgggaagatgtcaaacacccattttcattgtatttagtcacccaggtggggagctagcctgaaagagacagcggaaggagtttcctggactgcgctgtcgctcaccgacccgcaccaatcaccatgcagcttgccctcggacccgccccttttagggcgtgtccccagtgagtgatagacggagccgccctgccctgctcagcccagcccacgttgctgcttagattgaaatgcagaactcaagcctctttcatcggggcacagacttccttttacttcttccttttgccctctcgcctcctcctcctgggaagaagcggaggcgccggcggtcggccgggatagcaacaggccgggccactgaggcggtgcggaaagtttctgtctgggagtgcggaactggggccgggttggtgtactgctcggagcaatgggtgagtggcggcgggggactctgtcagagccgggaagggagggagggagcgagcgggcaagggagggagggagggagggagcgcgagggcgcgcgccactaggcgctcacattctctattgactttgctcgtgttcctacaagttgtaggaacacgctaagggtcagcggcgcacagcagttcaatgtgaacgctggctactgggtggctgttgatgccattttctgattttaagagaagggagctgtggcatcagcgagcccctcagcccgagtagcaaaccaagttttgtttcacacgcgcgcacacatgcaaacaaaacaggaaaagaaaagaaaagaaaacaaacaacaacaaataaaacaccctctagcttcccctagactttgtttaactggccgggtctccagaaggaacgctggggatgggatgggtggagagagggagcggctcaaggactttagtgaggagcaggcgagaaggagcacgttcaggcgtcaagaccgatttctccccctgcttcgggagacttttgaacgctcggagaggcccggcatctcaccactttacttggccgtaggggcctccggcacggcaggaatgagggagggggtccgattggacagtgacggtttggggccgttcggctatgttcagggaccatatggtttggggacagccccagtagttagtaggggacgggtgcgttcgcccagtccccggatgcgtagggaggcccagtggcaggcagctgtcccaagcagcgggtgcgcgtccctgcgcgctgtgtgttcattttgcagagccagccttcggggaggtgaaccagctgggaggagtgttcgtgaacgggaggccgctgcccaacgccatccggcttcgcatcgtggaactggcccaactgggcatccgaccgtgtgacatcagccgccagctacgggtctcgcacggctgcgtcagcaagatcctggcgcgatacaacgagacgggctcgatcttgccaggagccatcgggggcagcaagccccgggtcactacccccaccgtggtgaaacacatccggacctacaagcagagagaccccggcatcttcgcctgggagatccgggaccgcctgctggcggacggcgtgtgcgacaagtacaatgtgccctccgtgagctccatcagccgcattctgcgcaacaagatcggcaacttggcccagcagggtcattacgactcatacaagcagcaccagccgacgccgcagccagcgctgccctacaaccacatctactcgtaccccagccctatcacggcggcggccgccaaggtgcccacgccacccggggtgcctgccatccccggttcggtggccatgccgcgcacctggccctcctcgcactccgtcaccgacatcctgggcatccgctccatcaccgaccaaggtaggggctcagaggctgggcgtgtggatgtgcagcgtctgcccccgcactctcgcggaggtcccagtatctgcagcctcagggacactgtctttcccaccacctgaggctttttcctttggaaacgtaaggagtcttcctagggggtgttctgatctcattaacttgaaactcatgcccctggtttccttgccacacacagtcttctgcctcatctcaaactaccagacccataacatccccccatccccaacacatggttcgcattttccaccctcccccgcctctcgcgccgaggcagcctcagcccggcttgctcacttgg

SEQ ID NO: 94 - DNA, 6438 bp, Artificial Sequence
  subsequence of HOXD10
ctgaaatggaaaggtccccaaattctgaagacacatcctgcctattctggctcactgcagacctacccgcccgcaaggaattgcttgtttttagcctgtatgttttcttcatgtataaataaagattatgaaagggcatttgatgggcataaaattcccgattagattaaacagtcttgcctttcttagggtagggaaaattgggcaaacaagttcccagcagctcttctggccaagaggcaaaagggcgacactcgatactgctggagcgccaagctagtgtcagggcgcctgcggcaagcgagtgcagcgggcacttcattcagctttgggcacgcttagccctggcttgaaacaagatctctactatgtgagaaagcaaatttcagggcgctggtcagtggctgttagctttgaacagtaccttagcaacctagagtcaaaagttatgttttgtcttgttttgtttttccggccatcctcaacccccacccccaagctcgaaaacagccacccctgtggaaaggtaatgtttaaaccccaggctatgctgggatgctgcagccaaagcagttagaggcgccaggcttttaacctgacaatgatgttgtatttgaacagctgcgtaaaggtttaaaaggtctgtctcattgccaccgcggagttttttaaaagaggttattgtttgggcgagagcaccgagagggaacaggcgaaagggtcccaaggccgaaaataatgttcaacgcttgtttcaaccaggccaggggagattcctttttgggaagagggacaaagggttttttgggaaaggtttttgtaaaggagcgggcgggctactaggtcccccagaatgctgaggcgctttaatgaacctcaggccccaaagaaatgttctattgaggtggaaacccaatttacccacaagttcagtctctgggcctgaaatccaaggccagcccatgccccagcgagtacggggaaaagagaacacagatgccctcccggactgagaactggttcatggtcagagtttctgggaccgctttagtttcttggctggcaggaagggaacctggcaggccgaaggacggctccaagccctggccggcccctcactcagggcaagtctttggaaatcaaggttaaagctccccgctgctgccccgaggcccgggcttccgcagggcggctcacccgcctgcagcaagagagggagggaggaagttgttgaagtttctcataaaactctgagtttccatggtggtagtggtggtagtggtggtagtggtggtagtggtggttctttaatgagccggaccacaaccccagaccatatcctcttcatagaagtttccctcaccaaaggaaacagagaactaagattcccacctccttcccctcccttacccaagcaaagccttgtcaaataatttcagaaattgtccaaaactgtaaaactcaacttctgacaaaagtatagcttttaatatttgacaatttgtattaaaacaaaaatgaccttcttggttagcagcgaagggaaaaaaatcaatagtataattttcaataattcataaagcgaacgccattatggtaaatttaactattaatcttatcctttacaaagtctcgattgatttgttaataaagtatcttcccgtgtgtggcaacagcgggcataactctttaaaaaccttcagaagcaagaaaattaccaagtagcccaagaatgtagatgagaattttattgatcgccctgattcttcttaatatgtattaataaattccacaaccttttgtaccttgcacttgtcagaaaccagtgcttttacaaaatccataaaaggaaaacatttttctttgcagaagaaccaaaatgacacctttgcatttctctctgtccttcttggcccagtcagttttctaaaacttctggattctgagggtcagagtttccccttttcttaaattattttttcctttcttccttcctgtttgccctccattatcagggtgtggggagagaaacctctgtttagttctcctacagggagcccgagggacgctttcgcggatagtgaactgctggcaaagaattgtctctgggctgaaagctcccagaggtccggccccgcagaggtcagggtgtggttcctctgagagccgaagcctcgtgtagccctccggggcgcataggaacccggagccaggcaggaggaccgagcgggaggacaacgcagggaccaacccatccatggggatccgggcccggccagctgcttggcctcccggccctcgcggccctttttgcctccgccctcctagagacaccttggccgcttcttagccccaagggatctttcctttggacccctggggtgggatgtctcagggcccgcggaatccgactcaccttcccgctgggctgcccgggactaaattaaccagcctgcgcccccacccgcttgtcctggacccggccctcttaagcgcgttctgcctggttgtgtgtggggggaatgcttctgtgcgctggcgccagggcactctggcttccctccccgtccgtgcgtgtccacttggaggcccctagagctgagactttccttccgccggttgggcccaggggccgaagcgggggacgcgagtggggcgggctggccgagcgagccctggagaggcggacaggagggcggcggagagcgctgggccggttgtctccagcgcgcactatcgcgggcgcgtagtagatgtcgctgttgtccgtgcttacccggccggccggccaggctctggagcacgtgacccgagaggaggctgcggctcaaggccattttcaaatctcattggcttggttgtcatgtggtcggcagaggcatccacaattacacggggaatgttttcctagagatgtcagcctacaaaggacacaatctctcttcttcaaattcttccccaaaatgtcctttcccaacagctctcctgctgctaatacttttttagtagattccttgatcagtgcctgcaggagtgacagtttttattccagcagcgccagcatgtacatgccaccacctagcgcagacatggggacctatggaatgcaaacctgtggactgctcccgtctctggccaaaagagaagtgaaccaccaaaatatgggtatgaatgtgcatccttatatacctcaagtagacagttggacagatccgaacagatcttgtcgaatagagcaacctgttacacagcaagtccccacttgctccttcaccaccaacattaaggaagaatccaattgctgcatgtattctgataagcgcaacaaactcatttcggccgaggtcccttcgtaccagaggctggtccctgagtcttgtcccgttgagaaccctgaggttcccgtccctggatattttagactgagtcagacctacgccaccgggaaaacccaagagtacaataatagccccgaaggcagctccactgtcatgctccagctcaaccctcgtggcgcggccaagccgcagctctccgctgcccagctgcagatggaaaagaagatgaacgagcccgtgagcggccaggagcccaccaaagtctcccaggtggagagccccgaggccaaaggcggccttcccgaagagaggagctgcctggctgaggtctccgtgtccagtcccgaagtgcaggagaaggaaagcaaaggtcggtatgagcagagttgccaccccagcggggcgcgcagcccgggaacccggcagagagggagtgccggggtgcccagcgccgagccggagcccgacttggcaggtgctgctccgcctggttttagaggggtgatctcagccctgagatagtccccgcttctcccctgctgccctggccctctccgccagtcctggccccacgctgatggcgcccgggcagaggaaaagcttgccggttttatttttcctgagctagacctgaacacaacaaaagagcgcaaaggagacctgcggctcataaacacgaccacagagcctcttttctcctgctcagatttgcagttccagttttgccttgagcccaatgatcatgttaaggtgatccagggcaccgtgttcgtgttcaagtgtatgcaccccgcatcctgcgagcttgggggtggtgaggggaaagagatggctgggctggttggtgcttgagttgggaaacagggcttactgcctttgctgggctaggtaaccttggctttgtttaggaaaagtgctgcagtctttgcaatccgtcggcaaagagggcaaaggcggagggggagagtggaacccgcattgccctccctgcaaggccagccttagggctgggctaaggcaaagagccagggatctggctttttgagaaggaaccctcctcctctcccccagtgcttagaggtgggccacagtagggggctccctttctgggggaatgctttagtgtgggggcaagaagacatgaaaattaaggaaattctggggaatgcaacaatacccaggcaaggtgggggaaggtgtctcgcttccccatttatcttttgaaagagaatgggcacctataaacctgactgtcaggattcctgactgcctaggagaggtggggaagaagtggcagatttggggacctgaggcagcagtggggttggtaggcttgtccaggtcgtggcgtattcccctccgtccctgttaggagctgaacccttagaatgttgctggggagatctggaaagtttactattctactaatgttttgtacaagtgagaaagttgaaagagagagcgagaacccaaatgcagactgtcctgccatcatgtcatttaagtaatgtggcatcaatgtaagattcccttccaaggcccacttcatgtgagtaatgtttaatactagcattttccaaagcggcctggctgccagcagggtcacggccaagggtacatttgaacagtctgaagaaaaaaacaaaaacgaaaaccaaaaccaaaaccaaaacaaaaacaaaaacaaaaacaaacaaacaaaaaacctcttgatttttttcttcttctccctttaattttgttagaggaaatcaagtctgatacaccaaccagcaattggctcactgcaaagagtggcagaaagaagaggtgcccttacactaagcaccaaacgctggaattagaaaaagagttcttgttcaatatgtacctcacccgcgagcgccgcctagagatcagtaagagcgttaacctcaccgacaggcaggtcaagatttggtttcaaaaccgccgaatgaaactcaagaagatgagccgagagaaccggatccgagaactgaccgccaacctcacgttttcttaggtctgaggccggtctgaggccggtcagaggccaggattggagagggggcaccgcgttccagggcccagtgctggaggactgggaaagcggaaacaaaaccttcaccgctctttgtttgttgttttgttgtattttgttttcctgctagaatgtgactttggggtcattatgttcgtgctgcaagtgatctgtaatccctatgagtatatatatatatatatatatatatatataaaaacttagcacgtgtaatttattattttttcatcgtaatgcagggtaactattattgcgcattttcatttgggtcttaacttattggaactgtagagcatccatccatccatccatccagcaatgtgactttttcatgtctttcctaacacaaaaggtctatgtgtgtggttagtccatgaactcatggcattttgaatacatccagtactttaaaaatgacatatatatttaaaaaaaaaagattaagaaaacccacaagttggagggagggggacttaaaaagcacattacaatgtatcttttcacaaatgaatttagcagttgtccttggtgagatgggatattggcgatttatgccttgtagcctttcccttgtggtgcatctgtggtttggtagaagtacaacagcaacctgtcctttctgtgcatgttctggtcgcatgtataatgcaataaactctggaaatgagttcactccctctgctttctgaaatggaaatatgttatggtggaaatgaaagcctatggtgagattatcttctggttacactccctgtttggggcatttgggcaggggagtgatagactagtaggggaagggagatgggggagaaaagctggaggaggcctagggtgttggattttggcagtggttgggggagaggaattataagctagcttgagagtgaagttttcataattgggaggaaggggagtctcctctttcctttcccagtccccagtgatagtaacataattgcgctctcaatgggtgtgagctttcctctggcctgaacctggtaagtaagcctataccccaagccactttctcctcaaagc

SEQ ID NO: 95 - DNA, 4212 bp, Artificial Sequence
  subsequence of TBX20
taactaaaagtagaggaatttgagaaatggttactggttagtgtttttgccaacctcaactgaaaatgacgacagttataaaatgatgtcttggtgataagtctagagcttcagtgaataaaatggttcgtgtagggagaactggcttattctgctttacagtggtttcaaagagcttgctctgttttgtctattcaagtcagaggaaaaccaaaattaaactggtttcttatgaagtcctttagcgtctccgtttcaaacgcacaagcaggtgttacatgcacagtaaatcctgttgagccttaaaaggggttttattattatttttccatgaatgtttttaacccaacaaacatacacacacaccatatgtctgatctgatatatggattctagacaacttaggagaccgacgggcccagatataagatgcacattcacagcattcaacagactgaagcctccaaagaaaacttggacccaaaagaaaaagatctcccacccgcgatgtatggctcatggcttgagcatcagacgttgctgcgagccgcctgcagccaggggcacagacggatgcgcagcatccccagtcctcggcggacagccgggtagcccaacttacccaggggtttgattgtgttctccgtcgcctccttctccttagagccgccgctcgacatgagcgcggcaatggagaaggcgttggcccgagaggagagttggggcttgggggacgccgtgaactccatggtccccagcacgcggtcctggccagggacggggtcgtccgaactgccgtccagattccccaagggagacaaagacccgaaacacagctcaaagtttccgagagcagtcacagcggggccagggactccagaagtgtcagctccaacgactccagagctgcacactggcctctattccccaccgcaaagccccagagccgcagagacttcgaaggcagccggagaggagagggcccaccgagcactacggcgggtgcgcacgccccggggcgctcggcaggacgacagtctgcacagcccgaaggcggaaacgagcatcaactgcacaaagtcctggggtcctggagcatcccctccgcgtccttcctccctctggggctggggacagccgggatgtcccaggctgaggtggccaccagccgagcgcggctgctaggacgctggcgtggggagcgcggcgcggaactacggacagtgagccctggcgctcgctgccctgcgccttaatttgctggcggcggcgatcccggaggcccgcagccagtcagcgccgtctcacgtcaccgcttcctgattccgccgccgggggcggggccgcgggccgggcgcggagggcgcgcccagggtgcggcgcccgcgtggcctgtcgccccggctgttcggtaccccagcacaggttcagggaaaagggtgccaccactaggctgacgcagcagccatggacatccccacctggtctcacagccccgggcgggagggcggtgcgcgctgtcgggagaggacacatcaccgcggcctaacgcccgagatccgggcatggcccagttggggaagctatgaccagaccagtggaagcctcgggagttctcgctttttccattctttttcttacctgcgctcaaagttccaaaagaaagtagggaagcgctcagtagaatccggcgcctctgagccggcgccaactggccaggtccatactcggggcagatcccagggctgggactctcattcgatggtcccaaatttgatctctttgacagtggggctgagcaaatgcagccctgaaaaagataagcttagcgagagctgcgggcatttggcaaaggatgctgctctcagaaccgtggcttctgctcctcaccagtgcgtctctagcctggggctcctattttccctagagggaccctggaaaatgggacggctgccgaagagaaggcgaaggtcagggcgcggagctctacggtaaccacgcgacgcgtagtgggagagtgcgaaccttatggtagcgcccggactaagcggacacagacccctctggttttacaaaggcggctgtgacgaggacttcccacggccttgttggagggcgtcctgttagccctgctcagcctgaataactcaaattctccgaattcgcagggtaatccgcttcgcttggagccgtgtaaactcaggctgacatacacactcaagctgtatatgtaaatatttgttctcttttccagccagtcggtctggctattagaagcctcttcgtgggtcttaaaattaaaataataataataatttttaaaactccaacttttcactgcaccaccccctactcctgaaataaatttgtgagggaaaacggcaagttaaaatagctgtcgaaaacgtttgtgtgaacaaaatgatgacatctggaagagtcgtgatttcagcctgtcttggtcatcgtgtgtcaatagtttttaacaaggtgctggatgaaggtgactaaaaaatgcattctcatatcactatcgaagttcgaagtgtcgatttataaatgtttgaggaaattcgtaaaaccatagactttggtgctggaaggaatttacgctgtcttctagccggtctccatgtgcgtttgagagagaaaaacagggcccgacgtggcagagcgcgcatctccccccagtccacctcagcggctagaagcagacggaagggcaggactcacactccgggccccgaccctcatcagcccctggccctgcagctgtggctgggctgttagctgaagagccagagtagagttaacgacggctggcaagcagagggctttcagattaaaccgcaggatgcatctgaggatccgtttctattcttaaattttttgctggttttggacaacccagacccaatccagaccccttttttggttattaaagtcccccgccccaacctgtctctccccagacacaccttctcaatgtaagtgacatttctttgtattgagtggaaggcacacactgattcctttcctatatcaaatgcttaggatttgtccagaaagaaagatttccctcaagaagtggggattttggaaggtcggggaatgttatggttagtctagaccttgatatatgcttcaacagggtgtggcaaaccttgttagctgaatttagttttcaaaaacttgccgcaaaattatacttcataaaaaaacccttttgattgtttttctacacagaggaaaacaactgtgtcttttcttaattacctcaatgattttgactggaatatgaataatatcatgagaggaacattttcagaaaatttgatgaagcaagggaaaaactgaattgccacaaatctgtttcctcctcctttccaagtgcctacgcggccttagcccagctctgtgtctcttgtgtgcaggaaaccccgactgcgcatcctactacaggtaaaatactatacaagaaaagatgagtgatcgttaggaggcaggcggcaaacgagaggtattgaaaaggccactttaaacaaatccgggtgacccgtttggggatctctaggctatgcatcttgttggtgttgaaacctcggcagtaaaacatatgctgcaacattattatcgggggcacaccgtccctcctcctagatttattgcctttgcaaatcaatatgatgccataaaaacggggaaccggttctgggcagagaggtgctgtcgaaggatgattcaaagccttcccaaagcggagagtggggagttctgaggtcccttcaaaacgccactgatagcgcaggttaacaggtaaaaccacccgggggttggaacaaaacaagcacgttaacacatctctctaggcccttctcaggctgactgctggcagcggaagctgctgaagtcttaatgttaactttaacacacgcattagcccggagactttgtgtaggttactaaacctctcaaagcttcagtttcttcatctgcgttagaatagggccaatagttcattcctacctggaagatagctctttggattaatgccctaatgtgtataaaaagcctaacactcacaataaacccaacataagtaaagcataatacagaattttaatcatatttaattttgaactgcaaattcgcgattggagaaacatgtctctcgggtgctcatatataatgtagatagttttggaatgtaca

SEQ ID NO: 96 - DNA, 7272 bp, Artificial Sequence
  subsequence of CACNA1B
gccctccctgccggggccgctgggccggggatgcacgcggggcccgggagccatggtccgcttcggggacgagctgggcggccgctatgggggccccggcggcggagagcgggcccggggcggcggggccggcggggcggggggcccgggtcccggggggctgcagcccggccagcgggtcctctacaagcaatcgatcgcgcagcgcgcgcggaccatggcgctgtacaaccccatcccggtcaagcagaactgcttcaccgtcaaccgctcgctcttcgtcttcagcgaggacaacgtcgtccgcaaatacgcgaagcgcatcaccgagtggccatatcctgccgggcggggccgggcggggccgggcggggaccggggtgggggccggggccggggccatcttcccggtggccgggagggcgcgacctggggaggcgtcgggagacgggcgaggggggtacggagcgccccagggcccctcggagcggcgggtgcgggagcatttccgtgagtgcggcgggcgcggggcggagcccctctgctccggactcgtccctccgcacgccgggtcctggggatcctggtcggtgcacagtgcgcggctagcctggagggcaccgagggcgaagccgcgtccgtgcaggtgcgagcgctgtggggacgcggccgtgcgcgcgcctggctgcaggtgcctgcgtgtgcgggctgagctggagcctggcgctgcgcgtgcgtgcgctcgcgatgcgggctacatgcatgttcacgtgcctgtgtaggtacatgtggctgcgtgtctggagggagcagcgtgcgcctgcgcggggtctccctccagcctcgcctgggggcgctcggccccctcccctcggggccctggagtcgggcggagccgggccggaggcgctgtccgcggtgctgacggccgcccgggtgtgccgaggggctggcggcccagactgcggaggccccgcctcgcggccgcccctagggatgggggcagggagtgagggagaccaggccgcttccgccaggagaggggctccggacccagttgtctcagcccctccggagacggcctagcggtggctgctgcactgggctctgctggcgtcggcctcgtgtttccctccgtgcggcgtctgccggccagtccttaactcacgcactccattcgagtatatgatcctggccaccatcatcgccaactgcatcgtgctggccctggagcagcacctccctgatggggacaaaacgcccatgtccgagcggctggtgagtgcccggctgggcctgagggcagggtggtggggaggccgcgactccactttcctttatggtctgtgcctgagaacagcttcctcgggcagggtcgtctgggcagtgcccctcgcgtctgaaggaaaaggtaggcctggcagataacaccttcctcgagggccagggcagctggggtcaccggcttagccctgggcgtggccacgttagccctgggccagtctgccctgtgccacgagctactcctgcacctcaatggctgtcctggctttcggcgctagactttgatccagaaaaccatgttctaaacttggggtggggaaggggcattcatgtcttcgggaaggtcagctctgaatgccatgtgtgccctgctgggctgagatgggctttggcctggatgtgggaaccctgagcctcatcctccaagttgtcttgtgcgggcctgcttggaacctcttctccagtgggcctcaccatcctgtgggaagcattccttctcaaacattctgaatcatttttacctgtccccagattccagccaagaggcccccgtggtagcccccattggagcatagagtctgtgtgagtcagggtgccagggcaaggtctccgtggctcaacaggaggcaaggtggaaggccagccctgtggggtctctggaggggctgggtcagaggaagggcagcattttggaggtgagcagtttctgaggtcagagcatgtcccccagcccccactcttccctgatgcctggccccatgtctgggttccgagtgtgcctaaagactggagcctccaggtgagcagaaggcagagcaagtgggggcccagggggtgcggggccagaggcgtccaggagacggcctctctggggtgtcaggagctgctccctcttcccttaagcctggcttccgcccccactagcatcctgagacaagagctattcagactttagccctgaaactgaactccctttgaacctgggccaccgcaggcccaggagtgcagaaggggagacagggagcctgtcctggaggtgaggcaccaggaggtgagttatgggtggccgaggtgaggaggtcttaatggagcacagtctggaatgcccagtggtctgggttacggccgggtgaggaggaggagcatggacagcccagccacaccatgaggcaggcgtgagtcatggtccctgtgggggacttgggcaggaccctggtggggcccattgctttctggaggctggagaagagggtgagcttgagaggaaacaggcagagagccttgaatgccaagtcacaggaaggagggcagggccagggtcagagggacgcaggcccaggagccaggccggggcgggggcagggaggatcaagctgtcttgccctgccaggcagtgggtgtccagccttgcaagttcctgcctcgcaggtgtgggagggtttactttgtggtcataggttggggaggacacttctaggagtggcgagctaacctgttgggaaaactgcagaacatgcccgccctgagccagcctagaggtctggggagctcttgaccagtcccagtcccatgtgcaggcccagccattgatgtcccctgggatggaggggaggctgtgctgctgcccacagagcaggccgaggctgggtggtgcaggggcagcccctcagttgtctcccagcctggccctgggcgaggcctccctggttccctgcctctcggggctgtttcccacctccccgtcgactctggagctacctcgagccaggccccagcttgcagtgcaacaccaagctgcctgcacacccatccctcccacctaagccagccttcagccatgggctgggcagggcagagctgtgaggagagggctcgggctgggggctccttcccagctgagggtgctggctggtccttcctaggcgtcgggcctgttctctttttcaccaggaagtttcctgtgaagatctctgtctgctgcggccccactgttcccctggggcagatggtcagcaaccccaccccttgggaaaaggggtccctcctaaacaaatcagaccagaaggctcgaggccaggaagagcatgggcgagtcagcacgggtcatgatggacccttgggtgctggtagcttctaccaggtactgccagccaagccttgggccagctccaccacaggacaggaggagcccaggctgagtaaggtgggagtcagatgcggagagccctcgagagcctggcttcctggggaggaaggcacaggctgtggaactggtggcactcacctcacctggcagctctgtggcagcccagcagctgcttcttcctgtgacttccacagtcctgaagacgaaccctcaggggaggcccttgaagctggtctcctctccccaccccttcacctgcttcctaaggcagcagccctggagtgcaggtgtccgacacccccatgccaaccctgcacatgcagctccctcagcccagcttcccgggcttgccttgcacagggcctttccctgccagccccacgcgtgtgctcacgaggagtctttggggtctccctaagctccacacagccccatctccaccctgtttgctgcttccagctcggcactggtagggcctggctctgctctctcatgtccagtaactgttggctggagctcagcctggggtgcaggaaagggatctttttaggatcagctgtcttcattcctttggctgctctgttccctccacctggatccctttctcaaaatcgagctgtggaagccttgcctgcaggcgccacgccctctgggaggctccctgcggtctgagcccagggtggctcccagcttcaggctcagactgtggctggctgcctccagggtcctcacagatgtggcggtcgtcgctcagcacactcagggctgaggttgtgcttctcatttctgttgttttctgccgagatgtgcatgttctggttacccgggtgcatgttgaatgcataaacggggcctggactgagttcaagaaagcctgagctgtatccaggcaaccttgtgcaggttcccacccagaggctgctgtggcctctgcctggctcctgggcatctctgtgcctctgtctcccacatgttagaatggggatgacctcatggggtattaaagggccaccctagttgataaaggaaaaactacctgataagcacccacaactagtactgttacatcactgtcttccccgaagcaaggcccactgcatggtgctagcagggagattggggccccactgtgacgtgggcagaagctgagatgccagggtgggaggcacgaggggcctgcaggcatgactgggatgttgctgctgtaaacagtggtgtccccattaggggacatgtgcagacagcaagcaggctcagtgatgggaatggctccttggagaatctgcagggtgttgggggcaaggtgaggagggtcagaccctcacgatagctgtggcctgcacatggtggggtggggtcctcaccaaccgtctctgcccgctactacaccgggtaggggccaggggtgaccactgttctgcgcttctcctaggacgacacggagccctatttcatcgggatcttttgcttcgaggcagggatcaaaatcatcgctctgggctttgtcttccacaagggctcttacctgcggaacggctggaacgtcatggacttcgtggtcgtcctcacagggtaggcaagctgaggccaggaggcccagcgtgtgaggcccgggcgtgtgctctctgaagctcagttgcgccgtggagctggggcagctgcagtcccctcactggggtcccctcacagccctgctggagatgaacgaatgtgagacagtctgtttgccaccctgtgtgctatgggggtgcttctcccaggggtgccagtgctgtatttctcgctgacggatcacagtgacctgtccccaggaggcgctggcttgcagagcgcacaggccaggggccaccagcttccatggctggcctgagccagcatggtgcctgttggaggtggctttgctgcccaggtgaggggcttcctagcgaggaggagggctggacttctggcctcacccaagcctgtggtctgggaggggcacttggcggtttgaattctgtgcctgcctgagacgctcacctgtggtgtccacctcgctcagagcccttgtgctgcctgggatgaggctgtgtgtgtcgagtgctttcacagttcctagtgccaggaaggtgcttcggcagtttctcctcaaccacttaccctaacaacagcttgtgattgccaaagtaaccagcacatctagaagatggacccaaggggcctggatgggagctcaggtccagtgctctgcaccccaccctccagggtgttaactccccaacctgtgcagtgggcactgtgaggtcccctttcctgcttccctgactggcaggcggaaggctgggctgggctgctgtggctctggtgtggagagtggtggctggggagtgagtgcttggggagttgcccccacagagcctgttagcacttcagtgtcagaggccctgtgctgggccagggaccactgtctgctctttcctgagccttatggttccgaggctcagagcccagatggaagaggagggagcaggccccacagcaggcgagagctctccttccagagccccatcctcacccagtgactgccccaagatgcctggtgcacaggagggtatatggaggggtgtttgggctggtggcagaggaggaaggagatggctgtggagtcctcgagtctggggctcatgccttcaaggttctgtgtgtgtgaggaagaagcagtcggctacatggcctctggtctcttgggtgaggccctcagagggagcctcgcattgcctgcctggatcccggggtgctgcccccatctgctctgcctgctcctgagcctggggctggcccctgctgggtgagagcagcatgtacagaactgggcttgggggtgtcgcatggaaggctcagcccccagagctgtctgggcttgggagtgtcacacagaaggctcagcccccagagctgtctgtgatgtgctgggcacagcagcattgaggtggattctgtgcctttctgcagcacggccctggggtagaatttatggaaggccctgtgggggtctgtggctccacggccctggggtagaatttatggaaggccctgtgggggtctgtggttccgctagcaatgcccgttgggggctggggtgggaggtggctggtggagagtgtggcctctcagaggactgggcgctcccacatccagtgggcactcccagaagcagcccaggagtcatggtagctgtttacccctctctctccctgtggacccaagtccctgaggacaacggtgccttatttttttcaggaggtccctagagcctcacttggagtgggcacccaggaggggcagtgtgcctctgctgaagtaatgaattgttggggtgtaagcagtgctggggggtgcgggccagcgggcagctgggtagaggtggcagcacccggcctcatggggcgctgtccatggtgctgagtgtgtcggcccttgagggccaggagaggaggcaggaggagttgcaccaagccatgggcaggacccctggatctcccagcacacatagactgggtccagggctgctcctccttcccctccccttcttccccctccccctcctcttcccgcctccctcttctgtttctcttcatctctctccctctccctcctctcccctcttccccccccccctcctcccactttgcctgtctagccctttgtctcctctccacgctctctgtctctggccctcttggtgtcttggtgtctctctgcctctccctcttttcttctgcccctctttcccttggcttgggcacgtctctgctcgcctgtgtctgcagcagggcctgggcgttgctggggtggctcccagg

SEQ ID NO: 97 - DNA, 7265 bp, Artificial Sequence
  subsequence of ZIC1
acacacacagggcggacgaggaggagctgggtatatagattttttaaatgagaaacaaaaaaggtcggagaacaggaagccaaacctggtttggcggagaccttggtgctttcgaagccggagaaagtggctggctcccggcagccgcggaggcgccagctgctcaggctgcagacaaatctaaacccttgcttgctgccaacatctctctccgtgcacttcactgaggactttgccaaaggaaagagctgaggaaattgaggaggccgggttaagggcgtagaaagaaacaaaacagagacagaaagaattgagacagagtggggaaaggaaataatttgggattgaggaggcttttggagctttatgcatatttgaagagttcagttttagtagtgactggttttaagagtgggtttgaggggtggagaaagtccgaggaaggcaaggaagaacttgttgtctattagactccatgagggtgttttcaaaacaccagattcccctctttggcctttaaaaataatcaagacacaggtccggaacagttaaaaaaaaaaaaagttcccacgagctcagggttgtagcctggcatcagacaaaacattctgggccccctgcccccaagaggccgggaactgggtctcctttcctattctgattttcccgggtgagatctgagaaccatgcttgagacttcgggtttaacgcccgagtcagggaagaatttgcggcgttgagttctctccggcccagattacgctataaaatgtgagtgtatgtagggagtggggtgggttggaggaggcgaccaggggatgcggagcgtcggggagggggcagggggaggagagaaaagcaatagggcaggagaataagccgcaaacgtgaaaactagaaaccaggagccaggtggaagcaatccgaaatcgtgtgtagctctgggtaatacgagtttccagatctgatgctaaaaaccgactcctcctactattaatttttttaaacataaaaataaaatgtagatccaattgtattagggattacaatagagttaagatatttataattccactgcagatgtaagaatttattgacgttccgggtttttaagcttgcaaagtgctaatcctgggctgctggctttttgttttattttttttctatttgtttagtttttgaaaaacggccgcggtatttttttctaattagacccctctcattctactttggcaccaggggagaagcccttcaagtgcgagtttgagggctgtgaccggcgcttcgctaacagcagcgaccgcaagaagcacatgcacgtgcacacgagcgacaagccctatctttgcaagatgtgcgacaagtcctacacgcatcccagttcgctgcgcaaacacatgaaggtaatcgccgcactctcgtcgccccctttgaggcaggagctctcttggctctcggcttggggtcgggcggcgagtggcagacaggcggtggcgggagccagaggaagcgggaaggcaaaggttccactcagtggaactgggcagagaaggtagggcgggacctggaaaaggggatgggagtgtccaaggccgttttaaatttttggtttaataataaaagttaaaagaggcgagtatgagcaaaggccgccactgaatttggcccagagctagggcttttgcagggggttgacgctgcggaaactgctgcccttgcagctgccagtgagacgcaagaattggactcctgcgcccaggcctgagctctggctcacctaaacatggacaagcaaagttcagggaaagaaagtgcagtctctggcctcatatccagtctccctcttcccagacctatttttcttttgtgagtcttggggaccctgactttcccaggagcacggtttctgcaggcctgtgcagagaaaccaagcccaaagtcccgctgatcgggcctcacctgtgttcagggggctccaaggggtccaggaggaagggcactcgcggccttcgcctctctagtcggccgccgcactggctctttatgtccgtaaaaacgcgactttattcctgcaggtccacgaatcctcctcgcagggctcgcagccttcgccggccgccagctctggctacgaatcctccacgcctcccaccatcgtgtctccctccacagacaacccgaccacaagctccttatcgccctcctcctccgcagtccaccacacagccggccacagtgcgctctcttccaattttaacgaatggtacgtttaaaatcagaaacaaaacatcgaacaaaaccctatttaagagactgatcacacacgtatacacaacattactgaaagaaccctgcgaatcaaaacaacccccacacagaccccgcaatccttttttaaaaaatctgccaatagacccaggacgagtaagagaggaagcatcaaccttttaaaaatttcctttcgctttcattatttttctttttttggcaaaggcttggtacccaaggtgcggtagggggtcgagggggaggaggccacctgaccaaatgccgccaaccccgagggccagtttcttgtcgaattggtacgggctctctggggcttcggcttctttttttctttgttttcttgtaaatacagaattattagcttaaaactgtactgttgaattctgtaaatagttatatctcggttggagcgggtgggtgggattgtggcgttgtggtctttgcattgggggaggggggagggaccggatgggcggggggagggggagggggaggggtgggcggccgaaagccaactgtttgtactgaatggcaagaatgttctagtaaatgtgtaccaaaatgtgaattactttgtacgattacagtctccacgtcgacctaacccaatattattggtattaatgtgctttttttgtataaagtgcaaacatttcgtcccaaagtctaagtactttagtgcagtaaaatgttgtttcatgtcctgtcaagaattcgtatagtacgagcctggatctgcgtgtcaaactgttccatttgtttatgtaaagtgatattaaaaaagatataaactataactgtccgttacttttggcaaaagatacaaccacataatgtatataattcctagtttccatatttatccgcatgtaaagggccggtttatccatgttacagctcttcaatatttatggctagaagaactcgtatgtacactttagtttccagaactgtttggtaacctttcgtaccttattaaagattcttaaatctccgtgattgtggtaggaatttcttcttcacccaccagcaacctgctgcctcttctgccagtcttaaagggtctccagaaaagctctccagtctcccttgccttccctttctgtcactgcaggtcgtataaacgtgataaatgaatgctaccctgctggctctccgagagagtgtaattagtatttatatcaaaatttatgaaacaaattttcggccgcagtataatttaaatgacctttgcagatgtagaataacaaccataaaaataacaggaatagattgcacaggcgacatcaatattaatgtagacgaattgtcagaagctcaggggctcgctctgcaacattgcaaatgaacttgcagccgagggttccgctgccccctagattaaattccccgggctgaaactgagttgcagatttacaatatcatattttaaattgctgtcttcaattaaaccatttatgaccataactaattttcaggatgtcgatgcatgcttttccaggccttccttctttgtacaaaagtaaatgtccataaagcgtttcacttatattcttcaaacatgatgctaatttaaattaattacttcctatgatatgttattattcctatgattttgccactgttattagttctctcaaaaatacatctagggaagaggattattttaagtaatttgattatctttctatctcttttatttatttctcatttacttaagaaattcgttccattggttggcattgatacagtaaatttgtaaatgaggagacaatataaaaaatctaaattacttgtgcttaatgactgtagcagaatgccttttctctaaatcagattgtctttcttgcagtttagtttgatagatttgcaagctatgctgcttccatgaagttagctgcgctggtaggaacgcaggcttctttgtctctggttgtagcttgcatgatcgccccattaggcagacaacgtagccggagatcacaaatcaggcccttggctgtagttgctagtgtgtggaggtgcagagcaggtggcagaaactgacctcactgggcaagggtggccatggacctgattctttaatgcactctatgtgttcaggaagccacaggccatatttgactctgagaaagaaaacaagaggaaaaaccccacaaagtataacaaccccttaagatacatctattttaaagtgaaattaatttttcagtttataccattggccaattacaagataaaaatgttcaatttctttaagaatcctttgttgacttgtcttttcatctcttgctatttatatttgtcactgtttcaacaaagtcttatttgctgaggaaggactttgctgcacttactgtaccacatcaaacactggggagggtggtgtttaactttttaaaaaatgttattctgattataacaataatattggcttttttcatgaaaagagcgccaccttgcaaggtttagtgagatttatggaagttgaatacctaagcaggaattgctgctagctccaaaaatttgcgaagcaaaagctagccccaattggtttggaagtttgaaactgattaacagatttgcatttgaagtgactccagacattaggtccagacattagttaaaaatagaaagaggaataaagacatctcttctctctagaaaagataacaccacaattaataatccttcccactttcattgagatcagcttgtctgataacctgatatgagtgtgataatgataaacatgataatagtggtacttttgtaattttgctggtgcatttaagaagatagtaaatgatgagttcatcttttcttcgaacattcctattcctagatgtagtttacctcaaattgggaattataactgtctaatttttgttgtgtacctgatgccccttttgctttaataccacagtgtaacaattaaatatcacactatgacatatgatttaagtaggatattttaaagataaattttaggggtaaatgtttacttcaaaatgactccatatttcaaatatctgtttagactgtgaaggccaaataatttttaagaaaacatttgaagagtagtgtgtttgcatttgtgaataatcttactcacagcaagtaaacgtaataaaagccaacatttaagccaaccctcctgtgcattctcttttccaacacctatcacaaagaaaaagtcattaatgatgtaggtggcctaaaataatccttcgaagttaaatgtagtctattattttgctggtacctttaatatctgcttcttgagatgtattcttcatactttttttcatgggctattaggttttgaaatacataaatgtgaacagcaaaatatattgttagactctctttagcaggagctgaagatgctgcaaatagctgtttcctgtgtgtagctttagattctgacttaggtagaatgctgtcctggttcattttgcaattgcattgtattctgaatactatcaaatgattagaacagctaacaagttattaaaaagttatgttgtgtcaacagaaaatgcctgagtacaagcaatcatatttgagaaatgaagagaaatgagttgtggtatgtgtgtgtgtgcatttgtagagcaagcatataaatatacaagcaccatttatatgggggctaagtaatttcaaacatttcagatcctttgttttcttcttcaaaagctacccccaactgctttaagcgtttgcagctgatgattttgattttttaaagtcaagcattcaagttaacctttaaaaagcaaaccacctccaaaagaaagatgtaacctttcaattgccccatctgcttatcttttttttttctttctttcttattttttttttttcctgacaatgaaagtagcactaaccttctttgctgataggcctggcatttagatgcttttattgtgaagttttctcagaacttttaaagggctggccagagaattataccctcaagtacctcacctagccccaaaagcttccagaagttttctttttgaggccaacattaaatcagtgtctaggaccccttgtgagtcggtgctgttggagttgttacctgagcatactgcttttcaggaagtgagttggagaaggccctagaccttaaagagaagatttagtttaagatgttatgaggagttactgcaggtggtctggcacactcaaaataaaggaacttgtgcccttggctgtggactagatataaagacatcagctcttacacattcccaagttacatttcttttctttttccaacttataataccgattacaaatttatctcctcctctctaggtacagagttctggcttccttgtagcatcaagtgtagttcttagaatcatgtgttcgtatttgtggggaaaagcattttcataaagatagtcacagttgatatcaactgttttagaattattgaaaatagtgttggcaatggaaagattgatcttgtctgtgccgtcaagccgctaaaggtacaagttagccacgatagtctctctttcggcttttaaccacactgtccatcctctgtaatatgtaccatttaaactagttagatatagaaagtaagattattatgggtaaccatatagcaatttttaaaaaatgataagcactattttggggcaagaaatacaaaaaatgttaacttcttatgtcacattcaatccttttccttaaagtttattgcaaatacaatggtgtaataggtgcaaaatatgaataatgttctccttaaatctatgcaaggctggtttgctccagagtcccttccttagcaagaggaaacacatcaggccaaaccagaggctatttttactgtggaagctgggatctgtcatcagttactaaagttgatatccactttagagtgaagaactaaaacagtgtgaagtttccaactgatgttatataccaaaggtgagtttttaaaaaatcgggtt

SEQ ID NO: 98 - DNA, 6047 bp, Artificial Sequence
  subsequence of DLX1
ccccggcgcagacgccgcagcccattgtgcttcctgcccggcgcgctctgttgcagaggagccccggccgggaagtgtggatgcgtcttacccgaggccgggccgcctcgcccgctctagtccagcggagcccgagcgcctcggaccaatccccagtgattatgcaagacagcggaccaatcagctccgccagctcatgaatatttatgaccttcgctgagtcaaagctttgaaccgagtttggggagctcagcagcatcatgcttagacttttcaaagagacaaactccattttcttatgaatggaaagtgaaaacccctgttccgcttaaattgggttccttcctgtcctgagaaacatagagacccccaaaagggaagcagaggagagaaagtcccacacccagaccccgcgagaagagatgaccatgaccaccatgccagaaagtctcaacagccccgtgtcgggcaaggcggtgtttatggagtttgggccgcccaaccagcaaatgtctccttctcccatgtcccacgggcactactccatgcactgtttacactcggcgggccattcgcagcccgacggcgcctacagctcagcctcgtccttctcccgaccgctgggctacccctacgtcaactcggtcagcagccacgcatccagcccctacatcagttcggtgcagtcctacccgggcagcgccagcctcgcccagagccgcctggaggacccaggtacgtgcgcttgccagggagagggagaggaggaggtacaagggagagagggaaagaaggagcgggggagaagaggagagggagagagagagaaagagaagagaggagagcgaggtggggtgggggtggggagggcgcgggagcagtggaggtttcgaatatcaatctatagatccttgtcacagcaaataaatttttttaaaaattccctcaatttgcaactatccagccaaggataaatcccagagcgtctcctggcactggctgggcctctgggcggctcggtgtgcagagcacacaatgccccgctggaaaacagaaacccacatgtgcacgtattagtctcggtaattatttattgcgtagcgctataaacaatgtatgcaattaagggtaattaaacctcaactaccgcctgcaaaaatagcaaactttccctgcaaaggcaggagctgagctcctgggaacggctctatccctcctgcagcgtcccgggacaggccctcggattttgggggacccttccctggctttcagagtttcttgaacgttctctccctggtgctgcctccgccacccttcggtagccactcgctctcggctgttcgcactaaaggcggcccctcgtattaacaacgggccctacttctgctgtccctccaggggcggactcggagaagagcacggtggtggaaggcggtgaagtgcgcttcaatggcaagggaaaaaagatccgtaaacccaggacgatttattccagtttgcagttgcaggctttgaaccggaggttccagcaaactcagtacctagctctgccggagagggcggagctcgcggcctctttgggactcacacagactcaggtacctcgccgctgccgctccgttctgccacgcaggctttccgcggccggcctgcgcccgggtcttcatttgttgctcgctgggactcagggtcggggtgtcactgtgtgtatgtgtttgtgtccacccctggctctcagcgtgtctccttcctccctcattccctctgccctagctctgtcactgctctcggtatcccgagctgcctgccgtccggccctctgtccctggacaatctgattagggcgcaggaaggatttccccagacgatttgtttgggaactcagaggtcacacgtgcctaaacaactggaacaatagactccgggcttaatccctcctttgcctttaaattgtgtgactaatcactcggggcctgggtccgcgcctcagcctccctcctcctcctccttcttaccggttgggggtggggggagatcctttcctccgccctctcacctctcaagtcccagaccttagagaagaaacgggaccttccttcccggctttctgtaagactccggggagcccgtgagcgttcctgacggcggcgggcgcgggtttccgacgtccggtccgggatttggagcagagctggagaaagcaaacagacactagtgcaagaatggttttgaatccaaagagaagttcagcaaaaccttgaggcctccttagtccgtcccaactcaagggcagaaaagatggcgcatagaaaagttgggtcgcgttgcaaataaatttcctccactccttcctaggttttcgattctttttattgatgttgatattggaattgctggctcggtgttatgcaggcgctgtatcttccgcaggcggtagccacggtcggactgagcccctggcaggctaaggcctggatcccggttctcccctcatcacaactcctccctggctctctgagagctgcccccgtgggctgacggcggcgggaggttcggccttcgagcctttggctcttatgggggaagggaggaaggagggatgtctctgcttctctggcagggagctgccagctggcgcagggttgggaggtcctatctctgctgttctgcggtcccttttttcctccctgtgacctaggtaggctcagtggtcccagcctgagtcacgttgttgtccgctcttgcaggtcaagatctggttccaaaacaagcgatccaagttcaagaagctgatgaagcagggtggggcggctctggagggtagtgcgttggccaacggtcgggccctgtctgctggctccccacccgtgccgcccggctggaaccctaactcttcatccgggaagggctcaggaggaaacgcgggctcctatatccccagctacacatcgtggtacccttcagcgcaccaagaagctatgcagcaaccccaacttatgtgaggttgcccgcccgtctccttcttgtctccccggcccaggtccctcccgcctccaggtccatccatcccgtccggaaaagaaggacccagagggaagaaggaacagtggaggcgggacgccctccatctcctcggagccccgcgaggtccggcccagcaacttcccggcatccgcgctctagcctgaaccctggcctgggccgagcagtggcagcagagagtggcctcggagggaagccactgccacctgagacagcccaagcagcaagataaacccgctccacccgacccgccgaccttcagctttgtgggactatcaggaaaaaacaaaacaaaaacaaaatgtagaaaaagcaaaagctcttttctgtcctgtcagtctcctgtctccttttgctctgtctgtgcgctggtaaagtccaggtcctcatccgtccgctgtcctcattctgcggcctcagcaaaaagccacaaggtctgagcggcccgggtcctgccgggctgaccatctccggatcctgggacactctgcctgaccatctgtgtagctggtgtgggaatctgggggcattggagggagggggttttatttattgagaaatggacttcgcctgaggctgtttgccaattcagggttctgctgggcgcaaggaacgcactgttcaaacgcactgtttactttaagcgcacggggagaaacgaataaggaggacgtggtgatttttaatttatacagtaacttttgtacttctctggtatggagagtttggagccgaatgatttgcattttttacatgtccgacattatttaataaataatttttaaaagaaaagaacgataaatgaagccaacatgattttctcatttcgggaggaactctgttgcttcgcctggacaagaaggaaaatgctgatttcctccttgggtagaaagagggagcgagggcaaatggggagtagagagaaaacaggcgagaacaagcactctaattccagtgggctttaaaataagacaaaatcagctttacaacaatccctagaggctcgaccacagaataatgccagtcaccaccctgaacgcacaatctccagtgcaggatctaatgactgtacatattattgttattattattattgttattattgttgttctgtaaacatgttgcacaagcttagcctttttgcgttctgttgtgtgtggctgtaaaaccccatgctttgtgaaatgagaatcttgacatttttcttgtgaaatttggaaaatgtgatcaattgaaatcaactgtgttttgtgttctctatgtcaaagtttagttttatattgagaatgttaacttattgctttgtatcttgggaaaaaaactttgtaaataagttataaagtttctttgagacagtaaaattatgatttcttgaaagaactgctctcttgtgctgtgtgaggctgtgccagggggccaggccaggttcccgcctctggagacagttcatacagggtcagcgacttatcaacttatcggtgatagaatggagaccctgtaccccagaaacaccagggtatcgtcagaggcctgtgaggtgccccattgggctttttcttcctgccttgctccattgacccccaaggtgtctgattcctacctgaattggaagggtaaggagagaatgcctggcgagggttccccaggaagggggctcaggaacaggtgcatcagggcagggctgacgctcaggaaccaaaaggatgttgaagaccggctgagaggagatgaagtcagagttcaaagtcagccggccaggacgatttcagtttttcccacacccagccagctcttgagaggccgggaggttgggaggctgagaggcctgaaagcagagacactgctttgcctctagccttcctccggatcaggcctccctgcttttgcatgcccggaggcgctggattccgtcgcggaaaagacgcagccagacgccaagcaggggcccggaaagacacgtctgtcagactgcccctctatcaatcagtgcgctccaggggacagggcacagtcccaggcagccaccctgggagctccacagtgagaaaggcaggttcctgcctaatgatccggggcctttctctgcacctcacagaaatggaggtgctaaggaaagggtggctgacactttggaaccccaaaatctgaccaaagtcaagcacaccactcccacctcatcccagtccgaaagtcccaaggccaggcccttatgggagcacctctagtgaagcgcttgctcagattagtttcctccagaggaacacgggcttcaagggactagaaccagattggttcccttctcgtggccctgcgtcccagcccagccccaacccccaccccagatctcgcagccgagccgaggcagtcccggagagctgcgggcccagacaggctgccaagcgctgttcctacttctcccgcactcgccttccagcgctgctgcccgcgggagctggccctccacctttggggggtcttttcaggcgcgcggtggggagcagagcccggaaggcagtgatctgtgttgtgacaagcacccatttttcaattggtgctggtgaaagatcagatgcgccaggctcttccgacgccctttgggaaggggaggaggaagtggtggggctgctgggggtggggggaggcggtgtgatggaagcagggaaagtagtcgggggtgggggaatgatgccggggacctccaagccccttccaggcctgagattgggacttctccgcagcacctagaagaaccagcgctgatgggagagatcagacctcagaaaccaggatgtgggcagtcagatgggcctcaaagctgaggaaagaatgaatttcccagctcccgcgcggggtagggggtcttcctaggttcaatttcccctaggagatgtgactttgctagtgcgaagatttctgtccggcatctgactcaggtcccccagacggcagctagggcccaatgcctcaagctacaggcaaaatctgtttggtcaagcggattgtaa

SEQ ID NO: 99 - DNA, 6023 bp, Artificial Sequence
  subsequence of DLX6AS1
caggagattctttgacccaagagcccattcctccaacagtggcctccggcagacccgggaggtcttgtgttggcaatacacaagcatttctctctaaataacattgacactcgcaatacaaattccaacatctcaacaccttaaaaagcaaaaagcagcttaggcctcaaatcctgcctagtgaatatgaccctcacttactacaagccctaaaagagccttagggctcctactccagattgcagggtttacttttattttgaatgataaagacttcgagggccttgcccgccctcctcctcccacccgcaagggttggcccgcgttcccctgcgggcgagacaaagaagcaggagccaggacccggctggcgcctaacccggcgccggggccttgagcccctgaggtgtgcgccttcctgcaaggccccaaagaacccgagtttttgccccttgctgaagggttggaagtgcgggctggactagtgcaaacaagagtgactccaaccgccttacttcagctcattaccgtcacccatgaaaacggaatgaaggactgggaagccaatctgccgcgttcaattggagagaaatgactgtcggaagaggccctgcggtaaatagcctctgagccgcgaactctatgcgccgtggccggtggcagaggccacacctggcagccactcgtggcgcgccaccttggcatgttgtgtgcgggtcacactatctccagttttccattctcgatactggcaggaaagtctgatagtcaggcctgaagtttagattccatcccgcaagcgcagagatatcacaccaagtgggacctctcgctcgttccacttcccagcccctgactgtctctgagctcagactgggtcgcccagcaggtttcagcaggacctttaccatgcaccacaactaccacctcagtgcagctgcttcactggaacagagtgcaaggattttagccactaactattaggggaaggttgagagccctgaagctacaacccggacaatcccagccttcccggcttcctcagcaatcaaacaaatgagaaaaaaaaatccccttgcaagtagaggcagctgcactctggatacagtgctcaattgcagggaccttccgaggccctgccacgacatactctaattggggtgcagccagagttgcaggaagctggcgaggaaagcggtgcacctgtgagcataaagcgaaaaacatagacaagcacagggtgagggtgtagggggtgaaacgccttcacggtgttaacaacaagctgcagggtataaagcaataaaactgccacgtctacctgctggtattgaggacattacaaacagtctcggcgcgcagcccgcgtgtaccgagagcgcactagggttgggagtgggaaggtggggtgggaaatcttctcttttcctgacattcccttctgtcccccaccccccacatctcccccttacttagcccacctttctttttccatgaagcttttctgttgttgttttaattcattgccgatttgtaaacgtgtagatcgtgttactggttcgcgtgttaaagtgcacctcttgttaaaaggtggggaacagggcacgccacttaaaaatgaattcagagttactgaaccggctccccagactcaagaacttaagcgcaacgggctgggaaaaggagggggagaggagcgcaaacgccgctgacctgggaactcggaggaaactcgcgggcagcgagcttcaggtcttctgatacattgaaggaaagaaagaaagacagaaaaagaaaaaaacaaactgtcctggagatagctagacatccagggctgggagctgggaaaatcaattggcataagccgctgccggcgggcttcgcgcaacgtaaaaaataaagtccaagctgctccatctgcagccacccttttctggagttaaaggggcaagcggcaccttttctctatttctcagtttccttcggtcctgtaacttatggagtccagaagaagtaggatatacagaagtcctcagtagttttcccaaagggagacactgtctccttcccgcaacctccagacactgcagtacagggttgttagatattagatagtacgtttctccgtgtgggcaaaggctcgcggcttaggtctctaagcagatcgaaagtcggggtccagaccgagaggatcttcaggtctcgtccacccaatctcaagcctctggaagggcgggctgccggcgacctcctccagtcccgggacccggaacccgggaccctggacgccggtgcgggcgggcctgccctcctctgtgcctggcccccagtctggccctcctacctgttgaccaggcctgaaccacgcaccggggctccgctgtctctgcttggctgccttaacctgcgtgggtctggagaccggagggagaaaggctagatccgcagccttgggctgctccgaacttaatgtctttccccagtccatctttgaaagagaagtggttctaccacctggatgtgcggatataaatccccttgcaaataataaatggattaataataacaaggtatgaagttctttttatagaaaaaaaggagagaattgaaactaaatgcggcagttagacaaccattttgataagaggataattgaggcgacactggtgtataattagaggataatttatgctatatccacttttattccacctcccaaaataaacccagtccataatcattacaggcaaattgttctgaattttatagcagcaatttgaacaaagtactgcagttaatcatgggagatttttgtgtattcctgattagaactctaattgcctccttccagaaagtaaaaataactgtaaaacgactctatttttatcattaacaatgttgacaataaaataaaatcaattggaattgtaatcgagagacaaatttaggacgaaggcacttttacttgggtagtttatattgtaatcaagatttgccaaaccactaaccgcatgtatcatttgcatatatttgaaagcattacagtagcttctgttttcaataggaaaaaatgcattactgtcagtcctccaacgattcgttttcagaacacgctgctgcgttctgaaaagaaaaaaaagacgccccccccccccacaaccttttgtacaatatataagaaatacggcctgaaacggcagggaccgagccagaacagggtctgatttttctttttctgtaccaccccccagtggggtggagcccaggtgtgagggttcgtcttccttctgtggtttcaataaaatacgtctagaaaaatccacggtgacaaggagctcccacaagagtgtagtaggaccagagtggcagggacgtcaagaaaggggggcctggatttaatgcgggggtggggtcactgcttctaagcacaggcaacctacaagggtgcaaagggattgaaagagagcagcccccagttggctgtttcaaggctgagatattggcaactggggctccgggatttggggcacgagctgcggcgggaagcatcggcggccggccgggcagaggcgcctccctccccaacggccccgggcgccacacagcgcggcccccggctgcagctccggctgggattggaactgcggaaggtaggcgaagaactctgcaagtcgcgcacacgccagtagaagccgtgcgcctgtgacgtcagggggcgactgaccaatggggaggcactgccctttggagacaaaccattcgactcgtggcgtctgcatcaagtctgaaagcagacgcgcaactttcgcagaatccaccttaaaatctctgccttaaactgcaccagcccccaaaaaatccaaggggggaaagcaggcggggggagagcagattcccccctccccctctcctctcccatccctcctccttcctcctccctttgagttaacaaggccccgctcactatatctctttatattaaatatatatatatattagagaagagcgagggagagggagaaccacctccacccccctctttaaattcttttttttttttttttttttttttgcaaggatccaaagagctaaggtggctgcagaggggagagcggcgcgagccaagtgggggagggtggaggaaacccgggagaaggctttctccagcccccaaagtttttgatgatgaccatgactacgatggctgacggcttggaaggccaggactcgtccaaatccgccttcatggagttcgggcagcagcagcagcagcagcagcaacagcagcagcagcagcagcagcaacagcaacagccgccgccgccgccgccgccgccgccgcagccgcactcgcagcagagctccccggccatggcaggcgcgcactaccctctgcactgcctgcactcggcggcggcggcggcagcggccggctcgcaccaccaccaccaccaccagcaccaccaccacggctcgccctacgcgtcgggcggagggaactcctacaaccaccgctcgctcgccgcctacccctacatgagccactcgcagcacagcccttacctccagtcctaccacaacagcagcgcagccgcccagacgcgaggggacgacacaggtgagaggccgctggggcagctcgcttctcccgcctcccgactgccccctaccccgcccgcccgctcacttcctcgacgcccgggcctccgccggccccctcccccaggcggccccgcgcgcccttggccgggccccgtgcgcgcccgctcgcctggcgcctgcctgccggcctctcccagccgggccccttcccgccgccgcggaccctcagcttccgacgcgcagttcgggctgagtcccgggcccggcgcaggcttcgttcgacgagttagtccacactgcgctctccagcctcctgggtctgtgcgcccttttccttgctccttccctccaggctgtaacccacgtttgacccggctggggacatttctgggccggaactggggagcgtgttttgcttcccagcccacgctgggcaggcagtggcctactttgcgtggggcgccccgtgctcctcagtgactcggagggaagctggcctggctttcgctctggttaaactagtaacagtcaggctctttccagtgggctttaaagtgtccctcaccttcatccctgaccgggccccctatctagcttttcgctacagtgttggctgctcctttgttcgtggaggggaagcaaagaacctcgggctgatggttctcagcacccgagggggacaaagttgccgtgagaggcgcagcctgctcgtgggctggtctgagctgttggttgtgttttgtttgaggatttggtcctcctcaggagagtcatttcaaaacatgccgaggatgcttgatgcactgagcttggagctggtgacatcaagtcaactggccgcgtaaacacctgggtggctcaagcacagcttcaggtactgttaagccgggcacaggggccccgctccgcccggacagctgccgccttgctgcgctgcgcaccccagagagcctccggcaccgcctccgctgcggcaaagcgggctgtttgtctgagggcctctggcgctcccttggcccagacgctgcacattgttcgggccagggactgggtcaaggagattacgcagacgctgggagcacacgggcagagtggaccaagagaggtcggggcatcatagggatttttcgaggtaacccttattgggctttggggagactcgttgcatgccacgccaggagcagggagatggcagcagtagcctcccgggtgaccgctcctctgtattatttgcttacagatcaacaaaaaactacagtgattgaaaacggggaaatcaggttcaatggaaaagggaaaaagattcggaagcctcggaccatttattccagcctgcagctccaggctttaaaccatcgctttcagcagacacagtatctggcccttccagagagagccgaactggcagcttccttaggact

SEQ ID NO: 100 - DNA, 4118 bp, Artificial Sequence
  subsequence of MIR196A1
ccctggtttcatcccttgtcactgcatcagtcggggttgaattgtccaacaacctgggctccccattagcttgcaagtcaggcccctctccaaggaggtggcactcaggacctatgtgtacccccagcccagcccaaggccagtgggaagcctttggccactggggtgggtggggaggaaaaagtcaactgagggattaggaaaggaaggacttttcggacctacttctgtaggtctggtcccatagggggccttcgacaggaccctgagggctttaggctgagattgcaagagctctcagtgtttgcctttcagaatgagacctactgagccctcttcaaggacctgaagcttcctgctgaggtggagcaccagcccgcaaagagttacaaaaacctcaagaaccccctgcatttcttttgaaatcaaatatttgtgaagttggggagagtttctctggaaagttctggatgtagttgagagctcagagaccctaaggctggaagttggagctctgactgccatctttgggttgggctgaacagcccaacagggccagggaggtgcctcgggagagttgactgctcctcatcccccttcccctcctaacacacacacaaaaaaacattcagaagtgggaagacacttcccagatctcttctctgggggaacatccttgttgctcctggatgaaggacctcaaacctcttccccattttgcaaggttgatcttccagtcctgattctgctcccctcccccaactcctccagctaagcaaggagcagtaactgccgtgaatcgggtggtttaatgttgttgtgttcagaaacccaggcccaacaacatgaaactacctaattcactcagcagttccaattcaagctctaggtcaagagctcactgggggcaaaccctgtggccatttttttgtgggccaaaaagcggcttaacttcattttgctccacctcttccccaacagaagaacccagttgctactaaacaacacatcggaagaactgaacccaggactctaggtaaaaccattttggagccggtcctgatagctcagattccagagacatttgctgccttccaggagccctggccagagaagaagaccctagacacaggcacaagcctgggcagggcctctttgatatacctgctcagtctctgcctctcagcccagctggaggtctccacagataaaaagaattctcaacttcaaacagatacgaaggtgcatctatactcagcaccctgctagcccctgtattccaggtcacccagcctcccagtgtagctctgagaggccagatcttcaagtcctacacaccccccagctttgagattggggctcagacaggagagtgagacaaaagagtgctgagaaagaaagtgacagagagaaaggtggaaaagcagagtgtcagaaagtttcgggaattctagggaacaaacagaggaagaatgggatttggaggggaaagccggttgatctgaacagttgctgtgaaggcaccctgcccaaaatgtcccagggccctggctctgcagaggccgagctgccccaggtaagacaattcattccgaatcttcgcagaataaggactgagaggctaaggactgggattgggacacagagaacaaatttgcttcctccttcctgaccttcggtctgggtccttggccccctaacgtgcccgctcctcacctctgcctctccagacacccgcctgctcacaggtgctcacgctcacacccgcacccatcgcaaaaacgcagctgtgcaggccgagggcggcggcggacttacctgggcggcggcggtgccggcagtgcgcggccgtcggaaggtgcggagccagcggccgcggcccagtccaggctccctcccgccctcgcccagaagcgagggtccgagtggccacgtgtccggcagggaagtccgaggtagcgagggagtccacctggccgcccgctccccctcccgggtataaatcttggggaccggaaatacaataaaacttcaccgtgttgatgaacttcaaacggtttacatcccctcctgtcctgaaaagaaagacgtccgggggcggattaaaaggaaggggaaacaaatttacgagcggcagaagcacccgcctcggcccctttctttgcccgcacactttgtccgcgtggagagaagcagccccagcccccgggacttggcctccgccgaaccggccgccaggcgcgctcttctctcggaggagtcggcgctgacccagcccgcgcccggcagagactggaagccgccgcctacacggaaaatccacagagccccgcgcagaccctatgatcggctcggcccgccgggcttgggatgaggctccctgcttctcgctagagcagaactgggctccctggcgcttccttgcgaaagcccaggctctcccaaccacgcccggtggcctccattttttgcatctttccgctgaaagcgggttttttcttttttctttttttttgacagagtcctgctgtgtcacccaggctggagtgcagtggcgcgatctcggctcactgcaacctccgcctcccggttcaagcgattctcctgcctcagcctcccgagtagctggaactacaggcgcccgccaccacgcccggctaatttttgtatttttagtagagacggggtttcacaatattggccaagctgatcttgaactcctgacctcgtgatccaccctcctcggcctcccaaagtgctgggattacaggcgtaagccaccgcgcccgacccaagggttttttgtttttgttttttgtttaactttacttttctctttccttttccgtttctagcggccagacctttgcccagccctgcccgtttattgccgggtacttgctggaaggggacagaagataagactcggggtgactcccaaggcctgaagggggctgattgggccgggggctcccagaggataaacctaggggccggtcggtcttcctcggcgtggaagtgagagccacgcggcgtggcggagctccaccaccgtctccttatctctttaaagcctcaaaatcaaacaaaaccactactacccaggcctcaagtttccacagtttttgtctgctctggaccgtttactttttttgaaaaaagagaacttggtggaatccaaattctctactaggcctccgaaccaaaacgaaggaaaatccgttttcttcttgggcttcagagaactgggatcgaagtgattgacttcctgctccttttgtctgctccaggggcctggttaggtgcccttctggatgggagagcaaaaggttctccatcctgcctcacagttattcacctccaaaacagttttgagacacaatggatggctaagattagctcaggctcaggcagagtgttcaggtacaggagtgaggtccagctgcaggcccaagagggggtttagtgcactgaaggcacccaccttcccatagatacacacatagataaccccactccccaaccccaagaaaaggcaccaaagtgctgctggatattttaaaaatctgattaaaaaataaacgggcagggaaaatactaggcagtataggttttgaattttctgaagggttaactctgctgcaggcagtcccactcggccccagctctccagaggtgggtggtggtctgggggcagtgccctctggccccttcctagcaccaaaagggaggaattggggagctctttaacagctggagggcaggaagtatcttatttctggccaacattcatattccagtatttgcatggggaggcccctccagcctccctcatttgctctttatcatgttatattttcattcaaaatactgagatggcagctactggctgtcacttcttctattaggatttccctctgggaggacggcaggactgaggggccagcagtttccagaccattcaagagtgttattacccatcccctaccgggcacctggtgggggccggtgtgctggctcccagcctactgctggcctgggtctctgtggctccctggctgagaaaaggagatggaaaccttttatagtcttagactctttggaaaaactgaagaggc

SEQ ID NO: 101 - DNA, 5393 bp, Artificial Sequence
  subsequence of FEZF2
ccgcaagtggcgcacgtgaaaggcttcttgtcgttgtgggtgtgcatatggaaggttaggttgtagacctggtggaaggccttgttgcagatggtacatttgtactgcttctcgccgctgtgggtcagcttgtggttcttgtagttccctacaacagatcaagaacaaaaaacgtgggggtatggagtagaatggtggggaggaagaggcgggcgtcccaggggcagcccaggtgcctgctcaaaaaaggcgacgcttggctaggcgggcgcgacctcttcgagtgaagaagttgtcaaacttcgtaagcgtcaagccgggtgctctcccgacaagaccgagactgagtcccgcggagccgctctgcgctcctgctctgcccgccacagaggctggtgcagcttccctcccgccgcgctccgcgggccgggaaacttttgcgtagcccagagacgcaccgagtccttctcctggctgatgcctcgctagaagaaattcgcacgaacccgggcttcatcctttttcttttcccccttctcatttttaaagttacttctttctcgccccccaactaccaactgaagatccaaaagtgccttggaaaatccgatccaggggccaaggatcataccggtttcccccaatcttagattgttcccgggagggttattttgcctccaatatttttcatttgaaagggaagttccggatacaaaaggaacctttttctatagggcaataccctctccttttcctacatcctttccttctgtccccgtgcttccttcgacctctcgaattcggagtctctcagtgcacccagcctgcatacagcgtggtctactaaccccgctaggagagcttccccctacaccaggcacaacccgattctaaagaaatgctgcgcccgcgcctgcagatttcgccttctctctccagatccctctttgccttcctgccagccagccgcgacccgagtcctgaggtgaggtgagaagagaaggcctcgcctggcacgttacctttttggtgaaagcctttgccgcaaaattcgcagacgaagggcttgtagcccgcgtggatgcggatatgcgtgttgagcgtggagctgcggttgaacgctttgccgcactggttgcatttatgtggcttttcctgaggaaaggggcgagtgcacagtaaggagaggccacctcgggaacacctggaagggacatcccccccacccccactcaaccctagagggtaagggataatctttggccatcgtatccccggtgttatcactaagattctgggggttgcgcgcgggctaggcccgacccgggggccacgtacctgggtgtggataattttgtgcctgcagagcgtgctggcctggcgaaagcctttgccgcagactttgcacacgaacggtctggctccggtgtggaccggcatgtggcgggtgagattatagtgagcgttaaacacctatggaaagacatggggggccttgtggtgcgtctgtccgagggcctacaatcagccccgggggggccacagcctacctcccccaaccaacacccccttcagaaaccagagcctttttcagtttgtaaagtgctgcccaaactcctgcttacaccaatactgtgtggccgctgacaagggcatccccattttacagaataggaaactgaggcccaacgaggctcccagtttgggtagtcaactactggggagctcctcagcttgaaaaaggggcattccaggctgccccaaggaagccgccgccgccgatcgcccctcccggcccccctcgccgaaccctgggcctcaccttgccgcacacctcgcaggtgaagtttttgggcttgccatctgcggagcctcctggcagcttgctgtggcccttgacgcctccgcgctcggcagtcagggccgagttttccttcagtacctgctccagcggcgccggcaagcgctccttatggggatagggagccgggtgggggaacttgtccgcagccaggccggccagcttggcgttctccagcagaaagagcttggggtgagcagccagggcggcgggggcctgcgcattgaggaggccagacgggaagaggtggccgctgaggagctcagacggcgggtacgcggtcgagtccaggtagttgaagtagtagagcgagccgctggccggcagccccacagcctggttgatgacctgcggcttgatgaccctgcccgcgggcagcgcggacggcgccaggcccagctcggccttgcagcacacgccacagttggttttgcacaagccgctggcgccgcacactggggcccccccgccgccgccgccgccaccgccgccgccgcctccgccgccgcccgcccggaggctgcttttccagagctccgagtaactgagcagtgtctttgacggcacctcgtagcctaggggctggagggggatcatacagggcagcggcgagcagaggttgagcagtttcttgccctggctgccgtccgcctctagcgctccaggccggggctcaaagggcgcacggggctccgacgtcttggccatgatgcgctcgatggaaaaggccagtgtcttggaagtggccggcgacgctccggcgcgcgggcaggccgggggcaccatggtctccagggaagccgagcttgccatggcgcgcggagctgagccgagccaggctgggccagggcgcagcctctctcctctaagtctgcattccggaaaaggcaggggggaaaactgcaatttaataagcacctagtcgggcccgggtcacccatttgcattcaaatgaacaggggcaaaacaaagtgcacccaagggtaccaaattaccgcccattaacccggcgcgcaaaggaacccaccagcccctgccctgggactttgaaagggggaagaagggggagggtttacaaaagaaaagggggggggcggtgagaaaagagtctcaaattaacccccctgagcccttccctggacccgggcctctgccacgcgtgctgggagctggacagtgaaggggcaaagttaaagaggaccggagagccacctcgcatttacctctttcccccaccaccaaggagatgcgttccgagccatgcagcgtgtctcttctgtcacattttgatggcaaacatcttcccctccgcgtgagatcactgtcttttacattcagctgacatcacatgaagtcacttgaagtggaatgacatgggcggcggcgcggctcccgtagcggcccctgtgttcccccgcgcctgccggccgccgccaccaccgcccctcaaactttaaaaggaggcaactggcgcccgcgctcctctcgggaaagtgcgagcggtttgcgaatagggaaagagggaagagacgggagggggagggggaggaatcgtgatggttttgccggtggaaggaaagggggggggggacccaaacccaaacctaggcagagttccgtgcgtgattcacaactttggaggcctgcaggtttgggggacgcggggagggcggagggtcccggacgcggcgcccccaaagggcccctgggtatcagtctagtagccgaagtatcccttagccctccgcagccgagctgggcatcgtgctaataaactgccatttacccacggaaccggcgccagccccgaacacgcgcaaatgataattacctcattaggatgtggcgcatggacgcgggcgccgcgtttggaggggggaacttgttaatggggaaatattaatttatgcaaaagcaatgagctcgccttggctggcgtcggaggtcgggagaaagctcccactgactaaggacgaccccgaagcgtcacggagagcaaggccgctcgccggcatctcgggggcctcggcgccgcgcaggtgcgcctccagctttatggccagctctgggtctgaggctgggggagactaaaccgagagctggaagactttcggagatcctaatagatcagaattgttgatttatgatcgggtttctgaggcaaagccgagttctgcttctggtttagggctgcgtgcggggaggattcggagggcagctctcccagctgatgggtacttactgtttgtataattgagaaggtcccatctccacctgtttaaggagcagattgaaacagcagaacctccccctggatcctattaaaacgtttttcctcctaaggccattcagtcgaaccaattttccgaagtgattcatagagctgaattctgccaaggcagctctttcacttttagccactaaagcaccgcgtggaaccgggttttgtgtttttctaaaataaagagaaggattatcagagaggagagggagggggcctgaagggggacgggcagagacttagtgtggccagaggtacaagcagagggaagaaaagacccttttctagacaggccccaagtaagttcggaggaattcagcgttttgtgcctggcgcacaaaagcagcgcgctccgcgcttggtttggaggggctgaattcatctgtttgcagaccattccacctgcgtatcacaacaaactgctcaaagacgctccagcactttcaacaggccgggtgctcttggcgacaacaaaagtggtcgaggctgagggttcttacggaggggggtggtggtggctagcaagagagcgagcgagagaattaggtttaggaaagggggaggactgggtgcaagggttttttgaaaagttttggctggttttgttcgcgggacaattatatcttgctagccagcttttgcaagaccacgagctttgtagccgcaatcacagtttaagaggattaccgtggatataatatgagcaaacagggtttgatagtgaattccatctccaaagacacacgatcatgtgaagccagagaaagtggtggtagaggtaaaccctctgtttcttcacccaggaacaagtcttgagagggctgagtatcctgtcctaggcccctccatgctgcgaaacatccctggagaacgttaagggacgggggagaaaagctctagttttaacttcaggcaaatcgctccctttttcccttcaataaaagtctctttccttctgcccacccatccagttgcggctcctttgaggtgcaattttaggcaggatttggacatagcaggtaaaggaaggaaaagtgtacttggaaagaaaagagagggaacagagagaggtccctgagggaaagtggcttggaggtggactgcaataggctaatgctctcaccctgccaaactctgaaactgcccctaaattccgcaatcataagtctgttcccataacgtcaccctcccaccccctccccaaactaccagatttctaagccaagaggcttgctcatctggagaagaaca

SEQ ID NO: 102 - DNA, 5442 bp, Artificial Sequence
  subsequence of STAG3
ctcccaaagtgctgggattacaggcatgagtcactgtgcccagccatttgtcttatttatcattactatttttttgaggggggacagggtcttcttctgtcacccaagctggatggagtacagtggtgcgatcgtagctcactgcagccttgaactcctggactcaagcaatcctcccacctcagcctcctgaatagctgaatacaggcatgctctaccacacctgactaatgattattattattttttttttagaaatggggtcttgctgtattgcccaggctggtcttgaactcctgggctcaagccatcctcctgccttggcctcccaaagtgctgggattataggcatgagccacggtgcccagcctttgtcttagtttttggtccccctcacctgaccccagagttctagaaccattcccttggaaagaaagggactggtcagggctggggatggagaagtgctgtggtaggagccctttcttctctttcttccccagctggatcgccatacctaccctgtggtcctcatcttcctggcctcatagctcctcctctccaagcatgtcttccccgttgcaaagagctgtgggagataccaagagggccttgtctgcatcttctagttcctctgccagtctaccctttgatgacagggactcaaaccatacctcagaggggtaagtagatgttgcattgtgtggccacttcctgtgtccctggcagccttccccctcgttttcccacattgatgataatatgcgtgggactgtgtgaaaacaccagaagtgctatactcgttcagcacagtgacaccctccctccagctccaggtgttttttttggcggtcctagatgttgtagacatcaaaatagtagtacatcctgtttttttttttttttttgagacggagtctcgccctgtcgcccaggctggagtgcagtggcgcgatctcggcttactgcaacctccgcctcctgggttcaagcacatcctgtttttaatccatcatccatcttgtctaaacctctcttaaacacatttctatgttcagcatgtaccaaccctggtgggggctgagagctggcagatgggggagtaaagagttctttatttgttgcctggtaaattgtatatactttttggctagtgtcccctatttcttctacttggggattttgtaaataggtctgtgtatccttatttattaccatatatgagtttattctgtgtaggttataataatatatcttggttttttacctttccagaaggaaaaaagcgaatttcatacagatctgctttatcccctggctgttttaattggctttctctgaatcatttctgtttctgtcagtgctgctgtgggggaccagattatatcaaagttataaacttgaattgataagacatgtggtttatgtttcaagggggtgaaatttaactctagatacatattactctcccatttatggatgaatgatagatgacttcctgagccatgattatctttctctacaaagagcagtgatctcgctacctgctaagtgagtatcatttgattctcttcttcggagagaatactaggaagagttgtccttctcctgcctcatttcctcattcttcatctccattgctttcatgtgaaagttttcctttaaggctttgtcccggccgggtgtggtggctcatgcctataatcccaacactttgggaggccgaggcgggtggatcacctgaagtcaggagtttgagaccaccttggccaacacggtgaaacacctgtaatcccagctactcgggaggctgaggtaggagaatcgcttgaacctgggaggcggaggttgcagtgagctgagatcatgcgattgcactccagcctgggtgacaagggtgaaactccgtctcaaaaaaaaaaaaaaaaaagactttgtcccaacttcctactaacaataagctcattttttcttaaaatctggatatgtttttctcatggagatggggtgcggtgagagacagagaaaccataattaattagccttttatatggagggaatagggtggttatatttaaagagaaccatactttctcacaggaatggcgactctttgttagctgatgaagacactgactttgaagacagcttgaatcgcaatgtgaagaagagagcagcaaaacgaccaccgaaaacaacaccggtgagtcagccagttttcttttgtttttgaatcttgtgggggaagcagcccagctacttgggaggctgaggcaggagaatggcgtgaacccagggggcagagcttgcagtgagccgagattgcgcccctgcactctagcctgggcgacagagcgagactccgtctcaaaaaaaaaaaaagaaaagaaaacctaaaagaggttcaggtgatacggttcataaaaggacaagatttacaaagtattaagggatggaaataggaagaagagaaattttgaagagaaaagaagagaaaaggacgttaggatgtagagatacaggaaggggactcaaggactttttttttaagggaaaaaaataaacttcataacaatataaaaatcaattatttcaggactgagtctaactcagactctgctgtggaattggcagcttaagcctacttgtgtgataatgatgaaaccaagcgttaatgtcactgttaccttttttgtttttttttcatatttctgatctttttatacatattaggtggcaaaacatccaaagaaagggtcccgagtggtacatcgtcatagccggaaacagtcagagccaccagccaatgatcttttcaatgctgtgaaagccgccaaaagtgacatgcaggtaaagcagtgtctcacctctgttgataccatctcactttttgtaaggtggtaaggacaagtgtctacaaacttgatttgacgtgaacattttagtgagtgtaacatgtcaagaaagataaggttatggggtgaatccttggagtgatagaagggtaaccttgaatgagagagcatgttctttttttttttttagacagagtctctttctgtcgcccaggctggagtgcagtggcacagtcttggctcactgcagcctctgcctcctgggttcaagcgattcttgtgcctcagcctcccaagtagctgggattacaggcgtgtgccaccacgcccagctactttttgtatttttagtagagatggggtttcgccatgttggccaggctggtctccaacttctgacctcaggtgatccgcccaccttggcctcccaaagtgctgggattacaggcgtgagtcactgcacctggctttgagagagcatgttcttttcttaaaggtatcacaggagtgattatgcctttattgattgatggagcagatgaggagaggcattgcatgacacaggaaggaagcttggatgtgggtggcaccttgttcacccatgttattttttagctccatcttgacaattatacttaattattttttccttgtttctttttttataattttattgaagttctaatacccgaaagtgtacaaagcttatatgtagtttaaaaaataaaaatgaaatgattactcagatctctagccccagctcaagaaatgaaacattaatagtgctgtagagatcctttgtgtaccttctttctactccatttcacagtctccttattacccacaggtaaacactagagtgaattttgtgttaatctttctcatctctcattatagtgttaccactatgaatatgttctttaattatgtaaatgaatccattattcaggcttctatgatttaattatttgagttaacattgtttgagatttacccacattaatgtgtaattttatagtttctgggaaaatatttaaaattttcaaacatatagaattttgctagttatattttcgttatttgatttctaacttcattgtgttgtagtcagggaatgtggtgtttgaaatttatgtaggggccgggcacagtggctcacacctgtgatcccagcacttggggaggctgaggcgggcagatcactcgaggccaggagtttgagaccagcctggccaacatggtgaaaccccatctctactaaaaatacaaaaattagctgcatgtggtggcgtttgtctgtaatcccagccactttggaggctgaggcatgagaattacttgaactcgggaggcggaggttgcagtgagctgagattgtgccacggcactccagcctggatgacagagtgagactctgtctcaaaaaaaaaaaaagaaagaaatttatggagacttagccttatggcctagtattgagttggtacattcgttttatcttttctgtttctttttccacctttgcttgccttcctttggatttcttatcttctgcaaggacctgagcacattttaattccaaatgtcttttccaccttatatgcagttgtacagcgtgttagtttttttttttttttttttttttgagacggagtcttgttctgtcgccaggctggagtgcagtgacgtgatcttggctcactgcaacctccacctcccgggttcacatgattctcctgcctcagcctcccgagtagctgggattacagatgcatgccaccacgcccaactaatttttgtatttttagcagagatggggtttcaccgtgttggccgggatggtctcgatcttttgacctcgtgatccgccggcctcggccttccaaagtgctgggattacaggtgtgagccaccatgcctggccttttatttcttttttttagcccattctcccccttttatttttaaaattttattaaacatagtcattttataatctatgataaattattatctaaagtctttgtgagtataattctgtcagtgccttgtttctttatatgttttactaggttttattgtgagccactcattttccctggagttcttatgtgttggaattctttggggcctaggccaaagctgggtttttaagaaaggaacctgcttttgctttgacagttgtctggggacactccagaatcacttttttttttttaagacagggtctcattctttctaggctggagtgcagtggtgctatcacggctccctgctggtttgacctccctcagtggcgaggtggtgatcttcccacctcagcccctctcatagctgggactataggcatgtgccaccatgcctgactaattattctgtttttggtagaccagcctgggcaacatgagtttcactttacttgggttactgctcccagcctgaatcgcttttaattatctgaatgattattctgggctgggtgtggtggctcatgcctgtaatcccagcactttgggaggctaaggtggatctcacttgaggtcaggagttcgagatcagcctggccaatatggtgaaaccctgtctctac

SEQ ID NO: 103 - DNA, 5140 bp, Artificial Sequence
  subsequence of PTPRN2
agagaggttaaaagctctgtccaaagtgataaacctcattgctggcagagccagacccgcgcacagatctgcttttccacgctgctgctggacccatcctcgcaccctgcgcctcatgtctaagactccccacgccgtctgcgcatgctgccgctctgccaaacctgtccttctcccaccacaggcctcaagtctaagactccccacaccgtctctgagaggaacgcctcccacagcacgcacagagattccctagataagaaggacattcacaaagagggctgaaaggctcatttgagagggggtgattgacatttgatggcaattactaacggatatttttagtgtgcctctagtgtgaataccgttttgacaacagtggagttacaccaaatactggagcggcattctgcactgcaacaacactgaaggacccgagggtggcttctccgtggctctgaggttaacgctgcagcgtatgcagcaaacacctgtcaaggacccactgtgtgctcggcacaccaaggcaggtaacaaaggacccagtgcatgctcggcacgcagaggcaggtaacaaaggacccactgcaggctcggcacgcagaggcaggtaacaaacgaccagcctcagaagcagatgtgcttgctgcaaaccaccttcctacggcccagcagaggcacaacaagcagcgaattttttccagggcctcccgtgaacacggcaccctacgttgccatagcgacgccatcccagctctgagccgcaacaaagcggcagtgtctgtgtctcacctttggccatcttgttgagaaccatgtcgatcaggacgtaggtgccgctccggcctgcaccgtcactgccaacagaaggagagaaatgaaagtgctgccgtccacacggaagcccgacccacaacaaagctagtgacagttcatttccttcctgcttacgggggccggcgagaggaaaggatggcggatgtgagagggggaggaaggacgcgggctgggagaatccaagtgaggggagaagggaggcccctgggggcttcgagcctctgagcagcttgtagcttgtgggatgagctgctgtgctcagatgtgactccctcttgcttgttcccccctctttggccaaagatgtggtaaattttgccagaacaaaatgaactaagcgtttgactgtgtcagagttgatggcatttgtattgaaaatatctgcaaggtgccttctctagtgttgccgggcaacctcccgagcggagaggggagggcgctgggcggctgggccccgctggctcatgcacgcagggacacttcaggcacatccccctaggctgcctgccaccccttctaaacgcaggtcctccgtctcagaaggagaaattgacataacagtcgttactaaatcttactctttaaaaagcactctcatttcatctctttctcatcccaccagctataattggaatatttaccatctgggctagagttgtaaaaatgttttgaataatacttcaacagtagcaaaggaaaaaaaatttccctttttttctggaagaagagtagcctcaggatcatccttttcttatgaggaatgtgtgaagccatttcctgcccccgtgcagacgctgtcactgggttgcatgagtttgagagaccttcttaaaagtacatagggctcgtgttcacacccatgactggcttttaaacagaggaccttttacatttataatcctagcaaaatcaattgtgactttccggaaaacgaataaatgtttccatttcaagacttcaagaaagatgtgactacccagcagatatcacactttcggttctgctttctatgccgtctgtgatcccaagaaatgactggaatcctataggtgatcttttgatggtaaagaatcagcgcattttggctttaacatgtttcctcaaacaaatggttgaaaaaagctgcagttgggatggtaaatgtttaaaaaacggcacgttcacatcctcacaccctcactgcatcaccaaggaggagaggcggtcggcctgggccgccacgtaaccctcactgctcatttcaaagggccacggtgagcattctggttgctgagtgcctttctcacttgtctcctatgcacagcatatattcacatgaatattttaagatatacttcaaaaatcttccaactaagtgttgcttgtcttgatacatttgtgggtaaaaaagatgttctactctactctgtaaggataacaaaccgtaatctattttcatcctcctctctcatagacaggaatgcacacacaaaacacacatgcttcttgattggatttgacagatttggtgtttgttctttggagacaggtttcctttttattccaggcaggaagaacattctataagacagttctagaaaaatggaatatgagttcttcaccaaaaggagttgggtatgaagtccagcagagacagtactattaggttgagttttctttgcgtaaaatctattcttactggtgtggttttaacgtacttagggatatgagtcactgaatttttacccagaggcctgaacccacatgataaactggaggtggctgtacctcctgtaatgacagatttcgtccctgtacataactggccccaagcatttctcaccatctgcagagggttctgagcctctgctggacgtcctggtggttgagacaatgcaacaggctgaaaccattgtctcgatgtttctgtgtcatgggaccacagggtttaagaacaagcaaggtggcaggacatgctcacgggtgagtagaaggcaggacactgcaccgtgggctgctagaaaatattccatgtgaggcctcgcgcggtggctcacgcctgtaatcccagcacgttgggaggccgaggtcggtggatcatttgaggtcaggagttcaagaccagcctgaccaaatggtgaaacctcgtctctactaaaaatacaaaaaaaattagccgggcgtggtggcgggcgcaatcgcttgatcccgggaggtggaggttgcagtgagcctgacgagaccacgccattgcactgcagcgtgggcaacagagttaaaaaaaaaaaaaaaaaaaagcaagccatgtgcagtttatacagacataatacaagcaacgcccaattgtatttacccaaatggcatagaaaagtaagtttatatttttggtttcctttagaagtgccagttagttatatttattaagcaattagaaagttaagcttctgtatttaattgcatagattagtttttgaggtagccaaaacttcttaatccattaaaagttgtacttgcctgcaatgaacaattattggacaagaacggcccctgtagcacttgtttacttttctgaaataaaaagagatataaaaattatcgttgtgtactaagactttgcgttatccaaaacaactattaaaacaaagcgcaaggtctgtgtgtttgaaatcattttgcaatcgcttgttttgacggagaaaataaaaatcatacgcataatatcaaacatttattcttcttctcaacatgacgttattaatcggagctttaaaaccaatgttacacctctacactgctttcttcttccaaggaggggtgccaggctttgaaccagtggactcccggcctgtcctgcccgtcccacccctgcaggctctcctctttctgtttctgcttatgttgacttgaccttttgttacactacatcttgattcttcactaaaatttttgagttttgcaatttatgctcaaaatttcttagtccagacatcatattgaaaactgttatttccatactgtctaaaaacagcatcttcaagggcatttgtgacccgtcagcttttggtaaggatatctaaattacggagaaacctctatgaagtccaagacaagtcccttccatgcttataactttgagtatacaaacaacttcattgtgcagagtttagatcagaagttgtaaaaattagaaatgagcatatatttaagatttcataaccaacccctaaatcaaaacagaggactgatttaaaattcactgtgtaaatccaggtgtttttttttaattcagtgaaacaatgaaacatgtttatgaagtccattaaagttgtcagtgaactatttctgaataagtaaaattaaaggcggaacctcgggttattggaataaagcatgtgtgaaggagagtgttctacaatgtgctgcgtgaactcctacaagaaacaaattaagaaaaatggaagtatggaccatcaatgggaaaatgtcacgtttctttgcaaagccttgcctatccagcaccaaagagtccgtggaaagtaaacattccatcaaccggtgctttgctacaaacctttgaagccaggaggggcagggtggctgtggaaggagaggggaggtgagtgtccagtgagcatgaggggagggatgcttgaatacggcggagcccaaaccacagagctttctcctcctctcttcctattccctgaggagttaccagaacaaggcccttctgatgggagtgtgaatgcccagtctggagggcaccacgggagctgaaggagcagttgcagggactggactcggcgtgcccacctgcagatgggccgcggccacagcctagccaggacgcacttgatctgtgctgccctctggtctgtgaaacacgaggctgatgcccaaaaatgggcgggctcagacacaggcacaaccagcaacggcctccagggccgtgtcaccgtttctgttagaggtgtttgttgttgtttttccggggcacacagtggtgcgaaggctttggggagaggcggggaaggcaatggtgaactccttagaggcaacagcacttgtatgccagagtgccttgaacattcttggtccctggagaataaagaggttggaaaacagacccacttatgtctacttctacaattttccattcctgactcaggctgtaaagcatcgagggctcctgatgacagaatggataccaggcctcaggggtgcaccccagcatgggggtgggaagccctccagctcagtaaagaccatgtgtgtgtgcatgagactgcacgcatgtgtgtgacgtgagcacgtatgtgcacac

SEQ ID NO: 104 - DNA, 4606 bp, Artificial Sequence
  subsequence of BARHL1
cctccccagcctttctggtcccaaaacccgaggggggaactggccaagcccttgttccttggggacagggtgactgggaagtgggtgttggggcaccggacttgaactcgtttcctaatttccctcccgaacacactcaccagacgtagatgcaaatgtacaaacacagaggcatccacacactcaacccaaatagccacacaccgacacacacatcaatacaacttgcagtcacacacgcacgcacgctcagccccacagtcactcgcacgctcttagcagaggcaggaatggtgcttttcataaacaagcctcagaacacatcgccccattaataataaatactgattactgctccgggcatcaataattaaggcctgttacagtaattacacaattatgatgatgatgaataattcagggagggaaacagggctggtgtggctgagcccaccttagtgggaccctggctggtccgcctagcctcacctgcaggtgagcctagggtccaggcctgacttctccaaaccccaggccgttggctggccaaggcctctggactttggggccagacagtgcgcagggctcgcagtgcgagccctggaggatggcaggtgcagcctgctccagccggcagggcgtgcgagccgggagcgggtcctctccggttgccatttcaggcctgctcgcttctgctagcttgcagcccggccagcctgcagaggaatcaatcgcattcccttccctgaagagcacccccccatcccctcaggcctctccagggtgatcctaccttcataaagaggcacgcgcagggaggagcaccccctacccagctccaagggttcgttctgcgatctcctgggcagggtaaggcgcagttagagccgggctttggggtcagacagcagggcttaaaacccaggctcctttttgaaaaccggcccagacctcagttttcctctctgtaaagtggggtaagagccacggaaggccggtggaagataaaaggagaggatgcacgtaaggcgtgcgatggtgcctggcactcggttatttattaacaaatgagtacgatccctcttggcctccctacaggctctctgggccaagcagtggggaggggctggggtcgctggatgccctagccctgatcccgccatacgcgtttatttcggcccccaggactaaatggaagcgacagacggccgtcgggttggagctgctggcggaggcaggcaattactcagcgctccagcggatgttcccgtcgccttatttctacccgcagagtctggtttccaacctggaccccggcgcggcgctctacctgtaccgcggccccagcgcgccgccgcctgctctccagagacctctggtgccccgcatcctcatccacggactccagggcgccagcgagccgcccccgccgctgccccccctggccggcgtcctcccacgcgccgcgcagcctcggtgaggcgcccgtcggctccggggcctcctcccgcgggctcggcgtggccccttccgcccgcctttctgagggcgcaggttcgacgccctttcccgggagggggccctgcccggccctccctggcgccccagcccagtgccccccgaagggccaaatgccaagtccactgaggcccggaccccggactgcgtctccccagcccccctcggcgtcctctctcgcggccgctctgtccgggagccatccccacccgccgggtgtacatacgcgtctctgccactccccacccccagcctctgccggctcccctaggcaacccctttctccccaggagcgggtgcggctgattcccaggcttcgctctctcccacgccccttctacgctccaggtggagaacagcccctctccccgcgcccccgccagggagagaaggggagtgcggagccccgtctccctacccctcgagcacctgggccagcggctgagctgtacataccgtgtgcaaagtgtatatgaagttatttattcgtgacccatgagcccgtgaccgtgtccgtggattagtgagtctgtggcctgtgccctccccactcccaggcggggcaggaaggggccaagggggcttgcccacccaccccgaccccagcccccagcctcagccccggtccgggggcagccaggcctctcgggttctctcttttttaaatgtcgaaataaacttcttacaaatgaccaggcgcctgtccgcgctcgcgtcgctgggtccgcactcaacccctctcccatccctctcctggggactcggtttccttccatcctcaataacgaaacatttttgtcccccttctcttccccggtgctgtggacatgcgcgggggccccgacgggactcgctggggcccgggtctcccctccctggcctcagtcttcccatctctacagcgaggccagctcgttgttcccctcctcctcctctgtctccatctggttcctagcggctcccagacggtcccgagggccggggcgggggtccgtgccggaacaggcgggggtcagcgcggggcctcggtcggctgcgggccgggctgcggggccctcgccgagccgactcatctggccgcgacaagggccccggcagctggtgaccggcccgccgggcgcgggccgacagatgggctccgaggctgctccccccatcactcccaccctccgcccagcgtccggccgcgctcgggctcccgacgctcgcgggcgccaaggcggcccgggcctcccggcctcccgcaccaggcaggactccgcgcgccttcgctgcgaaccagacgccacatcgggtaaacccccactcccacatcttctcacctcccctttaccccgggaggaggttggaaatgagacccagaggggagccaaatcccagcgtctgccccatctcttctggctgccccagaccgcagctctagcatctcaggggagaggggtttaagtcccgagtcagactcgaggcttccagttcacgtccaaagggccacggtcacctgagactgctccctctctggggaggtgggcgcaggtgctcccttcccacacaccacctgcagctcgctaaccctcagcgctgggaagttttgggggccggcaagccgtggcccctctagtttgggggcagggtttctctgaagacgggggctgtgttcagactataacccctctcgaaaaccatacccacagccaggtccgctactgtttcctccctgccccgaaacaccctcgcacagcagctttctttcctgggatggcgagggtattattctaattttgcaaaatgcacagcagctaattaagtcaaggagcccctcggctttcgagttcttttgcatgtgaatgggggttggtaaatccccagctctggctctggtggggggtgaggagagactgtccccaactcagggttaatgaagtgggaaaggagtctctcatagcctcctgcaaacaaaaccccccatgcaacaaaccctgcccaaatcctacatggattgacttaaacccaggggataagtgctttaaattaatctcattgaataagaatgagaccaaacaaaactctttaaaatcatattaaaaatctatcaaaggacaacttgcactggtgtgcttttcattttgtgaaagtgaaggagatagaccgtagcaaccaccctcacatttacacagtggcagcgcaaaccacagacacattctcaactatgtaattgtccttgtacctcagaggcgatttcatatcctacattaatgaagaacaaggcttccctacaagtttataattagaatattttaaattgtcctgcacatcccatctgtaataataacttcacaacctttgcagtgaggtgggctcctgccttccatccacttagaaggctaaattggtttctgttcccaaccctgaggttgggcgagctctcgtgtaagaaaaaaagaatgaatgtgggaccccaacaggcctgacaataggagagggctgagaagccatcttcccccgctctgccactgacccatcccccctcataaacgccgactcaacagggagggggcaacaaagttgaaaagaagtttagagctccctgctggccctcggtcgcaagggaaattgaggactggggcaagttgagaacctgagctgattttcagggtgccccactccccccacagcgacaggcctggctctggattcttcctagtgtggagcagattaagagataatgtctaatgatcaagggggaggtttaacaagaccagttaagaagccttttcaagcagggcaacttctcccgtggaaaagcctccaacttgcgtctctacaaagcaacgcccggattttaatggcttccactgactgtggcctgaagggctaagcggggaggcccctggcagtttgggagatacctgctccgaaaggtctcatttactcccctcttccctaaagttctcctcccttcaccccagggggaaaagaaaaaaatcaaaataacccactgggcttcgttaaaaaaaaaaaaaaagtcctttactgagatttggttggttcgttgcttctctagagtgcaaggggctgtctgcacatcagc

SEQ ID NO: 105 - DNA, 3540 bp, Artificial Sequence
  subsequence of CCDC140
tcttcccaaaggttaagcagagtcgacagagcactttctggggtcagcggtaattgctgtgtgaaggaggtaccagaagtgtaatttcaagaaggcaaaagtaggctcaactctcagctaaaataaactcttggaccccgcgagcagttaaagaacatctagagctgagtctcatttgtttttgagccggaggcttggtctccaagccctcccagcgtccacccgtctctctcctgccgggagttttctctcctaagagccggcagatgctggagggaagcgcttgctgcaagattccttctcccggtcccgtagattgcagagtccgcgggaccgttgaacggaggtactgccggctgagctgggtcttaagtgcccatgggttcataaactagctgtcacttgctataaacatgtacaaatggaggccacaaggatgtgggggtgctggggacctaaagctccggaatcaggaggcgactcattttctctcctttccggcctctttcttttctgccgagcgctctgagattcatatgtacccagatgatcagcccggcccttctcaccggccagtggccagaggtccctggacacccggagaggggtgggagggcacccttaggctctggacagctgggccacatccaaagacttaatgaatctaaatttcttgtggcctgtgtccccgaagtccgacctgggatggccaggacagcaaagttggctgaggctgcctggcctagggcgcccgcacgccgccaaacctaacccggctcagagccgtgactccgcagaacagggcgcaacaggtctcaggaatgccgggtgattccagccactctttctctgtctccgagtcttgggcctcccctttatttctttctgaagtctctccggagcccaagccaccccacacccaaaccccgcagctggatgggagtccaggccacttccctatccgcagccggtgggccaaggagtcctggtgccaaatttggccgcggtacaggcgctaattggtaaagggatgacccagcggtggggcttggaaggcgagggcccgcgccctgcatccttgaaccctggtttgggaggcagtgacttttacctgggctaacaaattacccagaaagcatcagtgggactctccacaacggtgttgtgaacgagtgtagggtccactcacgctctgtgcacgttcgaaatgaaacgggagccttgaagacgatatttggataatttgacaaaaaaaaaaaaaaggtgggcgggggagatagcttctattgtcccctctgcgcctctgcccccagtttcagagacactacaggtgaaaataacagcgggctggctgtccaggcctgagtggagcgtgcccttgttagcttgaaagttctccctcgcagcccgtttggatgcgtgcgtctacagcccagtcgcactttggtgaccggcctgggctgtgaagcaccctttagcgaacagcctccgcacttggggacactggcacaagggtttcatggcccgtggacttctcagggcctctgagggttgacttcatactcagccagacacaggtcttaagaggaaattatgatctatgcaaaataatgtccctgacctagtggggagcgggggtggtgtctgccacccagacctttttcctcccgtctgaagggccgagctctggcaggctgacacggtcgagcagagaagttcctggccacccgcccggccccaggcgtgattctcaggatgcagtaaaagttgggcaaacgccgagaaaccctcaatcccacagaaaggctgccgggggctcacggggaggacatcaaaacgccaggttcgtgatcatgagcttccggtccggatgtgatgatacaggattggtgaatgcccgggttaaacccgtggtccttcgcagccgctgcctcagtgacagtcattaggccccccgcagttatttgtcaaaagcattggcgccgctcttctccccatcgaaaaatcagtcgggatgagttcggattaagggactagatgaggatgtggacatcccattgaaacatggtgtaggccagccgaagtgggtttgctccttcagctgggggagccccagggaacgtgtgagcgggtttacaataaggaacatatggtttgtgggaagataggaagagagaaggaaaataggaaaggaaaaagaaaagaggaaaagaagagagaggtacttttttttttaaaggcagtgagggagggagagaagaataaatctcacagcagctggtgtcctagttcatttgggtctgagaaaattatttttaggcaaacaaggaagacaggattccgccgcccgattctccagggcgggaagaataggatgtcttgtaaaaaataagtaagtcctgtctaatcttccaaaaaatgttctgctcaattaggtaaaagttcatggtggggtgggggtgatgtttagaagacagattcttcggtaactgctctttggtgtgtgtattcggggtgtgtgtattcggggtgtgtgtattcggggtgtgtgtatgtgtgtgtgtgaaagaatctggtgtgtgtgaaaggggtaagggttgaaggaccttatttagctgggggaccgtcttgtattgggagcgggcagcctaggccttggaaagaccagaaaatctgatctgtgcggaggcaggtgaaggctgtgagtgaggtgggggcgggaacagagctggaggaagtgaataaaagaaaccttggggtccgttggtttccttgactcgtggagcaaaaaagtaggcgagtgaccactccaggaactcctgcctccgggcgccggtacataaagagctggggctgtgtgtcctgctcttgggggaggagggtactgggaagggggaactaacaggtctttctttcgctcggatcaggactggactccttctgactccacgcggccccagctcctgaaccagcgcagtgagcctcagccgcttctcaaactgggtctcagaaaatttctcctcgagatggatttcagcggcaggaaagaggggccagtgacgcgaggagcaagaaaagagtaacatgggagatgaatgttcaaacccagatctcctcgctgagcctggaagctcgccaccgtgggatcacgggaaccagaggcaagaggctgcgaatgagtccaacacccgcgttcctcgagttttaaaagcacacctggggccagagactgcacagccaactaaacggagtaaacgcaacaggtggaggaggcagagttgtcaggggccaagcccggcgcgatctggccagttcttggggagcgcggacctgggactgcagagaggcgttttgaagagtgctgcgcgcacctgcctctcggagatatccaactccacccgggcgtctcctgagagcgcacagtccacagaccccgggagggctgcccgccctaggacacgtactctcccgacccctcactctttcaaaattggggaagaggcggaggagatgaaaaagaagaaagagagaaagagaaga

SEQ ID NO: 106 - DNA, 2301 bp, Artificial Sequence
  subsequence
atcataaaagaacctcattttacggctagggcaatgaggcccagggagagcctgcctaagggcacgcagagcaaagaatacaacattacacccaactacggagggccctgtgctccggacgctgcccggcgtcgctcagagtgggtgctcacaaattatttgtcaattgattggaggttgccaggcccatcttgcaagacacctcccttctccctggaaggagaaacccttgggagtctgttggttaacgggaaaagtgctttctctgagaggaaggcggggcaagccggaacaagctctcgctgggaatccgcacactccttctcccggtgtttcttaacccctttcttctcccgggagtggagagggggctcaaggatactagaaacctgtccccttggcggagacacgtagtcgcctctggccgccgcggccgactgatcttgcggagtggagctccccccaccccgcccgcgtttcgctggggctccctccgctctgcaaagggagcggggagctgggggagccttgcacaccagtcttcctggagctgcagacgaggagccccgcgccttcgggagcctctcggcggcttcccctctaacgcgcgactgtgcagcctctccccgccgcccccacccgcggctcgccctcgctccctccctccagccccgccagccggagcgcgcacaccgggactccggcacgtgggcgcgcgggaggtggcggccgctgctgccgctgctgccgctgccggagcccgaacccaagccccagctggagccggagtcggagccggcgagatcgccctccatgctgcgggagctgcggccgccttccgctcagcctctggtcccaggcgagcctggcgagccggcgaagcaccggcggggaggaggactagaacaggaggaggggcacggcggattgaagcgagctgggctgtgagcaagggacacccacagcctggagaaacagccccgctctcttgcgcgctgtctgctccagccgctactgggggctctaagcagcgcgatgctgcttcgcttcttctaggcggcggccggcggaggctttccgcagccgcttggccggcgccggcccctattccgttggcaagtcccttgtctatcccggagggcgcacccggacgctcgagccggagcgagcgcgaagtccgaagtccgcccccagagccgccaacttccctgtgagcccctctccccgccgcagcctgcgccagacctgggagcgatgcgcccccacccgggcggcgcgccctctgccaactcgccacccatgggatcgactgccctcagctgcccggcttggagtgcgtagccttcgccgcgtggcccaggagaggagcgagacaccaaggcgtttcgcggactccgcgcgcaccagtcggcttggtggccctgcgggatagcgtttatacccaggggtgagtaggccgctaatggaggccccctttacccccagctagcggcttgcatggacggcaaagagacgggagaaagttgggtctccttgcgcttaatctggcattggcagaggaatgcaacactgtttcctccaactcgattgccgcgggggtttccccagttccctccatctctaagccaaggagggagtccccttccgcttcctaaggagaaaaggggctccctagagcagatcgctgacttcctcaccaacgtgccatttggggcttttcagccgcccgcgcgttaagctagctcccagcataagcgcttagagatccgcagccgcctgggcgcgctaagagatcgtgggcagacctagcccttagggcagcctaagcgcgcttcactaaagaaaaaagactgttggtatattaaagaagtgtgtgtgtgagagagaaagagacagagaaagagacagagagacatgggtgggggcaccaggaaaggtagcccgagtaggaggtgctagtgaaatttatcttttgctgacggatccagcctccggaatgcccgattgtcttgatccgcggtgcggtgcgggttttaggggcgcacaatacagggtgtccagacagagtccaacaggtggcctgcgcgggcatcctgtggctaggcgcgggggaggggaacggctccctccccgagccccgggctgcctctgctgcttctaggggtgcatctgaacatggataaggaaatgcgctccctgctctcaggccctatttggggtgagtgtgtgaggcatccaaatgcctcctgtcggaaaacagcggcctcattgtgtgcccgattgaggtttcaacttgcaggc

SEQ ID NO: 107 - DNA, 5043 bp, Artificial Sequence
  subsequence of GATA2
aagcatttccctctttctccccaacttttctcctcttccaccaaagctctagaatttttctgagtcctggaaataatggatcgaagttgttgttctttaaaataaaataaataataagctctttcttttttagataagtggcctgggttttttttgtttgtattttttttttcaattaaaagaccatctggaattcaaataaaatgcaaaacaaacaggagaaaggaccaagaaaaggcaagctgacgggtctgagcagaactaggaccctgagccggggctcagcgggtgctggggccagcgggggctggggctggggaccaagttgagcaggatcactggctggcatcgtgttccccaggaagttattcttgatttagtttaaactaaatgaggagtacagcctggcaagagaaggtggttcctgcactcaggagtaactgttttaaaaaccttccccctctgtggctcaaagggattcgggaaagagacatggacagcaagaactccacactagccacgagtttctgggtttatgctctgtggccagattcttggacaaacccagtttggccccagccagctgcgggaaaaggggcgggggcactgcagcttcatcccctcactccagccctcagggagggagagggaagggcctggcgagggcagggagcaggagcaggtcctgggaattttgctctggggaaaatctcccgaggagatcagggagccatcgaaatcccaagatcagactgattgagttagagacccagattccttaatggtctggaacctccggagtgcctgaaacatgcacacacaacatgcacacagacacacgtatacacatgcacacacgctcccaaacacatgcacatacagagtcacttccctcgcttcacatactaagtcctgaggtggcttgaattttcacttaagattcagggagggaaagggggaattcctgttctatgttctggtcaggcagtgaccaaccctggggcaaggaactgaactttgggggtacactggaagcacttaagaaaatggcaaaagttttagagtctcctctccctgacccgggggtctcaaacatctgctgggggctattagagcgagacatcacccatccccagatctgggaaaccaacactgccacctctcccaagtcacagctccccaccacaaaaacgcaaatgctcccctcttccacgaagtccccagcacctgcctttacctgaacaggaacgagccttgctgcgctgcttaggggtgaagctggaggccggtccccccaggaagcctccggggtggaagagtccgctgctgtagtcgtgggcagccgccggcacataggaggggtaggtggggatggggtggtgtgtagcaggctgggtgcccatagtagctaggcctgggcgcaggggactgccactttccatcttcatgctctccgtcagtgacacctggtacttgacgccgtccttgtcctctcctcgggctgcactaccccccgcggaagatgaggctggagacgcagcccccgtggtgctagggtcaggagacacttctttgggtggcgtgggtgggaagccgaaaaggtgggagccagagtgggctgctgtaggggtgagggaggccactgagctcccgctgcctcccccgctcccacccccagcccctgggtacacagagagtgggcctccagggcctccagcagctgaggggtgcagtggcgtcttggagaaggggctcacggtccaggggttgtggtggtgggccgcagcggcagagagggctgctttgcccccgtccagccagggcaaacccgggctgtgcaacaagtgtgggcggcacatctggcctccggtcaggcgggctgcgggcaaagagagagaggatcagggtgggcagaaagatcagggtaggcagagctagggacgcccctgacagacattgagatcacgactcccagaaccagcagtcatcccctccccaaagaaagccagaaacataataccccaccggtaataatcaggaatgtcagtccaagctgaaggacaagtggcatagaaggaaccccaccggacagaccctacagggaaccctcacaggccagctggaagtgggcagaaaccctgtgggtcccagaccctccccaatcggccgctgctcccacctctcccgccccaatttttcagcagctcgattcctgcggatcctacatccgggaagcaagcagacgggccctcctcccctccctcgcctggcgcgcggcgcctgggttctcatcaccacgggcccagtgctcaccgtgcgcggggctgtaggagacgcgcgcccgcgcgtgagcggggttggcatagtaggggttgccctgcgagtcgaggtgattgaagaagacgtccacctcgtctggaggcagcagctgcgcgggttccatgtagttgtgcgccaggcccgggtggtgtgagtcggggtgctgcgcattcagcacggccgggtgcgccatccagcgcggctgctcgggcgccacctccatggccggcggcggcggctcagggtctgggtgcagacggcaacggccctgcgcgaggaagggggagtgaggcgtgccgccagcgcctgacaccccccaaagtcccaccacgaggtgtcccgcacgccacggagccccagcccagatccggcgagaaagagcaccagtcccgggtgggaggaaagcccaaggctcaaaacgaaaggaaggcgggggagggggttcagccacgcacactcacgtggtgacccgcggctccagaatcacacacccgtgcacatggggtcacgcccggggacgggtcccgacaccagtgaccccaacaaacgcacagagcagcacttcagtcagacactcacactgagcccccccgcccggtagacaaacacatgaacacagactcaaaagttggagacaggcgcccgggcacccagtgtggcacttgatcccagcgacacgcacacacccacacttggcgccagatacacatactgatctcaaccccgaaaacatgcacacgcagccccctgagcgcagtactaagcggcacaatcaggacctctcaacaaagcacaccaaagcagtcgcccgcagcctggccccccgccctaagtccccccagagtcccctcaaagctaggagcgccccaggcccccagccggctctcaaaccccaaacttacacacgcagccgtggggaggggagggactcggcctctgagagtgaaggagttccggcgggagccccgagggcgacgggcccagggacagcacgtccggaggctggcggggcttacagggtaggagctgggggtagagtgcgcctcggcctcgggccctcccggctccggcccctcggcatcctccggccgccctggcgccagctgccgactcctgcacagacatgaagcgggggccgcgcacgcctaagaagcccaagccagccaatcaacgccgcgcgcctcccagcctccgcctcccattggctgcgtccgcaattcccgaaccgctggactccgggactgacccgcgggccggcccccctcagccggcgggccccctccctgcgcgctcctggcggcccctgctgccaacgcgccccaccactaagggaccctcaccccaaggcccgacccctgcagcccctcttgcgaacactccgggatccctcgatgctctgggcctccctagcagtaactaaccaccaactgccccctccccaggagcccgggccgcacaccctctggatggcctctccccgagaccctaaccccgccacgctccttcaccgctgaacgtggtcagtccgagcgcagttacctacccagaccgttccctcccctagctcgggcgctgtctgggtggactgggggttgggatggttcggacgacagcggcggaacagcaggagccgagaggggcagagaggggcaggaactacagggctctagagggcacctgggcctcggacacgcggccgctcagggctgtgcttgacccagtggaggtggcccggccggtggctccagaaagggggagggggcacccctccccgggcgtggccttcgcaggccaacgggcccaattgcctggggcgaggccgtggagacccggactggcgccggcgccagctggagggagacgcccccgggcaagaggtggcattttttttcctccggggggggtccccgaggtggcctctggtgagggggaggcggtggtctgaggtctccgtcttctaagtcacctggaagtgctccccactcacttctagcccggagatcggctctatggttcgtgtgggccgggcgcacaagtcttcctccctcccattgtacagactggggagacggaggctcgaagggagccccgggccgaggagggaggtccaggacaaaggcattttgggggacctagacaggtgccgagtactggggggactcaacagcgtcctccagccctcttccctgttgggcccgaggctcccggggtagatgtccagagggcccccaggtgggtcgggggcaggaggagggctggggtcccggccacccccgggagagtgggggaggggcggcgggattgacagtcggtaattgggtaactggaggcggcttctccggccgggcggccccgccaccgcgacgccgagcccctgacgtcacccgattcgccaggaaatgaactttttaataatccgaggagggaggaaagccctcggtcccctcggctccgggggcgcccggctgggcccagctccgcgggcgcgcccccgtcaccccctcccaggccagttcagggcagcgccaaggggccgcgggctcaggctgaggcctcctcctgcctaggcgtctggcgtccgtttgtctgtccgaggcctcagcgcaggtaaagcgcggggctggggggcgcagagctccattgggctgggaaccagcgcgtctcgtgcccttgggggacccgcctgcccgagccgcctgctaagcctcccgctcccctccacgc

SEQ ID NO: 108 - DNA, 7737 bp, Artificial Sequence
  subsequence of ADCYAP1
ggttcccggaggcagccccagagtcgcggaccgatgtgccaggctgtggatgagccctgggtaggggagggttcgtaccagcggcgcctggggcagcgaggagcgcgcgttctgcctgcgaagctgccttctccgagccccgcccaggaacattagctctggggggccgctgatcattgatttggacggagagatgggttctgggttctgtattaggattccagcatctgggctcgaggcagggcaatatccagaaagaccccagggttcggggtacccgggccagggctgaggcgcatcgccgagcaaaggctgggtgcgaggcgtgcggaatgatgcgcttgccttgcccgggcctctccaaggatggagaaaaggcgagtgaagcagcgaagtacgactccaaccccgcccagagagtgctactagcgctggctgcacgccaagtctctccaggggtccaaagcgagagggatttgttttaacccatctctacccgtcctgtgtcaagaacggaggctgtagagggcgactgcgaagtcgccaggcactcgctggatctcggtccccctcctcgtgctctggggttgagatggggcaccgccatcgataacagatcagcgcgaactattcgtttagtggccttaaaacaccctggtttcaccctcagctattttcaagttcccgtgtgcctggcactttctccgtgcgagaagcaccggagggtgcggacgcgccacagtctgagccgccgccgaactggctaagtttaggggcatttattattcatgttcctgccagatcctcgcctgcccaaaatagaaaccgaggttctccgtgacctacatctgctcggagaagggctcccctgggctcggaggctggggtgggggtggctgaggagttggcccccgcacgccccacgcatcctctcctttgctttctgggcctccccattcgggtcttcgcgtgggtcagcgcccggtctcccagggcctttctcgtccccgcccgttgctgctttggggaggctcgggagccaggcggggaggggggcggtccttttccgtagacaggtgtgcgcgatcggcggagacgcctcggtttcccagcgcttgttgaggccgtggcccgcaggacgaccctttacccgcgaagggggggtgggcgggccgcccggcggggtaggagtggttgggtgtcgttgcctcctccttacctctgctcccacccccagtcctgggagaagagacaattctcagcggaggacttttatcacctgtgaaaatccgcgcgagccccttactttggatcctcgccgagctggggaggaacttgcactgaccacaccttctgtccccggccaccccgcaggccagaggaagaggcgtacggcgaggacggaaacccgctgccagacttcgatggctcggagccgccgggcgcagggagccccgcctccgcgccgcgcgccgccgccgcctggtaccgcccggccgggagaaggtgagattcgcgcggcctcgcgcacacccgcggctgggagctcgggactgcggtgacgggaggggcagtgtggtgacccacccaggatttttttttttttcccgtgaaagtcctcaagcctgtcctctccctggcccgatcctattgcagcgacagaaaatcagcagcgggcgggtctgtgtggacctgagggccgcgtggggaccgaggggggctgtggcccaaagagtggcagtgagtggcgtcaaggaacccacactccgcatctgccactcctagagccgggactagctcccgatcctagcagttgctctcgagatcatcccgggagttattggcgagttctgggcctctggaggtttccctgtcagcctccccggccgccgagggggcgcgcgcccaacaagggggtctctagcggccacctggggacagaaacagtgaccctgggcgcgcactttgcctccccgttagagatgtcgcccacgggatccttaacgaggcctaccgcaaagtgctggaccagctgtccgccgggaagcacctgcagtcgctcgtggcccggggcgtggggtaagagtttgtggaaggattaacctgcgcgcgccggggtgggtgcctgtgcggggcgcgcggggcgggcggcggtgggtgcccgtgggggccagggtgagtctgcgcccctgggtctggggtgggcatccgccacgggtcgcagttggagattttgaagtggcactttaaatttgcccagagagctctggaagaggcaaaaagggaacgcgagccagggagtttgatccgttttgaatgaaaagaaagagaaaccaaaccaaacctctcagtcatccaaaaccttcaggcttccagggaggttttgctataattttctctaagcatgactgtttctgggggaggggaaaggggtggttgtatttactgaaaattcaaatcgaaataataaatggccaaatgtggacacttatggacccaaacagttttgctcacgccagagaaactgagagcacagggcttgtgtgaagcctatctcggcagaaggcaacattctaataaagcccgtgggaaaacagattacattttcgccatgaataagtcatgcagtgaaaaatattgcctacagcctgtcgacttatattattatcacgtttttcaactcggcgtgaggagggagaggagtgttcatatttgactaggaattgcaggatcgatgcaaactccagggcagcagccagactggcatatgtagggctctccggttactttctctgtatgtcgcgggtgagaggaacagcgaggacaatttagcgcaaacacacgaagggtcggatctcaagggggcagcgctgggagaaaggttaggcttgaagcgcgcgtcgcctgcccggatcttatcccgggccccctccgcagggtttggtgccaggagatcctgcgtggggaggggggcatcgaggggctgccgtctcggccctccccacggctgcttccaggcagaggcgggcgacgcggtgggcagtgcgagccccgggccctccccgaaggctcccgcgtggggtggggcccgcctgctccccgcggcgattgaacctgtgtctcccgccccgccaccctcttcccgacccctttgcttgcagtgggagcctcggcggcggcgcgggggacgacgcggagccgctctccaagcgccactcggacgggatcttcacggacagctacagccgctaccggaaacaaatggctgtcaagaaatacttggcggccgtcctagggaagaggtataaacaaagggttaaaaacaaaggacgccgaatagcttatttgtagcgatgggttaccagctaccctgtgtatacagccctgacgcaatgaaaagtcgttttccaaactgactcaacagtcatcgctcgtgtgttctatccaaacatgtatttatgtaatgaagtaaagccattaaatgaatattttgataataatattgtttttctttctacaaagcactagagaatgcacagatatactttgtggaccaattattgatatatattataaatatatataaagaatatatatatatatatatatatatatatatataaagtatagagagaagttcatacaaagcgtgcacaaggattgaaaattcgcccgagctgtttatgtttttataaaaataaatagaaaagtagacaatcattgttttgaatattactcctatttttgtaaactggaattaaaaggatagtatttttatccatgacaggcctgaagatattactacttaccatttgctactgtacataaacaatgatgccctgctccagggagattttgaggtaaagatatggagaattgctgaagggcattctttcccagtgagtctctggggcaggctgcttcaatcccagcctaactcaactgggctctgtccccctggttgggtggcaattccaatatttctgctttctttgattctccttttatgtgtagttgtctctcttcagactctcagcccagaagaaaattctcctgataaaacaacagctcgatccaaattgtgcttctccccagaattcacgcctctccctaggagaagagttgaggaactgtacagaaaagggcggcttcgttagaccgctctcttttctgtacttcctgagtggccagggaatctaatatccccaaattagggcaattggaacaaagtgaaggacatagaggtatattggaagaggcagagcctgaggtggtaggaggaggaccctggaaatggactggtttgagattgccccaggtctgggaagctgagggcaaatccagtcccaatggtcctgactttgggcgctgggtattggaaatggatgcaaagtacaatgtgtttttctccagtgctgtccatgcttctcatcttgtgaaatggccaggatcctctcctttgaaacctgctctgtaggagctacccttttcctttgtggttttatggagacctctccttcctaccctcctgcactgtttaagtactgtttaccatttttcattcacttctcttaaacttgtgaatgcttctcactttttttttttgtttgatgcaggcacttattgtaaattttagaaacccctctgtagccactagtaagtaattatgcactaaatatgaaccctttgtttcttgtttattgagtttgtaggtaaaatgtatttttctacattattgcttattgcttagtaaaatttatttcataaaaccaacctttgtcatattagaatgtgtagtgttcacatgttgctcagttttgctaactgataaatcatttaatcctcttcttcatatgtatgagtactatcttatatctgtggtcaagagtgaggtaagcaagctccaacagaccctgagaacctacgcttgtatcctttctttggctaaagaaagcatgtctgtttcctgtcaattctttgaacatacagagtaatctttataaacaaaagaaccttcacccagcaatcagatcgagcagcaacagacaaaccagccagccaatctcccaaatttcaggcacaagtttatttatttatttttttatgttttgaaaaaagaagatgaagaagaagaaaaaaaaaagaacaaggaaagattaaacgttagcttgtaaagtttaaaggacctttccttttcctttacggatttgatcagtatgaagtcataaatcaaagaaaacagaattggatttgcattcccaggcgggatggatgctgccaggagatcacattgcaaatagtgaaaacagaggcattcggtctatgcctgagtcctgtgtataggatcaatcttcctttaattccgcagtctcctcaggcaatgtgacacgggatgcagtttgcagctttagtgcctttcttcgccttttaaattgccacgaatcacagatggctatttagtggccctacaatgctgcaacacatcagcttgcattttagtcttaattatttgtttcttggataatgggcagagttttctgtatttgtatcagctgttagtggtgaaatagggctctagttaaccttttatttatgaagtctaatttagtgttcccgtggctagttgcaagcattttacagtgatcacccagtttaatcttttgtatactttttagaaatgccaagagccttactaaactgaagcagatttatgatatagtgataatttaggtagatgttagtcttgaagctcttattttgtgtgcaactgattataaaaacaccttaaccaagtattattacacacatgatatctataactaggactttgataactgttatataaagtgtgtaaaatttgtatgaataaatttttgtaaacaatgcaacttggtctaatgtttgggaaaaaagacattcaggaaataattactttaaaatctcttaaagtattatatttctttagcaaccataagatttttttacgtctggaatatatatctatctaagcacccttgtattttcatgaactgcactttaataattgatgggcaactggattctgctaaaaatttaaagtagctactcagatggagatgcctaagaaggttttaagctcataaacaggcatgatgttgcaacattataagacacacaatttagattaatttccatcccctagtgtgtatatactttgctcaatattcagaaagttactaggtagtagtgggagacaatgctggagcattagttacacatctaaaatagcaatctaacattgttcttttattttttattttagtggccaggtctcactatgttgcccaggctggtcttgctcaagcgatcctcccacctcagcctcccaaagtgctgggattacaggcgtgagccaccacacccagcctaaaatagggatctaacattgttcttatacaagtaactctgcagactaaacttgtcttgataaaattttgtataaaatgatctaaataatcagtttttggaggttttaaaatgtgtttagagacatacaaactactgtctctgattaaaatgctttaggtagaaggaacgtgaacatgagtaagtaaagagttaattagatgcctttaaaagaaaatgtactttgaagtccaggaagaaacacaagaagtcatttgtggattgtatgctttcttagttcatatttacaaactttagggcaaagctttcatacgaaattccttcaaattccgtagtggtgtgtgttttggcacctttgactatttctggcttagaaaatgtatagaaagtcacacaataattgacataccatttaatttaaaatgccagggtttcatcctaaaaattaatggtctcaattagtaaatcaataaatatgttacgatagaattaaaggatgagtgaggattctaaaattatcttcagaatttagctcagtatttaaggcctagaatcaaatagggaggagcccacagtctagaaatcccgtttgtagtcaatgaaaaaatgaatccagtacagttcatatttgcatttgattttattggataaggaatttttcttctccatctttaactgcccctctttgtccttgaagacatagtgtggtagatgaaaaaatgaagaagactttattcggttggggctaggctaacgacttgtcaagaacataaagataaaccccagacttggctgacttcaagtgaatttcatgtatttagcaacttgccatattatcttcggtgataactcaaattacatctttttaaaggcagacttgatacatatgggtattcaagaagctgtaataggtgccttaatgctgttagggcggagaacacacttattcaatacaatgcacacttattgaacacctgaaatgggccaccgcactggtcgagagagcttgactaacacctgggagctcaggtagtatttttttcagaatgtttttctgaaatgtgatcatctttggggcggggggagcttaaaaatgcaaaattgtagggctctgccagatccagtgaatctgcattttaaataaaaaccctagattactgtgcactaaaatttgagactgcctagatttagaattggtgacatatgtaggcatacatatgtgctggtctgaatgtttttttcatatgaaataagcaaaaggtcatgttacctgcatacagtaataaatacataactgtgccatattcttccaagatatctggtcattaagct

SEQ ID NO: 109 - DNA, 8315 bp, Artificial Sequence
  subsequence of TBX5
ttatgcggggtttactgcttacccagaatagcggctactgctgcctactagggcgcacctaccgctggagcctccgcggcgactgcccacctccaacacacacctcctctgctgtgcgcttgctctccctaaatacttcccagttggcaagcgccaaagaacacaaaatagcctccaagagcaccggcaaccatataatctcagtgccccgctcctcctttacacccccagggagggaaagttggaagcccagtgaatggtcgaagtcctttctgagcgcagctttcaggattaaagttcccggattcgaggtaagagtcagtctctctcactctctctccctctctctctctctctgaaatacaagccaactcagctgagcacagtgacgttgggttgcctcgatgctcacaaagtactgaaatcgcctatccaactagctcccactgcactctgtcgccctcccccttctctctccctcccaccctcccgtcctcccttccccccaccccaaatttccactagatttcccgaacactcaaatcacaatacgactctcaacacagacctgcaataactccctcctctctacccctttcccaacctccatccatctctgcttctctgagcaagcggtggctgcaaaaactcctgcacaaatcatttcaaacgcggtcggcttctaatcgggaagtaatctcagtgacgctggcggtgcagagaaccgagtctggacgcacacacacaaacacaccgcgggcctccgcagccttgcagacattctctccaacgctgacctcgagaaggagagctgcctgaccccgcctggccggcgctcgccttcctgacatctcccctccaccccctactcatcacccctactctcaacgactctggggtgaaggcagggtgaaggtgcattgggatgggggccgagatcaaagatgctaagaaatcgctgcgggccctcaccccccacccagtggggccaccagacgtcccctgctccaggtgtacacaaggcagtgcccagttttattaaaataatcaaacagtcactggggactggctagggttttcatctccactggtctcctctccttgccctttccctctctgagatgtattttttttttttagggtgagttgaagaggtcaataaaagcacaaacacagtcagtaggtctcagtctgagcagacccagattgggacaccgaatattggtgcttggagtaaatgtcaggagtcctgttctgtttcccatccttacctcctgtacccccatcatactgatttttctagggttctgataagagacttgggcctgcaagtcaaggtctggagaaagggatggagggaggagaaatgccccgaggtcagcagctgtgtaaccctctgtgactgctctgctaaaatcccaggccaggccattgctgcaaaatgccaaagtggagaatctccaaccctgaatgtggggcaaccggggagaaagccagccctcctttgctatggtgctcactccaccttccaggtttgtttgcaaacagatattttccctttgcccaggcgatgtatttatttgtgaaaacaccctcaccctccaagtcagcttggaggcctttaggcttgctggcaaggcgaccctaggccgaagacacgaaaaacaaacatggcatcggaagaaggctgaaccgctacatctccagtagagggaaagggaaatccagaaagaccttcccaatccctttaagttctcagagatttggggataaaattaattcccataaataatcttcaggcccctccagagaggaaaaatctggactctcccaggtaatagcccagccagatttgcttagctcattgagcacagatggtctgggccaccaagcaaaatagggattttcaaacctttcgagagaatccattcttgccaggtgacacacgaagccattcttatttcgttcatgagaagtagcagcacagcaagagaagattcagcaagactaagacggggtgaaaagccaaggagggccaagtgcaaagagaaacctatttcccccctcagtcctccagggtgaaactcacctccaactatcccacctcttctttggagcgcaaaagccaggagtgcgcctcgctggagagcagggctcaggtgaagactttgaaaaggaccaccaaaagagacctctttaggccaggtcttcttccaacgtctgtcaagaagagcacgtacctcccagctcaaggttggtttgtggtctccgacaaattaaatattactgtttattaccaggcataccccagtaaaataaagaggcaaccaggcgatagcgactatctcaccagccgctgcacctataggacttggagacgtcacgagtcacgcaaccggcccgcgcgctgtcacgtttggctggggggcagcggcgggaggtaaatttctctccgtcttcgcctatcagtgccgggtctgcgcagccacaggttccggacgtcttggccccgggaataaataaagacataaaccaacccggctttctccggaggaatgagggtgatgaacataagacacaaatagagccaagatcgactttcttaggaagggggagaggagggaactcttcacgaagggaggtgggagtccacctcagacctctattggaaggaaatcgagttgttccgggggactgaggtctcttgcataaggcatgggatccttattattattattattatttttaaatcccccgcggaggagctctgggcaaatgaataccgaggcgccgctctagctggttaggcttgggatgcgataactcagtgccctcttgcagacttgcatagaaataattactgggttgtcgtggaggggacacgagacagagggagttctccgtaatgtgccttgcggagagaaaggtccaagaatgcaattcgtcccagagtggcccggcaggggcggggtgcgagtgggtggtggagtaggggtgggagtggagagaggtggtttctgtagagaataattattgtaccagggcccgccgaggcacgaggcactctattttgttttgtaatcacgacgactattatttttagtctgatcaatgggcacaatttctaagcagcgcagtggtggatgctcgcaaacttttgcgcaccgctggaaacccactaggttgagttgcaaaacgtaccgcgtagacgcccctggtggcgccgagagaagagctaggcctgcccagcacagagccggagagcgtcgggccttccggaagggtaagttctccgccaaggggtcccgagggagctggacgtctgaatctggacttgcccccagcttcggggttcgattctgggttttgcgcgtccccaacccccagggctttccgaagcatggcctggctccaggcccggtcctgtaaggactggaacggcagcaaaatgtgcagggaggcagtcggccggcagagctgcggcgggagccaaggtcaggcccgcggggagagcgggcagcttccagcgccggccacaagctcccaggccagctgggccgcagacccctttgcttccagagagcacaacccgcgtcctttctctcagccaggctgcagtggctgccccgagcttcgctttcgtttcccaagctgttaataacgatatgtccccaaatccgaggctcgtgtttgctcccagatgccaagaacgcaacccgaaatccttctcccaaaccctaggtcgacgagatgagttcctacttgacctctgagccgaggtgggccggaaaccgaggcctaggccccgccggggctgcaaggaaaaggggaaactccgagcgtagcgtcttttccttgtggttcctttctccggcatcccggactgcgggccctgcagccacctggaccggcattcaaaggattctgcaagtccagcttcacagactggctttcccagacgctccgaagcccgcaccacgaacagaataaaggagagacgagagatcgcaactagatttgagaatcctcgttcttttccccaatcgttcgggcagtaaactccggagccggctacagcgcgcatcctcccttcctcctttcggagaactgtcgctttcccgaagctgctcccagctgggttttctcccgaagtttatttttctcattttgcaaaattcctgccctgattttaatactgcaacaggacagcagaggttcctctttaaaaagtcaaaacccaaaccaaaggggcccattgctgttgataatttttttcttcaccttctccttccgtttttaagaaagacacttccaaaactacccattgttttcctctcaaaagagaactcgctttaaaatgcatccctttctatttctctccggatatgtccccacctgacccggtggcaacttgtggggcgtgggggtagtgaaaaatagaagtgtggacggggctgggaaaatgaataagaattataacaatagaaatgatgacaaaactaaactttgaccaattcaatttgcaaaagaaagggttggtctgagggtgagacattccctggtttctcaagggggtcactttccctctcaccgagttaaatctggctctgttatattttttccaggaacacagtatgtctcttcccaatgttttattcggtttctggtttccccacttttgaccggaagtatgtgggaagaatactggctgttattattatgattattgagtgtccaatactctcctccaatatttccaccaagaattattatcgctgctctcctcattcatgttagtgttgctttgtgtgctttagatgacaatcgtcctctttactctccaagtttggagggtgagggttttttgttgtggtggtggtggttgggttcttctttgtttttgtttttttgtttttcctgttcggggtaatgaaatgagaactggaagagaggatatcatttcgaggcccagctgagaaggatcccaatgcgaaaaatttacacacttcaaagagcagaaaggtggaagcgagtggtgcttggacacaaggatgccactgttcttatctcctccaatttgggaagtgcccagcctagaaaggtgagggtcccatctgggagaccatggagtacccccagggtcacactgagcctaagaacttcaaccatcctgcaggtcaaaacccactgataggtctcccaaaatgtttggggtagggggaagaaacatagggcattccaggtctgtaaccctgcaagagagagactcaaactaatatgtctaggtctggggtgaaggtggggggcctgtctggatacctcctccctcaattgaagggctcgttggaaacataggaacccactgctctctgggactctggaaagacaaattttctttggcaaacggaacagtgtcgcgctgtcgacagagcagactatttttcttgttccctcacaaggtgggggtggggggaaagaaaaggaagcaagaaagaaagggaaattaaatccacacgtgttaagctcgctcaaagggccagagtcaaaaccagagatgaaacttcgactccagttctggctgcccgcgggcctctttccaaccagccaggcctcacagagcaaggcatccccactggagagaattcgatctgatgtttcataaagcgctttatttaaggagaaggggcatgggtctgtctccaagtctgtgctgcagaaatccagaatttgtagcggcaaagaaaacaaaggagataacaattgtaatcataatgaccctctttatgaaaactcatcttgatgtcctccaaatcaaaacaacaattcaggcaatattcaagcaatggccaaaatcatccaggccattaaatcatccaggccattgttttacaaaattcctaaggtctgatcaggctttcggacttgggcctagctgggtcaagagaacctgaaatgctgttgtcaagagactctgaaatcaccagtttaatcaggacagctaatctctacatccttgaggcctctcttttggggagagactttcttgagagaggacactacaggactcagctacagagctctgctatacatgggtgggagtggaggccgccaccccacctggaactgtgagtgaaaactctagtaatgatcttgaggaggtgaagggaggtaggtgggggtgtgggtgatgagggaggccaaaccccaatctggaaggatctgtcactgaaacaattgcttggtcgagacctctaatttttcttcctctccagccagtctcctgtggctccctggtgctgggtttctggcctttggtgacatcctaacagaagggtccggaagcagggaccccagacaccttgctccctctcccaaatcacacccaaaacatactggggtgaaacaactgacagagggtctctgtggtgagcaactgactgaagtttccagtggaaaagttcctgacgattgtttccgcagggaccttgaatttcctggtcaccatggcgacctggaagtcccaccgaatgctctcaacaatggggtaccccgaggacattcgtgcaattggctgcgcagtctgaggcctgaaaagcgtttctgccaatcgttcttgactttctggagcctccttagtgggttcaacggagcagggatttttaaaactgcccccttttttaaacaggggagaaaattgagatttagtaccaggtgggttcaggtcctgagcaaaagccccatctttgaattcagaatgctgaccccagggccgatcgtgtagagcctatggtgtatcttaatcgaaacccgtggcccaaacatctcagccaggaacctgggactttaggtgtcacttaatctcttcacacctgttaactacacctatctgcataggaggctccccacatcagtccaggcaacttttttctttgcctggggccatttcttctaaatggaaggagaaaagtctgagcattagaaattgtggcattaatgtctgcaagggctaatggagtgaaaagaatacattattctccttttcttcttagaaaaaaatttcaattgtggatgtaatagaaataccattaaaataatatttctgattgcattgctttcttcttgaatgtttatcagaggggagggggaagtggatcttttcattttggggtggacagtggataatacaggctgattttcttgtgtccggttcggaggcactgcgcctgcagggtttggcagcgatgcaggcagcaaggagagaaagggtgacagagagaaggcgtccaggcctcaggtgccgacagaggtctttggcggtgggacgggagctactcctcctctgggtcctctctcagctttgttccattctgctgccaaccccatctttctcctgactgctcaggaaagacaaaatttaacttctctccccctgtttccaacaggacatctaatgtccctcaaagctgctggctggctctgtagtgcctccacccattcctttctcttctgagagcccaggcagcctacagaggctcccgcttctaacccaacgcctcctgtttccttccctccccagcattttgcattaatattttagaagagtcctacttatgtctacacaaccaccaagagagcaatgtgagtattttaggctcacaaatctgttagcatttgaggtgcaataatagccaacatttatggcaggccaggaaagagccattgtaacctggttttgctcacacatttagctctgaatcgctctatgagaagagagctcaattctcctcaaccttacagaagaggtttctggcgctctggccaccgccccactctggtgggattcgaacctatcagaaggcagggttcctctatcaaggcaggaaggggaaccggggagaggtctgttggattgggggagtgcaaagggcactttttcagcgtcgaaaagcacacttagttgaaaaccgggggggaattggtccttctgtcacggagcgaaggctcacatcatttctgatgtctcagtcttttctccccattcccactgaggccccagaagagagcctgggggcaaacagcccagattcactggcattaagcaagatgggagggaggacggaaagatgctgatgttctcctttccaaacctcactgttctattcccaaatcctggcccacattcatcatagcctcaaggccagtacacactgtcccctggctttgagggaggaagatgggtgggtgggatggagccgggcagagatgtgcccggctccatttttttttttttttttgaaacaaataattaggctgtg

SEQ ID NO: 110 - DNA, 837 bp, Artificial Sequence; identical to SEQ ID NO: 66
  subsequence

SEQ ID NO: 111 - DNA, 156 bp, Artificial Sequence
  subsequence of NECAB1
tttacctatgtaacaaccctgcacatcctgtacatgtaccccggaacttaaaaaatttttaaaaaagtatttaaaaatacacttagtcttactgttatcatacattaaaaattgttttcccacactgggcctaccctaggcaaaattgagaagatg

SEQ ID NO: 112 - DNA, 3718 bp, Artificial Sequence
  subsequence of ADRB1
gggaacttgggcaaaggagaaaacaagcacgcagaccaaggaatctgaaatcgcagttcattacgtcagcataaactgacagtacctttttgtttgtattgacccagctcaaattataaaatcacatgagtaataaaacacaaaatacaggtgttatcattgaaaagtctaaaatgtaattaaacgcgttttttccccctcgcggtggtatcgtttactctgtatctcaacgtttctgtctccctaagcctctcctttcatatcatgagcatacatttttgcatcatgctcacacgttcattagctaggactgaggagtgtgtacgattccaaagggccctcagcgttagctgttagatgcacaaaccttcgcttcctttccacatctactgcactcgaggttcaacagaggatccttgcaagaacagcgcccagagagcattcttgacagatgcgcgcttggctccagcaacccgctctgctgggaagtttcttctaaccactaacacccacctccaatcccccaagctgtcacgacgcatgctggctgggtcccgtcttgacgggggaagggttttacacacaccctgctaggctgccccacatcacaaccaagctcgcagggcaaactcctccaagcctggcggacaagctgtcccaggcgctctggcgcttcctgaacaccaaggtcccctccccgctcaagggagctagcgctctgttccgcagagaaccccggaactgcaggtcgaggggatgcggggggagcgggggcgcaggagggagccgagtgctggaggcaaacggggcgcaggagcgggtgcgggaggcaaacggggcgcaggagcgggtgcgggaggcaaacggggcgcaggagtgggtgcgggagcgagtgggggctgagggaggggacggggccccggggggagccaggcgcggaagggggcgcgggggaacagggaccaggaaccagcgggcgcaggaaggggtgcgtccgcaggaacccgcgggcgcacgggaggcactagctacgcgatcagctcgggactctcaggagccgctcaattgccaacgggaggggggtgcggggagttggaggtgggggtgcagaccagacgggggcgtgcctttgcccggattggctgcaggagcctgacgcgaggccccgggggttggcttggggagtgggagcggggtggggtgggtgctgggtgccggagctgcgggcccggcgcgctcagaaacatgctgaagtcccggcggctcttccagcagcggcagcggctccagcagcagcggcggcggcggcggcggcggcagcggcagcgacagcgctcggctcctgcgggaaaggcgcccggcgcccatgcctccggccccgcgccgcggctgccctgacccggccgcgacctccctctgcgcaccacgccgcccgggcttctggggtgttccccaaccacggcccagccctgccacaccccccgcccccggcctccgcagctcggcatgggcgcgggggtgctcgtcctgggcgcctccgagcccggtaacctgtcgtcggccgcaccgctccccgacggcgcggccaccgcggcgcggctgctggtgcccgcgtcgccgcccgcctcgttgctgcctcccgccagcgaaagccccgagccgctgtctcagcagtggacagcgggcatgggtctgctgatggcgctcatcgtgctgctcatcgtggcgggcaatgtgctggtgatcgtggccatcgccaagacgccgcggctgcagacgctcaccaacctcttcatcatgtccctggccagcgccgacctggtcatggggctgctggtggtgccgttcggggccaccatcgtggtgtggggccgctgggagtacggctccttcttctgcgagctgtggacctcagtggacgtgctgtgcgtgacggccagcatcgagaccctgtgtgtcattgccctggaccgctacctcgccatcacctcgcccttccgctaccagagcctgctgacgcgcgcgcgggcgcggggcctcgtgtgcaccgtgtgggccatctcggccctggtgtccttcctgcccatcctcatgcactggtggcgggcggagagcgacgaggcgcgccgctgctacaacgaccccaagtgctgcgacttcgtcaccaaccgggcctacgccatcgcctcgtccgtagtctccttctacgtgcccctgtgcatcatggccttcgtgtacctgcgggtgttccgcgaggcccagaagcaggtgaagaagatcgacagctgcgagcgccgtttcctcggcggcccagcgcggccgccctcgccctcgccctcgcccgtccccgcgcccgcgccgccgcccggacccccgcgccccgccgccgccgccgccaccgccccgctggccaacgggcgtgcgggtaagcggcggccctcgcgcctcgtggccctgcgcgagcagaaggcgctcaagacgctgggcatcatcatgggcgtcttcacgctctgctggctgcccttcttcctggccaacgtggtgaaggccttccaccgcgagctggtgcccgaccgcctcttcgtcttcttcaactggctgggctacgccaactcggccttcaaccccatcatctactgccgcagccccgacttccgcaaggccttccagggactgctctgctgcgcgcgcagggctgcccgccggcgccacgcgacccacggagaccggccgcgcgcctcgggctgtctggcccggcccggacccccgccatcgcccggggccgcctcggacgacgacgacgacgatgtcgtcggggccacgccgcccgcgcgcctgctggagccctgggccggctgcaacggcggggcggcggcggacagcgactcgagcctggacgagccgtgccgccccggcttcgcctcggaatccaaggtgtagggcccggcgcggggcgcggactccgggcacggcttcccaggggaacgaggagatctgtgtttacttaagaccgatagcaggtgaactcgaagcccacaatcctcgtctgaatcatccgaggcaaagagaaaagccacggaccgttgcacaaaaaggaaagtttgggaagggatgggagagtggcttgctgatgttccttgttgttttttttttcttttcttttctttcttcttcttttttttttttttttttttttctgtttgtggtccggccttcttttgtgtgtgcgtgtgatgcatctttagatttttttcccccaccaggtggtttttgacactctctgagaggaccggagtggaagatgggtgggttaggggaagggagaagcattaggaggggattaaaatcgatcatcgtggctcccatccctttcccgggaacaggaacacactaccagccagagagaggagaatgacagtttgtcaagacatatttccttttgctttccagagaaatttcattttaatttctaagtaatgatttctgctgttatgaaagcaaagagaaaggatggaggcaaaataaaaaaaaatcacgtttcaagaaatgttaagctcttcttggaacaagccccaccttgctttccttgtgtagggcaaacccgctgtcccccgcgcgcctgggtggtcaggctgagggatttctacctcacactgtgcatttgcacagcagatagaaagacttgtttatattaaacagcttatttatgtatcaatat

SEQ ID NO: 113 - DNA, 5583 bp, Artificial Sequence
  subsequence of OTX2
aaaccaaaacccaaaactaagagattctctccacaaccggcctaggtatgcactctgcatagaaggcatgggcccttcaatctaactttcaaagctcttttcctctcgaagcagggtccagaacggggaaaagaaataacttttgaaaaatccacgcctcactatgactgctcacgaggtggcctctggagaactcatacctagaagctgaccgcggtcgcgcggcgagttccggcagccggtcggcgaccgcacctccgggcgcgagtgcctgggtcccgcgttcctgcccggcagccccgcagccccgcagccccgcagccccgcagccccgcaggcctggcgcccgaggtcccgctccactgcccgcgccccccgcgcagccttatatctaacggtcaattcgtgcaatctgtcgcttctccctcccccacgccttgttttttttttcttccaagaagcccatctaccagttgctgtgtcctcgctcaacaataattacctcgtccgagaattaattataataaatgttttcttgataaactaacgagataatccgaggggcacacgtcccttaattacaggccgccatgctcctctctgcttctcgtccgggctgattaattttctgcatgatggaaaggaaacaaaactacgcggactggcgactggcctgcggctgggaagacgacgaagaggaggaaagaaagaaaaaggagacgtgtgggcaccgcggaaaacggccggcgctggcctctctccggcgaactcgagtgaaagtttctggcctcggggaatcaaataactctgccacccgcgagggagggaggaagaaacgtgccaaaagggttggccttgactattaattatcgttgggagaaagccccggtgttagcgctgaggtctgggtgtctaccttactctggggggaggagttccctctcctactcccctctgttgctaataacttttggtgcctgtaaaaagtcccgagctgagcaggagaaatcctgaccccgaagctctaggatggaggggagaatttctaggagcgacttccccgtcccctccccaagcaatccaccaccgcagggtcggcgccgctcggccttcgctccccgcgcaccagttctatctgtgaaggaagcaaaagccaactcggtggaatcctgacaggggacttgggtttccaaaaatatgtcccgaaatcgggcatcgatttcaagagtcacttgaacgcaacaacgcgaagacttcttgggagtttgcagagcgacccgtcgcccgcgcccggcgctggcagggaccttcggatggttcttactgggccgatccatggcacaggctgggcctcggcgaacccctcggcccccgcccggccccgagccacgacacctcattgtcctggagcctgggaagggggtgcgcgagcgcgcgggcgagccctgcctctccccgccagagaacagctgaggggccgcggtcccagcgggaggattccggtccctggcccggccgcggccttgggcggagcaggggccactagctgccacttctgcccgccccaggtgcgcgcggagggctacgtggggcgggccgcgacccggcaaagtcatgttgaaaaaacactcttcacgttcgctcggcctggtgaccagggtcggggaccacgacaaccgggggttgggaggctgcgtaattacaacccagggtggtttggattttggggggtggtggatatttaaaaacaaaaaggagatctggaagcttttgggagaaacagacaaccgagctgtgctaggctgagggagaggaggccaaagagagcgagcagtgagcgccggggcggacgagaagccagcgctcccagcctcctcggttatccgctccggtttccgctcacgttcaacaggggccgacaggggctcgagcggcggcccccggcccaggccgacccgcaagcgaaccgagcttccggcgcgcgggcccaaggaggcgcctggctttttattattgttgtttcaatccatccatctagttacatctgcatctttttgtctcggactctaaaaaggtccctgggatccatccaaacgaccccaaccaaatctgggggccaaaacgcaaagatcgcgggagaagcccagaacggcgttgacataaaaacaaaaccacaaacaaaaccttccaaaacaccccagattacattcgcagcgtttcgacgacgttttgcagaagcgacgacccccaggagcacgctctctgcctctctcccactaccgctctcatctctagatcacatttttctttttgcaacgatcgttattacacctcaaaatttgtaagagaaaaaatacatccgcctacagaactccacgttcgcagaggggcatcggtcggtctattggaggtactggggtgatggccgacagacacggggacacgtagatatggatatagacaagacagacggacacttaccttacagcctcatgggaggttagaaaaagtcaaatatcctttaaattccaaatagccagctatcctaaaagaaatcaagagtattgagttagaaaccttgcagtcttcacccttccatgaaaagtcaaacacaaccaaaaaaaattttttttaaagaacgaaaatgaggaaggcggctagagttctaaacacgcgtgggcccctctgcaatacatacaaagtagatgtggcgagtgagggctgctctagcaatttttatttttaatcacagtggaggctgtgttggagctgaggccggtcccgctctcagggagatttgctgagaaagcgcctctctggcaactttttgacgcaaactctccaaccaatggcagggagagaatgattgacacatctaagccagagggaaaataataaaaacacacaacagggggaggaaaacaggccgctgctgcacggggggacgagcaggcaacaaatccaggcctccgacattaccagaatgttctttaaagacactgggctttgcttaaaatatacattatgggccggagcatgtgaactaattgtataattaaaatgatggacagggagttcttctcttaccctcttttcccctgcttcctttactccgaaatttcctttcctctcttttttttttttttttttttgttgttgttgtttttagggaagggaagaaaggaaacccatgcaatgtaagatggaagataaaaatatttaagtaaatgctggagaatggcgggttagggagtgactgggttatcacattcaaccccagcaataagtgtgtggatgacaggcagaaagcaagtcagactgaaactcaaaaacaccactatgccgtctcagacagggccagagcacgctgacggccagaaagggtaaaggagggaggcctgggagtgcgatgtgggcatgtagggaaaacagagagagaaagatacacaagtccaagaacaaactattttctaaaactcagtgtcttctctattccctacgcccttataaatatccttacacatataaataaatgatccccgagtgagagaccccggcttctggtaggttcctggggttttttggaattgagaagcccacgacagactgcagggaacacgaaccccggaatctaatctcagggcccatttaggagaagtagctgggaccacatcgggcctcgaggatgcgagtgtgaggtcgacaagatatcgtggaagagagcgaacgagggaggcccccgttggaaacagtttctgtgttagaacaaacgccaccaaacgaccgacactgcgaggcctggagctacctgggctggcgccgcccgagccccgggctgcgagcccagaggctgggaagtgatgggacctgggggcccgagccggagagtgcgacccccagcccaacttttttgcctggcatagaaagcagggaccggacaggtttcaaacggatccgagtccctagaaaagcaaaaacagactgggcggagtgtggggtggggggtggctagtggaactggtgagtgtgtgtgaataagctgggtgggggtgggagcagaagacagctcttgcttcacaacacccagtgcaggaaaagaaaaataaaatctcttcctaaataccccaccccccgccacccacccaccaccaactaccatcaccaccacggccagtgggcccaaagaaacagctcgctgcctttaatttggggacctatgttaatgaagttggtaattaattcgtcgctttgttgtcggttcttatactgtatgtgtactcaaatgtggccgtccttgggatttacagcaattaacgaattacgggagtgcgcacgaggcagcaagctctcggcagccgggctccggctcgggctcggcctggggctggggactccgcggcagcggcccctgtcacaggtgtccctagagctttgggccctggcggcccctcgagcccccgaggggcccggagcccgcccagctccttcccggccctctgcagcagctccagtccggagacccgctggctgtcgcgttcccaggagtcaagagtttctaggggcccgggcgggggggagggtgagtaccgaccttttttctcaccccacccccactgtactgaaacacctggcggccgcccccgaagcctttaatggggatggtggtgaggagggggtaacaaatgccccgggcgttatgaccctcgtggcgctggctgtcggaggcactggttgggtgcgcttggtcagagtcatgatgctttcgatgaaggaaaggcaaatccacctcgatcacctgaagcagagtctccttcctacccctagaaaagacaacgtttcccccagtttgatcacaatgatgtttaaagcataaaagagccgaaaaagaaaaatggacgttgtgaatctggcagaggggaaggccggaggaaggccttggggacagtgggcatggggtgggatggagaatgatcagaacatgcgcttgtgagctaaaccaagtaaaccattttggactgggagatccatctgccgtagggtccagtgtccagggtaacctttcaagcccgatgtagaggtttgcgatgtcctcccagatggcgggggcagctgaatctccctaaaaatccccctgttctattcgacaggggcagatttatgcatggtggggcgtgagagggttttgcccttccagcggccggcagcagacagctcccgcttctcctttgccctctagtctaataacttcgcagaaatacagggccaataaactacgagttggaaatggacagtgttaaataaacaagggtctctttaaaattctcatccacttcagatgtctaaagtaagattgtgatgattttgtcacggtttggtaaatttacccctttaagaggctttcataaatcccagaacacaccttcagccagatttgaatatagatttaggttttaaaacccagaagctggaaacaccgctttatcaaagagaatttccctttagcttagcaatgtgctgaagctcttaaaagattggatctgagagagagagacagagaggagaaagagaactagagacagagag

SEQ ID NO: 114 - DNA, 7286 bp, Artificial Sequence
  subsequence of NKX2-6
actccgtctcaaaaaacaaacaaacaaaaaacaaacaaacaaaaaaaaaactgtgtgtgcatggtaaaccttcgctgtgaggaacaagtgtgagtggaggtgtctatcagattgaggagactttggaccctccttggaagtagagaaagaaggagaagaaagaggaagaggaagaggaggaggaagaggaggaggagaagaagaagaaggaaaggaaggaaaaacagagagaagcccgggtgtcaagaaggcgcaaactcggtgacaggctctcaggaggctcctgtctgcctcattttccttcgcagccccaagcgcactgcagggaacttggctgtaagtccaggagcgggagccttgagtgtctcctaccttcacccaacttttgtgcacactcttgtctttttgacgcagcgctccaccaacaccagggatgcatcccagctttcttggatgtgatgctttgtaatccaaattaacaatatatgatgaaaacaaaatatttattggctcctgacttttggctcagaaactgaggttctctttgagagatacataaagttgaggtccacatttggcttcttaaaaagtagcctctccctcctttggggtctttctggcaagcaggtggtgtgggcttcaccctgaagtcttcctttcacccagggcgacccctacagctgagactgtgcccaccaagatgcagcgttttcctcccttctcacttctctcctgtctgggcttaaaccccgttttaccccaagggtggatagaagggaaatgctgagttttcatgggatctcacgccaggagaaaatcaggagcatggaaggggtgcaagttcatggcaagacgggacaggactctaaatgagccagtgcgattggaaccagactcctaatacccaaggcactggcacaatctcctggagggggatggagctgtttggtatgtaaagtttgaggacagaacaacttccttcagagacgtctgtgctcagataaactgaggccatctccacttgcaaagaggaaaaattctgaggagggtttgttttcttagcgcatcgaaaggtaacaactgaccttcagccaggctgcagagcaaggaggaccccatttcaaagtcacagatcatgcaggccctggggctgcacagcaccgcagggtgggccagcaccctgcgcccttctgttcacaatcctggagttcttgagggcaaggtggttagctgcgatggaggaaggcatgaagcccaccgaaggtgtcttccctgtccggatcgctaccgcggccttgggctcagttcctggagccggcctcgggtccggcctcgggtccctcctcggcggcgtccactgctgccgcagaagagacgctcccaggatttggtttccagtgggagaaggaaggcgccgcaaataccatcggctgcgaggcgactgtggtggtcgaaggaacgtgatcctttgtcagctcagcggagccgaagtgatcgccgagttggctgagcagcgccgagggagtttagaatccgctgcagaaaacctaccagcttcttcgcggacacagcaggtaatgttcttaggcttctggagttagtgagtagccggcctgcaggccggtaaataactccgatctagccccttggtttatttctttcgttcgcgccttgaatggaggcgccatggcacagtctggcagaggaggcctgccctggcgggcgctactcagggcccctgcgttgagaatgccgagtgaggtgctgaggtttggagagaaaaaggtggcgttttcatcccttggaatatcgggcctctccagctgaagcctccggatcgacacaacacaactcccggatcgacgcaacacaactccccgccagccccttcccttccagcgggctggacacaggtgcgtgggcctcgcagcccggcgcgcacggttgcgcctttggatacctgcgacaggactcggccagaaccgtgtcccagggcagagaaaaccctggcaacctttaacgttctccctgacgcggagaatcctgcgccaacggggccttccacttcgggagactcaatcgccacccggtccccaactttcgtcttccagaagaaaaatccatgaggaggaatgggggggtcccccgaccagaccagcaagaaagggcccagttaggagtgacctcagcgccacgagggttccactgctttgatggccacacgcttttgcaaacggtttgggggtggagagacaccaggtgatggtagggaagggcggtggtgactggcacggctaagacactgcggagggtttcgctgtggagatgagaaggtggaggttctgggcactgtggctgcgagtgtgagcgatgcgtttgtgggaatcagaggagcggatttgggaaaagtgaatccttgagattcagggccttactttcgttaggggtgtgtgaagcacactgggtgtcaggagaggatgggaatgggattcgagaggcctttttttggactcctcgagagaaaatggagagagtctcgaacccaggagataggaggcgtattttccccatgcacccatggatcacgcccccgcccccacattccccccgtaggaggcaagacctgagcgcttactcacgtggctcccccatccgttccgcgtccatctccaagactgcctcacagggacccccaggaggctccgaaccatccagctttctgtcaccgccgccgccaccagcgttgtgaacctctgaccctcgcggctctgcgtccattctcaggtactgaaagttttccgggctcttccgcacccgcggatgtggcgaagccgcggggcagctccgctcgcgctccagtcgcaggatgtccttgaccgagaagggggtggaggtgacggggctcagcagcatcccgaaggcggatggggcggggccgaggaggtccgggtgaggagcggcaccctgaacttcccgtcttgtcgctgcaggccccgcagacagacccaagctctgggacagacgcccagcgtcccagacagcgccttcctctgggccatgctggtaggcccgggtccagggccgggtgacgagaccgtagccccccattggttctcgcagaaaccacgtgctagctctgcaccttcctcccccagcgctttcttcccgcgcccgtcgaatcctctccagtccccagtcgccttcctgggaggtttggttcgtattgacggttctcaaagcaaagaaaacgtggagagacagtgctgcgcgcggcttggatctccgtcaatacggtactagcgggagcttccgaggtcaacctagggtccacggggaccctcctagtggacatgcggggattggaggtggagtccttgctgtgcaacccgatccggtccatccagcctggtcttagctcaactctgcattcttatggcggaggaaagctaagatagagacagctgggacccgcggaatttgaggcgcgcgctgggatcttacgtgcgcagaggccggaccgcagagtagaagtgagtcttgacccaccagggcctatattgagatggaaacctctctctttgaacagaatccaggtctgcggagtcccgacccgccacttcctaggagcagcttctcagccccaggaccgaggaatgggtgtgggggctacatgtggggagccctcgacctcttaaagggctccgcgaatggtgggggagactggaaggcaatctctgcggcccgcgcaaagtggtcagaggcgggagtgggggtgggggggggtgggcttccgtcgcccttggcgtccccacgttctttttcttcctctcctttatcctccttaaagcggattgcctggagcgtgccagcttgtgtgcgcgtataaatgcggcgcccgccgaagggctgggaagatttgactcgcattagatctccagaaaaggcccttggttacggcgggcaccgagtaaatggcgcagtgtggcacaaaggttaccaacacggagatagcgccaacagatccagcccctgctgttactactcctggatcagggaaacgtgatttggtgtcagctgttccagcactgaatcgaagagggtttaaaaattgtgttttaatcacaatgggatctcattagagttcttttggggatttcagatcaaatgtttctttttgtttttctttccttcctttccctccctccctccctcctttttctttctttcttttctttctttctctttcttcctttttttttttttttttggttacagggtctctctctgtctcccaggctggaatgcagtggccggatcatggctcgctgcagcctcgacccggactcagtgatcctcccacctcagcctcctgagtagctgggaccacagatgcagccactaagcctggctatttatttatttatttattgcttgtagagccggggtttcgccatgttgcttaggctggtcttgaactcctgggctcaagtaatgtgcccacctcggcctcccaaagtgctgggattacaggtgtgagccaccgcgcaggcttcaaatgcttcttaaacctacttacgtgaattcaatgttacaacagctgtttgaatatgattatctcctgaaattcagataaacccaactcatctccccaggctaatgggtgcaaaattgcacacaaatatttatgcaaaatttcagcacatttgatcattcagctacaaagtaatgatttcctatacatggtaacatttaatcttcacatcaaagctatacccaaatatttccagctgctgctccttcttcttcttcctcctcctcttcttcttcttcttcttcttcttcttcttcttcttcttcttcttcttcttcttcttcttcttcttcttcttcccctcctcctcctcctcctccttctccttctccttcttcttcttttgttcagcgaggagtccagatcagagaggtggcccagatagttcaccaaatggcaagaccagactagcctctaaaccaagacaatttaccctgtctttctttctttttgaaatatacatcctttgctcttagagatctcaaaatcttctgatgacccatacatttatttgaatttttgtttcctgataaaagtcatcatgcgcaccttggaaaaagtgaagaaaagttaaaagaaaatatccacccagagacaacattttagtggaccttcttgtctttatttctgtatatatgagctcatagggtatatatgtttgtatatgtttaaatttacatcataagcatgcccagttcatctttagaattttttaaacaaatataatttaaaataggaatctaatatttcatgttattgatagaccgtagtagactgtgtttgtatttttagataatatctttttttatcactgtaaataagactttattttgtgccttcaattttcatccttgtcaatattttctgttattttctcaggatacatatgtagaagaaacatcaatcagtcaaatattttaatgctcataagacatgccattccagggcttcctagaaaaacagtattatcgtattttgttcccggaggtgcaggcgagtgcctggtctacgggtgtttacaatcatcaccgggcacccacaagagaccctgaacttagaatatttccgcggtaggagttccgcctcgtccttccaggggatactgacgactcgctgggttctcgccttccaagtgctggaggggggaagtagggccacccggggtagaaacctaacgccagaaaccttccagcgccttatcagttggtggaattttcgtggcagacagtcgcgctctacctaagtcgtagaagaaaagacaccttgtgggggacttggcgtcggaagccttgagttcaaatcgtagccctaggtccccagccttgcccttcctggcttgctgcgaggatgaaatgagatttttgtacgtgaaaatgctttctaacccctctcgaggggtggaaacgtctccattcgaccagagtccgggtctgcggagcaatttacccgccgctttccaagagcaggctccccagcgtagcgagtccttgttatggaaagggtcgtttcggctcaggatgcgcgctcccggcgtagacctggggataggggtccctgtcgcgctcgccccacccctgcagggagcaaggccgtccttctgcagcaccgcgccacgcggcgggaatttgcagtgtcctgctttctggtttcagcttcttcgctcgcttgggtctctctcggtcacctctcggaggggcctggagtccctcctccctcctcctacttcagcgccagaagcattgaaagccgcccgcccgccgagagtggaaccggtacctcgaatctcgctcattccgggtcaattggaggcgcattagcggctgccttgcagtgcaacagaggctcgagtgacaggccacctgcctaagcgctggcgcccaggaaagccggggaggaaactaggaagggaggcgacagcagaaaagccagagagtccagagactcctaggcaggcctccgtgcagccccaacagcgtggtgccgggaggtgtgtgtgtgtgtgtgtgtgtgtgtgtgtgtgtgtgtgtgtgtgtcccttactcaggaatggagacatcgtgatcacctctgttcttaggtgagatggagacggccgtgctaggggtgtgattgatccgctttgcttcactcaggtccgcagagtgttttaagcgcctaccgtgggccagctctgcccaagctctgggaatactgagaaaatgagaggtctcagccttcttatccgaacttgcattcttgcatagaagacagacttttaaataattcccatacattgtgttaccttgcacaatcagacggaatttgtacactatatttattgattttttttttttgagacggagtttcgctcttttgcccaggctggagtgcagtggcatgatctcggctcactgcaacctccgccttttcggtttcaagcaattctcctgcctcagcctcccgagtagctgggattacaggtgcccgccaccacacccggctaatttttgtatttttagtagagaccgggtttcaccatgttggccaggttagtctcgaactcctgacctcgtgatctacccgcctcggcctcccaaagtgctgggattacaggcgtgaaccaccgcgcccggccctgaacctctacttctccgtggttaacaaaagtcattatttcctgtttctttcactctcctgaaacgaagggattccctcc

SEQ ID NO: 115 - DNA, 7007 bp, Artificial Sequence
  subsequence of SIM1
caaactttctctggtgatgcccaaaaaaataaaacgctccggactcttgtggccgagttttaaaaatttaatatggagtcggctagagtacccttttgcggaaagaaaaaacaaagaaggcaaaaaaactttcgaagacctgtgttaagctatttatgagtattatctttttaatagtgctgctgctaaaattattttaactaggtagttaaatccttttatccttacaccattaaacaaagtttaacatgacctcccccatcccacccctcagaaaggtgatttactgcgttaaggagcaaatcaccaagaagtacacaatgatgaacactcgccttgtaatatgaggttgggggcagatctttcaaaataaaacatggagttggattttttaaaaggtgttggctaggagctgcttcctaagcaagcaatcaaagccttggtaaggaggaaccgtgagcgccccttaagctcaaatccggtctttctggttgtttgcacatctaaataaatctaacgatttccccaccactctgcaaacactgatgctccccgcccgcactcgggactcctctacctctctggctcccggtcaactcatcccgactctttagcccgcccgaggtttcctccccggagtgactccactgccctggtccctggggtcctcctggaccgttctggaagggcccccgccacagccacctgtacacaccccttggccttatcacatttatcgctcttcccctttcagccaacctattctccttcgtttctgtcacgacctgctcttctctttctaaatcccggctccgacatacccactcagaaggagtgacaggagggattggctgcggaggccacacgggggaaaggagaaaggaccctattgggaaagccgaggacgccggcgacgctggcccttgggcgctctggggcctacggaggccttaaaccccaaagattggcggggacgaagggccggggcactcgagcgagcctggagcgggcaaagactgcgttgcgactggggacaggtctcgcgcggttcccgaagggtgcgaagactgcgctgagcattttgaaggcctcccaaagcggctggaagacaccccgaagcggcctcccaaccagaatgatctgaaaatcccccaggctgggctcgggataaatactagttctgaactcccggcgccagcctaggccatttgttgtttcgggtttcggcctcattagtatgcgcctacgagggaaaatgagacttccccacaggttaataaacaacctgtccggcacaggttaacaggagcctctctcgccctctcctgccccacccccgccaccttttaaggaagcttttgccttcccggaggtttgccttctctttctgttccccgtagaaatcttacgattgtgtctgggttaatgttttataagggactggctactctcgtctacctgccgggctttcccgatctaatatcgaaggaacctccccaagtcctagtaaggggtcccccctccctaaagtctcgaagtggggtagagaccttctccctggagcccctcgcctcctgccttcggtgacgcgctctagcacacccaatttcagttggcgagggggtaagctgagatttcgtttctgcacttgacctaccgcagaaaattcgcaaatcctttgattgtctgtttaaaatgaggaggaaaccagctccctttgcggcgggattacagtgggaacaagatctaaagattctcttgcaattcggcgaggccgagggaacggggttttgcaaaagagaaaaggagctctgtgagggaggcgataactaaatcgggttttagacaaaaggattttcctcagctaaagtggccgaagacaaaggaaaacagaatctattttggaagatttccaagaaatgccacattaaccttagctgataaattttgcttctcccaggcccccctcttcccttaaagtctgctttatcatatttacataagtagcattagaagggatgtatctattatggatctaaagggctagctcacatttcctgtgaaactcaggcaagtttcactgtggctttaccctccgtgcttagttgagccatttccatttaaataccccctgacccaaggattacctcaatggactgactgcacgggttttgtaatttcctgaaaatgagatttcgatttataaaacaagaaaccaattagtaaccaaatgaggcgaagtagatccactaaaattgacctaatcccacaggcaccatttaggcccgttcttggcgaatgaatgatgagccccagtctagtgtgagctcaaagcatcatccagctgtgttattgcaggcagcaaaaataaattgatagagcttttccttcggaatgaatttaatacccttgacaaaatatatattacagacccgacatcatcaccgccctcactctgacaggaagaggaggaagataagcgtgtgttctgttcttttaaaatttttctttattttaataaataaacgctacatctcaatagaaatgtatcctccttgcagtccttcccgggaaccttcacctccccaactaattgaggtgccttgtaggcaatgggggagggtggcggaggccctgttccatgacctgactacgacttggtgactgaggaggggaaagccctcctaggccgaggccactgcggttcctgaacagcttgtctcaaccaactgtgtatcccttgagagagtgtaggagagtctggcccagggggtaatcctgaaaaccccaaatcccatgtatcctgccgggcctgcacatcctcgctaaatgtgtactgtgcaagtcttccccgggctgaggcgtcgagtggccttcgtgttcagcctccgggcgcctccgcagccgagctctttagagaaaaaaagagagggaaattggtgcaaccagcccgaatcaagctcctagagcagtcactggtaggaggtcccttcacgcaccaaggcgcacccgaccccacctctggcactgctgcccgccctgcctgcggccctctccggctaaggagcctgtgtggttgacctgagggcatcggcgagcgcgccgggccaggtcttgttccacgcagcagcctggaccccacagtgtgtgcctgcactcggcagtgccctgatctctcctgcctgctgatcccgggccagagacaccgcggccgcacccagggaatccactaatgttactgtaaatgtggggtggaggccgaaggtcacaccgctgtctgtctctctctttctctctctctctctctctctctctctctctctctctctctctctctctctctctctctctctctgccttcgcggagctccagccctcgagtttgggcttcccgtagggatagagcctgcgggccaacctggctgcccgagttggagccagccgcgaaaagacggcagaaacccaaggagggcggggttcggccagactaaaactgggggcgaaattcatgcagcgttcatgagacagtcctgcgtgacggccgaaaaacgtcaatcgatgtcgccctgggactccgggtcttcgaatgcggcccagctttggctatgccacctccctagaggcccgcgctggcgaggccgagcccgaacgcgcgggcgaatcccacttaggttctacttggcgcagggactcggacgatggcacctaacccgccttcccgggaactgcccaaacagactggatctggacctaaggtttagacgactgcttgcccttcagggacagtggccgggagggcaggaggggctgctggcacacacctgcacctgcgggacctctgatgagggcagggggcggctcctgggccggcctggggagtaaggagactctgtgctgaggccacgagctaggcccttggctggggccaccgcggacagaggatgggacacaccgcgcagacctggctgactgcgtgcttcgggcggtgcgggaggcgcgacggggacctcgacatgattgtcccctgtcggccctgcgccgccgaggccgagtgacaaggcgcaggaaccgcctattcggtggggctaccagcggaaggaagtttactctgcagtggacactgttttagcactttaagagtagcaggaccattcctaaataattgaggttccccctcctccacacaaaattttaaaatttcacggatcagacactggcaatgggtggcccattaaaatcattaggtgttagcaaggtacaagcctcattttcctgagaaatacctggcgggacggagaagtgcggtgagaatctatgggctctcattctgtgtccacatttgggtctgtaaaagctggaagctcccaagatttcttagaactggacaacaactcccctagaaattagatttgttctttagaaattcagccccgttttatcattagacgggtgattgcaccctgcttgaaagcatcccaccatagcttataatacctgtttttgttgttgtttgttgtttttattagtgatccctcccattaaagaaaaaagtattttttttattgatctgatctacaatttctagcatataaatccgccttgcaaatgctctgcacggagtttagttctgcactccacattttaagtcaacatcaaaactggaattaaacacagaaaactagcatggagggtaaactgtgcttaaaggcctttaaatgagaaaaacttctgtaagaaaataaacatggaaacctaatgctcaatcatttccccaagaagcaagaaaaacagccttaaatcaccgacccacgtgggacatggggcctctttttctttttcagttctctgcctcaaaaaaatataacaccattaagaatttcaatcttgaggtgaatattatagaaaccatctgtggaagtttgtttaatcacccttgtagagatgatctttcctgagtagttactaatttcaactctgtgattatttttatttttccaagacatcttgtcaatgaaatggcaatgtgatgttaccaagattctgaatagctatagatcagaaaatatatctgatcctttcaaagttgattatgaaagcctccacacccccagccaaaattgctttagagctggataacaaatatgtatgtctttctagttgaatttgtcctattttgcacacaaataaagtcatgctattttttagatcctgcccctctggctttgataataccaaagatttatacatttccatgtgcctcaattttttctttgcaaggctactttggaatagaatatgtcactaattggcagatatgaagtgttagtgatttctcagttatctttcctaattttcttttttctctgaaatctccaatctaatgctttattcttaattattccaggtacccatattccatttctctgttctcccactcccccattttcacctaaacagtttaatttcatctagtcaggcaaataaaagctgaaacttgcccccagacaaggaagctactagacttgggagaaaaaaaaaagtgtattcggcaaatgagaagggaaggaaattgcctgtatttaaggtgtatttaaggatatttcttctttcaaatataattatgaaatgattttgtttgttcatttaacttatagccttttggcattacagtgtgttagagatgaaatagtgtatgaacaaaactgaagttttacagcatttttatacctatagctatgtcaccagattaataattatttagattatataccttataaaatccatatattacctgtgataagacacttatacctatctttatttcatccttaaagctgtattgaggacctactatgtactagggtggcttcatgataaatgtaaagatgaatttcatcttccaacaaattccatttaacgccactagaaaagattacatccatataaagtgatcagtttccccaactgccttggaccccaatcttgtttgctctctgccttcagtcaacactgaacttaaatttggcaccccctataggttgtgcctggtcttgcgattgtgactattttattcctttgaaagctgttgttgttgttgttgttgttctttaatattttaaagagctgtgtttgattttgggtttttgaagcttgtccaccgtcaaaaattaaaaactcatccctaggagccagctgttctgatgaccctgtctagctcactgggtggaggctgagggtgagttatgagctcaacagtagctagagaaacaaatgatgtgcccagagttcacacatcgtccatcccctcctccccataaactcacactcacccacagaagggagagaaaggaggggtccggggctcgggggaaggtgagggggctgcagaaagcacagtcactgttaaagtagccagaggggaccgttctggccaccaagaggactccagcgggagccttcattggcgctctctttaaaaataacgagaggttggctgtaagagtttattttgttcctatttatttataacgagacttataatgtgtagagttagcacttaattatgcaaaaaggcttgctcttttaaaaacaaaaacaaaacaacagcagaaaacagcccgatttcctcccagctgcgcctgcccccgggtctacaccaagccgactagcttccctggccggccgactccccgggctctcccggccggctcggtgcccgccccagaacgccgccctgctattcttctcctcccgcgattactcgcagccccacaagcaacaccatatgctgcttctgatcaaacagcgagcgacatcggcaccaataattgacgagaccggctggaaatcacgcagaaagggagcccactgagaccgcaggggctgacaaatcactgctaataatcctgttaggaacagtgcggccagcggagttcgcaatagctttatttttataaagtaggcgctgacagtataaaagacaacgagatctcttttttaaatagaag

SEQ ID NO: 116 - DNA, 6193 bp, Artificial Sequence
  subsequence of DRD4
tgcggccgcacctgatgcctgtgcacacctgtccctggtggtctctcctgtggtgacttcttttgctcaagggttcacaagggcagcagactgatctgcacaagagggactgagcctggctgcggccgcacctgatgcctgtgcacacctgtccctggtgcaggcccttcccccgcagccccgtgaccttgtcctgtgaggctcacggtgcctgctccttctcagagtcctcatttctccctttaacgcacgccctgtcagcgcctccgtctagcccgtgtcctccagaccttcgaggtcaggggcctcaattcctggcacagcccctccactccaggcctcccagaaacagactagagcatcaggatgtgcgccgcctggggtcccacagagtggtgcccccttttagtgtcttctaggccccttagtgacagactacagaaaatacctctcaggtcacaggtcacccctctttggtgaagagtccatagaattctctgctgcgctttgcaagcactttctcttctgcacgtttggaacctaccccggcctgtcgtgtctttctcctggcctcctcgcgagccgaacctactgtccggtcccgggaccccctgcccagggtcagaggggcgcctacctagctcacggtcttgggccggagggaatggaggagggagcggggtcgaccgctcagctgtccgcccagtttcggaggcggccacgcgaggatcaactgtgcaacgggtggggccgcggctgaccgtggtggtcgcgggggctgagggccagaggctgcggggggggggcggcgggatgagctaggcgtcggcggttgagtcgggcgcggagtcgggggcagggggagcgggcgtggagggtgcgcacgaggtcgaggcgagtccgcgggggaggcgggcagagcctgagctcaggtctttctgcgtctggcggaacgggcctgggagggaggttttgccagataccaggtggactagggtgagcgcccgagggccgggacgcacgcacgggccgggtaggatggcgctggcgtcgatgcccgcgcgcttcagggcctggtctggccgcccctccatccttgtcggtttctcgggtcgcggaccccgcgcggcgccgggcgatgctggcctgcccgtggccaccacctcgcttcattcccgtctctttgggccgccgcattcgtccacgtgcccgtctctccctgcgcaaaattccaagatgagcaaatactgggctcacggtggagcgccgcgggggcccccctgagccggggcgggtcgggggcgggaccagggtccggccggggcgtgcccgaggggagggactccccggcttgcgacccggcgttgtccgcggtgctcagcgcccgcccgggcgcgccatggggaaccgcagcaccgcggacgcggacgggctgctggctgggcgcgggccggccgcgggggcatctgcgggggcatctgcggggctggctgggcagggcgcggcggcgctggtggggggcgtgctgctcatcggcgcggtgctcgcggggaactcgctcgtgtgcgtgagcgtggccaccgagcgcgccctgcagacgcccaccaactccttcatcgtgagcctggcggccgccgacctcctcctcgctctcctggtgctgccgctcttcgtctactccgaggtgagccgcgtccggccgcacgagcatcctcacctgctcctcggttccccgtccctgtccctacggaggacccggcgcgacccggcccctttctggtgcggagcttccagctggggcggcggcaggggcgctgcgccttgtccctcggcgatacacccaccgccgccacctcgcgaccttccacccgctgcgctgtctgtcccccgaccctcgttcctcttctccttccccgtctgtcttggcgtctgttatccaggagatgcccgtccttctatccagggaccccggaaacaggcgactttgtcaagcccagtcccctccgtagctggatttcacctccagggcagccagctggacagacaggcagatgcaggctcagccccctggctgccgtgggacacacacacacacacactgccacagccactgcccaccacacacacctagtgcagatgctggcacacccccagaaggaggctcacagctcgcaggggagacctgggctggacaaaacccaggggaggggagggtgtgtggggaccaggcccctgctgagaaccctggggggaagcctgagggggaattgggggatggagcccacactccacaccaggtctggccctcgagtgggtcggccttggtgccagcccctctgcggccagagaaaagcagcttagggctgagctggagacgcggtgtccccgactgtgggggagggggactcgaggtttccccttgatggacacagtgaatccaggcggctggggcagagaccagcagcacgggacacgcgtgacctgtgctcctttcgagccgcagacgtcacagtgacgacgtttaagctcctaatctccccaaatcggcgggaaggattagaggggctgcctgctcctttgcccttggagagagtcactccacgtggagtcctacgctgggcactgggcacggtcttcatatttttaattataatttatcttcaagacaattatgatgtggatactatcatcacccttgtcttacagatgaagaaacagaaatgaattaacgtgcccgagtctcccacagagaacttagccaacagagcagccagcttcgcttctaggcccagcggggaccctgcctaccccaggctggggaggggctccctttgagcccgatgatatcaggcccgcccccagggaattccccaggccgttctcatgtttgtaacaaaagggagaccaaggccagaagccgtgattcacgcctgtaatcccaggactttgggaggcaaaggcaggaggatagtttgagaccagcctgggaaacataccaggcctggtctctacaaaaaattttaaaatatcagccgggggtggtggctgcggctgttgtcccagctattcgggggagctgaggcggcagaatcgcttaaacctgggaggcggaggttgcagtgagttgagatctcaccactgcactccagcctgggcaacaagagcgaaactccgtctcaaaaaacaaaaagaaaaacaaatcagccgggggtggtggcgcgcggctgtaatcccagctactctggagactgaggtgggaggatcgcttgagctcaggaattccaggctacagtgagccatgatggagccacagcactccagccgcggtgacacagcgagaccctaactcaaaacaaagggagatctgcgtggggaaggggtgtttccctgcccggtcctctggcctctggctcacagccgggcccccttctccgtattcagccctggaactacccataagagtgggggcgggtcacaagggcccgcggtggctgggaaacctcagggcctgtggtgtcgccgcgcaggtccagggtggcgcgtggctgctgagcccccgcctgtgcgacgccctcatggccatggacgtcatgctgtgcaccgcctccatcttcaacctgtgcgccatcagcgtggacaggtgcgccgccctccccgcccgcgccccggcgcccccgcgccccgcccgccgccctcaccgcggcctgtgcgctgtccggcgccccctcggcgctccccgcaggttcgtggccgtggccgtgccgctgcgctacaaccggcagggtgggagccgccggcagctgctgctcatcggcgccacgtggctgctgtccgcggcggtggcggcgcccgtactgtgcggcctcaacgacgtgcgcggccgcgaccccgccgtgtgccgcctggaggaccgcgactacgtggtctactcgtccgtgtgctccttcttcctaccctgcccgctcatgctgctgctctactgggccacgttccgcggcctgcagcgctgggaggtggcacgtcgcgccaagctgcacggccgcgcgccccgccgacccagcggccctggcccgccttcccccacgccacccgcgccccgcctcccccaggacccctgcggccccgactgtgcgccccccgcgcccggccttccccggggtccctgcggccccgactgtgcgcccgccgcgcccagcctcccccaggacccctgcggccccgactgtgcgccccccgcgcccggcctccccccggacccctgcggctccaactgtgctccccccgacgccgtcagagccgccgcgctcccaccccagactccaccgcagacccgcaggaggcggcgtgccaagatcaccggccgggagcgcaaggccatgagggtcctgccggtggtggtcggtgggttcctgtcctgaggggcggggaggagaggagggggggggtacgaggccggctgggcggggggcgctaacgcggctctcggcgcccccaggggccttcctgctgtgctggacgcccttcttcgtggtgcacatcacgcaggcgctgtgtcctgcctgctccgtgcccccgcggctggtcagcgccgtcacctggctgggctacgtcaacagcgccctcaaccccgtcatctacactgtcttcaacgccgagttccgcaacgtcttccgcaaggccctgcgtgcctgctgctgagccgggcacccccggacgccccccggcctgatggccaggcctcagggaccaaggagatggggagggcgcttttgtacgttaattaaacaaattccttcccaaactcagctgtgaaggctcctgggggctgatggggagtggggaagaggggtttctgcctcagtggccccaggccccccagccagttaacctctttctccccgccaaggaagcccacagagcagaccccaccaagccggccgcctgctcagggtgaggggggaaggggcccccgagagccactcagttccgcagcgctggggcccagcttcccctctctgcaggggagaggaagcagcacccagcagggcaaggtgtctcctggggaagcccagttccgatgggaagaaacaaatggggagaggcggggtggggggctgtcagccgccaggccctgcccgggccaactcccacctctgagaaccaggcacagggggctccaggctcatgctgccccagcagaccccggcaggggagcccaacctgtcattttagaagctgccttgaggccagagcctagcttcctgccagtccctggccagaggatgccccaagccccacagcaaggggcctgtggtgatgggtggggccccaccaagtggcttccctggagggagctccgtgctcagtcacccctggtgcccagccaacctctgcccagcgtccaccaatgtggctgggccaaggggtgggagcagggaggcggcagcggggccaggggctgggcagagcgacccaagctgcctgtctgcaccctggctccatcaaccagtgcagcccctgaccctgggggaagaggggcggctcccagggccctccatgcaggaacagcctaccctggactggatccagctctctcccaggcccaggttgtgggagaaatgggggaccctccgcctcccaatcgtgctggctggaactttcctgtgctggggattcggcgtttgcagccagggtggccagtcagggtgccaggctcccatctgaacactgacagactgtgggctgtgcagtctacagcattgggcacaacctcagcttgctaaaatactcagtgcaggctgggtgtggtggtcacgcctgtaatcccagctactcgggaggctgaggcaggaggatcccttaaagctagggagtcaaagctgcagtgagccgagatcgtgccactgcactccggcctgggtgacggagaccctgtctcaaaaaagaaaagaaaacgagtattgggtggagagaggaccaagcccaattactactttagtgcggctgccccgtcccgtctggtgaccacgcacttctgtgatggcctcagcggctgcctcctccaggacaccttctccgactacctgcttcccaggaccagcctgtcccagtcacccccggaacagactgagtcacagtggattcctctcagacacccgtgagagtgaaggaggggctcccgccagctttgtcc

SEQ ID NO: 117 - DNA, 8064 bp, Artificial Sequence
  subsequence of TBX15
agggcttttcctatctcatttcactagcagttgagctgacgggtgcgtgcgagaatgcgagacctgccacgtgtacacgtgtacgcggagtgtcgatctgcctgcgtgtccttggatgtgcctgtctaggtgcccacccgcgcgcgccaccacatccccaggcctctggaacgcagctgctgtgtggcccggcccgaagtttctggaggaggaaatccctccacagaaggtttacattatttcgctccgcgggagacccggcttcggcagcacttagcagaagattttggcgggaaaggcccaagccctagctgaggactccgggtggagcaggggctgaggtccgagcgcagatggcgccgccgagcgcctgaaatatacttgcaaggccgcagcaatatacttgcaaggccgcagccggagcagctgttccagccgatcctagctcgaaagttcctctgttgctctgggagagggcgggggagagcaggctcgagagccaggctcctccgaggctggtcttgaggcacttctctagtagcttctccaaaagactgagagtgccggcgtaggtatgacagtgagggtacctcacagacccttctccaaagtctggcgggccttggggtttttcggggccaccaggctcggtggaatttttgaaacgctttcgaaatacatagtttcctctgtggagtgagtgcctacaacgcgcaggccggactgatcccccgttgctgcaggttggtgccccaagctgcgggtgctcgggcgccaactaaagccagctctgtccagacgcggaaagaaaaatgggctgtgaaaaagcaaaaggcctcgtctttgaatgaaagttaaacattaaaatctgaccctagagttgtctaaagatcgcggaattttgaagctccggcagagcggactaaaaaacggtgctatgagagatggtgagaatactctaggcatgaacgtgtgcgtgtgtgtttgtgtgtgtgtgtgtgtttcattcttcccgcaaaacaattttttgtttttttcctattcccggtttgttatcggcctagggcgggagaaccacgcagcggcttctgggccctaaggacaaaagagttaaaacaatgaggctcacccgggaagagacgctgccctgggcacaatagggtcgcctgcattactcctccatacacacatctttaaatgtgtccctgtgtgtgttcgttagggtgctgtattacagaaaaagaaaggcctaaaaacacccccagccctggtcgcgcctttcgctaccgcctgagtctggagccgacagctccacctcttctgctccctggaccgccgcgtctccacgccacggcgccctttttactaaaagatcttttctcatcctatcagcaaatcgttaagaaaggcttagccattgcgggggctccaacttaaggattcccccggcccactaaaaggctaggcccggcctgtagcccagctccgcagaaagccagagggtgctgggctttcagcttcttcctcctagacacttgccccacaaatatatttcgttttctctaatccaaatacccatctttttcttttttaaaaaatgataacgtaatgggaaatgaccaaccgaactctgttacataaagttagttctgttagatcttccaccccacccccatcccgcgggagcgagtaaatagaattcatgagcttagctccccaggttcacgctctggaatggtttctttttgcctcattccctaagttttctctcttctgcctcctgaatggagctcaggctaaggagaacggcagaaagagcaaactctgatctgaatctctaattatgaccccatgtattacccatttgaacataaggccctagacgggctccgtgcgatctggggcctcccaagagaaaacttccccgggacaggacgtctgccacgcgcagctaaacaacttctgttttttccgccgtggggaaaataaaagaaccttacaaattctaaggcgtcataacccctgcaagaacttctaactgtatgaaggcccacgcgagattttgacaatagataaatgagctgaggaaatagggtctggccagcgaagggaaacacacagtagccctgggtgcctttctggaatgcccacgcaggggtccgcgtggacaagcacttgcattcaaatacaggaaaaggcttggacggtcgaaataaatctccttttaattttcttttcatcgactaataaaaataattccccagcactaaactcaaataccgtaacgggccacaaaaacacggagaattcataaaactctatctctgcaggtcacccgctaatcgcattattattagcctcgggagcatggaaattgaactgtcactgcctaaagagaaaatgtaagcgacagctgtccctcctctgagttggacagctttgtggctgagatccccaagctcctgagccccagaccgtctctatcccagtgcaggccgctgccccctccccgggcttgtcagcgtgtgaagcggggtctactccccagctctggctgttcagcaggagcaccttccagcatggttttagaagtccgggctggaaagcttctgaaaccgctaaaccaagttgcgagcgttgtatgtgcgcgcgcgcacactcaagattcttccgacaacagctgttcccccgggctgtttttgcacagttgaaatcttggcacttaacacaaaacgttaaagttggcttctcccctcctagggttctgttaaaatacagacatgacatcccccctgctttttacatgttccgtgcacataatatacatgggttactgtaggatctgagacacaaatcaatcgtacccacaccctaaatacacagagatgtgggccctgaagagtgacccaaggagtaaggggtctaacatccattcttgtttccgtaaacgccaaaggagtagaaatataattatgttccaccatcgaaaagttggtgggagaaaggcaaggacgaggttgaaggctaaatgagacaactggtcattccccgaagactgaggtattggattggagaacgccgcgccagtcctcccgagttctcagaagcgagtcctagatctcggctcccgccgttgccttcggcccgcgcccctcccaatcccagggaccggcagcccttcatccacggacacccagaaagctgcgctctccacccaaaagaaaaagaaatgcaaacaaacaggactccttgcttaggctggcgacgaaaatgcaaggctcagtccagccccaaaaattggttccggtgaatttagggaggctcagggcatttgcgcgaagaaacagaaacctatgttggggcaaggcagggcgtcaatggcagggcctagctcctcacccgcgaccggcgactggcccttcggcgtcccctctccgcccgcctcccgcggtcggctgcgacgcactcacccgggtgaggctccaggccgtgtgccgccgcgtcctccgtgtctccgagtgggcccgcggggctcagcgcctccatagacaggtccagccccttctcctcccagtctcgcagtttccgttttttatttgagccgatcaaggcttcaacggagaaggcatgtgctcgcgagctcagggcgactgcagatcttctcctttcactcattttagccgcccacacccctgcctccgcttgcccccgctaccgagggagcagccggcgccctcaagctctgagcgcccaccgggcccggcccgggagaggcggaggcgcgtcggacgaggctgagactgcggctcgcgggtctctccaccctccccctgcgtcctcctccgccctcctctgccggatccgacctgcgcccctacgctggcccagctgctaggaactagcgccccgagcgccgcccgctcgctgcatgagcgcccgagtcctgcttcccacccaccggggcaggcgctcacagactgtgtccactgaacttcatcttgtttttgttattattattattctctctcctctctctctctctctctctctcccctccctctctttttctctcctccccctctctctctcttcctctctgccttcccgtcctccctgtgatccaaacttctgggaaacttttttttccgctaaattcctcccttcccgaggaacagggggcaggcggtgcgctcctgtccgaggggtgagggagagggagggggaggaagaaaaagactgagggggaaaaaagccagcccccaaccaatagcgaggagggaacaagagaaactccgagagcgcgaaccaatgagaggaagggagagactgaggcccgggccaaagcgcagcgccagtcgtcccctggatgctcctgggccgactttaacccctggcttcccggtttccccatgggttactccaagagggaggtaggacagttgaaagttgaggtctgatctgcgcctttacaaactcctgcaaatcccaaatccatacgtttttcttccagatctgctggtctcatagacgctgcaagtccagagtcactttagttgcagatctggaattttggggctctgacaaaatgttaacctgtccaaaatgccagaaaacgattctgataatttcgcgtcagcccctaggtgctttagaatattctggttcctcctggatttcgccacacaggttttaatgttcctactgaacgttttctaagcaaatctgggtaaggcaaaaggaaacaaacaaacaagcaaacagaaagccctgttactaaccagggtcttgtaactgaaaattcaaagaccgcttcctccttccagctctacctggtggagaaggagacacaggcgccttgagagcaaggggcgggcggcggagcgcggggtttagggcgagctcctcaggcgtattccagctgggccccctcacgccgcaaatactctctttccctacggcccgaacgctgggctgcgcttcgcctgttccgggctcttgttgcagagaacctatggagaggtgacaggcaagaacagctaggaactttaacagaagagaaggagctttttcaaaattccctgcaaatcccgttacctcaagaccatggctttcccggccagctgatctcccccctggccgccccctgccttttgcgatctctaaggactgcattcaacatggatttctaaggaattaaaaaatccaacgctcctggccattcttaattcccacacctcttcccaagttacgccaccggtcgaggacggcaggagacccccgagtgcagagaaagctcaaaccggcagcgaagtcggtcctagccaagctgaaaaaacgtctcggatttcgcggacagcggcctagacacagcccgatcttccagtcctagtgccctggtcgagacggttctatccttttgcaaagaagccggaaagagctgggtcccgggggcgggggacagactgagaggccaagcaggccagtcgtgacgacagccaggcccttagaagtctccaaacctgaaagtttaggttagggggcccacagcctgttaagatttcttgttgttgttttcgcgaggcccgggagaatcagctctcccaccttgcggcaagaaaagatgacttgtcaggcctctgaaacgccgaattctctgccggactgcggaggggcccagggaaatctagtctttattattacagttggaagtgttctggtgctgaaggcaaccacagtgttgtgaattcaccttgggcctctttggacaagaggctacttttgcccccttccttcacccccgccccaaattaggatccaaccaggatgtcaggaagctagcatcccaggcgaatgcaaaaagaacaatggaaaagccaccggatgagtgtgattcagccaagcctgacctccccggagcctgtgtctcaggcttggaggtccccagggagcacgaacatgaactctggggagctggaagcagggtactggtccccgcctcctgcagctctgcccagaggacttggggagcccggatggagaggcgcaggatctcccacttcagtcagcatttggcgttgcttccaggagtcgtcgctgaaagtcagcgcgcattcactgctaccgggcttcagcagagaagctggagacaaggcagacgggaacccgcaatttccttccccagcggctggggcctctctctcacctcccaactctggtgtcgcccggcgttttccgcctgcggctggagcctgcccctaccaagcttggtggggtagcaatggggccggcctctagactttcccagctcttttctcatccccatagccggtatctcccatctctctctggcagccttttgcctttcacagtttctcacaggcctggtttggactgagaagcgggtacaccatatgcctcaccctctctgagaccatggaattttctcaaaaaggaggacttagcctgggcaacatggagaaaccccatttctacaaaaaatacaaaaattagccaggtgtggtggtgtgggcctgtagtcccagctactcaggaggctgacaggggaggatcacctgagcccaggaggtccaggctgaagtgagccgagattgcaccactacactccagactcggtgacagagtgagaacctgtcttctcaaaaatagaaaaaaaggaaaaaaaaaaaaaaaaggaggactttttggttatctaggaacataattgcaagtccagaggcccgattgttcctgtgtgtccaaagacgcagcatctgagaggcatacatagaggaatgagcaatggtttcaacagcatgcatctgcatcctctccgaagcttgcactccgcagagtcaggagtcagccagaagagtttccacacccctccttcagattgcacataggctgctcccacccccattccacagacacacatatcctggaattgtaggttaggccactaaaaccaaccgaacccaaatgaaagcaggatggtttttaacagtcttgaaaataaggggtttcctctaagtaaatgggaggagcagtgaaaactcccgtgactctataggagttaatgtaaggtttttcccagaagcatgcactccttggtgggtgactgctgatgggaaggaaaatctggagaaagagtaagcaggatggcttaatatgtgtgcttaggtgtacactcgtgtgcagttgagggaggctttgggagattacatgtaagaatctgcaagtgtgatacaaattttccttctactgattacatcaacgggctttaaaagtctctcctcattaccccagcttatctctcttttaacctttatgggtaagggtggggtccgcagtttatgaggctaattccctaggcactacctaggtttccctgctacaggcttcaacttttcgccctgagtgcatcctacaggcgatccaccctgaaatgactccatttcagggctgtttttggcctgaaactgattgacaaagaccaagcaagatgtctgcctcccacttaccccctgcaggtcccccaaaaggaagcgaaggttattggatacctgggaagtctgaggagccctggggtttcacaggctacctgcaggggcttacagaggggtggaggtccaggcctagtcttggaaggggaaaaattagaaagagaaaggcaatacagtaactgttcacctacaactgaccaggtccagatattttgatttttcaaaggaagagcagagtcatgcgacaacagatcagagtcataaacacaaataggcattccaagaaacggagcgcccacatcctccacatacctgtcttttcctcccattaccccacactgaatagcaccttaaataacaccactgctaatgcctcaataccaaggtgaaccaccagccggctttgatttcagagttttgagtgagtaattgaaaacaaagttaaaaatagttggccagccggacatattaggctgcccttaaacacgtgggtaaggcaccctgtgggggtgagagaattacaatgaattcgcccatcaaggtaggtataaaacattatgag

SEQ ID NO: 118 - DNA, 5519 bp, Artificial Sequence
  subsequence of TRH
tcaaatcctggagtctagttgggagaccaagcctgaggtttcatgtttgcagtgtctccctcactgcctctgaactttttgagggctggggctgagcctcattcacttctaggccttcaggacctaccaaggagtctgacaccatagtgggtgcttgttaaatgtttagagatgggccgggtgtggcggctcatgcctgtaatcccaggactttgggaggccaaggaggaggattgctagagtctaggagttcgagaccagcctgggcagcataagaagactccatctctacaagaaataataataaaaaatagccataaaaattatggtgcctggctgtagtcccagctacttcggaggctgaggtgggaggatcccttgaactggggaggtcaaggctacagtgaggtcagattgcaccactgcactccagcctgggtgacagaatgagaccctgttttaaaaaaaaagtttcaagatggaggcagtccccagggctagatgtggcagtcccacatctgggactttgggaactgactcggggggcaagctccttggcacccatgtgtttctcctccctgcttcccctcccctcctttgctagagttgggtgaactccaatagattcctgtgcaggggctgcagactcgaatgtccctcctcagtgacaggggcaacacattggaagacattagggagtggtggagactgtggtggccgagagcagccaggctcagctccacctggctgttgacaggaggaaatgggggcccattctttttcaagagaagccataaatccaaaattttctaagttatcttggttttaaaatgttggttattcagatttttttcaaaacactgtggaagtcaatcaaaattgtccatgaactggttgtagcctacaggccgccacttttggaattctgaaagctttcctctggctcctattacacagaggagaaaactgaggcccagagaaacggaggcactagccaggaatgacacagttaagattagcaccctggagcctgcggggtggctcacgcctgtaatcccagagacgcaggagtctgaggcaggaggatgacttgagcccaggagttcaaggctgcagtgagccgtgatcgcgccaccgcactccagtctgggggacaaagcgagatcccatctctttaaaaaaaaaaaaaaaaaaagtagagctccgctcccacttgccccccattctctctctctctctctttctctctctctctctcttgctctactctcgcccgtctgcgttctacattggttctgcggccgtgtccctttcgtgtgtgtctgccctgtgtttctccgtcgtctccgtgtggatctcggtctttgtctcgccctctagctctctcgtgcgcctgtgtttaatcgtgcgcttctctcaatctctctgtccctccctttgccccctacacgcgtgttctcgtcaacagatctccagaggtggtgcagaaacgaccccgcgccggcgccccatcctgcggccagtgcctccgcgccccggctccggtccccaccgtccccgccccagatttccggaggagcaggcgggcggggtcccgcggggccggctgccgtcagcgccccttcccggcggccgcgacccctccccgctgacctcactcgagccgccgcctggcgcagatataagcggcggcccatctgaagagggctcggcaggcgcccggggtcctcagcgctgcagactcctgacctgccgactgcggatcccgagtccccggatcccggacccatcctgtggagcccactcctggcaggtaaccgccccaacccctctccttccgcagacggtgtccgggagcactggaaagggagccctctcggcccgccctcaccttcggttctctgagagcttcctggagaacagggccggtgcacaggcgggcgctgtgctcgcacccccgggtcctccccgagcgcaggccggggacccgacgggaggcacggcgcgggcacatcggaggctctcgctgctgggcactcaggtcgccagagtccgcagcgcggggtgggagctccgcggcaccccctgcctgggtgccgccggacagagctgggtattcagggcgtcggcctgagaacctgggagttcgaatcccaatctcaacgctagaaatagaattttagcgttgaagttaggattttagcgttagaatcagattcctggcttagtcatgaaagcttagcattagaaatagaatcttagctttgcaaatagactttgagctttagaacctgaatcttagcgatagaaatgggatcttcgcgttggaatgaggacgtcggccacggagcttggagttagaacgtggcgatggggacctttgggggagtcttggcggggacgcaaccgttagcgtcgcggctgtgcctggcgctgcaatctcaatggttgcactcccggcgaggcagtcccagcgttggcttccccagttccgcgtcacattgaagggtggcggtggcgctggcgatggggttcctacggcctcctgccttgcgcaagcagaactgggcgcaggcactacaggcacccgtgggggcgaggacgcctagaggtgacaggtgtggacgcagagccggggcgaacccgccgctgctcccgcccctgcacgaggggcagtggtcctgcttctgggagggcggttgaactgtgcgtggtttgtttctggcgggcgtcgggggagatggagcgggatgtgctgtgattcggtgcgctcaggctccctctgtcccctaacccagacgccgcgatgcccggcccttggttgctgctcgctctggctttgaccctgaacctgaccggtgtccccggcggccgtgctcagccagaggcggcccagcaggaggcagtgacggccgcggagcatccgggcctggatgacttcctgcgccaggtggagcgcctcctcttcctccgggaaaacatccagcggctgcaaggggaccagggtgagcactccggtgagtggatggggctgttgggggctgtggggctaggctattgggagagccgtggaaacctgccggcaaaggggaggggaggcttggtcagctagccttctgcctttcggaagctcagaaaccctccctggctgcgcctaggcgggatctggagttgaccattcctcggggtcagattcctcccctgtctcaatgctgggaatatttcacagagagcaggccctgggtggggaagcttctgtgtgctagggagagagtttctttgtgtgtgacagtttgaattactactgtctaggcacttctgtgccagacactattccaagcacttcaaacaccttatcacactgtttgatcttcctaacaacctcttagttaggtactgttattacgattttacacagaagaaaactgaggctcccagagatcaattgagtcgcttatggtcagacaactagggagcgccagagctgggattggaacccagaggcaatgcctttgactattgtgtgaatgtgtgtatctgtgaggcctgaggggcaggtgcaagaccatgcctctgagtgggagctgcaggaaatgtaccctgcctgggagaaaagcaggagtgggcactcaggcgcctgcctattacatgggtcaggggcccctcactgacctctttccttccccagcgtcccagatctttcaatctgactggctctccaaacgtcagcatccaggcaaaagagaggaggaggaggaagagggagttgaagaagaggaagaggaagaagggggggctgtgggaccccacaaacggcagcaccctggccgacgagaagatgaggcttcatggtcagtcgatgtaacccagcacaagcggcagcatcctggccggcgctccccctggcttgcatatgctgtcccgaagcggcagcacccaggcagaaggctggcagatcccaaggctcaaaggagctgggaagaagaggaggaggaggaagagagagaggaagacctgatgcctgaaaaacgccagcatccgggcaagagggccctgggaggcccctgtgggccccagggagcctatggtcaagcgggccttctgctggggctcctggatgacctgagtaggagccagggagctgaggaaaagcggcagcaccctggtcggcgggcagcctgggtcagagagcccctggaggagtgaacccagttttccctgaagtcgagtttgtggtctaaggatgtcttgagccctgtgtgccccaccattcatgacctctgtattctctagttagatccctgaccataagcctgagcccctccctcccagccccatattcacacacatcccagcccctggccttgccctcttcctttaggcatgtgagaaaatcagcctagcagtttaaaccccactttcctccacttagcaccataggcaagggggcagatcccagagcccctctcaccccccccaccacaggcctgctccttccttagccttggctaagatggtccttctgtgtcttgcaaagactccccaagtgggacagggagcccctgggagggcagccagtgagggtggggtgggactgaagcgttgtgtgcaaatccagcttccatcccctccccaacctggcaggattctccatgtgtaaacttcacccccaggacccaggatcttctcctttctgggcatccctttgtgggtgggcagagccctgacccacagctgtgttactgcttggagaagcatatgtaggggcataccctgtggtgttgtgctgtgtctggctgtgggataaatgtgtgtgggaatattgaaacatcgcctaggaattgtggtttgtatataaccctctaagcccctatcccttgtcgatgacagtcatcctaatgataataaaacctgcatccagataatcacggagctctgtggttgctgttctgtcgcagctggcatgggattcttctttcgcattgagagggatatttaaaaggggatgggactagagttctcagctctgctgcagagggaatcagggaccctgggaggatgacaagtcctctctactgtccccatttcagaacacacttgggaggtggatggggttctggagcccatttgactcctggggagactaaggcctggagagaaggaagggcttgcccaaagacacacagctggctgaggtggagccatgggtctgagaggccagctcagggatttgccttgagtttgcctgatttgggaggcgggggtggtggtgagaggggaggtttgaggggaggactagtctggctcaggtctgtaatcttcatggttctgttgacagcttgtgtcaccaaacagcctgttaatgaacaggaacaaggagggcagaggaccaggctgcagtcaggagacacaaaccaggggtcttctggggctcggtgcaggacaggagggagtggtgtgaactagagttaactgaagaagtcatgtgaagacatttgaattcaaaaactttaagaaat

SEQ ID NO: 119 - DNA, 10262 bp, Artificial Sequence
  subsequence of FBP1
caagatcacctcagtgtccagcatctagtcctgtcagctaccccaacaaccaggcatgcacaccagttccaagggtacagcactgtaatacccaaaggctagtaaaaaccaaagtgccccaaaatagagaaaaacttcaatacctcatgatgtgtgcaggggagcagcacacagcagttaaaaggaggtagatgtagatgtcccgatattaatggatgtttcttgaataatgttaaataacaaagcaaactacagaaatgtgtattgtgatcccattttgtctgctattataggcatatgtaaatatgtgttcatgtgtaaacttatatgactgtaaaagagtatccggaaaaataagcagtaaattatttgcagtggataccccatgggatatatatggggtgggtttcactcttcccttgaattcttttgaatggtttaaatttttgtcaatgagtgcaacatagtatttctttaaaacctggtattcacaactatctagtataaaagtacacatattggccaggcacagtggctcatacctgtaatcccagcattttgggaggccaaggtgggcagatcgcttgagcccaggaatttgagaccagcctgggcaacataacaaaaccccatctctacaaaaacacaaaaattatccggcatggtggcacatgcctgtagtcccagctacaggggaggctgaggtgggagcaccaattcagcctgggaggttgaggctgcagtgagccattatcacaccactgcactccagcctgggcaacagagtgcgactctatctcaaaataaataaataaataaaacgcataccttacgtagccaaaattaacatgcttcatccaggccccaccatcaaaatctcactatccaaggtcccactgtctaaggttacttagacagtgggacacctcaaaacacatcttacatttctcagtctctctaggggtgtgaaaggtactgacacattttttaaacaatatcagacatgacaagcccttttttttctttttttgagacagagtcttactcggtcgccaggctggagtagagtggcacgatctgggctcactgcaacctccgcctcccgggttcaagcaattctcctgcctcagcctcccaagtagctgggattacaggcgcctgccaccatgcctggctaatttttgtgtttttagtagagacagggtttcaccatgttggccaggctggtctcaaacacctggactttgagtgatctacccgtctcagcctcccaaagtgctgggattacaggtgtgagccaccacacccagtcgacaagccctctttttaaaatatatccctggtcctcaaaggcagttaaagctgtgagccacctatactagctgtaaattaaagcttaagatttcacctgggtatgtttctaaaataagaatccttaggaatgtattattaagaggggccagaggcaacagtaatggagtcatcaccttccttaacatgtctgcttaatattcaaaaataaatgtgatcataccactcctttacatgaattacctccaccagtccatactgtgggaccaaagccagacagcctgccagtaagaaaaggaatctagattgcaggatgcggggcggagaagagtttttaagaatggagaaatgcattccaaacccaagtagcagggttgtatttgttcaggtcagctctgagcatcatgcgtcttttttttttttttttaagacaaagtcacgctcttgtcgcgcaggctggagtgcaatgatgcgatctcggctcactgcaacctctgcctcctgggttcaagcaattctccttcctcagcctcccgagtagctgggattacaggcgcctgccaccacacccagctaatttttggtagagacggggtttcaccatgttgatcaggttggtcttgaactcctgacctcaggcaatccacctgtttcggcctcccaaagtgctgggatgacaggctagagcctacgcgcccagcccatcatgtgtcatttttatagtgtgcataagtgcggggaatgttagtaaagtgtatggacaatctgaaaacccagttacacttcagttaaaagtgtggatcagttagctagaaaatacctgcgcacggcggctcatgcctgtaatcccagcactttgggaggccaaggcatcaccggaggtcgggagttcgagaccagcctgaccaacatggagaaaccccgtttctactaaaaaaaattacaaaattagctgggcatggtggcacatgcctgtaatcccagctactcgggagactgaggcaggagaatcgcttgaacctgggaggcagaggttgcggtgagccaagatcgcaccattgcactccagcctgggcaacaagagcaaaattccatctcaaaaaaaaaaaaaaaaagaaaagaaaaagaaaatacctgtgcacaccaacacaaacgaaaggatgttgtgtgacttacaaaaaacctcacaagaaggggtcctttgagtctccactccacttgaccccttgctactcacaatgtgatgagtagacaaacagtatctgatgggcagcacccaccacaggagaacttcttagaaatgcagaatctcaggacctgtcccagagctatggaaggagggcacacatcttaccaagatccccaaatgattcctgtgcccagtgacgttcgagatgcactccatagcgcattcagaaccattctacaaaccacttttgagctttccactaattgggcagaggctgcacacaccatcattgcaaatcgataggggttttgaagccctgggtgtttcctgtttctggcacagcatggcaactgtcccagcaaggggcagcccacgggagctcctttgcacacaagccctgctgctcctaaaggctctggacacacaggagacctcccagcctgcttgcggggggggcgggggggacactcgctcctaacaggtcttgtttcaggtcagagataactggattagaaacctgacttgggtccctaattgcagaaagagtgaaggaggacaaagaagaaatggggaaggaaggcacctgagctagcactttcctgtctgaggctagggcgggtatgacgggcaggccaggtgcccacacttggccggctgagaggggtacgaggcaggctgctcagggcagagaagaggaatgcaagatggaatcaggtgtacacctgtgagacggacccccaggtgggcccctccaaggtcaagggaggagatgaggacttgagtgaggctgagccagcttctggagagaggggctaccagacagagagcgagagaggcgctcagacatcagacggacagacagaggctgacggcaggaggctcagagggcccaacgtcagcccgccgggcaggctccccaggcagacagacaggacggggcccaccgcccaaggcccgactcacaggtgcgcgatgcccgccttgcgcaccgccgaagagatggctttgactgctgtgcagagcgagttgagcagctgggtcaactcgcccgtgccgcgggccttcctgccctcctccatgacgaagcgggtcagggtgttgacgtccgtgtcgaagggcgcctggtcagccatgcttgaaccgggtagagcgcggggctgcaggtgcaagcggcaggtgcggggctgcaggtgcgggcggcaagagagggcagtaggcactggccgcaggtgcggagctgcaggtgcgggcggcaggtgcgggccgcgggacctggcgggaggactgacagaccgactgccgccccgagtgtccgcagcgctcgtggtgcaactgggccaggccaggcgccggcgggtgaatcgcggaaacctttagacgcgggtcggccccccgcccccgggaacactcttgcgccccgcctaccccgcggaccagaccgcggctccgcctgcttggatcttcagacaaggtcggggatcctccctgcggtctcccaacccccgcccccacgcgccctgccgccccctagtcttcctgggctgtcgccccccacacacacccctccgtgccctccacccgcactgtggagcgggactcgggccatcggactctgccagagagaaagctatgactgtttcctccaaaatcataaaacggaagttcagaaaggttaagtaacttgctcaatgccaccagctaggcagcgaaacccgcagccagtccacatggcctggctttagctctgcagctcctgccccgtgtggctgcctgcccccgccccctgcccaagccccgtccactctgcctggcctgtcacctggcccttctgtccccgctaggagacacagagtccccgtttctcacccatctgagggcccacgtctgaatccttaatccaggcctcttctcaagattcctagaattcgagagctattgagtatttgaatttccaagatgtgagtctcgcccggaagtttcccggaaaacggtcgctgacacagagtcctcggctaccacacaaaggccagagggctccaccgcccgcatcctgaccccctggtagccacaatgctgcaattgatgtgctgattcacgaaacaacacctattgagcacctgctgtgctgaacactgtcctaccttccaggggtggagcctgatccaaacagacaaaactcctgcccttttcgagtgtacgttttcacagagaaacagtaaaaataaatatataaacaatagattagtttgttacataagccataagtaccatagagagaaacgaaatagaaaaggaagacacggaatgtggaggggagaagagggtgagcagaggcctcagtaaaagcttctctgagaaagggatatgtgagcaaagaggtgaaggatgcaacgcgccggtggagatgggaaggagagcggtttcctcaccgggagagccagtgcacaggccctggggtaggagaccatgtttcaggttcagggaatggccaggagaccggtggagctgaaatagagctagcaagggtcagaggtggaggagataaggccagcgggaggatgcagaggtgaggtctagagggccaagtgaggtttgactttgactaggaggaacccactggagagtttggagaagaagagaggcatggtctaccctgtgtcttcatactgcggctactgtgtgaagatcagactgaagacagtgccctccaggttactaggagatagtgagccaggtgttagcagtggaggtggtggattctggacatattttgaaggtagagctgatgggattcgttgacagatgagatatgtgagagacaggagtctcggatgattctaaggtttgaggcctgagaaactagaagaatgcagttgtcctcgactgcgatggggaacaccgagaggggcgtgtgctggaggcaggactgacaattaggagctaagtgtgggacctgctaagtttgaaatgccttctagacatccaaggcaatgtcaaatagacagatttatgtatctggagttcagaggagagatccatgctgcaggtataaattggaaaagccaactggaaaaaccaaccaaaaaccaagagatgtgacatccgggaagccagatgaagaaggtaagtaaaggcgggctgacccatgtgccaagcggtgtggatggggcaggcaggacaagctctgaaaattgactgctggattcaccgtggagacctggggtgcagattcctgtgcccagggttgtcagatgcggcggcgttgaatgaaggaaggtggtggtaccaccaggaaagacagcgactgtctcctcaaagccccagaggggacttagatgcctggcaaagagagttgatcctttaagggtcttatttaactctttgttcctcaggcaacttttcaggaaaaaccctgtgttaaaaaaaatagtaagagaaatacatccttaaacataaaaactcaaataggcccggctcactggctcacacctgtaatcccagcacttcactttgggaggccgaggcgggcagatcacctgaggttgggagctcgagaccagcctgaccaacatggagaaaccccgtctctactaaaagtacaaaaattagctgggcatggtggtgcatgcctgtaattccagctactcaggaggctgaggcaggagaatcgcttgaacctgggaggcggagattgcagtgagcagagatggcaccattgcagtccagcctgggcatcaagaacaaaactccatctcaaaaaaaaaaaaaaaaaagaaaaacaaacaaactggaggctgaggcgggcagatcttgaggtcaggagttcaagaccagcctggccaacatggtgaaacccatctctactaaaataaaaaattagccgggcatggtggtgtgcacctgtaattccagctactcaggaggctgaggcaggagaatcgcttgaacccgggagacagaagttgcagtgagtcaagatcctgccgctgcactccagcctgggcaacagagcgagattcaatctcaaaaaaaaaaaaaagaactgaaatgtgatgactagtatttttggcatagtaactagttactaggggagagctagagctagtaactaggggagtgtgcccctttacttgccagactctcagtccctcaggatcttggattggctaggaccgtaaaagtcatctagtccagccaaccctcattggacaccatccctgataagaggtgaagagcttgggatctgcattaagcaaacttgtttgagtcccagctccagccctcagcagccagagatctcggaccagttacctaatctctgtaaacccagtttgttcatccatatagtggaataatggttccatctggcagtggtgtcatcgggctgaaatgagatggcattggcagagtgcttagctcagagctacacacaggggacacactgaatacgtggaggagacccctgtctagctcagtcacttctgcttgtcacccacgatgatgggcagctcattgcctacaaggcaagccattccccttgggactaggccacgtcgcattgtggtgaagtgcacagactctggggctgcatggcttgggtccaaaccctggcctggccacttactggctgtgcaagcctgtgcaattggctaaacctcaccaagcaaccattggctcatctgtaaactggggctaatgattgtagccacctcatagggttgctgggagaattatacaggcagtgctggtagtgtttaagaacagtgcccagcatgtagtaagtacacagtatgtaagtgtttgcttcgttacatgggtagggccaactgttgttttcatgtgaacagaagcaagaaagttccctggccatcaaaaggggctagagggatgtgggaattggcagctgagcctgtatttgcctggtgtgcagtgatatcccctccatcatattggtcgattgtgactcgctcttttctgggtcaagatgcataaagcccatcacccaggtattagcaagagacagaggaaggcggccacctcacatgggttcctggcctgtgggttgggcccctccctcctccacccaccaccctcgcagagttgcttcttgccacatactccaacttcacatgggattgcagattcaagtgatgtgagcagtattaccacatgtgtaacactcgaaatcctgcgaagaatcagtgctcatgcatttcctcacccagctcccacgatggggttatgttggaggcgggcagtggagaagtaacagtgtggacagtccctgcccctacaacagccgccctcaacccagggctccactgcttactttcccctctgtgggggcggttagtgccacaggaaagaaaaacaggccaggcacagtgcacacacctgtaatcccaatgctctgggttgccgaggcagacagaccacttgagcccaggaattttaaaagcggcctggacaacataaggaaaacactgtctctaaaaaaatttaaaaattacccaggagtggtggcgcatgcctgtagtctcagctactggagaggctgaaggaggaggatcacttgagcccaagaggtcgaggctgcggtgagccgtgatcacagcactgcactccagcctaggcaatagagtgagagtgtgtctctaacaaaaacacaaaaagaaaaacaaaagccaagtggtgtatgtgagagggattgcagtagcatggtccttccttaaacacctcccccagctcctgtggccccgggggcctggtgtggaaactaaacagcaaacatctatttagcacttgctaagggtgtggcacttgcccagggcttcagaagcagcctttaatcaatccagaaccactctggggtggcttctaatcaaacccctgtctttacagatgaagggactgaggcttttctttcttttccttttcttttcttttcttttttttttttttgagatagagtctcactctgtcgtccaggctggagtgcagtggcatgatctcggctcactgcaagctccgcctcccaggttcacaccattctcctgcctcagcctcctgagtagctgggactacaggcccccgccacttcgcccagctaattttttgtatttttagtagagatggggtttcactgtgttagccaggatggtctcaatctcctgacctcgtgatccacccacctcagcctcccaaagtgctgagattacaggcgtgagccactgtgcttggcccaatttttgtatttttagtagagatgggatttcaccatgttggtcaggctggtctcaaactcccaacctcaggtaatctgcccgcctcggcctcccaaagggctggaattacagatgtgagccaccacgcccggccaacaaggtcaaataacctgtccaaggcctgcagccaggcaggaagtgacagaacaaagactcaaaccctcatctgtctgattccaaaccccatattcccactgacttgctggttctttcctaagtggcagtttccctccacgtcatgcctccagggacaggcaaggctctgagcccgcctacggcagctctctggactctagagctatttctgggctcatgttcattcattctttcactcaacacatagtttttgaacacctgctgtatgccaaaaccataccacaccctgaggttgcagtggtgaacaggacagacacagctcagtccactttaggtttatattctttgtgggggagataagaaaaaaaatcatttaaccaacaaagacacaaaactgtttcagggagcagagtgctatgaagactgtaaagcaggatgaggtaaaaactcaaagcctttcttatgaaatgacttttgatcagagactgaacaacagaaaggaatggggcaaatgaagagctcatagaggaacatacagaagaacaagcaaggctacggcaggtgcaaagaccctggtgcattcaaggatcagctgggagaaggccagtgtggcctgaagggcaagtgagggaagaaccacaggagataaagttggaaagagagacgagggcagattatgaaaggcctcacagcaagtcgctcaggttctattcatgcagccagaagacaggggaggccaggtgcagtggctcacgcctgtaatcccagcactttgggaggccgaggcaggcggatcacgaggtcaggagattgagactatcctggctaacgtggtgaaaccccgtctctactaaaaatacaaaaaaattagcctggcgtggtggcgggcacctgtagtcccagctacttgggaagctgaggcaggagaatggcatgaatccgggaggcggagcttgcagtgagctgagatcgcgccactgcactccagcctgggtgacagagcgagactctgtctcaagaaaaaaagaagatgggagggttttaagctggggagcgacatgacttactaaacggtgtgagaatggaccgtaggtggtcaagagcagaagccaggagacccagcagaaggagtctgacctaacctctacttgatttacagtcaaatatgtgaagcccgctgtcatattccccatacatctttacttctccagttaaatattttcagctcctccagctgctcctcaggtggcaagattttgaagttcttcccttcctgttctggacctggtggccccttgaggctccttataaccccatgctctatttccacgattccacccatctgctccacctcatgttccaggggtcctctctcctaggaa

SEQ ID NO: 120 - DNA, 8338 bp, Artificial Sequence
  subsequence
tgtctctaataaaggccttttttgtttcaaattacatacgctttttactgcacaatttttgtattgaccttatttcaactgaagcgattatttccagcaggtttaatttcgacaataagatatattttaatagttttacctttcgctagaattttgtattgtttaaaacagtaaatgaataaatttgctgatgattcaagaatatttgtttggtttcgttttgtatccctcaaaaggtttatttccaaactttttaaaacaaaatcacgagaaaagagttgttttaattacgtttgatttttaaaaatacttttatctaaaacccattttgtgcattaggagatagtttgcttccatgctcaaaacatggagttcacatctgggggacatttttatccctcagtttccttctaactgacgtttttgtcgggaatctgctcagacttttccccttttcttcacccacctcccaagttttccttatgtaatttagtaaaaggccgcctgtttttcacaaacacggatttgttattttaaaaatcaatagatctttatatgctagtgttaaaggtgtatggtttttcttatttccatcttctctccttttctctctgtcaggccttcttttatggcctgcactctaatgacgtttcttgatttctctttgtcgacaccaagtttttgttgtgcgtgctttcgaccctggtcaaccttccttcctagaggcccgctccggacagcgtaggcctgggcgcctgggtggagggtgcagggtgccgggcgcgggacttcggctctcgcctgggccatcccgggctctgagggcccggcatccatccccaaggtccatggctttcaagttcggtcacccaggcagagagaccctgccttttaaagagccctggaaagttgcgccgcgttttccctcaaccctggaacacgcagggaaaactatgggaatcgcccgcgtcaaaagctttcgacggcttctaggaacccaagcgggcctgcctcttcccctggagcttgccctcctgggggcgggaggagggcgggagggaatcatttctttcaaatgaagcccacgccagctctgaagccaatttccgccgcggactgtccgtggagagttggcgaccaacactttctcggacggcataaccgcgaggggcttagactggaaatcagatgcgccaagaggacaagagccaggggccagaataccccagtgggggacgcgccttggaggacggttcgcccagggtgggcttcagccctttcccagagtgctccgggcgtctggggactgaccggagcgcagggcgggggacacttacttcgttatccgcacgccttcctcgttggcatcagagccggacaaatcccaacccgcgccaggcaaagataaatgactcctggctcccccggcagctcagggggtctgggcgggggcggagagggaaggaagccgtcggccgccggaggtagagactgtggaggtcctcctcccggccccaagcgaatgagcccctgcggcccgagcagagagatacgcctcagagggacgactgatggggaaggatggtgggcaacgagtctgcgctaggcggtgagcctagcaccccagaggcccgagggtctggggctagtggggccgaccgttcaggagccgggtgggcgggaagggaattgccaaggtcggcccaggagctgcctcaggcgaggacggggagctttctgcactgggcttcccggggtaggagatgggcgtcgggtgtgggcactgcctgccctgggggaagaaagcgaggagataggtttcagagctgggggagtcgttggtgggagatctggtgtcccttcggcggccgcgggccgggggaccggggaagacggagggtcctgcggcctggagcaccaccctaccacaccaggcaacgccccccggggcgcccttcattcttttgcagagcccagaacttaataggtgggtccccttctgcaaccacgctgcgagagaatgactgccctgctaatctagtttacttgtagaaatcgactgtaaaccgggacaacaaggcaagggtgggggaagaaaaggaagcgccgaaggagccgccgctgcgtccccgcccccagctcggagctgccggggttggggccccgggtggcgctcccgacccgccgcgttttccttagggaaacaccgagtgaggcagaggatctcaggcccaaggtggctgcgaagagccccgaggcctcggcttggcgtcaatgtcccgccaccctcgagcccgggtcactgcccgggtcccggcccggagccccagcgtcctctcccgacagcgccaccgcgtgggctgaggccgaaaccttcggcgccggctctgccggtcgcgtcccggagccaacccttccgcgtcgcctgcagtccacgggttaaggatgtggcgggggatgggcaggtccctggcccagggtaccaccgggccactcaacacaaaaacgccctggcgcgtgcaaaatacgaacgcccacagtttgtcccaaccccttgaaatgaaaagtacacctggaaagcccaagatagcacccggtccgcaccccaaatttcaggcaggccagcaggcgtccagaaatccgctcccacccctcgtaggggcaggcaagctcaggcagccgggtgcaagggggcccaaaccgcagttgcctcccgaacgctttgaggctatgggcccacgccggtcttgaaccaagcggagagggcgaaaaagcccgctgcgggacccacggtcccagacacctactggagccagggacgaggggggcagtgtatccggcggcccaaactcgtaaggagtgggggccaacttagagggcttcccgagctggcgcctcgcctgttttctcggtatcacgaatcccctcggacaccgtttcagtccgtcaagaccttggcctccgggaaaggcccaagtgactgtgacggcggcgactcgggctcagttctcccccaccccgtggtgccttccctccccgccctacagccaagcccagaggaacagggcatcgcctcgcgcggtcccggagccacatccggacttgggaaccccgtgtcgggcttagaggacttcactgggcgggttggggtttattttcaataaattcagctgttcacatacacccccaccaccatttccacgcgcgcgcgcgcacacacacacacacacacacagagggacttgtcaactattgagacagcgacccagaaaggtgtaaattcacctggtgcccacccaattgcaaagctcccagacccacacaaaacactagcgagccctggaggtctgagacgccccgcgcccgactcacggcgcgaacaccagcgctccggccgggtcgcaggggccggtgcccagcgggccggggtctggcgagccaggcagcgggccggctgagctcctgcgccccgcggtcgcgtggcctactcgcctactcccttattattggctgggacctgttcctttccaaagtgtgatgcccggtgtcctaccctaggccacgcggagctctctcccggcgtgtcgggccctgcgcccctgcccagtggctcacctcggctcgctgcgcccgccttcgccccaagtgcccaggacggagcgaggggctgtgggtcggcgcagggacgctggctgctcacctccaggagccgacagaaggtgccttcggcgtcacgcgtccaaccctggggctgatttaaataactaataagctcagagaaattttacgaggggaacttttccttttagtatcaataaagcctagtaattgggtttgttggttacctaagctcgagttcgactttctcagtctctctctctctctctctttctcattcagaggcaacgttttcaaaaaccggcaattgcgtgtgcgtttggggtgtgcaagtgtgagtgtagatgtgtgaaagttatttgtttcagcagtccttgtctcgagagcaatcatcattgtagctttgagtgaagagttttcaaaggtgaactgttgttatttctgtcaacagaaaactgttgacaaccattcaagtctcacaatacaagtataatataagggagggtggaatatctaaagactgtcccgttggatatgacagaaagacatctgcagtgtttccctaatagtttgcattttaattaactttcattacattctgacttccactcaatatccgttgttttcagtaaagacttctatatgataaaacgttgtaatttttgttctggttttccaatcttcttgaaaaccagttcttaattgtaaggaatttttccacctgggaaccatgccgtaatttaaaaatataaaagacctttcatgaacaataactgcaaataacccatttgttagtgtctgcggagttgctggcacctatacaaagtctctgaaatataaaggcaatctaagaatgtttctctccaaccatagtgatatatacttttttcgtttttgttgtgtggaagttaaaaacacttttaaagttactttttagaaaagtgttgtgctaaaatttacctgaacttaaattccttatcaatgttagcctaacgaaatgaagagtatttctgaatcagattattgttagagtcatatgctaaatagtaaaggaaaagaaatgggaattaaagtttgcaaaccaagaccagggaaaagtcggctccagaagttaccaggaacccacccaaacctgtgcactcatatctcctgtatttacatattatagacaacttttcctttccacttttagctagaaaagtggtgggctccccttagttcgtctcgttttatgctgtaagacccaaagtctgctgagggctgcccctgccaggtaacttccggagacccggagttacttggagacagacccggccctttgcacattccaagtgaaggacgtctcgcgcattcttcccagagctaccacacacctaacctcttctggacacccaacagctggggcactggagcacctgaccctactcaagatcatcccccagcccttgccggcacttagggacagcagaatctgagctgtgggtgtacatactccccattttctgctttcccagaggatcacagacaacttttcttcccatctgctcccgctggactcctatgatcacccatcatccccagttgttgctatctctgagctcttggtgaccagcccttgtcccccaagctgaccaagttgagagagtacttgtcctcccagcactgtctctcagtatcaggaagttgagatcagtggcagggaaagatggaaggattggcaaggaaagtgcagggccaagtagagtagctcagagcctcagcaatgggcacctgtcctcccccaaacaacctgtggtctctccggctccctgcttttccaccattggtcccatcctgggctaccagcctccactgagctgctctgggaacttagggtgtctcacattacttccctgctatggcatattttggtttcagttgagctattttctgaagatgtggatactccagttttattctttttctgtctgtgtctcagtactcttttccttttttaagaatgttccccaagcctggcttttgccagaccctgtgccatctccccaagctctatttacaagaacaagaagtgatttgtctgtttatagcaggtttaattaagacagttatgcgccgtgaactctttgggcctcaatcaatgcacttagatttggaaactcagatagaatcacatcttacacgtgcggccccggctggccgcccaggctgaggacagagctattgttttctacatcagcctcactggaactgggcaagtcccctgcagaactggcaccccctgctcctcccaagagacctcaagtcaggtctcccggccagactcaggcctttctaatacaggcgtgaagggcgggacgcccagagccctcttgttggccggtggctaaggagccaggtggataacttctgcggattcggctttcaggctgctggagctctccccagcccgaggccttagcccagcgcaatcccttgtccagaccggccagtttccgcgtggcgaaaaagggggaggcaagtgtgtcttttccaaggagcttttatccaacagcctcccctccccccaactctcagccttaggtgccgggcttcagccgaagcgtttttcaaatttgtcatcattggaaacctcggacaagtggagtgtaaaattttgagggtttccaggtaggctctgacttcaggcattcaatgaaaggggaagagggctgagggcgggggagagagacaagcacagagggctccctgtagtcggcaggaattccctccctctgcagcccagctgcacccactagcacacactagtcttgccttctcccggctttggaagaatccccaccacattctttagctctcagaaaggagagggcagtcaggtcaaggtctttcagcatccctaccgcaatatacccctcccagccccctcaccaccaccacgttggcctaggacacaggaccccggggccagggcctcagtgactgcagcttatgccacctaatgcagaatggggtgtccctgcctccactgctcctctcggtctcagcatccaggtcctgaaacccctgcgattctggcctgggaagccagacttgccaccaacatcatggtatcacccataattgatccactcagttttcagtagatgtggaatccaacaagagtaacaccaccctccacgccccactcttttttctttctttctttctttctttttctttctctctctctctctcttttttttttttaagaatccaaggcacttgaaacattctgagtgtgcctgcagtagggtctcagaggagttgctctgaaagctgttgagagcagccacctttgctgtcactgagagcttggcagggtcagctctggtgggccgtttgcacccaggctctgatggcaccaggatggcttcctgcaacccggtaggaggactggggtgggtgggtccagtatttcgtttcttcctcttcctttttttttttttaatgtccctctttatttctattgaagactaacctcagtatcaaagggtgcacttgtttgtcctaaatggcttgtagctctttcctactctgccacaggacattagctctgggagcaccgcctggcagggccttcgctttgggcctaagcatccaactgaggcccagcaattccacctgtggggaatcttgcagtgaggtatttgtgcatcaggagtggggagtgagggagagagagctgggctggtgcagtatccactctcgcacctcctccctgagcggagctccagtatagactaagtgaatgaatccatgaatcagctccatagccgaggggtagaagaagcagccgtcttcgttaaatgggctgttggcagttgcggctgactgctctacccctcgcaggcccgcctctgggcaggcctgaggtggccctggagccccgccagcagcccccgcccctcaggccaagctctggccctggcaatctctgcactttgtcatcacgcccgagtatttgacattcgcaattatctgcaaataccctgatcagtttgtatatgaaacactttttttcctgccttaaggttggaatctggtaagtttcagacaagtggttgcagggggagatgacccaggggaccgtgcgggacagggccggtgaacccgattccgcgaggcgggcgtctcgaagggactggtctgcgtgcctcaccgggttccccagcctggctccgaggaaaggccgcgcggaggcgagaaagggcccacatctcgagtctccagtctctccttgaaaagagcaccccctaatcccggaggaagggagggtgaaggaggaggggagagcccactacaggcaaggcaggaaggttaatcattttgttaaccggaaagggtgctgccccgcctggccgtcgtcaccgagcgtgtcagtcacccgctctcgatttcgccgcagaattacctgctcaaagagccaccccaagaagccctcagctccgaggtcttcccgcccgtcgtctgcgggaagtaaacggcgtcctccctccaaagaagtggatgccccttcgactctcctccgccccccggcggttcctaaatctaggaaagccagccccggcatcgctcactactcctgcacctcagctctgggatacccgctcagtacagacagaccatcaaccaaaaaagaaaagaagaaaagaaaagtggtggtgggggtgggggtgggcag

SEQ ID NO: 121 - DNA, 8717 bp, Artificial Sequence
  subsequence of BCAN
ggtcggggacagggagaagggagtgcctgcctggtctgcgccccccgcctgtcagcccttgcctcgaggctctggggcacccaactcgtcgactcctgacaccgcagcggggtaggctgctggacagccccgagcgcctgcagctgctgctgccatctctgatctacatgcttccagctctgccagtggcagcccccctgctgctcgcagtctgatcagcaacccctcgggtcctcgcatcttccctgctgcgcgctcctgtcccagcgcggccgccgagatttccgaccttgtcccaggcagggcggtagcgttccggatcagtccttgcctccgtgcccccacgcacaggcagctccaggagcagcggccagcaacccttctggggacaccttactgtagtccggcaggacagccgatcagagccgctctagggggtggtcggagtgcccatttcggctggaatcccaactcggctccttgctctgtgaccttggggtagttagttgacttctctgaacctcgggttcctcatcggtgtaatgagcaaaacataaacaatctttttctcacagttgaggttatccacaggaagcatttaggagaactggctcaggtagacatcagtaactattagctggaattcggttaccactattgcattccttcctagcactgccaggggcctgggaattccctctcccaggtatttccatatcctgtcaggtattcccccacctattggaatagctctgcctacatggttctaataggaccaagagattggcgtcaagtccaaggggcaccattattatctgcattacttagattgcagatgatgacagtaagatcagggaacagtgttacccttagacccacccacagtattaccagtgcctatgttgctatggctaactttgctatttataacagcatcatccacatttcagattctatacgagagggatctgcaactgctcggctggtgtcattgctaatagtattattagttttgcttccaataaaaaggactatttatatgatgattgcaattacttctacaggccctaaggccctgcttatattgtgtaggctcatgttgctcctcatgaagccgttaagggggtagcagagagcttccctcctgctatagccaaagctctggcttcttgtgcctccctgctgaccctgctgagtgctggagctcagttcctatgggacagaccttggctgccggctgatgggcattcagcatggaggtggtgggtgttgttagatgtgtgtacacacgtgcatgcctacacacacacacacacacacacacacagagagagagagagagagagagagagagagagacctggtcttaactctctgggttgggtctatgaagactgtgagggagatggacatcccgggtcagacagaaatgatgtgacaagaggaaagtttcctgaacagctcaagaaattcaaaacaagggcagagatacagacgctggagctgaaacagagagggggatgttgtggcgtcaagggaacggaccgcatgactgctgagctctcagggttagagttggagaggtgtggcctgctctggaggaagagaagaggaagtggagatgagtggtgtgtgggatagagaaggccacagaaccctggacccctgggttctgaggctggtaccggatgtggggaagtctgagtttcctcagggctcctagctgcaattgggaggctgaggcccgagactggagagacagagctctctcagaactgcacggggctaccctcttggcctcactggtcagtgactcccatttttggggtcaagggtaggttgccctccatgttccagagcagttaggtcctcattggccttaggccctcttccctcactctcccactgtcagacagaggtgaaagggtggtccagggtgttggccccaaaatgactccaactatatgggtctctgggctgcccgtcagagagatgggagccaggtctgtgagcagctccagctccagcccagagagaagggagggagggcaccagaagggggccaggcccaggccctggcacagctcagatgcatggcaaacagtcttcccagcacccggtgggcactggctgctcctgcccaatggtccccactccagccccagaacagtcctcccaagcaccccaatgcctggagctggtctccgcacctctaatctggccccatcaagaacctcctccctctgaaaggtcagagagaggccctaagcatctggttgtgccactcctctcccaactctgaccctagggaatgatatccagacacagtgggggagatgggggttatgatggcagggaggtgggaggatctgggaaaagtaggaaatttcccatcatctcaggcttaggaaagtgcagggacaggtatgaaggcagatgctgagagggcagggaagatgggggataaacagtgggcctggaatgggagtgcacagccagtggaataaacctgatctctaggaagtcctgcctgtagtctaaccttcaattctcttgctgcatcattggcctattccatggcatacctggatctccatgctcttctaagtttagcccaacccttaaagatgatgtagctctgagtcttctctcctgggagcacattgccctcgtgcctgacttggctttactagggatccagggtcagccctatccttctctgagcctcagtctccatttctcaatgtcacaacacatcctttttatgagagtgtaagtgcttcgagatctttggaggaatattctgggttctagagcttctgatagccaggggtaggaaggggtagcccctcccatttattctccccccccttagtccaccctccagcccaaggctttcacaaaaggtagggtgggggaagggaggggctggatagaggccagactggcagagacaggggctttgtcccaactgatttctgagccaagagttccggtgggaaagcccgtgccaggcagaaaggagaggctgggaagaagaagggaggaggcagccaaggaagggggatggagaatgttggggagtaaagagaggagtttccttacaaataatggtggggaggaagtagaggagagggtgggctcaggagaagctgtgcttacttgcgttcggtctaggaggccctcctggaaaaggccaggtgagtatggtgtccctggaggcagggacagtctagaaggcagaagaggctaaagagatactatgggagaaggctctgggttcgaggaaggagtctggcactgggaggagcagatggaattctgagtataagagcacccaccattcatgctgtaaactgagctcctactgtctgcctggtgctatgcatttgtacaggagttttaagatactaaacactctcaaagcacatggtcctatctcaactcatgagatagtaatgatgatgcttttttataagtaagaaaataaaggctcagagaaggtaaggagcttggcttaggtcacacagtgagttgactaggactcgggttttggttctgagaagaaatcacttgctgggaagatggggatcagaaacagagagtccatggtgatgtgaaggtaggggacttctggagccaggatatgtgtgaacccacatgggtgtggtagggagcaggggggaagtccatcctgaagtctaaccccatctttccttctcatgtccctctgtcagcctgcagcatggcccagctgttcctgcccctgctggcagccctggtcctggcccaggctcctgcagctttagcagatgttctggaaggagacagctcaggtaagcaaccccacttggggtcaccgtctctgtcttgttcagccctaaccaactgcttccaggcttaggggccccaggaagagagagaattggagggctgtggggaagcgtccaggctggaacacttggaaataagggctgagctgtgagcatctggtgggttggagaaatcatggggcaggactagggaagggcactgggtgcaaggctttgggcccctaaggtggaggataggggatcctgaagctaggaggtgggaaaggggtggaactgggagaaaccctgaaggaggccctaaagggagcagactgggaaactgggctggaggactcagggggcgaggttggaggaccctggggtgtggtctaggaattttggagaggaagtggaagactctgagagcagggcaaggaatcctgggggctgaattgactgggagactttgggggatgggtctggagaccgtcggggtggtcctggaggacctagaggtagggctgcaggaccctggcccctggcccctggcccctggtcctaggggggccggggaatcctggggccggaaggagggatcctggagcggggcttggaggccaccgggtgggactctgagggtcgacagcgttaagttccagccggctccacccgttcacagaggaccgcgcttttcgcgtgcgcatcgcgggcgacgcgccactgcagggcgtgctcggcggcgccctcaccatcccttgccacgtccactacctgcggccaccgccgagccgccgggctgtgctgggctctccgcgggtcaagtggactttcctgtcccggggccgggaggcagaggtgctggtggcgcggggagtgcgcgtcaaggtgaacgaggcctaccggttccgcgtggcactgcctgcgtacccagcgtcgctcaccgacgtctccctggcgctgagcgagctgcgccccaacgactcaggtatctatcgctgtgaggtccagcacggcatcgatgacagcagcgacgctgtggaggtcaaggtcaaaggtgagagggcagggaggttccagagggagggagggagggagggaagggaggactcttgccttcggggatcccacagtgtgagagggaagcaaaggtagctggaaggcgcagcctgggttggaaaaagagtgaggagacacgggcctttgttgtctcctttctctcttcaggtggaggacattctacccacaatctaacttaagtccctcatgctgtagagtgagcacaattgaactttatttacccttgtgtacagaggagtgacaaggagggtgaggggaggccagcgtgctgggtgctcacctggctcaggggtcctctctgccccacaggggtcgtctttctctaccgagagggctctgcccgctatgctttctccttttctggggcccaggaggcctgtgcccgcattggagcccacatcgccaccccggagcagctctatgccgcctaccttgggggctatgagcaatgtgatgctggctggctgtcggatcagaccgtgaggtgggcaggggctgtggattggggcttctattggcccctgaggtggccatggccccccttctgctgggtgctgcctgctgtgtcaggctggacatgcagggctttttgcctctgggggatgaggctggtctgaggaggggaggtgaggaccctgagcatgtgcatccctgcagtgctagaaggacagccagctgtcagcaagtgtctgcactgtggtggcagtggggttcaatagaatcaatatgggctggctccctggtgaaagcatctgtactaagtgattctgtccttcctccctaggtatcccatccagaccccacgagaggcctgttacggagacatggatggcttccccggggtccggaactatggtgtggtggacccggatgacctctatgatgtgtactgttatgctgaagacctaaatggtgattaggagtgagaggttcccaggggacaatttcctactcccatgctgcccataggtcctcccggggcctctgcaggaccttactatccctcctgagtttaagggggcaagcaggagtaaggagacaattggtgtccctctctccaaacactgtcacagaggcaagctcatgaccaaagtctcagccaggcagcaggataccgagtttaactcatctaccacctgccaggtggactctgtgcatgactctgcagaacaagaagtttgggccccatctctttgagctctaatatccatcttgaggttctattcagactatgatcctatgaagtagagtagttgactccctgccacagatgagggaactggagaagcttgcccagggttcccatgggagaccagagtggaaggagctaccagctgcctgataacccagccttctcttctccacccaggagaactgttcctgggtgaccctccagagaagctgacattggaggaagcacgggcgtactgccaggagcggggtgcagagattgccaccacgggccaactgtatgcagcctgggatggtggcctggaccactgcagcccagggtggctagctgatggcagtgtgcgctaccccatcgtcacacccagccagcgctgtggtgggggcttgcctggtgtcaagactctcttcctcttccccaaccagactggcttccccaataagcacagccgcttcaacgtctactgcttccgaggtgagcccacctccctgcagaagctgagaccaatctcagaaaggcagagttgagtcctaaaagtcctaccccagtctgatcagtttagctcagggctttgccatttgcctgaagtggtcgtgggtgaagtccagcttgtcatctagggttctaattctgggcatgccctctggtgtggtgtctgtcagctgtttggcccaaggagtagtcaccttttggcctctccttatctgccttcccaccagtagtccatgccttgtttgctccagctgggctgctgaataagctcccatctcctgtcagcttattggcagagcaaagacgaccaacattctgtgaattcaatgagtaatctgcccaagttcttccagtcaacaaccaaatgccctcaggagccctctggaggatttccagaaactacagcttaagaaggtgtcagatctttaactaccaaatactggtggatggatacaattcccccaaaagggagcaagaccttaagtacagttgggaatagagatagctttctgcccacatcttatggcttgtttctttttttgagacagggtctcactccgtcccccaggctggagtgcagtggtgtgatcatggttcattgtagcctcaacctccctgggctcaggggatccttccacttcaacctccggagtaggtgggaccacaggcttatgccaccatgtctagcaaatttttgtaatttttgtagagatggggtttcaccacatgcccaggctggtcttgaactcctgagctcaagcaatctacctatcttggactcccgaagtgctgggatttataggtgtgagccactgcacccaaacctgcccatatcttatgttgggagctggagcgggaggcagtttctgggactctcagatgcaaaaggcccaggccaagggtgaccgacaataagagaggcattgccatgcggtgtctcggtccttccccagttttaagcctgaaatactgttacaagagctggaagcagaaatggaaggagcagacacagccttgaacctcagggagcacttggtctgaaggatgaagacacagcttttgccatgggaacccccagcaaagggaagacaagatgcctcactcccaggatgaggagagactgagagaaaagcattacttccatttggacagatctgtggacatatttggctggggttggggaggggtggggaagtaaaagtccataggaagacaggtccatctgaaaagacctcctggaacaggggtagtagtagtagtagtagtagtagtaataataataatagtaatagctaaaacttctgtgtgctggctatgattgtgtgccaagccaagcactgttttggaaagaaatggcctggatcatgaggaggggcaggggagggggaatatgactacagttgggactacgattggtggaggacacaggcagcaaggacacaaggtctggtgaggagtaaggctcactggagcaggtgatgagggcagggactcactgtcctgtcttgcctggctgagcacagacagccctcaggacttttcttagcccaattccaccttcacttcattggttttctgctcttggctcccttccccagaggacaagtaaaccattctaaacttctggttatttgaaaggagtaggtcccagaaggaggtggccttttcccttgcctacttgccccaccactgagatcctcaggtgatgcctgaagttattcctgcactctgccctccagctatcctgaggggatgacagcctctccccttctatttcaagaattttggaggctcggtgcagtggctcatgcctgtaatcccagcactttgggaggccaagaccacttgaggccaggagttcgagatcagcctggcaaacacggggaaaccctgtctctactaaaaatacaaaaattagccagttacggtggcacatgcctgtagtcccagctacttgggaggctgagacgggagaaccgcttgaatccaggaggcgaaggttgcaatgagctgggatcgtgccactgcactccagcctgggtgacagaaggagactctgtctaaaaaataaaagaatttggggatacctgggacacctcacaccttgccccaagcccaagatcacaaggtggtaaagctatttcatc

SEQ ID NO: 122 - DNA, 8797 bp, Artificial Sequence
  subsequence of TP73
acatgcatgcactgcctcttggcaggcgagggagcttggggaaggctcttaacattacacagcctgtttccccatcagcaaatggccacagaagtaccaggctcactccttgtgaggaataaatggtgcaagacctcatcaggggccccagcacaagccgggggctccattggatagagtttgggcccccttcccctggaaggtcctcatgtgggcaggaccaagcatgttcccagtgccgtgagcaagcacccccaggtgtttcctgaggccctgggatgtggccagcactccagtgccagctgcgattgcccttacaacccagtgccccgtacgcacggtcacccccgtccctactaggcggggcgaggagacagggccccaggtgttcagcccttgctcaagcctctagctggcaggggtgatgcccagcgtcacatcgccaggccttgggatggctccctggtgtccagaggtgtctggagcctgggtggaggctgcacctggatgcccagcctggctgccctgatggccccacctgcctctcacccaggccccgggatgctcaacaaccatggccacgcagtgccagccaacggcgagatgagcagcagccacagcgcccagtccatggtctcggggtcccactgcactccgccacccccctaccacgccgaccccagcctcgtcaggtgcgtgggctgccgagggcctgagcatgtgctgtcaccctgtctgttcacctctgtccttctggccatgtcagctgccctgccccaccctgtgtgctcaccactcgcaaccctggatcagacaggcgggcgggggcagtcaggccaggagcatctgcagatgctggggaaatggtccacttagaggaaaagcacaaaaagccggggtcctccactgacctgtccccagctgagcacgtcccctccctgagggatgccgtggccacctgtgggctggagccacccttcggagacagcggcagtctccgccccagccaggccactctcagagatgggggctcgcgcagccctgtgctcggaagctaatgctgcttcctttctcaaattctctctgcagttttttaacaggattggggtgtccaaactgcatcgagtatttcacctcccaagggttacagagcatttaccacctgcagaacctgaccattgaggtaacgcccgggtggaccccgctctgcagaggcagtagctggaggggcccctgtccggagggcaaagagccttctcttccttgctctcgtggctgggaaacttggaaaccctttcccacgggcaagcagatgcgatgatttgactcttgagagcttaggcagatgcagccaggcacgtggctggtggcgcgggacacaggcccaggcctccggatgctgaactggtcatttgagcctttttggactcccagcagccagtgtgcctttgattttaggggatgggctgtttccaaggcacaaagaacagaagaatgtaaggccccgagggagtcagtccagttcagtgccatttacagagaggtcagcgccatttacacagacaggaaaggggacctagggaaggcaagcacctggcccgaggccacacagctcttggcacccatggcagctgactgcaggcaccatgattaaacagccacggcttgtctttgggttagagactagtggagtacaaagcctgctggtagcctaggacggtgtgaaccacagggcaccgtcagtcaaggaagagcaagccctctggtgggaacctgccccccagccagtgccgcggcccaggtccaaggcccgtcccagaccatccccagcctggggctgcagacagagatgagggtcagtgcgagctagggccagctgctcagcctaactgtccctcgtgcagagagtggccgcgtctgtgtccactaaccgccctccccgcaacctgtccccagtgacccacgctgagccagctccaggtcacgttaacccttgcctcccctgagtgatgtgtgtgcttggtgtggtgcccagagggtgttgggagctcagggatgagctgggggtccactccagggggcagggacatggagaccaaggagggccctgccctgaggctgggaggcagttcctcccccagggccaggtagatgctcagggggctccatgtctaacactcccaggtcagggcccaggccccgcacaggccaggagtgactctggtgggctctccccctcccccgtctcctgcctactctggttgggggtgtaggggccagggtgtggtgtggccagacctccaggcccagggcgaccccccctgctctccctgctccactgccccctgcccctaatgcgccggcctctcgcaggacctgggggccctgaagatccccgagcagtaccgcatgaccatctggcggggcctgcaggacctgaagcagggccacgactacagcaccgcgcagcagctgctccgctctagcaacgcggccaccatctccatcggcggctcaggggaactgcagcgccagcgggtcatggaggccgtgcacttccgcgtgcgccacaccatcaccatccccaaccgcggcggcccaggcggcggccctgacgagtgggcggacttcggcttcgacctgcccgactgcaaggcccgcaagcagcccatcaaggaggagttcacggaggccgagatccactgagggcctcgcctggctgcagcctgcgccaccgcccagagacccaagctgcctcccctctccttcctgtgtgtccaaaactgcctcaggaggcaggaccttcgggctgtgcccggggaaaggcaaggtccggcccatccccaggcacctcacaggccccaggaaaggcccagccaccgaagccgcctgtggacagcctgagtcacctgcagaaccttctggagctgccctagtgctgggcttgtggggcgggggctggcccactctcagccctgccactgccccggcgtgctccatggcaggcgtgggtggggaccgcagcgtcggctccgacttccaggcttcatcctagagactgtcatctcccaaccaggcgaggtccttccaaaggaaaggatcctctttgctgatggactgccaaaaagtattttgcgacatcttttggttctggatagtagtgagcagccaagtgactgtgtctgaaacaccagtgtattttcagggaatgtccctaactgcgtcttgcccgcgccgggggctggggactctctctgctggacttgggactggcctctgcccccagcacgctgtattctgcaggaccgcctccttcctgcccctaacaacaaccacagtgttgctgaaattggagaaaactggggagggcgcaaccccccccaggcgcggggaagcatgtggtaccgcctcagccagtgcccctcagcctggccacagtcgcctctcctcggggacccctcagcagaaagggacagcctgtccttagaggactggaaattgtcaatatttgataaaatgatacccttttctacatggtgggtcagcttttttttttttttttttaactttctttctcagcattctctttggagttcaacctagcgcccatgagccaggctgaggaagctgagtgagaagccaggtgggcgggacttgttcccaggaaggccgggtggggaggaagcctagagggaaccccaggaagggcaaatccaggcaaatctgcaggaatgctctgccatgggagcagctcctcccttgccacggccaccttctctagcactgcaaggtccacagggcattgctttcctttctaggcggtggcagtcagggaacagactgaggtaggtgtaggggggtctaggccttcgtggagcaccccagggagttagtaggccccggggagacagagtctgcacaggccctttctggggccacctccatccacgaggagcagcctgagccttggtggccgaaccttgaccgtcccggagcacagcttcagggcagggaaccggagcccctggggggcctcacgggtgtgacgaggcccttcattgcaggcaggtgggccaatgggagccctcacccacgcaagccgagacaccacccagagtgcaggctgcctggccccttctggcacggccagctccacaccccctgcctagggtatgtgtggtcctaagggctaggagcttcccctactaacatctcccagaaaaagcagttaagcccctcagggcacagcaaggttagacacagcccccatccccagatcaggactccatcttgctaagtggcatcaccgtcaccagcctccccttatttaaaagcagcgactggtgttgccgcaggtacctggtctacgaagacgcaggcatccctctcccaccgtccacctccccgggggccgctgacagcacagtcgcctgggtgcacgcttgtgggggcagcaggaacggggctgtcggctctcaggggatctggctgcagccagggcgagggcctggcccttccttccagctccttccggctccttccagctgaagggcaggaagctctggccgcttagcttctagggttccatctccctagaaaggtgcccacgcccagggcatcagtcagtagcggcagcagcagcagactcggggctttcccagggtggcgcagccaccccagctgcatgtcacctcagctctccatcttattgccattttgtagatgaggaagctgagaccagaaaggctaagacccatgccccaggcaccacacccatctcttgggggctgggcacctgctacccgaggccacctcctgaagcccccactcttcccccatgttccacttcaggagccgcgggggcccatcctgacacccggggttcctcagcccagcgcagatgtgcttcagttccagagggcttgttgatttgtttcttaggtacgttacctgtccaccctgagtccagtgaggctgtcccaagagcccctgtagtgtgctcctgggaagggctgggggggctgggggggctgggagaggcccaggggcagctgtcactggaaccccagccagatgtccaaggaagccggccagaacacggagcagccagatggccccagctgcacctgtctagggagcccatgcagcctccttgcactggagaagcagctgtgaaagtagacagagttgagacttcgccgtggtcaggagaaaatgcaaattcccaggaacaagaatcctttaagtgatatgtttttataaaactaaacaaatcaacaaataaatcttgaaggcggatggttttcccagcagtgcaggggttggagggaggctgctggcactcctggggccaagggggacaggcagtggtcctgagtctgctcagagaggcaaggcagaaggagctcgccaggcaggtcagctcacatctgtccaagtcgctctggtcagaaacagcgactctcccccattcccccagcgttcccaccaggcctgggctgctgggaagcccttgctgtacccaggagcccgacccgcagtatcctggcacagagccacttgtcactcagaacagtcagtgtctccaacgcacaaacatccactcctctgttaccagttaaagcactttaatgctttaaggtgaaaacgaaatcccatccgtgtttttcgtgtaagatcgtgcttctccgagcagtattaatggacgccctccaatgacataacaactgtttttggtaatgtaatcttgggaaaatgtgttatttttttagctgtgtttcagtggggatttttgtttttgtaacataataaagtgtatgttccaatgaccggttctcatgactcaacctaaatctccaaagggctcagacaaacagggcggctcctcacaggcaggaagcccgtggcctctgtggccggccctggcaccccacttgagtttctctgtgtcgtgagtctgatgggtccctggggtgtccctctgccctgtgcctcggaggacctgcgggccaagccgagtagcctcatgggactgaccgggcctctcaggcctcctgaagtacaggcccatgagccctcatccaagccctgtggggcccaggccttctggactttagctaggccaagcagggtctcagggcgtcacaaacaccgacacagaacgcactcccgtttctcagcaaaacctaagaaaacaaaaggcagcagagagcctcatgttggctcaagccaggctgagaccaacgggcttcatttcagttctcttggttctcaggtttcttggtttcagagttgtgaacagggactagggacttgtcacagcaaaaacaaggctctagaaatctgttcaaccttgaaggaggcctcagtctttttagaaattggcctaaaacaaagatagaaaggaccaaggcaagagggggagatgccgccaggaagctccgccgagttcccccacaggtgaggtgccatgccaagccctggccccatcttcctggctagcgctcacgccgtcacaccagagcccgcccacccctttccctaggctcctacctgtccccacgtccaccaaggagggctgggcggtggtgggcccaccccctcatagccgcaggactctggatcatgaaggtgttgaggcctcaaactagacaggaagtggagggattctggatgttccctcggcaagagggtgccacatagaacgtagaaacggggactctaaaacgccctttcaggaatgaacacagaaatgtgagtgctttcagcacaagggtgagtttgaatatctttgtttaaaaggttagttattttttttaagtatagcgtgagaaatacaggccattattttcaaatatataaaaacatctccagtaagttccacacagaattttggaaagctaagctggactcagagcaggtctgctgctccccaaggcactacccttcgaaggaaggtttccacccgcccccggctgcaaaatggaaaggagaaagcccgtttccaaaaggtctccacgcccctttgggtggaaaacagccactgttcattcccgcgttcacatccaaagaggaagcctagattcaggtgacaagaacagaatatgggcttttcataccacacacatatatttcctatttctcaggaatggtgctgtgtcattactatgcacaaaatcggattcttcaagaaaattgttttttaggccgagcatggtggctcacgcctgtaatcccagcactttgggaggccatggcaggtggatcacgaggtcagtagttcgagaccagcctggccaacatggtgaaatcccatctctactaaaaatacaaaaattagccgagcgtggtggcacacgcgtgtaatcccagctactcagaaggctgaggcagaagaatcgcttgaacctgggagacggaggttgcagtgagccgagatcgcaccattgcactccagcctgggtgacagggcaagactccatctcaaaacaaacaaaaaaaaatgtttttaaatactggtgtaattaccccaaaaaaggcctaaggaggcctgcagcccgcctcatgcatgcgacatttagccttaacagcttcaccagccctcggccctgtttgccacagaaaagctgaaaccgcaggtttctgagtcaatttacaccgcccaatccctgacctgccctcttcctgagagagccaaccagaggcctccaaggccctgccaagggaactctgaccggaagagcatctctgaggcctgcgcacaacacaaaacacctaagcaagcccaacttgtgtccttggtctgaagtcccatcctgaaaagcctggttaaaccagaaatgaaacatacatggtttcccaatgcttccccttctgagtctccagtgaggacaagattgccatgaggttttgtctccctctcccagtaacagtaacaagtgaaacaggcaactggatatcaggcaggatcttggctccagcctcgagttggttcacggagcttctgtcttcaccacggaggcctctgccgattcgcagggcaggtccacagctgaccggtttcaccacgactgctccacggccacggtcacccggaaggccctgaggaactgctctttggtgatttcaggaggttatttccctgcacatttgcacagattcaggacaaaacccaacactgcggagccagacagtcttcctcttgttggggcatgtgaaggggccactggcctctgggtgggacactgatcctagagaggcccacctgcccctcttggacaagccccacccaggtccaggaattctgctcaacctctctggttcccagtcacccccaggactgacagagggtagaaagtgtcctatcttccaggatacatggtatccactagatctcaggagttcagaagtagttattttataaactcagagtttaagaagatttctcaggacgtgtcaggcaacatggtacacgcacagaaccccaaaggagcatctctcagaatctccctcaagtacacgcaacgtaaatgatcactgagatggacaatttcaaatctgaacccggtatctggaatgcaattttccacctgaaattggcatatcatctgcactgactgcagcctggaaggcatctacccattgagcatcaggacatcccaggttcctcctgaaaacgtcacccacctttaagggttctgacaaagtgtctgaagagctctcgataggagtcctggtagcggctagcctgggtctgggagcgaagggacagggacatgccccgcccggtgatgcccaa

SEQ ID NO: 123 - DNA, 8476 bp, Artificial Sequence
  subsequence of MIIP
gtatgcgccaccatgcccggctaattttgtatttttagtagagacggggtttctccatgttggtcaggctggtctggaactcccgacctcaggtgatccgcctgcctggacctcccaaagtgctgggattacagacgtaagccaccgcgcccagccaatttttgtatttttagtagagacggggtttcgccatgttgcccaagctgatcttgaactcctgacctcaggtgatccacccgcctcggcctcccaaagtgctgggattacaggcgtgggccactgcgcccggccccagtttttctaagttatatagtttaggtttcacaactagatctatgatccattctaggttaatttttgcatatgggtttcttttttttttttttaggatgagtgtgtggatatccaattatacctacaacatttgttgaagacaccatctcttcttgttttcccaagtttccacacacattattgataaaataaatttttttggggggggtgctgggtgtcgctgggctgtaactccttacctcaagccatctgcccacctcggcatcccaaagcgctgggattacaggcgtgagccaccgccccgggccgaaggcattatcctttctccactgaattgcactttcatttttgtcaaaaattaattgctcacatatcggaactctattctgttgcattgatccatttgtctacctggacgccaataccacactttctttcttttttaaattaatttatttattgagacagggtctctcagtcagggtggagtgcagtggtgcaatcaaagctcaccacagcctcagcctcttggactcaggtgatcctcccatctcagcctcccgagtagctggactacaggtacgtgcctggctcattttttgtagagacggggttttgccatgttgcccaggctgggtatcttttttttttttttcttttttgagatggagtcttgcgtcttgctctgtcatccaggctggagtgcagtggcgcgatctcggttcactgcaatctctgcctccctagtagctgggttcaagcgattctcctgcctcagcctccctagtagctgggattacaggcgccggccacctcgcccggctaatttttgtatttttaggtttactggcgtgagcaaccgcggccggccccaatactacactttcttgtttactgtgtagtccttatcttctggcgcaaagcgggcactcgctaaaaacctgaatgaaagtataaagcaggccgggcgcagtggctcatgcctgtaatcccagcattttgggaggccggggcgggcggatcacgaggtcaggagttcgagaccagcctggccaacatagtgaaaccctgtctctactaaaaatacaaaaaaaaaaaaaaaaaaaaaaaaaaaaaaaaaaaaagccgggcatggtggcgctcgcctgtagtcccagctactcgggaggctgaggcaggagaatcaatcgcttgaactcgggaggcagagattgtggtgagccgagatcgcgccactgcactccagcctgggcaacagagtgagactccgtctccaaaaaaaaaaaaaaaaagaaaagtatgaaacgatgagtacaatgagtagccagccgcctgccccacctaccccgccgttccggactgccgcctgcgccgagcctaggccgcccagcctgactgaaactgccgctgctgaactcagcgtatccagtcccgcagctgaccaatcggagctcgcccttccggggcccgccccattccaggaatcgacctccgcaccggcctcgaaaattgaccaatcggttgtgtagctccgctcttagtcccgcccccacgctgaaactgacacttcggatcgccgagtaacgctcaccagacgtcccggccctgcccctcacctgaccaatcaagacggccggccgaggcccctggaacggctcaggcggctgcggctgctacggcggcgcatgctaggggattctgccgggtgagtgctgggcggcaggactggggtggggcggaagggctcggcaggaggccccacgtgcattcccgcgaggggctcgggggccgcagtggaaaagaagggtaggctgcatctgcctctgcgggggtcccgcctcggcgtccgcccgctcgccctctgttacttctgcggccccggtgtttctggagcgtcgctttcccggtgtctccgctcagcttttccctttccaaagcgcggccggggccaggggagggcaaggcctgctgtgccctttgaccccgtgcgaaaacggcgaccctctgactataggggtgtggcccagagccacttggccagttaggggtgggggccgggatctttgtcctgcggatcaaacagttggcccctctggactgcatctccgtgccccccggccctgcggggtaatatacgtgtgtgggggaggttccggggtagtcggctactctgtgctccagaccttgcacccgatcctgaggatccttggaggtggggggcaagggctgggaggaggaggcggagttttcccaggctcccccacacttccagggaaaggctttccaagaaccctgaactcatggaccctggagtcaaattttggttcagatctagcctcttgctagctgtgtgacttggggcaagttgcttaacttccctgagctttggtttcttcatatgtaaaaagaaagtgaaggaggaagggagggcaggaaaggaggaagaatcccttttgaagcctgatttgtgttggactcaccagttataaagcaagcttgtccaaaccactgcccaggaggcggaggttgcagtgagccaagaaaaaaaggaagcatgcccttgccccagccattttggtaataatagacgtttattgaatgcttactgtataccactgtaagcactgtattaagtaagcactgtactgagtgctttgttttttgtattttgtgtgtgtgtgtgacagtcttgctctgtcacccaggctggagtgcagtagtgtgatctccactcactacaacctccgcctcccaggttcaagcgattctcctgcctcagcagcctcctgagtagctgggattactggcgcccaccaccacacccggctaattgtttgttgttgttgctgtttttgagacggagtctcaccctgtcgcccaggctggagcgcaatggtgcgatctcggctcaccgcaacctctgcctcccgggttcaggtgattctcctgcctcagcctcccgagtagctgggattacaggcgcgtgccaccacgcccggctaatttttgcatttttagtagcgacgaggtctctcgccacgttggctaggctcatctcaaactcctgacctcaggtgatcctcctgcctcagcctcccaaagtgctgggattacagacgtgagccacttggcctgttttttgttttttttacagtgatgcaaccatggctcactgcagcctgggtctcctgggctaaagctatcctcctgagtagctggggccacagacaagtgccaccatggccagctaattaaatttttttttggccaggcactgtagctcatgcctgtaatcccagcactttgggagaccgaggcaggcggatcacaaggtcatgagatcgagaccatcctggctaacacggtgaaaccccgtctctactaaaaatacaaaaaattagctgggcgtggtggcaggcgcctgtagtcccagctactcaggaggctgaggcaggagaatggcgtgaacccgggaggcggagcttgcagtgagccgagattgcgccactgcactccagcctgggcgacagagcaagactccatctcaaaaaaaaaaaacaaaaaaacaaaacaaaaaaaaatgtttctacaaatgttgtccaggcttaacatgctttctttaattctaacaacaatcgtatgaggtagatactgttgtcgtccagcagatgaggaaactgaggcacagagaagttaaataacttgcctgaggcagtacagttaaagagtgtcgaatgggggtctctggcaccacagggcaccctactgagccccgtgtcctgctgtcttgacttcaggtagaagagctgggcctggaacccagccctgaggacatcctgcggcccaggggcaagtgacacctgctgagagaggcccaggatggtggaggctgaggaactggcacagctgcggctgctcaatctggagctcctgaggcagctgtgggtggggcaggatgctgtgcggcggtcagtggccagggcagcctcggaggtgcgtgcccgccttgggaaccccagaggaaggggctacctgaccttcaggccagcatccaggcttctgggctcatcttgttcaatacacccattttactgatgatgggacattgagggctggggagggaagagactggccttggtcactgctgaggccggagcaggatgaggatgcttgccttggtgcctggcgtaggcccggtgggtaggttctggcagccactccctgggtgacccggcccctctctccagtcaagcctggaatccagcagcagctacaactcagagactccatcgaccccagagacgtcctcaacttccttgagcacctcctgcccacggggccggtcctccgtgtggggcccaccagatgcctgtcgaggggacctccgtgatgtggccagatcgggggtggcctctctcccacctgccaaatgccagcaccaggagtccctgggccgaccgagaccccactcagcaccctcgctgggcacctcaagcctgagggacccagagccctcagggaggctgggtgatccaggaccccaggaggcacagaccccgaggtccatcctggctcaacagagcaagctgtccaaggtaacgtgggagagcgggacatctgctgatgggaggagcttccttgggcctcagtttccctatctgacacatgtgcttgtgggtagcctcccttgcagaataagaggctcctgggagatactgtgagttgggtcttgctcagcctaaatgctcgctaggtggtagctgtgagtatctcatacagtgctttgagaagaggccaggatttgttcacagccacacataaagtggggccaaacgtttcccttcttgctcttgtgcccttggctgagccctgggctgcaagtcagggtgtaagttaagacacagtctctctgtccctcgaattgcggcttcctctgggccaggcctcttggcttagtccttgtccctctgtgcttccttcctcagcccagggtgaccttctctgaggagtctgcagttcctaagaggagctggcgcctcaggccatacctgggctatgactggattgcaggtaaggcgtgctgttgccctgcacacactttgcctgggagtgggaggtggaggcctgggatcctccatgctcctgtctgagcctccacccggtgctgttgcttgtttctctgaccgtgccatcctccgtggggagcaccctcttttttttttttttttttttttgagacggagtctcactctgtcccccaggctggagtgcagtagtgtgatgttggctcacagcaacctccacctcccaggttcaagtgattctcatcccttggcctcccgagtagctgggattacaggcgagcaccaccacgcccggctaatttttgtattttaagtagagatggggtttccctgtattggccaggctggtctcaagctactgagctcaagatatccacctaccttggtctcccaaagtgctaggattacgggagtgagccaccgccccccacagccaccttctttgttttcttatttatttatttatttatttatttatttatttatttttgagatagtctctcgctctgtcgcccaggctggagtgaagtggcgcaatctcggctcactgcaagccccgcctcccaggttcataccattctcctgcctcagcctcccgagtagctgggactacaggtgcctgccaccacgcctggctaatttgtttgtatttttgttttttttagtagagacgggatttcaccgtgttagctcgcctcagccttccaaagtgctgggattacaggcatgagccaccatgcccggctttttttttttttttctttgctttttaagagaagacaggccgggcacggtgactcacacctgtaatcccagcactttgggaggatgaggtgggcggatcacgaggtcaggagtttgagaccagcttgaccaacatggtgaaaccccgtatctactaaaaatacaataattagccgggtgtggtggcacgggcttataatcccagctacttgggaggctgaggcaagagaattgcttgaacccgggaggcggaggttgcagtgagccgatattgcaccactgcactccagcctgggtgacagagtgagactccgtctccaaaaaataagcaagcaaaaaaaaccagatgagcagcagtgagaagaagggggaaagagtagaacaaagagtttggtctgtcactgactgtgagtatacaattgcgataactcactaccttcacgccagcctctgagcaccttctgagccgtatctgctctctcaacctcaggcactgagacggtgcatctgttgaatgaatgaatgagtcccagctgccgtatgtttgaacatttgttatgtgccaggcccctgcacaacttcataccaatgccagctcttttcacgttattgtccagctctccccgacagcaacctaacctcagctgccttctggctggtttccccctggcctatgtcccattgctgtcctttgcatgtgtatgtgtgtttgtgtaaatacataacataaaatttaccactttagcattttttttgagatgaagtctcactcttgtcatccaggctagagtgcaatggcgtgatctccgctcactgcaacctccgcctcctgggttcaagcgattcacctgcctcagcgtcccgagtagctgggattacaggtgcctgccaccacacccggctaatttttgtatttttagtagagaaggggtttcaccatgttggccaggctggtctggaactgacctcaggcgatccgcccgcctcagcctcccaaagtgctgggattacaggcgtgagccactgctcccagccacatgtagcgttttttaagtggactgttaagcggcgtcaactatgtctacactgttgagctatcattactaccatccacctccagaactttttcatcttcccaaaaacttctctccccattaaataattactcccattccccctccctccagccctggacagtcaccattctactttctgtccctatgaatttgactcctctagggacctcatataagtgaaatcatatagcctttgttcttttgtactggcttattttatttaacataacggcctcaagatttattcatgttgtactgtgtgtcagaattcccttcctttttttttttgttttttgttttttgttgttgttttttttgtttgttttgagagagagtcgcactgtgtctcccaggctggagtgcagtggtgtgatctcggctcactgcaaccttcacctcccgggttcgagtggttcttgtgcctcagcctcccgagtagcaggtattacaggtgtgcgccaccacacccagctaatttttgcatttttagtagagatggggtttcactgtgttggccaggctggtctcgaactcctgcactcaagtgattctcctgcctcggcctcccaaagtgctgggattacaggtgtgagccgctgtgcctggctggaattcccttcctttttaaggctgagtgacattctgttgtgtgtagatgccacatgttgtttatctgttcattcagggatggacacttgggtgctttccatctcttgactgttgggaataatgctgctggtgacatggttgtgcactgtcacttttgacatagcagccagagggaatttttaaacatgggaatcagatcatgtcactcccctactcaaacctccccatgggcttttcccagcacttactgtaaaatccaaaatccctatctagacttacgaggcatgatctggcctctactggccccatgatgtgacctcccgtctttcttccagcctcgcggcctcctccttttttatttttatttgttttctctgttgcccagagtcaagtccagtggtgttatttctgctcattgcaacctccgcttccttggttcaagcaattcttcctcagcctcccaggtagctgggattacagacgtccactaccatgcttggcttatttttgtatttttagtagagacggggtttcaccatgttggccaggctggtctcgaactcctgacctcaggtgatctgcccgccttggcctcccaaagtgctgggattacacacataatggggtggccacaggcatggcaggaccagaaaggaggccacgaccagg

SEQ ID NO: 124 - DNA, 7991 bp, Artificial Sequence
  subsequence of HOXC4
attgaatcaggaaatttttctgagaaaggcaggtgggtatgggcaatctgacacgatccaaaaggcttactgccttgcacccctccccgcaaaaaggaagtagagaccaagatcttgggctttaattttatttttaattgtaaaaagatttcaaataagccaccatttgaactgggaagggaaactagggatggtcttgggggaaaatgtcattctctctaagaaagggaccccggggatgtgggtcgttttgagggtcctagaagttgaccccaattctcacctctcctgctgcactgcaggattgcccagggtaggtctagtcccctaggttcttcagaccactccaggtcaggtttggttgggtggctgccagtggtcttccactactgttcctgtctagggtggagtaggagctttcaggggtacggcatagaggggatgttgttctcttactaaaaaaaaaaaaaaaaaaaaaaggtaggggtagggaggcaccctttcaatccctgcaattcaccagccatcactgcctcaaggccacaaatctttgcaaagctttgaattccgcctgatccaaccttaatgcccccatttattaaggacaatatttaaaactcggcaagccaggagaggcaaccgaccctcagtgcttgaagctttctttcgcctgggcgtccgccctcagctctttctgcgctcgcctgcagcagcctggcccgtggggagtgggcggtgggtgggggtaggggtggggtgggggtccggggatgctccctctatgagagaattgggtaaacatggcgaccgcggcgcccatttgcacacgctacacaaatgcatcgcattcccggttgtttgcagaaaatttacagctgagtaataaaagtttacgatcgactcacaagttggattggccacaagaagtcatgtggattccatccatgaacgtgaactttttattgtggtttgtccgttccgagcgctccgcagaacagtcctccctgtaagagcctaaccattgccagggaaacctgccctgggcgctcccttcattagcagtattttttttaaattaatctgattaataattatttttcccccatttaattttttttcctcccaggtggagttgccgaagctgggggcagctggggagggtggggatgggaggggagagacagaagttgagggcatctctctcttccttcccgaccctctggcccccaaggggcaggaggaatgcaggagcaggagttgagcttgggagctgcagatgcctccgcccctcctctctcccaggctcttcctcctgcccccttcttgcaactctccttaattttgtttggcttttggatgattataattatttttatttttgaatttatataaagtatatgtgtgtgtgtgtggagctgagacaggctcggcagcggcacagaatgagggaagacgagaaagagagtgggagagagagaggcagagagggagagagggagagtgacagcagcgctcggtaagtgtttccttattggttcaaatatgtaactaatggtccgtggcggtttcaagaataggacagcagcggcttctcttggttagggagaagagggggctggcgagagggtgggcgcgtagttaattatggggaggaaaattggcggggggagagaaacggggttaaactggaataccggtaactggtagtggggcgattgtgttgtcctgatgtcactgtgtgccaagttgggggtggggaggcaagggaacagcacctgtggggctcaagccggcggtctagggcgccagctctctgctgcccactgtgtcagtacctgcttattatagatcttcggtctcttggctaatggaactgggtcggagcggaactggaagctcaagctccaggcaggagagagaacttagaggctgtgcccattgccccctaagcaaagttagccccccaacccccaaacaaactttccagcttcccctccctgtctggcagccccctccctcccagagagcgcgactgctagagctcacacatgcgcagtgtgggcccagggccgggccgccgagcaggaagccggcgcagctaggcggccggcggggcctgttaattggcaattaggggggaggctggtggctggtgcgcgtcagccgagaggagagcgtctgcccaccccctgctcccgcccccactcgggcggatggaagggtgggaggtgccctgcgttgggtggagggtggaggttgtagggtgggggtgggggatgctgtactcaaaagccatcttgtgctcagagaaaagaggcctaccggctttcccttccggggtccggcgcccctcacccccagccgcggccatcccagccgggatgcccactggaccgggatgcccgctcgccacgcatggctgctctgggctaggacctgcctcgcctcggggggaggtggaaatggggaaggccctaggctgggcggggacaggcccagtcctcctggtagagtctcctaggtgctgtggaggcagtgaggattccgggggctgctggcttatggggtagaggcgtcagcctggggcggcgggagggtcctgggcactcgggatctctctaataattggtgctaatggcctgttgtatagtcttaacccgacgcatatggtttcataacacagtggcttaatttcttccaaatgtacgtggccctgaatgtgttgcagtttgatatatgaccccgccctgctccccggcctgggtccgaggctccgaggcggccccataagtgtgaatttctgtttataaacggcgacgcacacgcaaacgcctacacacccaggcagacacacccggaggcgtgggggaacatattccagacgaggtccgagagaacctgggggccagacttaccttaatctaagccaagacaccccctctacccccaccctctcccagaggcgcgactgggattctgcgccaagtcccagtgggggaggggatcgctccacgatttcctgtttaaaccctgacccgtcgcctgtgggggggcggggatgggggaagaaacctgtttttatcaaatttttaaaaatacagtttgcattcagatcaaaccgtttgggccagagctgacggtgaattttatctcccctccccccacaacccccttcccttccttttctgcccccgctaaattcccctttcgcagccatcataaaggcctctgaggtattctcccgcgggaagaaatggcattttctctccccctcccccacccccccacccccagtaggacttgtgtgtcggcagaggcgtctgacgaggggctaatttcgctttccttgtttacgatcgagaaaagcgcttggctctccccaaatgggcccagcccgccgcctgctcaggctgccgcgcgctctcccgccgctcaggcacggcccagtggctgatgccccgcggatccagcctgcggcaggccggaacccggagtctgtgggacctgaaaagggcaaagggagtgcggtgggacacaagaggggcccgagaggcccgaaaaagggagcctttctcctggagtaatgtgggaatcgccgaccggtgaggcctctatttctctctttcgcctgcattttgtccgcccccgcccctgtggatggccgctgatgggggggaacacaagtgtcctttgtccgtccccgaaagaaaaccttttccagagaaggccattcaggccagtggagattcacctagaatattagaagggccccctcccacccgaggggcgggcctgggcgaggctgaggtatttctcttaatcctagaacgacctcactgagtgtacccacagcgagatttggaggtgctagagttcgaggttggccgcttaacagcaccatcctgaggtgtctttatataatattttaattgattttctgtcccttcctggctacagccctgcagctcccccacccccatcctatgcccttcacccctagacccatccttacaagacagaggcaagcagagaaggcatagcagcagcgaccggcgctctgttttcattttccactctggccaggggataaactggaccccagtggactccaacaccaactctctgcttcccagttactttcgattttctttcccttctccttctttctctccctctctggcattcaaacagaagcacaagaggacccaccagtggcaactctaagcctccttgcaggccacattccctgctgacgtggtccttcctgcaggagagcccttctgtgattatctaataatagccagggtggctgagaatagaatctggctcaaggactctgcacacccggggcagagacactgaatctgtgggtcagggcctggcaacattccttggagcctccccctctgagcccactctttgggcacccttaggcttgcctgccccccttataaggggctttgtcagccctgccatccgctgtatttcatgtgctggttcctagctaaggagaattgggcagagcaaaccctttctcaccctggtctgacagttgtgatcccgacagaatgcgaccttgtttggagaaggcgaccttgttgggttggctgtgttctgaaaccaggcttgggagtgttatatatttattatatacaggcttaaatatacagactcaggcttatgcatgaatatatacagactcatatttccttggtggttaattgtatattaccatgcctatattcgctcaaacaccattttatgttcatgcaaaattttgttagtcctcactagatgagagtgggctcatggaggcaccgggtgcactgagcaggccctctgtgcatgctctgctggaaatatgtgctcactggaatcggagtatgcgggttccagtaaccaatggatgccataaaggctttctcagaccttattgcttttgttgcccaagcagctggactggggaaatactaaatcccttctgctttctctccacacctcctggcaaactctcccaacttagaaattattttacaagggagaccagttgtcttgaaattgagttctgcgggattcttttcacgggcatggtggggctgcaagcagttcggagtagtcagggccctggcgctggaagcctcactggagcgatgaagggatcagagtggttaataaggtggcctctggacagtgatctggggcagctgctggccagggtgcttggagaagcttgtggaaaaggcaagccaaaaggggtagggatgcagtgaatatctgtttctccccctgcttgccccagccggccgctcaccccgccccagcccgatttgcctgcatccgtggcggcagattgggagttctctaaggtcccccaaatacccagatctggttactggatgaactgcgttttaatcctcgtcgctatctgagccaggacaagacctggtcagggagacggctggtccgggcagcacgggagaggacgctggacccgctgcctgtggcctggagcactgagtatgggctaccaaggctgagaattgatgggcctcctttcccagcctttttcccttccagagacacaaaaagacagagcagaggggaaatatcaatgtcagtggaaaaccccataaaagaaagcagggaccagagcggggctggaggggttttccgctactctctctaggtgatcgggttcctcccaagactcttgtccagacaggctgcaccaagaggtgtgcagctttcttccaccttcctcccgcccttcaaggagggcagccttaggctttctgggccttggtcaccccaggcactggggtgacattactccaggattgtgcccctcgcccagcccacggcctctgccacggcgccgcagccgctcctgtttattgtgtctgtgagttgtttacttgttttgtctgctgccaccctgcgtcagaaacccgccaaaccagcgaactcgcccaggagaacaaagtgctgtgctatccccggactccctcccctttccagcaaccccctcctgccctcacaagctcctgcattctccctttcggaggggaggaagcagaaatagtcttaaaacagggcagctgtttatagggtcaggggaattatggggacaccataaacctctgggtgtccctgtggtggacagacttctgagcagcccttcccttgcctaggcttttcttccttcccctggtgaccacttggttaagggggccacactcattgagaaagttgagcccacccccatcaacccagtcccccactaccccactcctttctgcaggagtttccctgagacacaggttgttgggttttaaatcagggtaatgttggtggattcataaagctagatatagcatgtcattcttctcccacactccctctcctcagccccccaaaattgcagtgaatttaagcaaatcctacaaaattaaattgcccctttgctaaagatcctatatgtctccaatcctgccaggtgtagagtcagatagttggcttttggcctttaattttgctgctagctattaaatttaaaagagtatcattgaagtaagtaatattctcatttctgaaattaattttcccctcccagtctctctctctctctttttgccagcacagattaaatggttctttcagatctgcaaacaataaaggataaaattatttatagggaaatgaggatgctgttttattgttggcatattgttccagaacataacaacattttattttcaagcaggagaggttagaccagggggagaaagagggggaaaggaaaaaacatgaaaggagggcaggaacccacacacaaaactcctgccatgtataactggtaggacatttacaatttctatatgacaactcactgtgatgtcataataccgagttcttgaattttataattctcatgaacctctcaaatgggtccaagcagtgcttcatgtggaggggtatagaagaagccaggaggctggggatcctttgacccagtgcagagcagcacaccccctattgcggcttcttcctcatgtgacatcctcttgaggccctattctgggggctgaaaatattctggatattctgcattttaatttttctcctgggccaagcagggccacttgctttgcccccctcaagtgtccctaggcatctaagctctctccccattcccagatcacagagagctgtgtccccaggctctccccaagccccctcctcagctaatactcagctgcttggaatagaggtgggaggcttgggcaccagcccccaaaaagccagaaatgattttttccagatggagctggaagggggctcagggctgagcgtgatggggtagagatgtttgggacctattttacgttttaaccttaagtcagagaagtgaattgagaagccaaacaaatgccaatgtgagagtttgtatctgctgatggtagcagcaataagtgaagtgctggtaaggaaaggtcaggcagaaatctggaaagagagagggaggagaggaaatgtgacatgagttagcagagcccttccatatacctttcttctccgtttaattgtaataaagcaaaagcagctcgggtagcctctcaacctcttagctcaaaagaggaatcaccagcgcaggccttggaggtgtttgggggcagttctcagcagcttaacatgcccaatctgccctcttcctcctttccccctccctgctgatccccagctcccttcaactggtcagcccgggccctgtccccaaaatattagcacccccaaatgatatccatttctgtgttaggtgtgtcaaatttcacttctctccatgcctaaactttgaaaggaggagtgtacctttttggaatgcggtgtgtgtagcgggggcaggtatgtgctcagacagcttcccccatcatatctatgggaaactggaagccccttaggtgagccatgctttggtgttcccaaacagcatt

SEQ ID NO: 125 - DNA, 8141 bp, Artificial Sequence
  subsequence of HOXA7
ggagctgagcagggtacaggacaacacaggagatgaagggcattgcggagggcattggacctccccacccactacagttaactcaagacaacataccatgctacaaagtcaccccattaacacatcctttccaagtcaagacactgccttacaaatgaactccaagactatagaaatgataaaaaaaaatcttgttcaaatatacagtatctgctattataggaaacatcagggcgtacatatttaacacagctgaacagtaagatacaggagccagaggaaaggacagcgaagctggaagcatctccacagtcctgctaagcagaagctaacccacagatctgcagccagctcaggaacattcccctccagaagtgggggttgatgggcctgagctgtgggtgccaagccagagaaggagggattgattctagggtgcaagcacttaggatgctttttggaataaatatattatttttcgatttaaatagatgccaataccctgatcctggacctcagcacattctcagggcagcctcagggaccccaaaagctgcgggctgtaagcagcaggggacttgcctgggagcagtcggcactaggtagcaggcaagccagccagcacaaaataggtagttttaggggagtaggtagtagtgagattcactttcttgcgggtctgggagggtggtgctgggtgtctgccagtgttgggatacatagggacttcctgggaatggaggccctctggggctggatacataggtagtttgggggtgcctcgagcagaggcctgtgctaggtagtattttggacgcgccagagcagggccggctggcctggggttgggggtgtcttttggggtcctcggaggcagagggaatccaaggcgacccagtctctgcggccgctcagtccacaaaagttgggagctggagtaggtgatgggggtgggtagagtgcaggttggggactgggttgcttttttgtttttgtttttgttttttacattttcttttatttttcccatttttgtaagtaaaaccagtgagtctcttaaagacgcttttccgactgtccggtgcagagagggccccggatcggcccctcattcctcctcgtcttcctcttcttcatcatcgtcctcctcgtcggccttgtccgcggcagcagtggcggcggcagagggcacggcgccctcgggagctgcggcggcagtcggaccttcgtccttatgctctttcttccacttcatgcggcggttctggaaccagatcttaatctggcgctcggtgaggcagagcgcgtgggcgatttcaatgcggcggcgccgcgtcaggtagcggttgaagtggaactccttctccagctccagcgtctggtagcgcgtgtaggtctggcggccccgcttcctgtcaggtcctgagaacagacatgcagacacatgaacacaaggacagacaagtagacagggcactcgttaggctgctgtcccagagcccgcaccttcctcctggcctagtccccagcgagcatccccctctgccccaggccccgaactgagctaggggaggagggggagtgttagggaaagaccccaactgcagtgccagacgcgcaggcagctctgtaatgagcaaaggcacagaatctcaactttacaaccgacctttccagccggctaagcttccacaatgtcctgcttcctctgacaaaggaaaactgtaaatatagagtgtgagcaagtgggaaacgctgcacttttgccattcaaagatgagcccggccattcccctgccttgctaggcaagtgggcgactcttcccagcagcctgagccctcatccccaggaccttcctagggcaccccgaccctctgtcctcattccctcgcccccatcttgaaatggaccctggcacagggtcgggtgagaggccctggagggcttggctctcctagcttttgagaaagaaatgtcaggcagcaaggaaaatgaggagagagagaagaagaaagggagggagggtgacagaggagggagaaagagagacagaatagcgaacaaacttaatgttaaaattccaagacaaatggagttaaataaatttacgaggatcgaacccattaattgggccataaaaagttttatgagcctcatttacatacaatgctatgggctccacgcaatggcgcctccgctccaattaaaaccagaaaggctgcgccgggagtcacggggctaccggctcgcaacagcctggctccgctcttccggccccgcgccccgcgctccgcgctccccagcgctgcgctccccgctcccggtcccgctccgccagcctggcccgcctagcgactgcgcctacctgaagaccgcatccaggggtagatgcggaaattggcctcagccgcgccatgcagcgcgccctcgtccgtcttgtcgcaggcgcctttggcgaggtcactgcagagcccggggatgttttggtcgtaggaggcgcagggcaggttgccgtaggcgtcggcgcccaggccgtagccggacgcaaaggggctctgataaagggggctgttgacattgtataagcccggaacggtcgaggcgaaggcgccggcgcccgccccgtagccgcttctctgtgagttgggagcaaaggagcaagaagtcggctcggcattttggaacagagaagcccccgccgtatatttgctaaaaagcgcgttcacataatacgaagaactcataattttgacctgtgatttgttgtccggcagctttcagtgtcggttttacgaggtagagtgatatatgataacattacacccccagatttacaccaaaccccattttcttttggacggagctcgccgcagcacgtgaccgcccacatgaccgcctccgccaatctcagcagtcctcacaggtggtctcgctccgcagggcccgcagccgcctagaatggaagggcaagaggctcaaatatgcggccaaagaatccgcccgcgcccggcgggcctggcgcgtcccgcggaaaaagacctggaggctccgcgggagcgcccagctggcggccaacctccgcactggggtctgcggacgccaggcggcccggccccacgcagcaccccccaccccgcccccccgccgactcctgctagtgagccctggaccaagcttgggatcctccccatccctctcctgtccgcctgcccagaccctggaagggtctctgtcccccgcaacagcctgccccgcggtggccttgtgggcaggactcagctatgagcagatcgactctgcccaagtcttctctcacccaggtccagtgggcgacaggccggacttagactcggatccagacggggaaggcgcagcatctcttgcagctgcagagagattgccaccgcaaactggagccatgtggttcgaataaagtcaacgtctcccagcttcctttccttaatcggaggcacactgtttatccgccctaaaggaagcagtgaaatatttatctattaatgagactcatttgccaacagatttattaacgtggggttcccctccctcctcccggacgctgtagtgctgcaggctctgtgccttcgctcctgggcacctggctggctccagcagtccgataaattgctaaagattcctttgtcctttccacaacttctggttcccctctggcgcatggggagccagggctgtttcccccagcttggaaaaatctcgggcctgcacccttccaggcactcccaatactggaaggtttctggggtaggccggggtgcctgggaacaatacatgctttagagcggatttggagagggggctctggcgtctagggactgcaacccactgtggacttccttttcttttgaagacaccgaaaacaaataggggaaaccaccccctaaaggccacccagctgtggaggcttcacctatccaagtaccagctcacatggagctgagcgcacagtggtctcacttcctcccatccaggcctccaattcctaccttccaggcctccgacccctgcaccatgttgcaccagctgaagcccctgccgcccaccgctcggtggaggatggtggggagaacccttcccctaaacgcctcataaactgcccggctgcgctggaagcccggccaccttttactgctcagctcgattacacaccataaacccgacctcacaatggaattgccccggaaattctcctgtaaattgtagagtttagttccttgtgtactgagcacttcccatcactttcagagggtccaggccgtccccgtttaccgcaccctctcagggggccccaggaatacaaaaggtggagggagggttcagatcgggacgccacggagccccagttcctgcgcagtgaaccaccggggcttgggtaggaaggcgggggctggtggggcaggtgggcgctgggctgtctcctcccgggccacggaagcctgggggtaggggtgtggagtgagggacaacatccggggacgcctttatggcggatcagatgataccttgtctccgatggagaatagagggagtaagacaaaaagaaaagacctaaataatcccagtcgcatcgccttctggaaggaaataaaaacccaagaaagttaaaggaagatgaagcaaacaagaaggctaggagatcaaagaggcagaattagaccgttttagaccaataaatttttcctggggtgacacacagcaagacgcaaagagaaaagaccaaggcccccgccgccgccgtctgtctagactcaagcgactgaaggggccaacagagctggtgtttaaagtagaacctgcccagtccaacagcccgagcagggagcgatttcggggatcgcgggaaggaacgcacttcgccaagggagggccgggtgccctcgccaccggctcattcctgctccggttttgcccgatgcgcgtccaggaggttctggcaggacgcactgcccctctgccccggccaaggaggatgcggatactgcccgcaaggcttcggcctttatggacccaagtcagccaactgggccgagtcctgcggacaccgaaacctccctttcgtttccaggcttccttctcccctcttgccctctgtggtctgatttaaaacgaaaaggtcggataaaatcaggctttcaataaggcttctttaactgtgtgttctctattcattggttctctacttatttgactgaaaagacacaaatgcactaggttatgtgagataattttcacagaaatactcattgaccctcagcctgaagcaggcacatgtaggcgggtttctaatcagtagagctatgtttagatagacattttccactgccgtccctgagcttccttcctacctactggcagagcgtgttcactctgcttcttgttaccaaataccaatatttaaattcaattatgaaggtaaagccagctctaggcagggaacagcgccttccagagatttgggtggcaggcaaattgcttcctaaaggtttccacccttgcctctctcaccagctgcatctgttccccatccagtgagtgagtgatccctagcctgggtgcaaagacaaactcgtacctgtcgtgtacaaatgagattgggttggtgcggggtcttgcctgggtgaaggtccgcagcggggaagccactcccaggcttcccagaggaaaagcagactcccagccaccagcctgccaagggcaagggaggagcctttggacagtccacccaggcctgggagaccctgggcggcctgcacctacctgaggcctccgtgatcagtggagagacgcagtcgccaccgatctgtgacttcatttatttgtagttacacaaatcgagctttctctctgcatccacggatctgcgacttcactatttatttgcagttaacataaattgagctctctatctgcggcttgaatacaaagccacggttgactcccagggaagctataaaacccttcttacaatcagacgttgtgaaattatatacggaaatgtaatgaaggtgtgtgtctgtaatatctgtatctatctatctatctatccatatatatatgtatatgtatatatgagatgagagacagagagggagagagagaaaggagagatattgtgtgtgtgtgaaaggaaagagagaacaaacacccgggagagacatcaaccaaaatccagtccccagttttacagcgtgaaagcactgggatgcgggtcgtaaacattttgtgggcttggcggagactattacgacccaaataaatgcactgtgtagcgtgttcacagggctccggggcctttcgaaaggttctctgtttgcttttgcgttttgcctctggaaccattcgacatccgtggctgatgcgcgcacccgagaggaggccgaagcgtgttccccgcctagggtctgggagaggctgggcctggattggggtcccctcccttctggcctcctgatgggtgaacgccagagcagcctcggttcctgtacagcggagggcatgccgcggccagagacagcccgggcggcttccacactgtgtgcgacacttttggtgctacggtgtgattgttatattaaacatcacattaaaaaaataaccaaagcagtccctggtttgtcccccaggattctcctcccagccaactcggcccggcccctatacctacagtggtcagacaccgagattgcctttacgcccaattttcaccgcctaattttattgtctcgattcaagccagccgagtcccggggtcctggctctgtcttgggttctggctcgccgggccctgacccaggtcgcaggtttcgggggcctcctgggcggccgcggaccccgcggtcacggtgtgagccctcggcacgcaccgtgcacaccctctgggcggtcatcaagttctggggctgcaggcgttcctcctgtgtccgccagtcagccggggctctctggcgcctggctgtgtcaggcctgtcccagctgaggacggtgaccctggagccgcgcccgcgcctggagctgcagccccgcggccgcccggacagctgcagcccggcagcactgggcccccgggatggggtcagggaggcgcgagcggtgagggtcgggcaagcccccgccgattccttgtttcccagcgaggcttctagccaggcttgagcagcccagaaaatatagggcggctgttcactaaaatctggggctcccattccagaaaggctcgtgtcaagtcgacatcttaggaacttcacaagggtcgcggaggcgggagatggcggcgcggaagcctcttgcatggagccacactgccatctgctggccgccgtttggtactgcagcctcagctacctccgccggcctgagctttgggagccgccggctagcccaccgcaccccactcccaaacgaggggcgtgggcctaggtcccggggagtctgcgtggagcccggaatctactgcagaggaggcaatgccaataaaagaggtgtttccgcagccgctttatcggcggcagacagaacaaatgaacaaatgaaagggctttggtggaatatcctaattggggctggacagttgtaaactcattaagggacgaattccagacagttcgcagacccggcctttatggcacactcttactgcctattctttgaagttccttctgtctgcaacaacagagggcgtcccaacctggcggcggggtgggggtgggggttaggggacgcctcatccacccgcgccctggttccccttttaagcttagaacacatccaactttgcagaagtcgtggagtgggggaagggggtcgggcgagggaagcaagggggtggaagcgaggccgaaccctccggccacatctggaaagcgctcaggcctccgaagttgtggccgttcccccccccccgcccctcgtagccctttacaccccataaacggtaacagccctcattttcttttatggcgcttaggggctcgtcaattgcctcagccctgcctctgttaggccttgtgctcgagaggtgcttgcagtgcaggacccagattctcttgggccaggctggcaggactccgcgggggtggcgggcggtgcgaggatgcagggctttgtt

SEQ ID NO: 126 - DNA, 7667 bp, Artificial Sequence
  subsequence of BST1
aagtagttgttacattggattatttagggaatgatgacaaggaaaaaaaagtccgtacatgttccgtacagatgcaagcattctttttttcctcaaatgtttctcatccgtggttagctgaatttggatgatgaatccgcaaatctggagggccgaacatgcttaacttccctgagtttatccattgctaaagcgagagaaattacaaacttagctaggaagggtgttgcggaaagtaattaatattatacttgcaaagtgcttggcacgttgttgtggttattatttcctgaaaacaaacaaacaccacttattggttggtgtgaaagagggcatctgtcaaagttgtcgtcctttggagccagaaaagtatttcttctgatgatgactgacctctcctcacctctccttcaaccttgcggcttctttggggctccctccccgtggacagcggtcaagattagcctgggccacagtgcactggtcctgtcctgggtgatgttccaagctcactcttttttaattttatttatttattaattttttttttagacagagtctcactctgtcgcccagggctggagtgcagtggtgcaatcactgctcgctgcagcctcgatcccctggggtcaagcctcctcacatctcacctcgcaggtagctgagactacagatgcgcaccaccaggaccagctaagttttgtatttttttgtagagaggaggtttctcacctgtatgttactcaggtttgtctcgaactcctatactcaagcgatccgcccgtctaggcctctcaaagtgctgggattacaggcatgagccgccgcgccccgccccacgctcagtcttgaaattgtctggaacgggaaacggcaaacagcgagatatccgagcgagagtcccgccctgcatcagtttgcggaaccgccttggtagaaggagagaaggggagtggaggaagcacgggactggagggaccaaagttccccgatggcggcccaggggtgcgcggcatcgcggctgctccagctgctgctgcagcttctgcttctactgttgctgctggcggcgggcggggcgcgcgcgcggtggcgcggggagggcaccagcgcacacttgcgggacatcttcctgggccgctgcgccgagtaccgcgcactgctgagtcccgagcagcggtgaggcagtcggccgggtggaaggggagccggaaagaggcaacggtggggagggcctggggaggggaaaactggcgctaaagttcggggtgagggggcaatgagagaggccttgaggggagaggtgagtgtggagacagcgatggtcctgaacgatgggggcgagtgaggagggggctgtgaagtgtgtctgcaggtgaggggtgcgctgtgcggggtctagagatgagtgtgtgtgtgtgcgcgcacacacacactgtagaggtgaggggtgtgtgcgtgtgttctagaggtgaggggggtgtgtgtgtgcgcgcgctctagaggtgggaggtgtgtgtgtgctctagaggtggatgtgtgtgtgtgtgctctagaggtgggggtgtgtgtgtgtgtgtgtgctctagaggtgaggggtgtgtgtgtgtgttctaaaggtgagatgtgtgtgtgtgttctagaggtaaggggtgtgtgtgttccagaggtgaggtgtctgtatgtgtgttctagaggtgaggggtgtgtgcatgtgtgttctagaggtgaagggggtgtgtgtgcgtgcgctctagaggtgaggggtgtgtgtattctagaggtgaggggtgtgtgtgttctagaagtgaggggtgtgtgtgttctggaggtgagatgtgtgtgtgtgtgttctagaggtgaggggtgcgtgcatgtgttctagaggtgtgtgtgtatctgtgttctagaggtgaggggtgtgtgtgtgtagtctagaggtgacaggtgtgtgtgtgtggtctataggtgagggatgtgtgtgtggtctagaggtgagggatgtgtgtgtggtctagaggtgaggggtgtgtgtgttctagaggtgagggggtgtatgtgtattctagagctgaggagagtgtgtgttctagagatgaggtgtgtatgtgtgttctagaggtgaggggtgtgtgtgtgttctggagttgaggggtgtgtgttctagaggtgagatgtgtgtgttctagagatgatgggtgtgtgtgttctagaagtgagaggtgtgtgtgttctagaggtaagggatgtgtgtgtgtgtgtgttctagaggtgagttgtgtgtgtgttctagaggtgagatgtgtgtgtgtttgttctagaggtgaggggtgtgtgtgtgtagtctagaggtgacaggtgtgtgtgtgtggtctataggtgagggatgtgtgtgtggtctagaggtgagggatgtgtgtgtggtctagaggtgagaggtgtgtgtgagtgtgaaggagggtggagaggtatccctctagaagtgagggtggggtagaggtgaactgggtaacagcccattgccacccagcagatgtttagtctgaatactcagaacccagaatgtgatctcaggttggaattccttgagtccagtccttccagaattcaaatttcagatcccctaaatctggaggatttctgaagtttgggtctttcttgccagtgctgcatttcttactgatttttgttccttctgtggccccccttttcttatgtttgtgatgtctttcttgtgctgatcatttttattgtcgcacatttcaggcaaataagaaacagcagagaaccacctgtgttacacaccacccagtatgagaaacaaagttacaaatgctatgggaaatattttttgaaaactagcatggacctcaagaggggcttgcactggagggtgcacctgctttgccagaggtggaagccttttgcagcattgggcctccctcctaacactacacatcctgctggctggcctggcctcacctggtccccgagctccacactggaactggactatgagactggccccaccgttaggtctaaatgaagaggcacctgctgtatagttgactgaatttgtcacctcctgctcggtgccatttctgcttgtctccgtgagcctggggcaaggctgtattccttagctctgagaaatctgtgcagtgccttcagagagacaattccagtgtcagatttctgaatctgtcacctaagccatgacaattcgttgtcttttttgtaagcctacttctgcagttactatatgaaaaatctcttgtaaagctcttagacaaatgggcatacttcacaacacattatgatgtgcatgtgtgtgttcttcccaacttgtacttttgcacaggaacaagaactgcacagccatctgggaagcctttaaagtggcgctggacaaggatccctgctccgtgctgccctcagactatgacctttttattaacttgtccaggcactctattcccagagataaggtaacaccacaaccatcttgggtaaaactgtgttctctgtctctacagaaatggatggtgcatgggccaggttgacattagctgtcccctgcatcctgcaatgtcacagaaacatcaggcagcacacataatgtgtgtgctgagctctctgtgggaagctagctttgtttctgtattagtccgttgtcacattgctataaagaaatgcctgagactgggtaatttacaaagaaaagaggtttaactggttcacagttccacaggctgtacaggaagaatggcaacatctacttctgggaggcctctgggagcttttacttcagcagaaggcaaagtgggagcaggtgtcttacatggcacgagcaggaccaagggcagagggaggtgccacaggcttgtaaacaactggatcttctgagaactccctcaggagaacagcagcaaagggggaaatccacccccataatccaatcacctcacaccaggccccacctccaacataggggattacaattttacaagagacacaaatccaaatcatatcagtttccaatagtgattgtagatctcccgctggttgtgggcagaagaaaatttcctaagttagcaagttagtgtgagaatcaacatgaggacatcaggacatggccatacctgtcacactgggcctccacatctggccagttctaaataaccttcatcctaactggcccaatggcctgaaccttgagtaattcagaaaactctcaatctcagtatcctcccgggagaccagtctctccatttaacgggtcttaagattatatttatttagtaccagtttatttaagaaaaccacatatctatattctgtatacactctcaggtctaataaaatgaaaataatgagaaaatttccataaaacccttgcttaaaacaatacctcaagtttaaggaatgctagacaccatttttgtttctgtgacataaacattgttaacctgattttttccattgtgtgttatttgtaaaggcaagtaaatggaactgtgaggttcaaagatagaatagactgaaaacatgatttttgagtatatgctgtcttttgaaccttgctgccctcctgtcactaaaagtggggaagctgactttttaaccttctgtttcatagattcggtgctagttgatgaactcagtaaatacttccggggctatttgtttgccagtcattggtgctaagggttaaggatgtaacagtgaaaaacagccctcacccttggggaccttctagtctaaatataaactgattggactactgagggtcagatgaaatagtgactgggggatttgtgttattgttatataaaaacactatggtggaaactataaagtataatataaaagcaatgtgtttttgaggcacttgacactttaggaagtgctttttgtgactgcttattatcctggccacagctctggaagaagagaaagggctcatgctctgcattttccagaagtagaaactgagaaacagggagattgcatgccttgctcaagattacatatctaatacatgacagagccaggattccagcccagttcccttgatcatttttaatgtaggggatcttaccacatgcacgtatatttagtactagtgagaaaatattccattaacatttgcatgataccctgggaataaagggaggagagatgctagcagtctttgaatgaataaataaagacaacgaaaaagaacgttcagttgttgtgcagcaggtcagagttgaatgagaactggattgcccaacttgccttgatgatattgtgcctgaggagtcggttttgattctgttttgtattttgatgttttgtttgtctttccttagtccctgttctgggaaaatagccacctccttgttaacagctttgcagacaacacccgtcgttttatgcccctgagcgatgttctgtatggcagggttgcagatttcttgagctggtgtcgacagaaaaatgactctggtaagactcctgcacaaatcacaggagacttaagaactcctatttactatgcattaccatttgtgctaaatgctttcatatgcatttatttcacttgatcctctccaagtcctctgagataagtggcaagaatagttaataataacaatactagagaatacttaactttgcaggtgccagtctaagcactctctctctctctctctctctatatatatatatatatatacacatatatatacacatatatatacatatctatacatatctatatctatatatacacacatactcatttgatgcccacaacaacctcatgggatcctatcataatccccattttgataaatgaggaaactgaggcacagcaagattaagaaatctgctcagggggcatagctagtaagcagcagacagtctgactccagagcccattttctcaactttgcacaactctgccttactatcctcatttgtccagagggggaagctgaggcttagggaggttaaatgactggaagtggtaaggctgggtctcagtcctgtcctgatggattctgaagcctgtgctctgtaacaccactccaggccgccggcagatatttcgagatccaagtcacaaggaaagttagagtcacaagagctggcctgaatgttctgcaaacactcctcattcatccaactgtggtgctaggagctggagacacagcagtccccatcttcagggaggttatagcctcatgggggatatcagctcgagtgatatgggctataatgcaggaaaaatggtgttcgaggagtagcagagtgagacaccagcctccaccagatcatcagggaagcttcagaagggaggctagcaaggaaaggaggttagggagtgtttccattatgaagactggagatccttcctgggtatcagagttacttcaaaagttaacctaatatcaggccgggcatggtagctcacgcttgtaatcctagcactttgggaggccgaggtgggtggatcatttgaggtcacgagttcgagattagcctggccaacatgaagaaatccaaactctactaaaaatacaaaaaaattagccaggtatggtggtgcatgcctgtaatcacagctactcgggaggctgaggcaggagaatccctcgaaccctggagaaggaggttgcactgaggcgagatcataccactgcactccagcctggatgacagagtgagactcggcacacacaaaaaaaagagttaacctaatatcagttctgtttatttctcctccattcatttgtccatcaaactaaaatttatagtgtctactatgtgccagaccctcatcttctagacagtaggaaaacagcagagaataaaacatgaaattaataccccatgcttacattataggagggcagataagacaataaacaggcaagtgaaatatacagactgccttaagattataagggctatggagaaaattaaaacaggtaataaggacaaaaaagattgagggtggagggccagggaaaggaaagtgttgcatttttacctagatgccgagggaaaacctcactgataagctgatatttgaacaaggacctgaaggagatgagaaagagcattttctgatgggagaacagcaattgcaaaggccctgaggtgggagcgtgtgtgacatatttaacagcaaagaggacagtgggcaaagaggaaagtgtgagctatgaggctagaggaataaaggagggccaggtggcacaggatgttgtgaggcctctgcttttcactgtgagtgagatgggcagcattgcaggttccacgtcaaatggacacagccattctttcaatggagaacttccaggaagcttttgtttgatgatgctgcagagggtggggagaaggaggggaggaatgtgatgaaaaacacataaagaaagggagagccttccagaaaaccaccagttatttcttcttcacctcgctgcccttttctatctatgccctcctatcagggctctttgtttcagaaagaagtgaagtccagcagttcaggtcagctaaataaccatatgtgtatgtcatggaatcctgtggggccagcagcaatggtgatggggttttttatttattgacccagaaaggggcatgtttttaagcaaaaaataaatttacat

SEQ ID NO: 127 - DNA, 7594 bp, Artificial Sequence
  subsequence of C1orf114
ataaatcatgattttactatttatttatattatttaaattataattttataatggtcactttagtttattaaatgctagcgtaataactgttctctcactaacctgccctatgccttaggatacaacatttaagcaatctacgcctcatttttcttatctttaagatgaggataatagtaatttgcccaatgtagatcaaagaaattttgtgatgtttagatgagataataatgtgaaaaccttaaagaattgcaaagcactttgtaatataattattatgaatgctgttggcaatatatacctctattatgctggcatcacttttttcattttcattaattaaccactccaggtccttttcaaagtcatcttcgtattcttcacttttctttgaatcagtatctttattttcattcattttctgtttgtgaaggaaatatgctgtaagattttaaaagataaggtatatgttatgcccactctagaggaggaatggagtatggagattaatgctgtaggtaagctaattaacacagagaaacacaaaatagaatgttcaaaatgaacatgcacttgaatacaccatgaaagagagatctgcaatggcaagacatttccataggtaaacattcctaaaaactctcccaccttccccctgttccccaaatagttattgatgttggttccttttccctctcaagataaagttaatttttggtacactttaggtatgctgaattaataaataatccaccagctgttttagccattagcttcgctttgttctccccaaacctttggccagactaagttattactgaataataactgttattcaacttaattattattcaaaaataactgttaattgttcaactggataattattgtttttttctaaactattcattggactataattctttctagatacttatttattttaaactaaaaacacaaaatagatttgctaaaggactcaaaagtaagcccttcaataatttctaaatcaggttgagcacaaattttgaagtgatctggagaaatcaagtcaacacttcagagtgagtttcacttcctaactgcaagacaagctaaattgcttaagctattatatctaactacctaccaattaaaagcaagggcaccatgaatgatacagaataaaactcactgtaatccgaaatacttacagtaaaaatagtacttttcacagtcacaatgccttggaataatcagttttcttttcagagcagggatcttgaaatttattattttaagatgtttgagttacataaatattataagaatatttctttggaactcttcagtgctttcccttattttatgataaacatagttctgaacttataaataaatggttgcctgaagactttagtagatatgttttattgtttacagagaatcacacacacatgaaaactaaaatttaaaatgaaaacataaaatctgtataataaaagcacagtaattaaaaatttaacaggttaggggtctttaagtcatactattatgccataattcaaaggaaaaaaaagccatagttaaggtaactctgagaagtaaattaagtcacatcaaatctgaagtgcaattcttttgttgtaacttaaaaacaaaaaaacaccctcatggccggttctcaagtaaacaaagaacataaattacaaactctggttatcaaatcccttaagcctttttcaaatgcgtcacaggatattcaaccccttcaattcttttaatcttcatcaccagggtactgtccatatggtacagaatcaacaagctagaacaaaaatacatcttatacaaacaaaatcacttaacacttcctactttatgcttgtgagtttcacacatttaaatttcaacatttatcatcagtaaaaatctaggtaaacggcttagaccagctctaccctcttaatacggaactgtagtaagagacggaaataaattccttcctccctgagtgtctggtaaatcccatgtggataggtgaactgccgatctttcagtaggagtcttaaaccaagtccacatgtatacataattttgataactttcttccagaattcaggatattcaaaaatagtttaaataattgggtcccatcttacagcgttttaaacatatgcttgcttaaaaatctaagaactgaaagcatgtcaaagagaatgccttttaatataaagtaagtacttaagcaaaaactaatccatacatcatgaaaccatctggcccattattcctgtgtatcctgccaagactgtgatcctataagtaagtttttaaaaaatcataaactgtcacaaagtatgatgataaatattttatggactttaggtgataattttaatctgtattcaggatcccaaggtaccaccaacgaaatgaataccattgcctcctcatggaagctacaatttcgggagtgactttttctcccagggacaaaattattactttccacgttcaagaactttgagaggggaaagaatatgacaaaaatttagtctaagctactctcagacgagtatccttcatacatagtgaagaaaggtgttaccagacttccccaccagtgccagactcggtggacctcggactccagaggataaggcgccaccagaaagcttcttccctcactacctaccctccctcccagctataccagacgtttatacctttaccctctatcccaccattaacatctccgcatcgtccttcccttctctccctctatatccctcttgcctgtgtaaaatgcggcggctgggatcacagagatggccgggggagttctcctctcctcctctttctaagctcttcacattgaggcaaaggagaccccggcacctgcctccgcggcagccaggaccacactgccatggcaacagcgtgcctctgcgtcctccatccgggcctctctaactacgagagcgacaaaaatctgcgcaggcgcatgcaatatcctcagaccaccgacccctcccggcacccatcccggtgcttgcgaagggccagtgaagctgaggtttctaaggggacgactaaggaatccacgcatcactaacgttatagagactcgcgaagtgccgctgtgttggttgtgaaatttccctcttgtagctgtctctcgtcagatttagaatttcttaggacaacttctaaaactatatttctatatgttatgtgcttcacagttaacgtagaaaagtagtttttagttttcattagtagataagcaaattgctaatgagttaccatatttttgaccctcagcttctttttttcctaatcaaaaccaaaactttacccaagagagttgccaaagaaaataggatttttgctctagctttgaggcatgtcaaaatggtcaactagaattttctcaaattctgcttatctttatgtataaaggcaaagcaagatgaatttagattgtggtgaaagttgagatgattttaacaactatccattcccagccagaaataaataagaactgggagaagtaaaaatatttcctcagtacaatccagtgtgttcggattatttttaaattgtttattattaggatttctatcacttgatgtgatggagagcaccttttctccaagagaggcaatgtaaaattaaatttttagatattcttcaagttatagacttaaggtcttttaaaatggaaggttaaaatgaattgtaatattgagtgcacttcctagatgtggtgtagttgtaatgacctaatgttgctactgcttcagcgcttgaaaaaagacgctcccaaaaaaggttattcactgctaaaggttgaaggaattttagtcaaatctcctttaatggatgtagagttgtagagttacttaccaaagctggaagtagaccctaggtttcagaactcctaggttaatagttttttcctctgaccatcctcctaaatttgtatttttcaaataatgggtgatagcagctttttttttaagtatcaggttttgggggaacaggtggtgtttggttacatggataagttctttagcggtgatttctgagattttggtgcacccatcacctgagcagtgtacactgtacccaatatgtagagtttttttgtttgtttctttgtttgtttgttttgtttttgagacagagtctcgctctgtcacccaggctggagtgaagtggcacgatctgggctcacttcaacctccatctcccgggttcaagcgattcttgtgccttagcccccagagtagctgaaactacaggcacgccaccacacctggctaagtttttgtatttttagtagagatgggttttcaccatgttgcccaagctgttctccaacaactgagctcaggcagtctgcccacctgggcctcttaaccaatatgtagtttttttatgcctcatcctgctcccaccctttctcccaagtccccaaagtccactgtatcatctttacgcctttgcatcctcatagcttagctcccacttacaagtgagaacatatgatgtttggttttccattcctgagttacttcacttagaataatgatgaaataacctccatttccatccaggtagctacgatgccacaatttcattccttcatatgactgagtagtattccatggtatgtatatgtaccacattttctttatccactcgttggttgatgggcatttggtttggttctttatttttgtaattgcgaattgtgctgcgataaacatgtgcaagtgtctttttcacataatgacttcttttcctctgggtagatacacggtagtgggattgctgcatcaaatggtagatctacttttagttctttaaagaatctccacactgttttccatagtgattgtactagtttacattcccatcaccagtataaaagtgttccctgttcaccacatccatgccaacatctgttgttttttttattttttgcttatgaccattcttgcaggagtaaggtggtatcgtattgaggttttgatttgcatttccctgatcattagtgatgttgagcattttttcatctctttattggccatttgaatatcttattttgagaattgtctattcatgtccttagcccactttttgatgagcttattcgttttttccttgctgatttgtttgagttccttgaagattgtggatattagtccttagttagatgcatagtttgtgaagattttctcccactctgtgggttgtctgtttactctgctgattatttcttttgctatgcagaagctttttagtttaattaagtcccatctacttacctttgtttttgttgcgtttgcttttagattcttggtcatgaagtctttgccaacgccaatgtctagaagggtttttccaatgctatcttctagaatttttatggtttcaggtcttagatttaagtatttgatccatcttgagttgatttttgtataaggtgagagatgaggatccagtttcatttttctacatgttgcttgccaattatcccagcaccatttgttgaatatggtgtcctttcctcactttatatttgtgtgtgctttgtcagagatcagttagcttcatttcttggttctctattctgtttcattagtctatgtgcctgtttttatgccagtaccatgatgttttagtgactatagccttgtagtatagtttgaagttgggtaatgtaatgcctccagatttgttcttcttgcttagttttcctttggctctgcaggctcctttttggttttatatgaatttgagggttgttttttctagttctgtgaagaatgataatggtattttgatgggaattgcattgagtttgtagactgcttttggcagtatagtcattttcacaatagtgattctacccatctatgagcatgggatttgcttccatttgtttgtgtcatctatgatttctttcatcagtgttttttagttttccttgtagagatctttcacctccttggttaggtatattcctaagtattttattttttgcagctattgtaatggggttgagttcttgatttgattctcatcttggttgatgttggtatacagcagtgctactgttaccggtggagggtgtccatgttcttggtattttgaacaaagaattggaaaaaaaaaaacacacaaataaagcaaggaaagaatgaagcaacaaaagcagagatttttattgaaaatgaaagtacactccacaatgtggcaacaggcatgagcagtggctcaagggctccagatacagaatcttcttgggtccaaatacccactagaggtttcccattggacactttacattggttcaccccatgtaaatgaagtggtggcccgcaatcagtctgattggttgtggaaagcaaccaatcagaggttgaagtgaagttacaaagttacactcctatgcaaacattacactcctatgctctttgcaaccaatcaggggtactttcaatttcccatctgcaggaaagaggatttgccaaggaagtagcctctggtccttttgttacttaaacatggcaagttagggttttcctttcaactgcattctaggaagtcagtgtgaaatggccttaggttcactgactccagaccctattctcctgcctcactactgatttgtgtacattgattttatatcctgaaactttactgaattaatttatcagttctagaatctttttggatggttttctagtatatgattatgtcactgacaaacagcaacagtttgatttcctctttaccaatgtggatgccctttatttctttctcttgcctggttgggatatagcagcatgattggtagccaaaagtggaaatgactcaaatgtccatcaaatgatgaatggataaatgttatatatctatacaatggaatattattctgcaataaaaataaatgaagtactgctggaggattctaaaaagatggtggaataggaagcaccaggaatctatctccccacctggaaaaacaattgcactgtcaaaacctatctcttgtaactattttggaactgtggagtctattaaaggcttgcaactttcaagggaaggcttggacagaaaactgaacttattttggtgaatttcagctcttagttcagtatcatctacccaaccccaaaccccagctccctagcaggcagtctgtattacttgcaggagcagctttaacatagttcatgagagtcaatgagcagtaaggaccctgtcctcctattgatgagggtctatgttctgataattgattactgcttctgatcaaggagatgcaaacacagaggtagccgccattgttgttgcaccttcccccaccattgtaagcttttactcctccagctgaagcaacttccagggaattttccttgttttcttccttttggaagacaaacattaaagactaagacattaaaaagcaactacatttacagagaaaagtataaagttaaattgaacacccagagaaaggcataaactcagaaaaatacctgagaagaccttaaatcataaagatgctcaaataactaaggaaagatgtggaga

SEQ ID NO: 128 - DNA, 5644 bp, Artificial Sequence
  subsequence of FOXG1
ttccaattcggattagaagctgaggctggagcggcgaggagaaaacgacatcgagtcaccccgcgcgtgagcgacgctctggagcaggagagaaggaaaaggaagagacacacgtatatagcatgtgttacctgatttatttcgagattgtttggtactgttttctctctgggcacctctcatttcggaaggccatcagaggcgcccactactgagcggccccggccgccgcagcagcacccggagccccagtcccggtttccccgcggtgccggagcccggagctcgccgccgcccaggcctcaggaatcgagtaagtaacccctgtttggccccgcgctcctctgcccacttcctcctcctcatctcatcgctcccaaagctctcccacaccctcctcccccgaagtaaaggacacccccgcacacacgccagcggtgggccttatctccccccttatccaaagctgcgctagactattacctacaaagggcacaattttcctgctggctcagaaatgccagacactggcctgcaaggccgactcggaaaagtagtgcctcgcctctacctcctccatttcctgccctctcgcatcctctccctgcactcccactcttcccactaccaccaccacccccgctttcaaaaataaaattggatacaaactttaatcactaaggacaaatattgacgcttaaacgaaaatgacccagtacaatgaggaggaagccggaaatgtgagctattggccctaggaggggaatttcggtggagcggagccggcggggtggagggggtggcgggggcgcagggaagggctgcggcaccgcgtgctcccgccggcgtatccctacgcggctccgcgcggcctcggggtccgaggcccgcggagagggggaggcgagcgcccgagggggcggcagccggcgggcggggcgggggtgggtgggcccggcccctccgattggtcgacggcgagagagacgctcccgcacgccgccagctctgattggcccagcggtaggaaaggttaaaccaaaaatttttttacagccctagtgtgcgcctgtagctcggaaaattaattgtggctatagccgcctcgatcgctgtctccccagcctcgccgcggccgctccgggacgcgcccgcccgccgcccggctctccccccctttgggctgctgctgctgctgctgtgactgctgctgcgagaggaggaggaggaggaggaagcagcgggggggggagcggggggtggggggggagaccaagaagtacagttgggagcgagggagcttcacccccggggcggtggttgtttcttttttctttctttcttttttcttttcctttttttttttttttctaattcctgaggggtggttgctgcttttgctacatgacttgccagcgcccgagcctgcggtccaactgcgctgctgccggagcgctcagtgccgccgctgccgcccgcgccccccgcgccccgttcggcacccaccggtcgccgccgcccgccgcgccgctgtcccgctcccgcgccgccgccgccgtttccccccgacgactgggtgatgctggacatgggagataggaaagaggtgaaaatgatccccaagtcctcgttcagcatcaacagcctggtgcccgaggcggtccagaacgacaaccaccacgcgagccacggccaccacaacagccaccacccccagcaccaccaccaccaccaccaccatcaccaccacccgccgccgcccgccccgcaaccgccgccgccgccgcagcagcagcagccgccgccgccgccgcccccggcaccgcagcccccccagacgcggggcgccccggccgccgacgacgacaagggcccccagcagctgctgctcccgccgccgccaccgccaccaccggccgccgccctggacggggctaaagcggacgggctgggcggcaagggcgagccgggcggcgggccgggggagctggcgcccgtcgggccggacgagaaggagaagggcgccggcgccgggggggaggagaagaagggggcgggcgagggcggcaaggacggggaggggggcaaggagggcgagaagaagaacggcaagtacgagaagccgccgttcagctacaacgcgctcatcatgatggccatccggcagagccccgagaagcggctcacgctcaacggcatctacgagttcatcatgaagaacttcccttactaccgcgagaacaagcagggctggcagaactccatccgccacaatctgtccctcaacaagtgcttcgtgaaggtgccgcgccactacgacgacccgggcaagggcaactactggatgctggacccgtcgagcgacgacgtgttcatcggcggcaccacgggcaagctgcggcgccgctccaccacctcgcgggccaagctggccttcaagcgcggtgcgcgcctcacctccaccggcctcaccttcatggaccgcgccggctccctctactggcccatgtcgcccttcctgtccctgcaccacccccgcgccagcagcactttgagttacaacggcaccacgtcggcctaccccagccaccccatgccctacagctccgtgttgactcagaactcgctgggcaacaaccactccttctccaccgccaacggcctgagcgtggaccggctggtcaacggggagatcccgtacgccacgcaccacctcacggccgccgcgctagccgcctcggtgccctgcggcctgtcggtgccctgctctgggacctactccctcaacccctgctccgtcaacctgctcgcgggccagaccagttactttttcccccacgtcccgcacccgtcaatgacttcgcagagcagcacgtccatgagcgccagggccgcgtcctcctccacgtcgccgcaggccccctcgaccctgccctgtgagtctttaagaccctctttgccaagttttacgacgggactgtctgggggactgtctgattatttcacacatcaaaatcaggggtcttcttccaaccctttaatacattaacatccctgggaccagactgtaagtgaacgttttacacacatttgcattgtaaatgataattaaaaaaataagtccaggtattttttattaagcccccccctcccatttctgtacgtttgttcagtctctagggttgtttattattctaacaaggtgtggagtgtcagcgaggtgcaatgtggggagaatacattgtagaatataaggtttggaagtcaaattatagtagaatgtgtatctaaatagtgactgctttgccatttcattcaaacctgacaagtctatctctaagagccgccagatttccatgtgtgcagtattataagttatcatggaactatatggtggacgcagaccttgagaacaacctaaattatggggagaattttaaaatgttaaactgtaatttgtatttaaaaagcattcgtagtaaaggtgcccaagaaattattttggccatttattgttttgtccttttctttaaagaactgtttttttttcttttgtttacttttagaccaaagattgggttctagaaaatgcacttggtatactaagtattaaaacaaacaaaaaggaaagttgtttcagttggcaacactgcccattcaattgaatcagaaggggacaaaattaacgattgccttcagtttgtgttgtgtatattttgatgtatgtggtcactaacaggtcacttttattttttctaaatgtagtgaaatgttaatacctattgtacttataggtaaaccttgcaaatatgtaacctgtgttgcgcaaatgccgcataaatttgagtgattgttaatgttgtcttaaaatttcttgattgtgatactgtggtcatatgcccgtgtttgtcacttacaaaaatgtttactatgaacacacagaaataaaaaataggctaaattcatatatatcttgatacttttgtctcttttattaagtagagctaattttttaaagaccaatcaacttatagggaattcaaaggctttttcagccaaactaaaatttaaactgctcctttaatttgaactgactctaaaaatgaaaatagtatttttccctttgtgaacaaattttacaaggagcagcctatttaataaacactagctttaaacaaagtataggcttttcagctgatacctgtaagtttctgtggatatacagcaaaaagagatataatttaattttctgtgcatagctctttaccctgtgtttatttccaaatccattaatagaatgccatttatatattttgtttcaggtatattgttaatagagcttggcaaattataaataaatatatgtatatggttagatagaagtgactataatgcacacatatgtaatatatatagacacacagagcccttcagttcaggtacaatttgcgctatgaatgctgcaaacatttttgtttaaatatttgtatttatactttctaagtcagcatttatttttgtggctgtttacccacaatgaaagagttctaataaagatgtgctgaagttgcaatatagattttgctgaagtgatcacctgtttaatgacttgcagatcaatgtttatattttattttaaaattataacaatttagaattctagatattcagaagtaaaatgcctctttttttaatttttacaatgtagaggtatttatttgattcccttttaaatgtctgtgtaattcaatctagagatttgttccttttgtttagtcataattttaactttccatatgcatatgtatgcatatactgtatatgcgtatatatgtgagacaaaatgaaaacattttttgaattgtttcaggcagcccaatcgctataattgcagaaaataattagaaaaccttagtaaaaggtttagtaactaattggatcctgtggtgaatctgtggaggacaagttgttcatttgttacaattgtatagtctgaaatgtgttctgcagtattggaataagctggttacttcttacaatgggcccagtgaaaaataatctggccctaagatgttatcagcaaacacttagacagttgctcagggggaggaaaaaaaaaaaaagcctaagggagaagcaagcttactggaatagatttgaaactgaaatgctgaatacttaatattggaaaatagaagggggtggactgtggagtggagagagggaaagagagagagagaggatctttatggtgaaaaaataattaccaccaaaaagaatgcatgagagagagagacataaggtgaatgatagagagagagaaaggcctaagaaaaatatataagggccaggaaaattaaaagagctggaaccaaatatacacaaatggggaatggacaaaaataagccaagacagctagtttaattatctcctttaagcaattagacatgattttattttcttagtataaaaacagtttcaccagaggtccaaattttcttgaaatttaagttcttcagaatgaagcataaaaatatttcacaaaaaattattgtgttaaaagtcaaatttatggctgatattaaaaatagtaataaagtccaagtgaatggttttatgcaaaggaaatccccattacacatt

SEQ ID NO: 129 - DNA, 7260 bp, Artificial Sequence
  subsequence of ATP4A
tgtctcgctgccttccgagatgatgcccacactggctgcaatggccttggcggtgatggggtggtcacccgttaccatgatcacctgtagggggaaccagtggatcactgaccccttcagatcagcccaatctccctgtcctccctgggagacatctgctgatacacgtgttcatttacttgaccaagcgtgaccacctcctacgtgcctgggatatagcagagacaaaagagacaaaaatccctgtccttgaggagctctagtgagggtgacagaaaataaagaaacgaattatatagtgtgttagaaagtggaaaaaaacatattaagcttggtgaaggaaacggtgactcgattttaagtgtacccagggaagggcttattgagaaggtgatatctgagcagagacctgtaagaggtgagagagtcagccacgtggaaagctgggagaagagtgctcctggcagggagaacagcaggtgcaaaggccctgaggtgaggacaggcccgaactgtcggaggaacagcagggaggacaccataactgcagaggagtgaacaaggaaagagggctaacgaacaagcttagaaaggtaacaaggcccgatgtaacagggccgtagagacacgggaagggcttgggcattgcctgcctggccttggctttcccacccttgttttgtgtttggggaaccactcctctcccctacaccatcagttgcagtgaggtccctggctaagattgggtaagtaagcccagacctggccaatcaaggtcttccatcccccagccccagtgactggctcagggataaatgagtgacccaatccagtgctactgcaaaagaggcactctctttttgtggggtggctaagcaggtgggagttaagtttgagctgctggagcaggggtgtgtgtgtccccaagtgaagggagtgcctgcaaataaagccagcaaagagaacagcagagctgagacatggagaaaggaaaattcctaatgacactgagctcctggatctggctagacctgaagcttaattccccagaatttttcagtatcataaaccaatgcattttggttcaagccagtttcaggtgggtttgtcatggggttcttcaacccaaatcctgctgccatcctctgtcctcactccacttgttcctccccacagtggcatacccggatgcctgcggtgcgacacttgagcacagcatcagggacggtggcccggggtgggtcaatcatggatacaagtcccgcaaagcagaggccgctagatggaaagttcatggcctctacgtcgaaggcatagccaggcgggtagtccttctcattcaggtagagctggcagaagcctgaccggaaacggggaagtcagggaagagccctgggcacaccctttcttagcagggccaggaaatgggtaaaataaccaggccccttgcaccaaacacctatggatgcctgaccttgtgctgaccccttcactcacattatctgaatctaccctcacaaccaccctgtgaggcccattctcatcttacagatgaggaaactgaggctcagagaggggacatttcttgccagaggtcacacagcaagtaaaaggcccagaattggaccacagatctgctttctagggtagaggcagcgaagtttaaggcgtcaggacaaaaattgggagaggttagaggtcaggatacggataaaagtccaggtgaggactggggtcaaggtagaaagtgaggacagacaggggtcaggactggtacagggaaagtcaagggtgaggctgtggactgcgacaaatcagccagcagccagggatgaggacggtcagggctgggccgggagtggtgggcagggtctgtgctagctcctcctcgcacctggagtctcctcccctgcccaggggtctcaccgagcacgcgttcgcccaggcctcccaggctgaggtaggcggtctggaaggcctcgcgccactgctcgtccagcggcagctcctggcccttgataaggatggagctgcagcgctccagcacgcgctcgggggcgcccttcatcaccagcaagtgtcgcgggtcccgcgggtcctccagcgtatggatggacagctgtgggcgggggggagaggcgaggctgtggacgggggaacggggcggggctgtggacgagggaacggggcggggctgaggagaggggcggggccgagagctcggtgcgggctctgagagctgcggggaagggtgaaggtggaagatggaggccttgtgtggaggggtccttggtagaaggtaagcgttaaggcggggctaggtgcagatttggagtcctggacgcagggaatgaacagaattagggtgcggagttgggctgggggcggatttggagagcgaggtgctccccatggacagtcccgccgaggagaagctgtgggcggggctgggtggtgggcggggccttgcctctggtggacggggccataggcggagcgggagatggggtggggtttggctgcggagagaaggggcaaggagcgaagcccctcgtggcccgctgatgtgggtgtggcctggggcggggcccgaggtgggcgggcccaggccgtgggcggggccggctgcgcacctggaacttgttggtggagttgaagggtatctcgcagacttttgggaagcggtcccggtagcccatggcgttgcccagcgtcagctccgagaacttgagcagcgccgtctccgatgcgtctccaatcacgatgcgctgggagcggggaccggtgtcaggggcgaagccggctacaccagcctcccgggattccctggaggccccctggctctcaccttgggcacaggcactgcatcctggccggacttgaaggcggcgcggttgcacagggtgagcacccggcacagcgcccgccacgtctccgaggactggtcaaacgtctgccctgcagaccaggcgtccaggctgggtcccgcacggcggctctcccggaccagaaccgagccccctcctcctaggctcatatcgcgggccccctccccagacctgggtggaattgggttccacccaaccctgagggacccagcccccggatgacccttccctctagacccggtagcgagtctcctttgagacctggagccgagccgccccgccttcgtacaaagccctccctacctccctatccctcttcaggtctccaccatccaccagatcctgccctggcgcctgtgccctccctcccccacacctgactggtcttccgtggtgtcagctgtgtggatgtggttgtcaaaccacagatgggacacagtcatgcggttctgagtgagagtccctgtcttgtccgagcagatcaccgaagtggagcccaatgtctccaccgcctccaggttcttgaccacgcagttcttactggccaggcgcttggctgtcagggacaggcagacctggggaaggggtgagcaccgcaggctggggacccaccctggcttccagtcctcttccccgcgtcaaagaacggggaaggctttaccccagccgcggggctgcgtgtgcaacgtgcttctgcaaacaccaggtgttttcttggccccagcttttgttcagccagtgctttgtttgggactccttccccagtctgcccagatacagtagcgaggcccctctctgagctgtcccagccgaggttctgaaaattctcttcacacaatcaaaatgagaagaggaaccttccccgcacctccctggggactggtctggagctgggtgctgactgtggaaggtctggtgacatgctggctgcctgcacaggacatcagcctcttccagttaaggacccggcctcgtcatctctgcgccctcaatgtgtggcacaggacttgccccagggttgcctcgggaaggacttgctgaatgagtggatgatgggaaggcaggagaatggatgggagctaagtggacagatagacaggcagggaggtgatgggggaaatgtggaggaaagaacagatggttgagcaggcccctcagctccctgcatccccgcctgcccccactcactgtgacagtggccagcagcccctcaggcacataggccaccacgatggccatgaagaagaccatggcccgcaggaaggtgtagccaatgcacatggccacaataaaaaatgtggcaccgaagagaatggccaggcccgcgatgatgtccacaaaatgctcgatctcgatagcgatgggtgtcttctcgttttccacccccgacgccagcgatgcgatgcgcccaatgatggtgcggtcgcccgtgttcaccaccaggccctgcacggtgcctgcaggggggccaaggcgcgactcagggatagggggcggcagtggggtgtgcactgccgtgtgagctgaaggacagccagtcactgccagtggaggatgtgacctgggagagggtagtgacagtgggagacagagaagcagtgtgccctggggaggtggcagtcacggggaggtggcagtcatgcaggagagagacagggaggctgaagccccctgtcctagaagatagcaggagagaggccagtggaggcagcagttactgggcaggcaggcgggggcttcacagaccctcaaggcacatggtggagaagaaggcgatgttgcgggtctccagagggctctcgtgcgtgcactcgggtgagcgggtctgtggctcagactcccctgtcagcgaggagttgtccaccttgcagccctgggccgccaggatgcggatgtcggcgggcactctgtccccacctttcatctccaccaggtcgcccaccaccagttggtcagcgttgatctggaatttgtctccatcgcggatgacagtggcttgctgcggggcaggggcaccaaagttgaggtggacgggggtgggggtgggagctgctgcatgtggggaggtaaaggatgaggagagctgggacccatggggagagatggaggccacagatgagggacaggggcctgatggaaggaggctacaggagcagtttggagtctctgggatctggagtggctgggtgctggggaacccacctgtggcacaaggttcttaaagctggcgatgatgttggtgctcttgaattcctggtagtagccaaagcagccggtgacgacaaccacagcaatgagagcgattgccaggtacagctggggacagggaaggggtggggttattcagaggggccggaagctgcctgcctgaggccaccgacctgctccctggtgccctggttttcttggttttccccatgcttttccccacctactaggaagctccatgcaccattccctgtagcctttagccccctcccatgtccctcatgtcccacactcgcctgctctgtcttctcagtgtcttgtgtttctgtgtatatttcatatcctctggccctgaatcctcaatcttccatgtccccatatctgtgacttgtgccccaaatcactgtgtgccttggtctgacgtgttcccttctcctgtgtccccaagccttgcattccccatgtccactgtcccatgtctcctcctgtccccatggcctgtattccccgtgtctccagtttcacatcctgggttttccataatctgctgccaccctctgtgtgtcccctgggcccccttgtccctgcatcctcacatccccgtccctgcgtgtgctgcagaccttgtacgtcatggtctgtgtcctctgtggccacggcccccatgttctagctccccagtcactgtgtcccgtgtctcccatgtctgtgtatctccgagttcccatcctgtgtcccatggccatgacttttcgagcctctgtcccatgtcacatgtccctgagtccccatgtcccttgccctcatctctgccatatgtccaatgtcccttgccctgcacctccatttcctctctgtctctgtgcttctatgtctcatgttttgtgtctctctatgtgctgtgtcctgaggcttgggtccctgccctggtgtcctatgtctgagtcccagggtctcctattccccgtgcctcagtctgtcctgtgtctgcactgcatgtcctctgcttccaagtcccatctcttttttttttttttttttttttttttaagatgcagtctcgctctgtcgcccaggctggagtgcagtggcatggtcttggctcactgcaacatccacctcctgggttcaaatgattctcctgcctcagcctcccaagtaactgggattacaggtgcccgccaccatgtctggctaatttttgtaattttagtagagatggggttttgccatgttggccaggctggtctcgaactcctgacctcaggtgatctgcccgcctcggcctcccaaagtgctgggattacaggcatgggattacacgcccggcctccaaatcccatctcttacgtatcacattgccatactctttatgcccccacctatgtccccatacccaagattcaccccagtgtccctgtgtcctgtgtccttgggtctgccccatccatatcccaatgtccttcaccctccatgacccctgtcttgagactgcctttcgtgttcgtctatccccatccttctctgcccctcttgtcccaagtcccaggctcagtgtcttccatccccaggtccccatgtcctgagcctgtccccacaacatggctcacattgtcgtcggtggtgaggtccccctcactagcctggatggcaaaggcgatgaggcagatggcggcggcaacccacatgaggcactgcaggcccccggccagctgcctcgcgaacttgacgtactctggggtgccccgtggtggccgcagtgcgttgggcccatcccgcagcagcagctcagcagccaggctcgcagagaggccctgggacagaggggcagggcgaggcggtcctgggggctttcctccacatgcacaccccgtggaaagccccctgcttcagtttcccttctccagcttggtctgtcctgctccttctcatctctttgtctcttggttcctgcccccaccccatctctccctccctccttcatctctccctttgtctctctctcctcgctcccctttctatgtgtctctctcctgctgctctctccttatttgtctctgccttctctgtcttgctgtctcttttcagctactcctctctccgtctctgtgtgtcaccctttctctctaatgctttctcccttctctccctctccctctctctc

SEQ ID NO: 130 - DNA, 7809 bp, Artificial Sequence
  subsequence of NOTCH1
taaaaatcaacatcttgggacgcatctggtcatgccccctggggatggcaccacgcggcccccgtagagccgggggaggctgccctgaggagtgcaggcggcacggcagcggagcgtccccagtgcatgggcggctaaggctccccgagctgagccaagtctgacgtccctcactggcatgacacacaacagactcattcattaagattttttaaacaaaatccacctttaaaaacatatttacagacattttttctgccataggctatacttggtattgcaaaaatctgctcctcccaaactaggaggggtggcccaagggcagcccccgcctccctccagcccctgcccgaccgcatgccccctgccagggctgcggggacaggaccaaaggacgcagcccacggcgttgcacagctcaatgtgcccggctctggcaagtctcctacaaaacacgggagcccacggggggtcgggtcccgcgagctggggcccaggctgtgttgctggagcatcttcttcggaacctgggggacactgtgcaggctgaggtgctggggccgccaccggggtcagcccaggcagtgtctttccccagaaaagggtaggatgcctccgtgtgtgacccaggcaagtgccacagtccacacatctcatgtttgacatgcatgatgcctacatttcaagaacgggcagggggccggggtggttctggagggaccaagaacttgtataaccaacgaacaactacataatactgaacctgaaacaaagattcatgattggtaccatgggtgcactcttggcatacacactccgagaacacattttcacaagcatgcttgcaagaaaccatctaaaacacatggcaacatctaacccatatgctttcacttgtttcctatttcagatgcaaattaatccgcgtgcggaaggtgagccagctttgcctccgtttgcctctggatgcagcttctcctaacaggcaggtgatgctggtggagcggccgggctggcttggggttgggtgggcgtcggggaaagggcgcggcctggacgccccaggagctttttggactatgctcgttcaacttcccttctccaacatcatttctttttggattttgaaaaaaggaatcaataaataaatggcatttataaatcatgaatctttgtttatattttataaacacagaagaatcttttcatcctacgtaggaaaaccctggctctcagaacttgcttgttttctcagaatagataaaagtttctacctggggccagataaaacagtacatataaataaaaaggcagtgtttctgtgtaaaataaaagtacataaataaatactaaaaaaaattaaaatcctcgttcttattttgtataaaaacatgtgttttaaaaaggctcctctggtcggccctggcatccacagagcgcacacagacgcccgaaggcttgggaaaggaagccggggtctcgtggggcgcgccgtttacttgaaggcctccggaatgcgggcgatctgggactgcatgctggtgggagggctggagacgccctcggaccagtcggagacgttggaatgcggggacgagctggaccactggtcaggggactcaggggacggggtgaggaaggggtgctcaggcacctgtagctggtggctgggggtgttgtccacaggcgaggagtagctgtgctgcgaggggggcgtcaggaactgggctgcggtcacgggtgggaccagcgaggatggcagcgacgtgggcagggcggggctctcctggggcagaatagtgtgcaccgccaggctgctggggcccagtggctgcacgtctgcctggctcggctctccactcaggaagctccggcccaggtggccgctggctgctgagctcacgccaaggtgcggctgtggtggtggtggtggcggctgcaggctttgctgctgctggatgtttgctggctgcaggttctgctgctgcatctgtaagttttgtggctgcacctgctgggtctgcaccaggtgaggctgggtggccagccgggtgctgggcaggccctggtagctcatcatctgggacagggcgctggcagcaaggctactgtgcagcgggcctaccatgccatgctgcagggagggggcctgtgtgctcagggggcctggtgccacactcccccgcagagggttgtattggttcggcaccatgccgctctgcagccgggacagccactcgcattgaccattcaaactggtggacccgcccacagtgaaattcagggcccctccgctgctggagcccaggacggtgctggtgccagaggccacaggcaggtgggagagacgaggtgggccagtctcaaaggccagccggccgcccccacccagcgccgccatctcgggcttggccgccacgttcaggtgcccgatgcccaggtgggtgtcgggcatcccaggcaggtggttgaggggcacggacggagactgctggaacggggagggcagcagtggcggcgaggccacgtctgacaggtagccatggggtgactccagggagtccacgggcgagagcatgccggagctgtccagcaggcagcccttgccgtcctgggacttcttcctccgtgccttgaggtccttggcctccttgcttccacaggccaggcctttgctgctgggcttgcggaccttcttgccctgcacgccgggcttgaggctgcccaggtagccgttgggcgagcagagcgggggcgacagggtgggcgtgccccccagcggggctccgtgcagctgcgggctgcgcaccaggttgtactcgtccagcagcctcacgatgtcgtgatgcatgcgctcctgtgcgatgtcgcgcggcaggcggtccatatgatccgtgatgtcccggttggcaaagtggtccagcagcaccttggcggtctcgtagctgccctcccgggcggccagaaacaggggtgtctcctcctgggggatgagggcgggggccggtgaggggggccaggccaggcgtggggaccctccccaaggttccatcaccagaggaagcagcagtacaacctcctccgcggggtgggggcaggcaggctgctcctcaggaccccaccccagcgtcctgcaaccacctagcctgactcttgttaaatgttaaggctttgatacatcttctgaaacccacccagagaggggatctgtgcagtcctctaccctagatcagcggggctccacctctatgggggggtcacagaccccactgaaaatctaaccaactgcaggccctcttccctgcccccaataaggcacaaaaggaaattcctggagcggttcagaggcaccggcgagggcaccagggagggagctcgtcatctggacggccatcaagccaccctggtggccaccaagctccttcctggggtctcctctgtgcggtggacacgtcacaggtctgggtgaggctgctgtgtgggagtgggaaggggcttcccaggccttgatgccctctggggcccagtctctgtggggccatgctgccacggactggggagcgcctgggccaacatgccccggtgcccaggcccgctgtgtgccctcacccaggagggagagacgcctgagcctgacatgccaagggggcagcaggagttgggggcgggggtgggggttctggcggcagggaggtgggggtgtctgcacctgtgccctgagcacccaggggaaaccaacagcagctgcagggccaggagctgcagggccaggatgagggctgggggtggctccccttggatatagtcctgagacttcttcctctgagccttgaggtccttggccttggtgaacacaccaagaggccccgccccgcagggagctgccgccacgcgtgttctggctcaatctgcaccacctgcgtcaccacattcccatccccacccccgcctggtgacagctggggacagaaggtgaggtccaggtgacggtgacacagcagtggcagcagcagcgttccccacgccaggctgtgtgccccgccatgactgccgcccaggagggtagggctgggtctgaggggcgagccgccgtgtcctgacagctggacctgcacttggaagggctccataaacgggggctgaaggaaggcaggagcactaacgaggtgcccgcatcatgcgggtggggcccacatgcgggcccagcgaccctcgagaccctgtgggtcaggcccttgtgtccctgcgccccgtgggtttggccctcacttctctgtggattcagccctcacgtctcccctggcatcccagcctcgcgctcaccctgttgttctgcatatctttgttagccccgttcttcaggagcacaactgcggcatccacattgttcacggcggcggcccagtgcagggcggacttgcctgcgtgaaagaagcagatggggtaggttggagaccagctggaggcaacccagtcccacccgtccctgtggcggtcccgccccacgacagagcagccgtgcccccgtgggctcacccaggtcatctacggcgttgacgtcggcgtgtgagttgatgaggtcctccagcatgccctccacggccaggcgggcagccaggatcagtggcgtcgtgccatcatgcatgcgggcatccaggtctgtggctcggttccggatcaggatctgggcaacagggagaggctcaggcgggtgctgggcagacgtacaccgatgcctcctgcccagaacgaacgcctggacgggaagccccactgtcttccggacacagacgagaccctcctgagatcggcacggccgggcaagacgaaacgccatggggctgcccctgaggaggggcccggatgggggcaggggctgtgctgcccacagacaggccccttggtgacagtgggatccatcgtgaccacgtgtggcctcatttaatcctcactgtggtcctagctgccatgaccacctacaaaacagagaggtcaagtccctgcccccaacggcggttacagctggcactcaggaagccgggctcacggccctacagccgtctcagaaccgccgagctagtgtccggctctgcccagagagggggtgggcagcccttgtaatgcagccgggtcttggcatctggcaggaggaatggcccctgctcactggcgggtgcaaaaggcaacttggcctgattcctgcaaagcacctgggaacttccacatctgtgcaaagaaggcagctgagagaggcacacaccaaacccgcacggggctcccttccacgctctttctgctcacctacatttatttctgcgagatgacaatgtgtcacctgagctaagaaatcaggaaatgagaagctctgtggtaactccccgggctgtgcccatctgaacctgcttgctccagggccgcctggagcctggggactcgcagcaggggtgactgcaaaggcagcccctgccagggacactccctggagacccaggcatccaaatccctaaatccattcttgccacgagctcaccggcaagctgagccctaggtctgcaggcaccgagcggcagcctctaaaccctgcttctcactgccacaggctacgccggcagccaaggttgagggaggggcggggctgcgaggggctgcagcagtggaacctggaccttgagcaaggcccacaaccctgatggagcctgttttgctgggggtggggaggtgctgcctcactcagcagatcccccaggcctcctgccagacccgcctctgcctgacttccctggagaacacagatgggcccgacgccctccccctcgcacctcgctgactgcgaaggtcccaggtggaggcaccagttgtcccggactcagctgtgctcggggtcaggctcccagggccacgtaagcctggccactgccccagaccaccaggcggccctgaggagggcaggtgggcacacaggcagccactgcctacctggaagacaccttgtgcgtcggcagacacagccgcatgcagcggggtgcggcccatgttgtcctggatgttggcatctgcgctggcctccagcaggcgcttggcggcatcagagcgtgagtagcgggcggccaggtgcaaggcggtctcgcccgtgcggtctgtctggttgtgcaggctggcgccctggtagatgaagtcggagatgacggccggcgcgtcctcctcttcctcgctgttgcccgtctccaggccgcccccgctgcaggaggcgatcatgagcggggtgaagccatctgcagaggcagagacgggtgctcagtctggagggccggtccccagctgcagcccagggggaggggggcagcagccccaagctcaaggggccacggtgtggatgcaccacccagcacttggtggccccgtgcacacagccaccaaggggcagctgaagtccgcctgggctgctcagtggacagagccgaatccagcttaaactcctggcgggcaactgcttcctgacctgcccaagacctggcacccaaaatccacccaggaaaaagaggaccccagaagcatgcagttagaaaattaatgcttcagcaggatgcggaggctcacgctgtcatcctagcactgggggaggccgaggtgggcggatcacctgaggtcaggagttcgagaccagcctggccaacatggtgaaaccccatcgctgctaaaaatacaaaaattagccaggtgtggtggcaggcgcctgtagtcccagctactggggaggctgaggcaggagaattgcttgaacccgagaggtggaggttgcagggagccgagatcgtgccactgcactccagcctgggtgacggagcgagactccatctcaaaaacaaaaaaaaaagaaaaaaaaaaagaaaaagaaaatcaacgctttccatgtctcaagaaggtttcagaaaagagtaatttacagggacagagtggccctgcggtatcaccccaggaaggggttggtggaagaacaggaggactccaggacccccccacgtctactctgaatgggaaacaccccaaggatgaaagctctcacccccaattctaagtttccagagtatcaactgtaccccagcctcggggcttaggggagagaggcaggtgggccacggggctagggaagccctggctgctggcacccttaccaggcccgcggacattgacgtccatgcagtcggcgtcaacctcaccctggggcggtgtgggggccatggcagacatgcgcaggtcagcggcatccaggtgctgctgagtccactgccggtggtctgtctggtcgtccaggtcaggcagaaccacgggctcctcgaactacatagagggagtgagcagagcctgtcagggcagcccggcagcaggtgcccgggagcccaggagcccgggagcctcgcgactcacccggaacttcttggtctccaggtcctcgtccccccactcattctggttgtcgtccatgagggcaccgtctgaagcgttcttcaggggcctggggggtgaggggtcgagaagtgaggctgagcgagctccctaggaagcccccagagacccctggcccgggcctggcgtgggaggtgggccctgggtcgggaggggcagactcccggtgaggatgctcggccaggtcccacctcccaccggggacccagaagcaggggcggcgtccgctcacttgaggcccacggagtcctcgccgaggggctcccgccgcttcttcttgctggcctcagacactttgaagccctcagggaaccagagctggccatgctgccgccggcgcttgcg

SEQ ID NO: 131 - DNA, 6917 bp, Artificial Sequence
  subsequence
agttaataaatgaaaagagctgtaaatgttcatagcagttgtatcactgcctagcataagaaccccttaaaaacctgtttcttaatttgggaaacagatatgacgatagttagcatttattaaaggatgacagttaacaactgctatgtgccaggccttgttctaacagcttttcatatttagcccacttaacatatttctattttcatatgaggaaactgaggcagagagaggctaagtaacatacccaaggttttccagctagaaaatggcagagccaggactcaaacccaggcagtctggctgctgagccctggttcttaattatgacattaatgcttattctgcccagtgaggataaaatgagtgaaacataaaatcaaacaggatgttttggtagggagcagtgttttttccctctgaaaaatgaaaaattaggttattgtgattttgtaatttacagcagtgaatatgatgtgaaaaataagttatccatataataatttatgtcaggagtcatgcagcagaaagatttctgtccatcacgtaaactttcatccattacataacccatatgtttctgtaccattaagacacttggttcaacaagacccttggagaatgaggttccttttgttccctggggttctctttttattttatttttggattaatatttgatagtaaagccaaggatttgggacaggaaacttagatgacatctagttcaaactccttgatttacatatgaaaaaattgagacagagggaaatgaagatttccccatatcatataactggctaaagggagctatgtaggtaaaaccaagatgtcctgatattctagtctaccagaaagtgttctttttttctacccaacttattcctgatttaaaggctagtatacgtgtgctgatctcccctcagtgggaggggcatggacgttgggagtagtctctattcacaacaaattaaaaatcagtaatcagccgtataatgggttgtgttagaaagtaaactaaggcccaataaaatatttaagagtttatttgagcagtgatccagaagtggctagggagctccccagagagaacatgaggaggaggctttttaggacaaatagataaaagcaaagataatatttcattggttacagttatacagttacacagttatacagttgccttatttggtctatcccatgaggaagtcctagttactaattacgtttttgttggctgcttctgattggttgagcttaagttctgtgtttctttaacataggcatttacaagaaataccacaaataaagtttcagacatgcttgcaaatcaagcaaggttaaggtcacttaggaggcccaactggctctgtctgctcaaggattcttctggcctcgtctccattttacatgaactgttgcataaataaacacagagtacctgaaacaacggaggtgatcattctgcctaccgagtgttggccaggccaagcttggagtgttgctcttattcttagggagtttatttttaagtaatctcatctgtaaatgggattacaatccacaaactgaccttgtatatgattccattccttctcccagcccagccccacactccaaggttttccctttgcttataaggggtagtcacccttttttatttcgaccttccaaacattctgggagttttcctcctttaggccaactacagcgcagaggagcgctttctcctgctgggtttctccgactggccttccctgcagccggtcctcttcgcccttgtcctcctgtgctacctcctgaccttgacgggcaactcggcgctggtgctgctggcggtgcgcgacccgcgcctgcacacgcccatgtactacttcctctgccacctggccttggtagacgcgggcttcactactagcgtggtgccgccgctgctggccaacctgcgcggaccagcgctctggctgccgcgcagccactgcacggcccagctgtgcgcatcgctggctctgggttccgccgaatgcgtcctcctggcggtgatggctctggaccgcgcggccgcagtgtgccgcccgctgcgctatgcggggctcgtctccccgcgcctatgtcgcacgctggccagcgcctcctggctaagcggcctcaccaactcggttgcgcaaaccgcgctcctggctgagcggccgctgtgcgcgccccgcctgctggaccacttcatctgtgagctgccggcgttgctcaagctggcctgcggaggcgacggagacactaccgagaaccagatgttcgccgcccgcgtggtcatcctgctgctgccgtttgccgtcatcctggcctcctacggtgccgtggcccgagctgtctgttgcatgcggttcagcggaggccggaggagggcggtgggcacgtgtgggtcccacctgacagccgtctgcctgttctacggctcggccatctacacctacctgcagcccgcgcagcgctacaaccaggcacggggcaagttcgtatcgctcttctacaccgtggtcacacctgctctcaacccgctcatctacaccctcaggaataagaaagtgaagggggcagcgaggaggctgctgcggagtctggggagaggccaggctgggcagtgagtagttggggaggggagaaagtattaagccagaacccaaggatggaaataccccttagtgagtcagtttagacttcaggctgttcatttttgtatgataatctgcaagatttgtcctaaggagtccaatgggggatatgttttcctcccgtgaggaaatgtttagttcttgagggaaaatccctaaatcctctatatactcaggtttagggaaggaaaacctacccctcacaactccacgcgcagggaaaatgatggacgtgatgctcgcctttagcttcctccctatctgatggaagaccatggaagacctcttggtctctgcaatcagaagtctcaagttgacaagaaaatcatagtccctaccctgcaggagagggtacatccagaaaaagcgaccatggactctattctcagaaatcagtccaacttagtgcagacctggccagatgaccagtgccctccccggggcatttcacccataaatgtgatgaggaaagcccataaatggtggtgaattttgctgagtggggttaagactggaaacccccctgcaggagttggttcttgagcaagttttaaagaaacaaggaactaggatgagtgtggaagaaggcgggcacgtctcagcccgtgaaaaaaactcacaggtgatcagtagtgagtcatgagagagagagcaagagagagagtcagagagaggagtaaatggagggaggaagatggaggaagggactcaagttctcaagacaggaacagggatctcctcatgaaaaaaagaagagaggaaaatgctcaatcagcagaacctgagcagaatattgaggtcaacccagaagccagctcctcacccaccctcacccagactggcgccctcatcctggagaagacctgctagaccctaaggcaggtaggagagagggtggtccacagtcccccagctttagaaagtttgttcgctcccaatgtccatctacccctaggaatccccactagttaaacagaattgctagatccctgtggaaaatacctttccttgcccaccatcatccccagaaataataactattttagttgggtgtgagacatagagaataaaagggggcatggtgccagacttcatttcatacaaatagctttaaaggagaagaggggggaaggagtttaatttagtttctaaaatgtttagtaatttgattgtgatcatgtcagagcaactaattcattttataaaatatcatttcactatgctctataagtagaaattcaatttggttcaaccattattgagtgatataaataaagcactggacttaacaaagacagaaatacagaaatcagtagaacatggatcccaacctaaaacttactctcttgtcataaaggaaaggagataggagtttttgcataaataacaaggtatcaagacagaattaaattccaagctggctttgaatgctctattttgccttaaaaatttatttactagtctcagtaatacattagtaaaaatcatgtcacttaattaattgtgttagaatcaaagaaacatagagttgggcaatatacttcatcctacccatcccacccaaatcttactctactcatctcattctcattaattttgggaaatcatcagaagatgtgttcgttgagtaagagattaaaagaaataagctttttgacccctgccaacaccccatgcccagggtggtcaccctccaatacaataacatgccaggaagagtaagttgccctttctgatgccgtaatctgccatcatcttcccatcttccagtctctttccattgcaagtcacaatctgggtctcagggattatacccgtcttagtctcgatcattgctttcacttgtgccactgagctggaccttcgcacctggaggaggtgcctctttgcctcatcacctgactccacaagaaacaagggcagctcctcatcactgggcttcaccactttcagggtaaggtggatggtcttctctttgtcaatgccataagatgagaggcttctccgtggctttaagatcttggagcccagcaaaagaacctggtcctgcacaggaaccttggtcttagaccggacatgttctttgatttttttcacgctgtcatatgggttggcatcaaaggtcattaaatcccattcctcggaacggacatgcacctgggaagtgaaagccacaagacagttacctaggatgcctgcctcctttacacttctactccccaccacaatggctccccctcttccactatctatctggtcctctagctcctattcagtagccagtgtccctctctttcttggaacttcttttttggaattaccaagttacaacacaaataagataatttgtcccattcctttataatcacacctttttttcgatcttgagaatggaaaataaaatcctgagcccccaaccaactgaacggacgctcttttgctcagggggaccctagagaaactttaaaaacttagtcattgggccaagggtggtggcttacacctgtaatcccagaactttgggaagctgaggcaggctgatcaattgatgctgggagttcgagaccagcctggtgaacttggtgaaactctgtctctactaaaaatacaaaaattagccagtagtggtggcaagtccctgtaatcccagctactcaggaggctgaggcaggagaatcatttgaatccaggaggcagaggttgcagtgagtggagatggcactactgcactccagccagggcaacagagtgagactctgtctcaaaaatataaataaataaaacattcagtcatgatggaacaggaggttggatatgcctcattgtatcttctcccttttgcagtttagacacaactgaccagcaaagttagagattataagactgagagaatggattctttgtggcaataagatagcaaattataaacaagaccgagggctataacaggcaaaagttaagtcatgcatcccttacacttaaagaataaactatgttctgccacaaagttttttcttttttctctagcagctaaacaagcactggccttgacaggaacaatattaaaacaattacagctcaccctgtgttggggaacacaggctaactgaccccgtgttccacaagccataactacagttttaattggacaaaagactgatttcagtaattttctcctgataagagaccactgaccatggactggttctggctagtttacagaagctgtgcatttgaatgcctttgtgtccctgcttcaccttttcatgtataaggcctaactgtaatgcaattaaatgttaagtctccacttcagagtgaccatgggtggtatgtaacatgcaagcttattcaatatgcatgcattaggaccccctccatgaatattcattgcctctgctataacctattggatatgtatacttagcaaaccccttcagcataaattcctgtgtcacctttcctcctgcaaagtgcttgcttttggttttcaatcagaagcaaaacttcccagcctgtcagaatggctaccttgcagactataacctttcataagaaataaactccccttctaaatttatgaattgtgtgattttttttagttgacaatctttacatttcgtttttctgtgcatttcaatggatgtaaaaaacatacctttatccatctcaaaatgtaattagtgattttccaccttatttacctgcctctcctatccagataaagtttgtcaaatgtcaacaagtaaatacgaggcttcaaaagatgtacatcagactctaaaaacaactctcaaagagaatttccaaaatatgacagcctcatgaagatactcatagccataggataccctctgtcaatacttcagaaggaaatcctgggtaggacacataatcactgaactgttagtttcttttcaaatatcccactgctttataataataactcacatactaccgtgacactatgttcagtgtttcttgttaatttatatttcttgtgtttttatttctatctaatgagagacaggactagctggatttcctaggccgactaagaatccctaagcctagctggggaggtgactgcatccacctttaaacacggggcttgcaacttagctcacacctgaccaatcaggtagtaaagagagctcactaaaatgctaattaggcaaaaacaggaggtaaagatatagccaatcatctattgcctgagatcacagcgggagggacaatgatcgggat

SEQ ID NO: 132 - DNA, 6914 bp, Artificial Sequence
  subsequence
tatgtatacatgtgccatgctggtgcgctgcacccactaactcgtcatctagcattaggtatatctcccaatgctatccctcccccctccccccaccccaccacagtccccagagtgtgatattccccttcctgtgtccatgtgatctcattgttcagttcccacctatgagtgagaatatgcggtgtttggttttttgatcttgcgatagtttactgagaatgatgatttccaatttcatccatgtccctacaaaggacatgaactcatcattttttatggctgcatagtattccatggtgtatatgtgccacattttcttaatccagtctatcattgttggacatttgggttggttccaagtctttgctattgtgaataatgccgcaataaacatacgtgtgcatgtgtctttatagcagcatgatttatagtcatttgggtatatacccagtaatgggatggctgggtcaaatggtaattctagttctagatccctgaggaatcgccacactgacttccacaatggttgaactggtttacagtcccaccaacagtgtaaaagtgttcctatttctccacatcctctccagcacctgttgtttcctgactttttaatgattgccattctaactggtgtgagatggtatctcatagtggttttgatttccatttctctgatggccagtgatgatgagcattttttcatgtgttttttggctgcataaatgtcttcttttgagaagtgtctgttcatgtccttcgcccactttttgatggggttgtttgtttttttattgtaaatttgtttgagttcattgtagattctggatattagccctttgtcagatgagtaggttgcgaaaattttctcccattttgtaggttgcctgttcactgtgatggtagtttcttttgctgtgcagaagctctttagtttaattagatcccatttgtcaattttgtcttttgttgccattgcttttggtgttttggacatgaagtccttgcccatgcctatgtcctgaatggtaatgcctaggttttcttctagggttttcatggttttaggtctaacgtttaaatctttaatccatcttgaattgatttttgtataaggtgtaaggaagggatccagtttcagctttctccatatggctagccagttttcccagcaccatttattaaatttcttttcttgttctcccgtgacttttgatatcactgcacacaactgttactgtaagatgaacattaaaaagtcacgtctggccagtacggggatcgaacccgcgaccttagcgttattagcaccacgctctaaccaactgagctaaccggccccgcttactaaaaccccccctaaacctcttgagaagtttaaaggcgaacgttatttcaatcaccaaagaaacttttctgaacttctcggaactggaaagaacctgcgatctttgctaacttgtttatgatcctcggcaaatttctccgaaccctgacatttcaattaaaatacaattctgaggaaggaaagttcaaatgtcacctgcttcactgtttcatgacaaggggtttcagtgaccacccttttaaacgcaacgccatcaccttccgccggtactttggcctgcccttctcactcctttctactttgcttccgtagcttctgagcaacccgtgaagaaattgacggaaaacggaaggaattaccgccagtttctttccacgggccgtcaaggccaatataagtccccacccaggctcctctgctcgtaacttccagcacgattcccactgtattagcccatgtttcccagaagtgagtatttgatccctaccccaccccatttttagaaaactcaggaaaacgctctcgtatttctatctgaaaaggacactttagagaaatacgttccattacagtctttgtgttcgcattgtattccttctcgatgaaacaggtataagtccattggtattttacgcacgacaagacaactttgcagcccgactcatgacctttagattaagaaacactctccgggagctctgctgatcgctgggtcttacgaggttgatgccttctgtcccaaagagaactatttccctgcgtgtttccgcctggctgcccacttctccagtagagaaacagctgttcctcgggattcatttttggaagttctttgggtcctgggtaatggggccgcatcctgcagcgtcgacaaggtggttgaatacgcaggaacacccacagtacccagggactaataaatagctcaatagatacgtttcgaataattaaataaaagaagtctcaaccaacccccttgctgtattacagatggtccagctctctgcctagactattgtgctaatgtcctgttccttctcccggcttttgaactagattctcacctctctccaatccatctttcgcagggctggcctgtctttccgcctcacttctgaaattctatccattgccgcctctgtgcaaaccgactctggttaatacttcagtcggtatggctcccctcttccgcactttgcactgcgagaaatgcccttctttgaggcagctggaggcctcctcctcctgagagcttaattgtggacacagccttgagtagaggcgaaaaggaaagaaggctgggagacaatcggggaaaaacacacacctttggtctggtttgaaagctggcgcccgaaaaggaacaagaaaaaaaacacgcttcggaagtgtctgagattgctgcggccataaagcagagcactaaccctggtactgatacgggaggggagcaagactccacccccgggcctgtgcccatgaacctaggtgaggaggggcacttcttcctccgcgcccaaatgttgcatttcccaagaccaccctggcccgccacgcccccatcctgtgcctataaaaacccccgagaccctagcgggcacagacacaagcggttggacatgaagaggaacacaccggcgggagaacacagaacacccaccctctctttagtcaccctggaggcctcggagaaggcggtttcagtgatccgtgaagagaccctgagtcttttacatcccggagaatgacaagagagtacctgggcgacgtaactttctgggttttccggagatgcggttttctacacgccaggggccaagcctgagaaataggtggacggcaaggacaggagctctctccgcgccacaaacgcccctgctcacacctgggttccttgattttcctgcctatataaccgagccacccatggccgggctccgagctctcattctgcggactgggacaaaggggttaactgtgatgtgctttgtataaccccaggattctgcacttgcccaagggcgaggtgcaaatccaaaatcacgcacgactgaacgccgagatcagctgagtcctgagtgcctcacgacacaaaatccgtatgatttttaaaagcgctgtatttgtgctgacaatgcatgtcagatcccatctgtctttagctcaatgtgtgacgttagacacgtcgttttgctcctcaactttcttatttggaaaaaaaaaaacgagtgttctagatttgcagagggccttttcagagctaagttccagtagctatactgtaagttgaactcgggcagtcctgttggtgaggaaaaaggacaaattgagaaatgaacaaacacagaagttgcaaaagccctgtgacttacagcacaggacaagtctacaaaccctgccatgccacactaagctcaagttgttttaacatcagtttactcagacccgatgatccaaggtaagaccaaagccaaacggatccagcaactgggcagatcttcatgttccagcagctaagttccacggaataaacctatgattcgcctagtttagaaattgtctagtccctcctcagaaggaccttactaactttccccctaaaagtgtcctatgaatagctccagtccccagaccctttaaattctggtctctgactcacccttgttttaggcagtactgggactccatagaggtacggctctttgctcagcaagtttaataaatccaaggtagtagaatcaatttgttttcttggtcgtcttgtttggagggagtgggtcttctcaatgttggttctgatccctgcctatggatatttatgaataaatagatatttgcactccatcatcatgtggagctacaagtgttaaatttaacgatctaattacctctaaaataaccactaaattcaacaatctgaaacttatctaattagttccacatcctggaatgaagggatttaataggtaataacaggtctcagtctctaatggagacataatcacacagacaccagatgaaagatgagtaaagtggaaagcaataggtagaacaataatttgctttatgctatgatttttggagcgaagcaagaaaattaatcaaggaaacaaagaagaaatccaagacttagtagtgttggatttgcgtttttgtcatatgacattacttgtattttacaggattcacttggtctccatctgacctcctcagagtagactgctctttcccaatcactcctgcaattaccctaggagatatgtgatcctaaagtaacggggagttttaaatttacttctaagtacacctgcatgatgccattagtcagggcagggtagctgaacaaactcagctctgaatcctttaagcagaggtaataattgctgacactatttaatcggattctgaacatgatgtgccacttttccttttgcgtctgaagtgacaccagccattttcacagtttcttccactaggaggtcctgggagaaaagtgataaaggtagattcaagaatggttagtttgataagagaaacataaaggcaagtatctttttcactcagttcaccttggttctaagagtgggtctatataaagaaatggaacatgcttctgctaattaatgttcaggcagaaaaagtcatgaattccactacaaacccatgtcccttcttccgaagacatgacaaattgatgagggtatgctttcttctgtcggtaaaacgaagtctgggatatagattgcaatattagcagtgccatagtgcagaatttctcataattaacacttttcacttgaatacataagaaaatagaattggaatgtaaagttaataaagtaatcatgttataaacaatatgaacataaaagcaaaaattacatggtctttggcatgcagtctttgatttggggaatgcattttttctattgttatcaggaagaaagaacagaaacagttcatattcacatggactagacaaaagtatgcatttatgttcttactccagaggtatatcaagtcccccaatttttcctaatctagtccaaagagaattgaactgtctgcaccaacagcaaaacattggtacactgtattgatagtatcatttaaatcttcgatgagcaagaagtgtcaagtaagttgcagattttgttaagccctgcatgctccagagggtgggagagaaacacagaaaccattcatcgacctggttcgtgaatgaaagtttttaggatctgtgaaattctgagacatttcctccaaagtaaagtctcattgttgtatctcgaagctcccgtcacttagaagggagcactgtgctcaccatgtttctctgagctgtgaaagcggcgcgttccacacttggagacccttctctgacacatttaccaacagatactgaattaaaatattaacaaattgaatccagcattatctgtaaagcataatgcaccatgagttaggggagattgcctcgggaataaaaaattagttaggcattgaaaagtcaattaaatgtaatataccacattaacaaaacaaaaaatacatgtaatcatctcactagatgcagaagaaatattggaccaaatttgccattcattcgtggtgtttaaaaaatatcccagtaagctaagaatagaaggaaaattcctcagatgaataatgggcgtttaagaaagtcctacaactagcaatagagttaatagtggaagaataaatatgtaccctttaatattggagaaaagtgcaaaatatctgtccttactacttctacattttactgaaagtcctagctagtgtcagaaagtaaggaacgcatgaatgaagaataaatggcatactcactttagaataagaaaaatatattcgtttgcaagcaacatgatcagatacacaaaaaatcctagtgtatccacaaaaataagcattataagtaaatgcagctatgtcacagattacagtatacaaaaattaattgtatttctatgtactagcatcaaaaaaatggaaaattaaattaccactttcaataggtttaaaacaaatgaaatatttagagataaacttgtcagtgtgcacaggacttgtacctaggaatctacaaaagatggctgagaaaaactcaggaaagcttgactaattggtgttgtttgacatatttacagattgaaaaaggtaatattattaagatatcatttttttccctctgagttgatctatagatttactacaatcccaacaaatatcccagcaggagatttttgttttgtttgttttgttttcttttctttttgtttgtttgtttttacagaaattgacaagcttattctgtaggacctagagtaacctaaataattaggaaaagaaaaacaaagttagaggacttacaccaggtgatgtcaagacttattataaagctaaggtaatcaaaataatgtggtattgtctcaaggatacttacccagattgacggaatagaacagatagtccagaaacagaccaacgtatgtggtcaactgatttatgacagaggtaaaatgtttttttaaacaaatgg

SEQ ID NO: 133 - DNA, 4834 bp, Artificial Sequence
  subsequence of HOXA7
aaaaacacatgcacccaattatggacaccaaaatatatacaattgtggaattaggtaaaaacacacacacagaaatacatacacagaaaaataagcacatactcatacaaatacacacataaaaatacattaaaaagatacatgacaccaatacatgggtacccaacacttggaccatcacaaggacagccaccccacttttgcttccccactgccccctgccctccagccatactcacctcccctttcccagtcccctctggataaggcagtccacatttttctttgtcaccacgcatctttattttcggttacataaaacacagctgggctgggaagtgtgccttccctgaaccccaggatggagctgagcagggtacaggacaacacaggagatgaagggcattgcggagggcattggacctccccacccactacagttaactcaagacaacataccatgctacaaagtcaccccattaacacatcctttccaagtcaagacactgccttacaaatgaactccaagactatagaaatgataaaaaaaaatcttgttcaaatatacagtatctgctattataggaaacatcagggcgtacatatttaacacagctgaacagtaagatacaggagccagaggaaaggacagcgaagctggaagcatctccacagtcctgctaagcagaagctaacccacagatctgcagccagctcaggaacattcccctccagaagtgggggttgatgggcctgagctgtgggtgccaagccagagaaggagggattgattctagggtgcaagcacttaggatgctttttggaataaatatattatttttcgatttaaatagatgccaataccctgatcctggacctcagcacattctcagggcagcctcagggaccccaaaagctgcgggctgtaagcagcaggggacttgcctgggagcagtcggcactaggtagcaggcaagccagccagcacaaaataggtagttttaggggagtaggtagtagtgagattcactttcttgcgggtctgggagggtggtgctgggtgtctgccagtgttgggatacatagggacttcctgggaatggaggccctctggggctggatacataggtagtttgggggtgcctcgagcagaggcctgtgctaggtagtattttggacgcgccagagcagggccggctggcctggggttgggggtgtcttttggggtcctcggaggcagagggaatccaaggcgacccagtctctgcggccgctcagtccacaaaagttgggagctggagtaggtgatgggggtgggtagagtgcaggttggggactgggttgcttttttgtttttgtttttgttttttacattttcttttatttttcccatttttgtaagtaaaaccagtgagtctcttaaagacgcttttccgactgtccggtgcagagagggccccggatcggcccctcattcctcctcgtcttcctcttcttcatcatcgtcctcctcgtcggccttgtccgcggcagcagtggcggcggcagagggcacggcgccctcgggagctgcggcggcagtcggaccttcgtccttatgctctttcttccacttcatgcggcggttctggaaccagatcttaatctggcgctcggtgaggcagagcgcgtgggcgatttcaatgcggcggcgccgcgtcaggtagcggttgaagtggaactccttctccagctccagcgtctggtagcgcgtgtaggtctggcggccccgcttcctgtcaggtcctgagaacagacatgcagacacatgaacacaaggacagacaagtagacagggcactcgttaggctgctgtcccagagcccgcaccttcctcctggcctagtccccagcgagcatccccctctgccccaggccccgaactgagctaggggaggagggggagtgttagggaaagaccccaactgcagtgccagacgcgcaggcagctctgtaatgagcaaaggcacagaatctcaactttacaaccgacctttccagccggctaagcttccacaatgtcctgcttcctctgacaaaggaaaactgtaaatatagagtgtgagcaagtgggaaacgctgcacttttgccattcaaagatgagcccggccattcccctgccttgctaggcaagtgggcgactcttcccagcagcctgagccctcatccccaggaccttcctagggcaccccgaccctctgtcctcattccctcgcccccatcttgaaatggaccctggcacagggtcgggtgagaggccctggagggcttggctctcctagcttttgagaaagaaatgtcaggcagcaaggaaaatgaggagagagagaagaagaaagggagggagggtgacagaggagggagaaagagagacagaatagcgaacaaacttaatgttaaaattccaagacaaatggagttaaataaatttacgaggatcgaacccattaattgggccataaaaagttttatgagcctcatttacatacaatgctatgggctccacgcaatggcgcctccgctccaattaaaaccagaaaggctgcgccgggagtcacggggctaccggctcgcaacagcctggctccgctcttccggccccgcgccccgcgctccgcgctccccagcgctgcgctccccgctcccggtcccgctccgccagcctggcccgcctagcgactgcgcctacctgaagaccgcatccaggggtagatgcggaaattggcctcagccgcgccatgcagcgcgccctcgtccgtcttgtcgcaggcgcctttggcgaggtcactgcagagcccggggatgttttggtcgtaggaggcgcagggcaggttgccgtaggcgtcggcgcccaggccgtagccggacgcaaaggggctctgataaagggggctgttgacattgtataagcccggaacggtcgaggcgaaggcgccggcgcccgccccgtagccgcttctctgtgagttgggagcaaaggagcaagaagtcggctcggcattttggaacagagaagcccccgccgtatatttgctaaaaagcgcgttcacataatacgaagaactcataattttgacctgtgatttgttgtccggcagctttcagtgtcggttttacgaggtagagtgatatatgataacattacacccccagatttacaccaaaccccattttcttttggacggagctcgccgcagcacgtgaccgcccacatgaccgcctccgccaatctcagcagtcctcacaggtggtctcgctccgcagggcccgcagccgcctagaatggaagggcaagaggctcaaatatgcggccaaagaatccgcccgcgcccggcgggcctggcgcgtcccgcggaaaaagacctggaggctccgcgggagcgcccagctggcggccaacctccgcactggggtctgcggacgccaggcggcccggccccacgcagcaccccccaccccgcccccccgccgactcctgctagtgagccctggaccaagcttgggatcctccccatccctctcctgtccgcctgcccagaccctggaagggtctctgtcccccgcaacagcctgccccgcggtggccttgtgggcaggactcagctatgagcagatcgactctgcccaagtcttctctcacccaggtccagtgggcgacaggccggacttagactcggatccagacggggaaggcgcagcatctcttgcagctgcagagagattgccaccgcaaactggagccatgtggttcgaataaagtcaacgtctcccagcttcctttccttaatcggaggcacactgtttatccgccctaaaggaagcagtgaaatatttatctattaatgagactcatttgccaacagatttattaacgtggggttcccctccctcctcccggacgctgtagtgctgcaggctctgtgccttcgctcctgggcacctggctggctccagcagtccgataaattgctaaagattcctttgtcctttccacaacttctggttcccctctggcgcatggggagccagggctgtttcccccagcttggaaaaatctcgggcctgcacccttccaggcactcccaatactggaaggtttctggggtaggccggggtgcctgggaacaatacatgctttagagcggatttggagagggggctctggcgtctagggactgcaacccactgtggacttccttttcttttgaagacaccgaaaacaaataggggaaaccaccccctaaaggccacccagctgtggaggcttcacctatccaagtaccagctcacatggagctgagcgcacagtggtctcacttcctcccatccaggcctccaattcctaccttccaggcctccgacccctgcaccatgttgcaccagctgaagcccctgccgcccaccgctcggtggaggatggtggggagaacccttcccctaaacgcctcataaactgcccggctgcgctggaagcccggccaccttttactgctcagctcgattacacaccataaacccgacctcacaatggaattgccccggaaattctcctgtaaattgtagagtttagttccttgtgtactgagcacttcccatcactttcagagggtccaggccgtccccgtttaccgcaccctctcagggggccccaggaatacaaaaggtggagggagggttcagatcgggacgccacggagccccagttcctgcgcagtgaaccaccggggcttgggtaggaaggcgggggctggtggggcaggtgggcgctgggctgtctcctcccgggccacggaa

SEQ ID NO: 134 - DNA, 6555 bp, Artificial Sequence
  subsequence of ZNF529
tctacctaagcaattggtctcctccgtaacaaatcaccgtgtgaaggcagactatttctatgtcatgagaatgcttaaacaaaaagagcacacaggagaagtgaacatactgtcaaggtgttatatgaaaattaactctaggaagggcatctgatgaggtactggaaagaaggagatctgtcttcataatgtcatcagtaactgggaagagaaggactagagaccaggtaaatagataagtcactatttggtgagcatttcaaatgaagttattccacatcctgaaaaacaaaaatgcatttcataaaacaaagaaaaaaatcaaaatgacctccagctttgctttaaaatgtgcaactacaatgcttttcttctctcagagctcttctcttggaatacagcaaaatgtggaaagaaagggaatcacaatatactcagcctttcttggagcccagacaggctaaataagaacacattcttcaccaccggcaagcttccataacccatgctgaatatgaccagatggaagtatgagaaagactggaatattgttgactcttcccttcataaagaaaagtcaggttcaccaaagcctgggactgaaatgtttctgtattcacaataatttcctttagacagctatgaaaatgctgtggatctgcaatattcaacttgcccccacagagcttccaaaagggatcttttggctaggcacggtggctcacgcctgtaatcccagcactttgggaagccgaggcgggtggatcacctgaggtcaggagttcgagaccagtctgaccaacatggtgaaaccccgtctctactaaaaatacaaaaatgagccgggcatggtggtgcatgcctgtaatcccagctactcgggaggctgaggcaggagaattgcttgaacccggaaggcggaggttgcaatgagccgagattgcgccactgcactccagcctgggcaacaagagcaaaactccatctcacacacacacacaaaatctttggagaaacgaatcctactcctggggcctcaatatcatatcttcccagaaccttgccttgggagcaattccagctctaacatctccatatcaaacacgaggctgtgcatatcagaacacagccttgtccatgtgaaacacaaggctgtgctttttcagttggaaacttcattctggatctcaaatatccaactttcttttcgatagccatttgactgcacactgtgcaacgtggttataaggtgaaatgactgaggcagtgaaagaaatcccagtataacaaactccaagaaaccacgtaacttaaaattggccccagaggttggcgaggctgcatgccactgtgtattatgcattatgaaagcgacaggggccatgctttagaacagaaggtctcagagtcttcacagacacagatcgagccatacggggaccttgtccacgtattcctgagccccagaactgcagaaatcaaactctacaaaagctgcaccaggccagttttgatcacagtctccagtgggtcacaacagcgctgtcacaggatcactgataacagcatgacacattcatagtcaccgctcagcgccgtcacacaaacggccccgcccccactcagtcccgcgggcccaatcggggacagtcagggctgtcccgggctgtgcacctgctgtgcacacacaccccctgctgtgcacaccccccgcccccccgggaccatcacaggcgcgcccactcacaccaccacacacggacgcagccacagaacggcacacacaaacacaatcacacagtctccctccccagcaggtgacttgcacacaggcctggggcttctgcctccacaaaccctctccgcgtcccatgaacccaggtcccctgccgtgagctcttctcgcatccagacccgggtcacctcaactcaccacatggaaaacgaacaccaggtcaacggaaaagggagccggggtcctggcagaagcgtagtgccagccgcaatagggcggccgtgggtgcaaacggaggggagcgccggcagctagcaccgcgcggcgactaacgggccgccccggagactcctgggagctcaggcccacgcgcgagtgcgcaggcgcagacgactcaccctgggccgggggtgaggcttggtgggtgccaggggtgctgaggaggccaaggagggcactgggagctccgttccgggagagctgtctaaggacgcggaaccgggtggggaggccagggaggtaaccaagagtccgagccgggcctggaaattctgaggaggaaaccgggaccgcggtatccagacgctccgatctgtacgagccgggcctcgggcgtggtccatgggcgtgaccttgagggtgacccggagcgagctccgcgaagggggattttgcccgttctgatcccgcggaagcgccatcgctggcggcgggtccccgcgcggagcgggcgctgtgtgttcgcgcgcgcgggcgcgcgctgaataggggtggcctcctgcgcccaacctgctgcattttaggtgcttgcctctctttgggatgttgtggccgattgtgtgtgaaaagtgaacggagtagtgttgctgcgcgaggtttcctctgcgtgtgtctatttttagattaggtgtgagtcgcatttgagactgcctttgagtgtggagaattgcaagtgatttgtaggtgtggttgtgactgcctggagtcgtgttagctgctgtctgaggttgtgaatgacaagtggggcctgtaggttggtggttctctgaaggatgtttgattgactgtgactctgcatgtgtttgtaacctactgttacttctggtggttttgtggccttagtgacctaaatatttgaatgattgaggaactctgttatgaccatggctagttggttatgtaagacttgattatctgaatagtagccattaagcctgcctccaaaactgtaactaagtagcaatttagcaaataaaatagagataacagtatcagaggggaagagatgattttcataattcccagattcatttcctggaaacaccatattaactaaaaccagtatgttgaaatgaatagcattccattggggacatgcaggaaattttttttttttttttttttttaccataactaccacttttgttgttgttttttgtttgttttaagacaaggtcttgctcttttgcccaggctggagtgtagtggcatgatctctgctcactgccacctctacctctgaagttcaagtgattctcctgccccagcttcctgagtagctgggactacaggcttgtgccaccacgctcggctagtttttgtatttttagtagagatggggtttcaccatgttgcccaggctggtcttgaactcctgacctcaagtgatcccctccccccgccccctcggcctgccaaagtactgggattacaggtgtgagccactgtgcctggcataactaccactttcaacacttgtatatgagtgaggtttcctactcccttaggcttgctaagataataaaaagtatttgatagatttttaataagtccagtctcactgtagtaattaaaatagttattttgcgggcctggtgcagtgactgatgcctgtaatcccagcattttgggaggccaaggtgggcagatcacctgagatcgagaattcgagaccagcctgaccaacatggagaaaccccatctctactaaaaatacaaaattagccgggcatggtggtgcatgcctgtaatcccagctactcaggaggctgaggcaggagaatcgcttgaacccgggaggtggaggttgcggtcagtcaagattgtaccattgcactccagcctgggcaacaagagtgaaactctgtctcaaaaaaaaaaaaaaaaaagattattctcaactacaacatagaccagataggcaaagatttaaaagttgtcaactgtcttcatcagggcttgggaaggtattctcatccactactatcagtgtaaattggcaaaaagtccaagaagaaccgtttggaaatacacagtaaacctgtggttagaggtagatggaaggcagagctgcagagggaaaaacacagtgttccctctcttcaagctaaaacaggttccccagaatcctgtatactttaccaagagactgggtttctggtgtttgtgagggagcctgatttgtctgttttcccactaactaccatcctggacatctgaagggtacacagggtggacaagtgctgaaatagtgaacattcatgcagatttaactgagttaattctgggagttctgagtcaagtatggtctcacatacgtatatcctccatctttgctttctcaggactgtttctttttccaaaagaggagctcaaaagagaaagttcatctagaaatctcaaagccatgtctcaggtgagatgatgtttcctctctttctgaaataactttttttcatggtgtatgaacatgagcttcactgtcctttaaccttccctgatattgggatttgcttccatgaaattagtcttcagtcagggccagattaggctgaggcaggcaagtggcatgaggtgaaatatttaaggggtaccctcagggctgtgccctcctaaattttgcattctaggtgcctcacctgcctcaccctgtatccagccctgttcacaatttctccattccaaccaaatcaacttaagccttccccaagtgtaccttctggttgtacatattcattgggtatatcattcatcatctcctttctcagtcttctcacaaacaaactgctggaatagaaaggtattgtcttgatttaaatgggaatatatggcttgaatgaatttaacttgtcctgatgctgatttgagacctaagctgtgagtagtcatggagcagacgtggaaaaaccttgatgatctccgctagcctaggttttgcaatggtacgttgggaaatagaagtggtagatcccagcattagtttctggaaagatgtcctgctttgtgaggtgtttaggatagcaatttgattgcaggcttgtaaaggaaacacgttttatgttcctcctctctgatcttttttcattcatgtctgctagccattcctacaaattgtgggctgccagtgaaaacctttccagtattccaatgctgttagagatttgttattttctttttagtttcttctaattttttatttgcgggtgcaggagaaggaaatccatatgccaggccacttttgaaatattctattgttgatcaaacagtactttgtcctcttttcatatctttcagaaaattcctctttagctcatccaccaacctttaaaatactggttttcctcagatgctaattggttctcttcttcttcacagtccgtttttctctacgcacaatcagattcactctgaaggctacacttagtgtgattctagtgactctcaaatacccctctccactctagacctctgtccagagtgtcagaaccgaatattcaacctccagtagctatcaccacctgtatgttccacagacaaagtacatttccaaagcttacctcattacttcctttggtccagcttacattttcttccgtttcccattttcactttctagtcccagcagccatgcatttgcctatgcagataaaatgcctgtatcttttccactctacagccaatttacgaccatctctgttgtaatggtggtcatgtaggagcagttgtcctctgtcagcccgctgacacttccttaatctaggagacatttctaaccatggttacttaattgtcatttccacctaacatgtgataagccttttccagtcttcaggagtattacctcaaaacttttatcacataacgtgtgtcaacttatgtttattgatgttctttacattccttaaagcaacagacccaaagtagggcatgcctcacagtagaatgtataagacggtctattggaaggaaataaaatactaacaatttacattcgagagcagtattcattaacaatgtagattttcataaatgcctattgatggtttataaatagctacaatgttgggaatgtgttcagtatatctttaagaccactgttctgtaggaaaaaaaaatctagtatcatgtcataatatccccattgcctatctccatataccttttccttcttagagctcaaagactgtttcctaacatactgtgccttttgctatttcctgatttactaactggtttttttctccccatgaatttttaaaagctgatgccctgtattcctacaaaacaaattcgttgtgagtacaaaacttttatgtcctcaatgaagcctcggagtacaaaatgaaatttttccttgttttgtgacactttaccttgtacgtatttctgtcattgcatctgtaaaacctactaagtgcatgtatttacatgtatgcccctctcttagcctataacttctcatgagcagggtcagggttttattcattttggtctaccaggcaaccagtcacattcaggacaaatagtgtgatctcagtatg

SEQ ID NO: 135 - DNA, 4378 bp, Artificial Sequence
  subsequence of PRLHR
ttgatctacacatcatgtgggtggtagcttattcttctgttctgtccttaagtaaacttctgccggtccttgatttctgggttgatcatgttccaagaatcactacagagcaggtgctgagcagtcagatgacagctgttgatctgttgcaagtgagcaattagagactgcaggagaatgccacgctacacagtttacattgagtattcagaaaaccaaatatttgagtgcccactttgtggcaaacactgaatgtgtacccacacatacacacacatacacaaacacacatacacagaggatgtctgtccttaggtacaattgaatgacctcttaagtgaattggaccttttcctctttatttatctatctcttcattgactaattcgtctcatcatttttaaatagtagttggggaggaaaggggagaaacaatagcaagacctttctaaagggagcttgtaggtgtttttgtactataaactcaagtggttttaaaacgaaacccttttggcatataaaggtcttactcaggaaatgctgaaatcctagatgtagagttttaatacatatttacctgaaattctaggaatgcaagggttcaaatggactaagcaatatcatggtactctcagctgggtcctttttctaaaggcaaactgaaaatctttaccaagcccaatgcattccttttaaatcccattcatattgttcatttcaccaacgagcaggaggaggggacgccaggaaggcaatcgtggttctgaaatacttttctgaacgtggagaaaaagttttgtttgtccttcaagggcataaagaagaaataagaaatcctcttccctctctttggcctcccccaagcaaagagcaagactctcaccaaagcccgcttaacattttacaaacacacaaggacaagacagacagccggacaagagggctgggctggaaatgttgccctatgttggcttagctagctctggtgctgagaataagcaccagattgacctcgagtggtgccctaggaggccagttgaagtggagctccttgaccaaggcctggctaagtggcatcagatgaccacgctgacggtcatattctggccatggggggctatcttgcggggccaagcgaccaacagtttgcgcagctcctcgcggaagctgtcgtgcagccaggcgtagatgaaggggttgtagcaggccgaactcatggcgagccagtggcagagcagctgcaccagcccaaaggcgtaagggtcgatggcgtgggggtcgaggtcccgcagcaggttgaagacgtgcagcggcagccagcagacggcgaacaccaccacgatcaccaccagcaagcagaaggtgcgccggcgccgagcgcggtcccagtcggcctggctctgggtcacgcagcccggcaccacgcggttgcggagcttcactgacacccggacgtaagacaggaggatgaccagcagagggagcaggtaggtgaccagcagcagcccccaggcgtagagctggcgctggcgctcctgggagccccagaactcctcgcagaggcgcacgtcgtgcggcttgagctccacgtgataggtgtgcacggcggcgggcagcgccagcaccgcggacagcgcccagatggccagcacagcgtaggcgctgaggcgcagcgagatgcgccgcctcagcgggtgcaccagcacgacgtagcggtccactgcgatggtggtgagcgtgaacaccgacacatagacggtgaccggctgcaggaagaagaccaggtggcacaggccgccgccgaacacccagccgcgtggctcgaaggcataggccagcgtgagcggcacgcaggcggtgcacatgagcacgtcggacaaggccaggttgccgatgaggaagttcgtcacgttgtgcagccggcgcacccgcgcgatcaccagcaccagcaggcagttgcccaccagccccacgaccaccacgacgctgtagagcagcacgatcagccccttcagctgatgcaccagctgcaggctctggaagggcgtgacggctggagcgtccgcgccagccaccgacccgttgcccgccgaggcctctgcgctctggttggcgggagttgtgaccgccggcggcagcccagaaaataagtcagaaaccctggggccccgagtggtcgatgaggccatggccacctgttcaaaggtaatcaaagtccgtcacttcccttgccatactccatccgacctcctacaccagccgcgcccctcccccatcgcctgagtcctcccttgggaataaccggccacagaacaacagcaaaagtagcaaaaagtgttgtcctctcacctctgtaaaataaacctaagcacggttagaacatacggtttatttaaacgcttccgcctctatttacggtcctcgcagtccacgcaggcagactcaggagcgcgatcctacctgggagtggggtttggagagcgggaaagcactcgcgggaagaaggggcagaatttctgctggccctcggtagtcctctgcccacgtcggtgatccggtctcgcttctccgcgggagctgaacggatccaaatgtttcccagtgggctagcagcttcttagagggactgggagcgcctcccctcagctccgccccccactccagctcccatgtatggaaaataggggtggagcgcgctctgccatgctcggtgcttagagaactagtgaagaggacagtgtggggaggatggaatccgaaacgggaggaggggccggcaaacctggccagagcagcgaagaggacgaatctctactgcaggagcttgcacggcccctggagggtcagggtccggaggagcgcacagtggaggagggcggaggagaggcgcgaagcgtcaggctatcgggaggagccggtgcagtcttaggagggaaggagcggggaaggaagtagcggtgggagattgcaatgcagctgggggcttgagagaggcacgactgacccgttcttaaaggctggatcctgcctagcggccaggttgcggagggcagagacgctagagggctcgggctgggatttaacagcagagcctggagctggtcgcggacctgaggaccctcaccctcccgtggccccgccacacgagccccctgcttggctgcagcgcgctcagcgggcagcgggtccggccaagccaaaggcaggagtcagcaccacggacagcttccgctggatctgccgcccctcgggcggatgatgtggggaggagcaggggaaaatgactagggaattcctgcccctctctggatccgggtgtttggggaaggaacctggtccggttcaaagacctgcctcgctgcctgctttctgggctggggctgagaagagtagggtggagtggaggcagctgagccgggggcctgggggtcggagactcatgacttttgctcctcttggtggtcaccgcactcagtgccaaggacggcgtcgtcttttacctcccggggtcagaaaatgcagctctcctgccagttattctacacaggcacacttcagtctggcccagcgactccccggctcaccctttctctcgctttctttctcggctaccgcgacctgtgccgtatctggctgcttctcccagcacagagtagttcctggactgagacttgacccctccctccttgactgaacacccacaggcctcttctcttcattttaggattttttaaaaatactggtaattgcagatttcagctagggtaacaaaagtaacaaacatttgagaagcttaggcgtttcataaaatcttcagtagtattaagtcctcattgaaatgcaaattagcctggcccacggggcaagagccaggggaggaggggcctttgtaagctccctccttagaagctatctcattccctcagcctcttgtttcctttttccagagcatggagcttcattgtctcctctctgataagtccttgtactttgtcctctggctgcagatattccagttagactggaaactaatatcaatttattccaccctccaaatttaaatgaatcactcatatagaaaaaagtcaatattggaacaaaagtaatcaatgttatgcacctctgtccatcctaagctcacggtccctgagttataatcaatttagctaaaaccagtgtgtgtgtatatatacatgtatatgttaggacaagatctcactctgtcacccaggctggagtgcagtggcacaatcatggctcactgcagcctcaacctcccaggccaaagccatcctcccacctctcagcctctcaagtagctggaactacgggtgcacaccaccatgcctgactaatttttgtttatttgtttcttttg

SEQ ID NO: 136 - DNA, 6673 bp, Artificial Sequence
  subsequence of ARL5C
tgtcaaaatgcagattctgacccagtgagtctgggcaggggtccaggcttttgcctttctttctttctttctttctttctttctttctttctttctttctttctctctttctttccttctctctctctctttctttctttcacagagtctcactctgtcgcccagtctggagtgtaggtacgatcatgtctcccaggttcaagcaattctcccgcctcggcctcctgagtagctgggattacaggagcacacccccacgccaggcttatttttgtatttttgtagaaacggggtttcgccatgttggctgggcgagtctcgaactcctgacctcaagtgatccatccaccttggactcccaaagtgctgggattacaggcatgagccaccgcatccggccacagttttgctttttttttttttttttccttgagatgtagtctctctctgtcgcccaggttggagtgcagtggcacaatctcagctcactgcaacctccgcctccctttgtcgcccaggctggagtacagtggcgcagtctcagctcactgcaacctctgcctcccgggttcaagtgattctccttcctcagcctccagagtaggtgggattacaggcatgtgccaccacgcccagctaatttttatatttttttagtagagatggggtttcgccatgttggccaggctggtctcgaactcctgtcctcaggtagatccacccacttcagcctctcaaagtgctgggattacaggcgtgagccaccttgctcagccctttgttgttgttgttgttgttgttgttgtatttttagtagagacgaggtttcaccatgttggccaggctgctcttgaactcctgatctcaggtgatccgcccgcctcggcctcccaaagtgctgcgattacaggcactttgagagcaacagcgcccggccatggttttgcattcctaataagctttcaggtgatgcctgtgtgactggtctgtagaccacactttgaggagcaagagtttagaaaaatgagacagacacagtgagggacatcagagaggtgctttgtttaaagtgacatagaaaatatacacatgcttttatatgtaaataatgcttctgaaaagttacgcaaagttacaataggaggaaaactaggagccagaggcaagaaggaaacttacttttcaccgtgtattcctccattgtttgaaattttcctttataattttttaaaatcattacatgtattactttttcatggaaaagcttctcctaagtaaagtactttggaggctgtaaaatgggagaggtgccatccagagagcgaatatcggggaaagctgcgatcggtatttactcagcaccacccatatgtgccaggcttgctagaccaggagctacagagcctcagtgagcctttgggtttgaagaaggggaagaaagttaactggcagaggggacaggggtgagaaaggagggacctgccgctagagggagcgaagagcagggaggcagtttgggacacttggcaggcctggagctgggtttggcagggcccccgggaagatggaggaaagcagtgggagctagggttgcctgtacggtgcaggatttgaatgccagaccgaggagccgcagtactaggaaggtccaagcagcgtgcccaatcgctcctccggactacagaggagcccgggaacccagggaagagctccagtgattggtccccctgcctgtcagtctggtgggaggcccagctctctaccctccccgcccgagagtcacttacaaccggtagagaatggtggtctttccttcattgtccagtcccacgatgatgaccgtgtgctctggaagcgtcggaggaagggcagcgtcagggccaaacccgaagaccaagggactgtgtgcccccaccagacctcccaggaaggagatagcgctccccgcaggctggggacctctgcccaccgtaccgcgtctgcttcccacccagctccgacacctgccccactccgggacggtggaaaagacagctgagcccccacctcccttcacattccagaaaagtgtctgaaaggcccggggcgcttcggggcttgccaagagacggtgtttagagaaagagcataacgcgaagtcacaatcgcaggaaactcgcagcagccccccatccccgccgctggctccgtttagcggggagaaaggagggtcgcccagctttgcgtcctggggcgcaccgaagcgccgggacccaagaggagcaggcagggacgggggcaggggaggccgcggggcagtcgaggagcgcccatatacgaccctcggagcccgaggtccccccgtgcgtccgaccacagatcagaggagtcccagaagagggcgagatcaaagcgctcgcttggatgccctgtgcgccccttaccctggttcccgaagatgctcattaacttggcgatcagctgtcccatggcacttcccgggccggacaggtgcaggagggctcagcggcctcaggagcggagtcggccctggtattcggagctccgctcccccgggagggtctggcagattttgcctacgaagttagggaagccccacacgtcaccaacctgacctgggaaccctctgggacgctggcccttcgtgggcactatggacaccccagtgactaagggctgcctgtcccgggcccaagaggtgcaaggaatatgggggttccaggctccagccctccccctcgccctgcgaaaactcctgagttctccgggtggactgctccactaccgcaaatcaggggagactcagcactgcgcgcggaaccggatcccagctctccctcctctgagtgccatgtctagggcactagactgaagcaaaaccccaggcgacccactttctgtacctaccagctgtgtagtacagacagggctcaccgatcctctctgagctgggagaatattccaaccctccacagatgtgcagttggttcactagcgtgggtcttgtgggcccactcaaattgcattcccctggggaagggcagggtctccccttgatgcttggcaacttctaggataaatcagtactcctacaattcacggacaaacctactgcccaggcacagcttcctgatccccaaaagtgggcgcctgaagacaaggatggagcatgaagagagatcctccggctggagaccctgcagagaggccccagatacctggcagaggagtacatgggccaacagagaaccaggaggccaggcctgaggagggaatggaaggtggagtttcctgctgttgcttgtgaatttctttctttgcttaagctggggggaaaaaaacaaaaaatcagataacaaaaggagaagtccaaaaggcaacgtgccctcaggctgcaggaatggttagcaggagatccagccaacacaccagggagccagctccttccacccgactgtactgccttcctgcagcctccactaaggtaacaaccctccattaaggtaacaactttctaactggtctccctgcatcttcctctcctttcccaaggcatcctctccatggcccctattaaccttcctaaagcacagctcagggtctgtaactcccccagctcatagatcttcaatggctccctattgctcactggattcagatcagtctccacttgacattcaagagcttccacgaacagcccccacctgccttcacaggtttatctcccaggctctgtatctactggttcctgcctatacatgcctggctctttctgatggtgcctttgcttctgcatttcctccttgagtgcctttcaccttctcagaaaggagaatgcctgagacccattagctgccctgccataaaagccacctgcttccccagccctgacttggttctccagccacatggggcttctccctacactgggcttatagacgggcaagtctgtttcctcccatcaactgtgagtaccagggtgggattcatatattgttaaccagcatatgacctcccccgccagcccaatcactccctgcctggtccagaaccctgcacacaggaggaatgtgttgctgtcagactgatgtagaatgagttaagctacagcctgagaaatggcacttggagtattaaaaaaggaatgtgaacacaagtttaagaggattgaggaaggctgggaagtttgcgggaagaagaaggaaaatagctgactaaatacagactttcatcccaccctgcttggtgcccagagttagaaggatagagttgactgccagagcccatctgggctgattgcatttcagccttaggagagaaggagccaagtctggggctggggggtggggcaccaagggtgctgagggaagcagcagtgtcttaagcattttaccatctgtttcctggggttagtgggatgcggggaggaacatcttagtgcatgctgccctccccacctcctctttgcagaattgaaagtaacactctgcaagctggaaacacattcagtaaacagacaaggagagggcatctctctgagcatactctggctctggaagctgcctgattaaaaaaaataataattaaaagagaaaagaagaaaaaaaaaagaaaagaaaatagaaaaacagacgagaagatctgcctccactttgaggcccaggacctggatcttaagaagcattcattcgttcattcattcatttgacaaatatgagccaggaaatacatgaagtagacaaaacagacctagtccaggtgtttatgtttttgttttgttttgttttgttttgtttttttgagacagaaccttgctctgtcacccaggctggagtccagtggcaggatcgcggctcactgcagcctcaacctcccaggctcaagtgatcctcccacctcagcttcctgagtagctgggagtagaggtgaaagccaccactcccagctattttttttttttttttttttttgtagagatgggcttcgccattggtctccaactcctggactcaaacaatctcccgcctcagcctcccaaagtgctgggattacaggtatgagccactgctcccattcccagtctgggtctttatggagcttgtggtctagagagagagacagatacacacacacacacccctctgagagacagtaggaaggcctgatttagaaagaaagcaaggcacccttctctgaagaaaatgagaggtgaacctagctggacttcctgggtcgagcggggacttggagaacttttctgtcttacaagaggattgtaaaacgcaccaatcagcgctctgtagctagcaagaggattgtaaaatgcaccaatcagtgctctgtaaaaacgcaccaatcagtgctctgtagctagcaagaggattgtaaaatgcaccaatcagtgctctggaaaatgcaccaatcagcactctgtaaaacgcaccaatcagcaggatcctaaaagtagccaatcacagggaggattgaaaaaaagggcactctggcagggtgcagtggctcgggcctgtaatcccagcactttgggaggccgaggggggcagatcacgaggtcaggagttcgagaccagcctgaccaacatggtgaaaccccatctctactaaaaatgcaaaaattagctgggcgtggtagtgcccacctgtaatcccagctactcaggaggctgaggcaggagaattgcttgaacccgggaggcagaggttgcagtgagccgagatcgcgccattgcactccagcctgggcaacacagtgggactccatctcaaaaaaaaaaaaaaaaaaaaaaaaaagaaagaaaagaaaagaaaggaaaaaaaaagaaaaagaaaaaagcgcactccgataggacagaaacagaacatgggcggggccaataagggaataaaagctggccacctcccagccagtagcagcaatgtgctcgggtcccgttccacgctgtggaagctttagttctattgcattcttttgctctttacaataaatcttgctgttgcttaatctttgtgtccgtgccatctttaagagctgtaacactcaccgcgaaggtccgcggctccattcttgaagtcagcgagaccacgaaccccaccagcaggaaccaactccggacacaaaaagattattggagctaagacaaaatttttctctaagatactgaactgggacagccccttgtccctggaccatggtggcctcagcctagttctctttagtgtagaacagtggaaaccttaagccacatgtaggacctgggcctctcccacatcacctcattctgggacagaacccactgcaaaaacaggagcagctagtcagggaaggaaacaaagggtcccaggtagcagaagtccccagtccctcagttcctgcctggtctcagctgacttcatggttgtcgaaatcctcacacatggacaaccactaacttgctgatggtgtagccagagttaattgagagcttctgattaccaagaaacaagaatctgcccccatctctcgctatctccaagccagctagaaatgcctttcctgcaagttccaggcaaatgcaatttcttttctctcttttttttttttttttttagacagagtctccctccatcgcccaggctgtagtgtagtggctccatctcagctcactgcaacctcccc

SEQ ID NO: 137 - DNA, 1006 bp, Artificial Sequence
  subsequence of PAX9
cggagttcggtcgattcgatgttggggtttaaagtttttttagttatacgtttgggtcgagtcgtttttagagttttcggtttttgttttttttgggcgggtgtatataaggattcggttagcgtcgagtgtattggttttttttatttagtgtagtttttttttttatattttcggttcggtttttagttttttattgagtaaatatttatttagagagcgagtcgtttttcggaggaggtttcgacgcggttagggaaaggttttttggtttttttttggtttgagttagttgtaggttttattggtgttttggttttggttttaaatttttttttttagtcgaaattttttcgatttttttgagattttttgagtttagagtgagtagtgtaattaggcggtagattttagttgatttttgtttttgttttaggttttgtatttttatatttatcgggattgattagattttagtgttttttttttttttttttttattttttttttttgttttagattcgtcgtttttcggtcggttttagcgggtcgttgattatttcgttttagtattcggttcgcgtttcgggaaggttttagtattatttttttttgttgggatttcgttgattttgtttgtagtttcggttttttttgtttttagagcggggttttcggtttgtcgcggatatttagtggtttaaaatatttaaaattgattttttttgcgtttttgagaatgttaagagtatttagtatttgtaatcgtcggtatgagtggggtttgcggggagtcgttagagttgcggataggttttttgtttattgagttgttatttttggtacgtttaggggattcgtagtagttgaggttatatggttatagttaagtttagtaggtggaaagggagagatggtattgaatttatgtgagaattgggaagatgtgtggtagttgaaggagttggtaggaataagagggagttgtatgttatttttatataat

SEQ ID NO: 138 - DNA, 1001 bp, Artificial Sequence
  subsequence of HOXD10
tggtttttttgagagtcgaagtttcgtgtagtttttcggggcgtataggaattcggagttaggtaggaggatcgagcgggaggataacgtagggattaatttatttatggggattcgggttcggttagttgtttggtttttcggttttcgcggttttttttgttttcgtttttttagagatattttggtcgttttttagttttaagggattttttttttggatttttggggtgggatgttttagggttcgcggaattcgatttattttttcgttgggttgttcgggattaaattaattagtttgcgtttttattcgtttgttttggattcggtttttttaagcgcgttttgtttggttgtgtgtggggggaatgtttttgtgcgttggcgttagggtattttggttttttttttcgttcgtgcgtgtttatttggaggtttttagagttgagatttttttttcgtcggttgggtttaggggtcgaagcgggggacgcgagtggggcgggttggtcgagcgagttttggagaggcggataggagggcggcggagagcgttgggtcggttgtttttagcgcgtattatcgcgggcgcgtagtagatgtcgttgttgttcgtgtttattcggtcggtcggttaggttttggagtacgtgattcgagaggaggttgcggtttaaggttatttttaaattttattggtttggttgttatgtggtcggtagaggtatttataattatacggggaatgtttttttagagatgttagtttataaaggatataattttttttttttaaatttttttttaaaatgtttttttttaatagtttttttgttgttaatatttttttagtagattttttgattagtgtttgtaggagtgatagtttttattttagtagcgttagtatgtatatgttattatttagcgtagatatggggatttatggaatgtaaatttgtggattgttttcgtttttggttaaaagagaagtgaat

SEQ ID NO: 139 - DNA, 468 bp, Artificial Sequence
  subsequence of TBX20
gtggtttttgttttttattagtgcgtttttagtttggggtttttattttttttagagggattttggaaaatgggacggttgtcgaagagaaggcgaaggttagggcgcggagttttacggtaattacgcgacgcgtagtgggagagtgcgaattttatggtagcgttcggattaagcggatatagatttttttggttttataaaggcggttgtgacgaggattttttacggttttgttggagggcgttttgttagttttgtttagtttgaataatttaaatttttcgaattcgtagggtaattcgtttcgtttggagtcgtgtaaatttaggttgatatatatatttaagttgtatatgtaaatatttgtttttttttttagttagtcggtttggttattagaagttttttcgtgggttttaaaattaaaataataataataatttttaaaattttaattttttattg

SEQ ID NO: 140 - DNA, 1003 bp, Artificial Sequence
  subsequence of CACNA1B
tcgagggtatttaggggcggtgcggtcggtagagtgggtttcggggacggttcgggttggcgttgagcggtcgtcgaggatttataggttcgttcgtttttgggttcggtttagtttcggggtgggaggcgcggggcgagggaggcgtagtcggaggggtcggggcggggcgggggcggtcgcggggcggggtcggcgcggtagggtgggcggggtcggcgcggattggtcgggtttcgttacgtgatcggttttttatagggcgtggcgcggggtcgcggagtcgggtgaggcggcggcggttgcggcggtggggtcgggcgaggttcgttgcggtttcggcggtttcgtggttgtttcgttttgagcgtttggcgcgtttcgcgttttttttgtcggggtcgttgggtcggggatgtacgcggggttcgggagttatggttcgtttcggggacgagttgggcggtcgttatgggggtttcggcggcggagagcgggttcggggcggcggggtcggcggggcggggggttcgggtttcggggggttgtagttcggttagcgggttttttataagtaatcgatcgcgtagcgcgcgcggattatggcgttgtataattttatttcggttaagtagaattgttttatcgttaatcgttcgtttttcgtttttagcgaggataacgtcgttcgtaaatacgcgaagcgtattatcgagtggttatattttgtcgggcggggtcgggcggggtcgggcggggatcggggtgggggtcggggtcggggttattttttcggtggtcgggagggcgcgatttggggaggcgtcgggagacgggcgaggggggtacggagcgttttagggtttttcggagcggcgggtgcgggagtattttcgtgagtgcggcgggcgcggggcggagtttttttgtttcggattcgttttttcgtacgtcgggttttggggattttggtcggtgtatagtgcgcggttagtttggaggg

SEQ ID NO: 141 - DNA, 1058 bp, Artificial Sequence
  subsequence of ZIC1
aagtaatagggtaggagaataagtcgtaaacgtgaaaattagaaattaggagttaggtggaagtaattcgaaatcgtgtgtagttttgggtaatacgagtttttagatttgatgttaaaaatcgattttttttattattaatttttttaaatataaaaataaaatgtagatttaattgtattagggattataatagagttaagatatttataattttattgtagatgtaagaatttattgacgtttcgggtttttaagtttgtaaagtgttaattttgggttgttggttttttgttttattttttttttatttgtttagtttttgaaaaacggtcgcggtatttttttttaattagattttttttattttattttggtattaggggagaagttttttaagtgcgagtttgagggttgtgatcggcgtttcgttaatagtagcgatcgtaagaagtatatgtacgtgtatacgagcgataagttttatttttgtaagatgtgcgataagttttatacgtattttagttcgttgcgtaaatatatgaaggtaatcgtcgtattttcgtcgttttttttgaggtaggagtttttttggttttcggtttggggtcgggcggcgagtggtagataggcggtggcgggagttagaggaagcgggaaggtaaaggttttatttagtggaattgggtagagaaggtagggcgggatttggaaaaggggatgggagtgtttaaggtcgttttaaatttttggtttaataataaaagttaaaagaggcgagtatgagtaaaggtcgttattgaatttggtttagagttagggtttttgtagggggttgacgttgcggaaattgttgtttttgtagttgttagtgagacgtaagaattggatttttgcgtttaggtttgagttttggtttatttaaatatggataagtaaagtttagggaaagaaagtgtagtttttggttttatatttagtttttttttttttagatttattttttttttgtgagttttggggattttgatttttttaggagtacggtttttgtaggt

SEQ ID NO: 142 - DNA, 851 bp, Artificial Sequence
  subsequence of SIM1
tttttgttttatttatttttagtttttataagcggtagaggtttcgggggcgtttattttttaattgtttttatgtttatcgtttaatttagcgatatcgtcggttttttcgttttttatcggtagagaggagtagagtattttcggtttttttttttggattatgaattggaggaggggtgcgtggtagaaagaggaggatgtaagttttgggacgagtgaggtgattttagaattttggtttttcgtagttgttacgaagttagtttattattatttttaattggaagtcgaaaattgtttttcgtaatttttttatagtttaagggtttagttttaattttatttcggggtcgtttttttttcgtttttttttaatgttatttataagttttttcgttttttattggtttggcgcggttaggggcgaggcgtttattggttaatagggttgagtgatacgagtcggtttcgagtcgtttttcgcgcgtttaggtttcgggttttgaattttattattcgcgggatcgttggatttttaatgagtttagggtgtcgggtcggcgttgttcggttgtcgtcgttgttcgcggttttttgggttttttcgacgtcgtgcgcgattcgcgtttttcgagttttttggggtcgggtggttgagcgtttagtttagcgcggcggtttagtagaatcgggaacgttcggaggtagcggaggtcgggtttgcgggttaggtttatcggcggaggaggtagggttcgtttaaaggtttatttcgttggtagtcgttggtcgacggcgtgcgcgaggtcggtttggggagttattttttttttttcgtttttttgaaa

SEQ ID NO: 143 - DNA, 1068 bp, Artificial Sequence
  subsequence of DLX1
ttcgtaggcggtagttacggtcggattgagtttttggtaggttaaggtttggatttcggttttttttttattataatttttttttggttttttgagagttgttttcgtgggttgacggcggcgggaggttcggttttcgagtttttggtttttatgggggaagggaggaaggagggatgtttttgtttttttggtagggagttgttagttggcgtagggttgggaggttttatttttgttgttttgcggtttttttttttttttttgtgatttaggtaggtttagtggttttagtttgagttacgttgttgttcgtttttgtaggttaagatttggttttaaaataagcgatttaagtttaagaagttgatgaagtagggtggggcggttttggagggtagtgcgttggttaacggtcgggttttgtttgttggttttttattcgtgtcgttcggttggaattttaattttttattcgggaagggtttaggaggaaacgcgggtttttatatttttagttatatatcgtggtattttttagcgtattaagaagttatgtagtaattttaatttatgtgaggttgttcgttcgttttttttttgttttttcggtttaggtttttttcgtttttaggtttatttatttcgttcggaaaagaaggatttagagggaagaaggaatagtggaggcgggacgttttttattttttcggagtttcgcgaggttcggtttagtaatttttcggtattcgcgttttagtttgaattttggtttgggtcgagtagtggtagtagagagtggtttcggagggaagttattgttatttgagatagtttaagtagtaagataaattcgttttattcgattcgtcgatttttagttttgtgggattattaggaaaaaataaaataaaaataaaatgtagaaaaagtaaaagtttttttttgttttgttagttttttgtttttttttgttttgtttgtgcgttggtaaagtttaggtttttattcgttcgttgtttttattttgcggttttagtaaaaagttataaggtttgagcggttcgg

SEQ ID NO: 144 - DNA, 1008 bp, Artificial Sequence
  subsequence of LMX1A
ttaggtcgcgagaagagggcggtatttatgagacgtcgattagtttcgagattaaaaatttagttttgggtatttttaattatttgttatttagacgtttacgaataagttcgttcgtttttcgcggttttggggaattcggtgtttagtgcgtgaggtttggggcggtttgttggatttatttgggtagggacgatttataagtattgacggatagatagtgatggggtttaatttagtgtatgaagaggggcgttagtttttttatcgcggattaggttttagagagcggggttttagagtttagcgttaagcggaaagagagtgcgtttaggacgtacggtttgaatatttatttagtagcgaggagaaggaggtcgaggtgtcgatcgcgttttggaagtttttttttatttttaggtcgtttagtatgttcgggtcgggtcgggaggatttgtagaggagaagaaacgatgcgtttgacgttcgtgttcgttgggattcggcgttagtagttatcgtatttttgggaaagaattgagggagtgtttagggcgattagaattagttaggaggatagggtttagttaagagaatgtagggtgggaggagagattagttatagcgaattgttttggttgatttgattttatttgaagttaatacgttatgtatttaggttttcgttttttaattgcgttttttttttttttgttttttttatttttatttatattttttgttttaggttttttatttcgaattcgatttcgttttaatttatacgaaggtgggttttcgggacgtttttgtaggaacgtagttattggggtatattgggtatataaagagtgggtattttttttcgagcgatcgggtttaggtacgcgggacgatggggtttgtaatttcgcgttttagtcgtttcgttgcggtttttatttgttttaggtcgagaaggggtattgtaagggattcggagggcgtttcgttcgtttttggattttt

SEQ ID NO: 145 - DNA, 1007 bp, Artificial Sequence
  subsequence of DLX6AS1
tcgtggcgcgttattttggtatgttgtgtgcgggttatattatttttagttttttattttcgatattggtaggaaagtttgatagttaggtttgaagtttagattttatttcgtaagcgtagagatattatattaagtgggatttttcgttcgttttattttttagtttttgattgtttttgagtttagattgggtcgtttagtaggttttagtaggatttttattatgtattataattattattttagtgtagttgttttattggaatagagtgtaaggattttagttattaattattaggggaaggttgagagttttgaagttataattcggataattttagttttttcggtttttttagtaattaaataaatgagaaaaaaaaatttttttgtaagtagaggtagttgtattttggatatagtgtttaattgtagggatttttcgaggttttgttacgatatattttaattggggtgtagttagagttgtaggaagttggcgaggaaagcggtgtatttgtgagtataaagcgaaaaatatagataagtatagggtgagggtgtagggggtgaaacgtttttacggtgttaataataagttgtagggtataaagtaataaaattgttacgtttatttgttggtattgaggatattataaatagtttcggcgcgtagttcgcgtgtatcgagagcgtattagggttgggagtgggaaggtggggtgggaaattttttttttttttgatatttttttttgttttttattttttatattttttttttatttagtttatttttttttttttatgaagtttttttgttgttgttttaatttattgtcgatttgtaaacgtgtagatcgtgttattggttcgcgtgttaaagtgtattttttgttaaaaggtggggaatagggtacgttatttaaaaatgaatttagagttattgaatcggttttttagatttaagaatttaagcgtaacgggttgggaaaaggaggggg

SEQ ID NO: 146 - DNA, 973 bp, Artificial Sequence
  subsequence of MIR196A1
ttatattcgtatttatcgtaaaaacgtagttgtgtaggtcgagggcggcggcggatttatttgggcggcggcggtgtcggtagtgcgcggtcgtcggaaggtgcggagttagcggtcgcggtttagtttaggttttttttcgttttcgtttagaagcgagggttcgagtggttacgtgttcggtagggaagttcgaggtagcgagggagtttatttggtcgttcgttttttttttcgggtataaattttggggatcggaaatataataaaattttatcgtgttgatgaattttaaacggtttatatttttttttgttttgaaaagaaagacgttcgggggcggattaaaaggaaggggaaataaatttacgagcggtagaagtattcgtttcggtttttttttttgttcgtatattttgttcgcgtggagagaagtagttttagttttcgggatttggttttcgtcgaatcggtcgttaggcgcgtttttttttcggaggagtcggcgttgatttagttcgcgttcggtagagattggaagtcgtcgtttatacggaaaatttatagagtttcgcgtagattttatgatcggttcggttcgtcgggtttgggatgaggttttttgtttttcgttagagtagaattgggttttttggcgtttttttgcgaaagtttaggtttttttaattacgttcggtggtttttattttttgtattttttcgttgaaagcgggtttttttttttttttttttttttgatagagttttgttgtgttatttaggttggagtgtagtggcgcgatttcggtttattgtaattttcgtttttcggtttaagcgatttttttgttttagtttttcgagtagttggaattataggcgttcgttattacgttcggttaatttttgtatttttagtagagacggggttttataatattggttaagttgattttgaatttttgatttcgtg

SEQ ID NO: 147 - DNA, 1050 bp, Artificial Sequence
  subsequence of FEZF2
ttttaaaaggaggtaattggcgttcgcgtttttttcgggaaagtgcgagcggtttgcgaatagggaaagagggaagagacgggagggggagggggaggaatcgtgatggttttgtcggtggaaggaaagggggggggggatttaaatttaaatttaggtagagtttcgtgcgtgatttataattttggaggtttgtaggtttgggggacgcggggagggcggagggtttcggacgcggcgtttttaaagggtttttgggtattagtttagtagtcgaagtattttttagtttttcgtagtcgagttgggtatcgtgttaataaattgttatttatttacggaatcggcgttagtttcgaatacgcgtaaatgataattattttattaggatgtggcgtatggacgcgggcgtcgcgtttggaggggggaatttgttaatggggaaatattaatttatgtaaaagtaatgagttcgttttggttggcgtcggaggtcgggagaaagtttttattgattaaggacgatttcgaagcgttacggagagtaaggtcgttcgtcggtatttcgggggtttcggcgtcgcgtaggtgcgtttttagttttatggttagttttgggtttgaggttgggggagattaaatcgagagttggaagattttcggagattttaatagattagaattgttgatttatgatcgggtttttgaggtaaagtcgagttttgtttttggtttagggttgcgtgcggggaggattcggagggtagtttttttagttgatgggtatttattgtttgtataattgagaaggttttatttttatttgtttaaggagtagattgaaatagtagaatttttttttggattttattaaaacgtttttttttttaaggttatttagtcgaattaatttttcgaagtgatttatagagttgaattttgttaaggtagtttttttatttttagttattaaagtatcgcgtggaatcgggttttgtgtttttttaaaataaagagaaggattattagagaggagagggagggggtttg

SEQ ID NO: 148 - DNA, 974 bp, Artificial Sequence
  subsequence of STAG3
cggatagggggcggggttcgaggcggggtttcgttaataatggttcggagtcggttttaggggcgggggtaaggaagaaattaagttaatgtagcgcggaagttcggtaggggggcgggattcggttggtatttaggaggttggtgaaataggggcgtggtttttttcgggggcgtggcgattcggtttaaaaggcggggtttgggtggaatttagtttatggtaattgagaagttagattaaaggggttattagtagtttggtttaaaattcgtttaatggagtaggagattgagggtagcgggggtgggatttgggtgggggcggggttaaagcgggtcgttcgcgtgtttaagtttacgtgagagggtaggacgtttgagagtttgaggttatacgaggttgtggagcggcgtgatttaaacgtggcgcgtattagttcgtatatttttaaatttcgcgatagttattggttttgggcgagtcgttgggattgcgtttgcgtatagcgtgttttgtacgttttcgcgtttttttggaatttttcgttttcggaagggtagcggcgggcgtttgtgtggaaggtggggtggttagagatattcgagggatttgaggtggggattttttttgaattttgttcggttagaagttatttttttaggttttgataggtttttttttgatttaagaataggttttttcgcgattttttcggttttgatattaggagttttttcgggtcgtgttttaatggttttcgttatagagttggagaattttttttttaggtttttatagattgagagtttatttttttaagcgtttggaaggttttttattttggagtcgtttattttaggggtagtcgtagatatttttattttttggaaaaataggaaacgcgtatttgttttttttttttttgcgtttttagttttatttttatggcgtttttatttttaaatttttaa

SEQ ID NO: 149 - DNA, 981 bp, Artificial Sequence
  subsequence of PTPRN2
taataatattgaaggattcgagggtggttttttcgtggttttgaggttaacgttgtagcgtatgtagtaaatatttgttaaggatttattgtgtgttcggtatattaaggtaggtaataaaggatttagtgtatgttcggtacgtagaggtaggtaataaaggatttattgtaggttcggtacgtagaggtaggtaataaacgattagttttagaagtagatgtgtttgttgtaaattatttttttacggtttagtagaggtataataagtagcgaattttttttagggtttttcgtgaatacggtattttacgttgttatagcgacgttattttagttttgagtcgtaataaagcggtagtgtttgtgttttatttttggttattttgttgagaattatgtcgattaggacgtaggtgtcgtttcggtttgtatcgttattgttaatagaaggagagaaatgaaagtgttgtcgtttatacggaagttcgatttataataaagttagtgatagtttattttttttttgtttacgggggtcggcgagaggaaaggatggcggatgtgagagggggaggaaggacgcgggttgggagaatttaagtgaggggagaagggaggtttttgggggtttcgagtttttgagtagtttgtagtttgtgggatgagttgttgtgtttagatgtgatttttttttgtttgtttttttttttttggttaaagatgtggtaaattttgttagaataaaatgaattaagcgtttgattgtgttagagttgatggtatttgtattgaaaatatttgtaaggtgttttttttagtgttgtcgggtaatttttcgagcggagaggggagggcgttgggcggttgggtttcgttggtttatgtacgtagggatattttaggtatatttttttaggttgtttgttattttttttaaacgtaggtttttcgttttagaaggagaaattgatataatag

SEQ ID NO: 150 - DNA, 1004 bp, Artificial Sequence
  subsequence of BARHL1
ggggtatcggatttgaattcgttttttaatttttttttcgaatatatttattagacgtagatgtaaatgtataaatatagaggtatttatatatttaatttaaatagttatatatcgatatatatattaatataatttgtagttatatacgtacgtacgtttagttttatagttattcgtacgtttttagtagaggtaggaatggtgttttttataaataagttttagaatatatcgttttattaataataaatattgattattgtttcgggtattaataattaaggtttgttatagtaattatataattatgatgatgatgaataatttagggagggaaatagggttggtgtggttgagtttattttagtgggattttggttggttcgtttagttttatttgtaggtgagtttagggtttaggtttgatttttttaaattttaggtcgttggttggttaaggtttttggattttggggttagatagtgcgtagggttcgtagtgcgagttttggaggatggtaggtgtagtttgttttagtcggtagggcgtgcgagtcgggagcgggtttttttcggttgttattttaggtttgttcgtttttgttagtttgtagttcggttagtttgtagaggaattaatcgtatttttttttttgaagagtatttttttatttttttaggtttttttagggtgattttatttttataaagaggtacgcgtagggaggagtattttttatttagttttaagggttcgttttgcgattttttgggtagggtaaggcgtagttagagtcgggttttggggttagatagtagggtttaaaatttaggtttttttttgaaaatcggtttagattttagtttttttttttgtaaagtggggtaagagttacggaaggtcggtggaagataaaaggagaggatgtacgtaaggcgtgcgatggtgtttggtattcggttatttattaataaatgagtacgattttttttggtttttt

SEQ ID NO: 151 - DNA, 1064 bp, Artificial Sequence
  subsequence of CCDC140
tgtttatgggtttataaattagttgttatttgttataaatatgtataaatggaggttataaggatgtgggggtgttggggatttaaagtttcggaattaggaggcgatttattttttttttttttcggttttttttttttttgtcgagcgttttgagatttatatgtatttagatgattagttcggttttttttatcggttagtggttagaggtttttggatattcggagaggggtgggagggtatttttaggttttggatagttgggttatatttaaagatttaatgaatttaaattttttgtggtttgtgttttcgaagttcgatttgggatggttaggatagtaaagttggttgaggttgtttggtttagggcgttcgtacgtcgttaaatttaattcggtttagagtcgtgatttcgtagaatagggcgtaataggttttaggaatgtcgggtgattttagttattttttttttgttttcgagttttgggttttttttttatttttttttgaagttttttcggagtttaagttattttatatttaaatttcgtagttggatgggagtttaggttatttttttattcgtagtcggtgggttaaggagttttggtgttaaatttggtcgcggtataggcgttaattggtaaagggatgatttagcggtggggtttggaaggcgagggttcgcgttttgtatttttgaattttggtttgggaggtagtgatttttatttgggttaataaattatttagaaagtattagtgggattttttataacggtgttgtgaacgagtgtagggtttatttacgttttgtgtacgttcgaaatgaaacgggagttttgaagacgatatttggataatttgataaaaaaaaaaaaaaggtgggcgggggagatagtttttattgttttttttgcgtttttgtttttagttttagagatattataggtgaaaataatagcgggttggttgtttaggtttgagtggagcgtgtttttgttagtttgaaagttttttttcgtagttcgtttggatgcgtgcgtttatagtttagt

SEQ ID NO: 152 - DNA, 1780 bp, Artificial Sequence
  subsequence
cgtttcgttggggtttttttcgttttgtaaagggagcggggagttgggggagttttgtatattagtttttttggagttgtagacgaggagtttcgcgttttcgggagtttttcggcggttttttttttaacgcgcgattgtgtagttttttttcgtcgtttttattcgcggttcgttttcgttttttttttttagtttcgttagtcggagcgcgtatatcgggatttcggtacgtgggcgcgcgggaggtggcggtcgttgttgtcgttgttgtcgttgtcggagttcgaatttaagttttagttggagtcggagtcggagtcggcgagatcgttttttatgttgcgggagttgcggtcgtttttcgtttagtttttggttttaggcgagtttggcgagtcggcgaagtatcggcggggaggaggattagaataggaggaggggtacggcggattgaagcgagttgggttgtgagtaagggatatttatagtttggagaaatagtttcgtttttttgcgcgttgtttgttttagtcgttattgggggttttaagtagcgcgatgttgtttcgttttttttaggcggcggtcggcggaggtttttcgtagtcgtttggtcggcgtcggtttttatttcgttggtaagttttttgtttatttcggagggcgtattcggacgttcgagtcggagcgagcgcgaagttcgaagttcgtttttagagtcgttaatttttttgtgagttttttttttcgtcgtagtttgcgttagatttgggagcgatgcgtttttattcgggcggcgcgttttttgttaattcgttatttatgggatcgattgtttttagttgttcggtttggagtgcgtagttttcgtcgcgtggtttaggagaggagcgagatattaaggcgtttcgcggatttcgcgcgtattagtcggtttggtggttttgcgggatagcgtttatatttaggggtgagtaggtcgttaatggaggttttttttatttttagttagcggtttgtatggacggtaaagagacgggagaaagttgggtttttttgcgtttaatttggtattggtagaggaatgtaatattgttttttttaattcgattgtcgcgggggtttttttagttttttttatttttaagttaaggagggagttttttttcgttttttaaggagaaaaggggttttttagagtagatcgttgatttttttattaacgtgttatttggggttttttagtcgttcgcgcgttaagttagtttttagtataagcgtttagagattcgtagtcgtttgggcgcgttaagagatcgtgggtagatttagtttttagggtagtttaagcgcgttttattaaagaaaaaagattgttggtatattaaagaagtgtgtgtgtgagagagaaagagatagagaaagagatagagagatatgggtgggggtattaggaaaggtagttcgagtaggaggtgttagtgaaatttattttttgttgacggatttagttttcggaatgttcgattgttttgattcgcggtgcggtgcgggttttaggggcgtataatatagggtgtttagatagagtttaataggtggtttgcgcgggtattttgtggttaggcgcgggggaggggaacggtttttttttcgagtttcgggttgtttttgttgtttttaggggtgtatttgaatatggataaggaaatgcgttttttgtttttaggttttatttggggtgagtgtgtgaggtatttaaatgttttttgtcgga

SEQ ID NO: 153 - DNA, 1038 bp, Artificial Sequence
  subsequence of GATA2
gtcggtatataggaggggtaggtggggatggggtggtgtgtagtaggttgggtgtttatagtagttaggtttgggcgtaggggattgttattttttatttttatgtttttcgttagtgatatttggtatttgacgtcgtttttgtttttttttcgggttgtattatttttcgcggaagatgaggttggagacgtagttttcgtggtgttagggttaggagatatttttttgggtggcgtgggtgggaagtcgaaaaggtgggagttagagtgggttgttgtaggggtgagggaggttattgagttttcgttgtttttttcgtttttatttttagtttttgggtatatagagagtgggtttttagggtttttagtagttgaggggtgtagtggcgttttggagaaggggtttacggtttaggggttgtggtggtgggtcgtagcggtagagagggttgttttgttttcgtttagttagggtaaattcgggttgtgtaataagtgtgggcggtatatttggttttcggttaggcgggttgcgggtaaagagagagaggattagggtgggtagaaagattagggtaggtagagttagggacgtttttgatagatattgagattacgatttttagaattagtagttattttttttttaaagaaagttagaaatataatattttatcggtaataattaggaatgttagtttaagttgaaggataagtggtatagaaggaattttatcggatagattttatagggaatttttataggttagttggaagtgggtagaaattttgtgggttttagattttttttaatcggtcgttgtttttatttttttcgttttaattttttagtagttcgatttttgcggattttatattcgggaagtaagtagacgggttttttttttttttttcgtttggcgcgcggcgtttgggtttttattattacgggtttagtgtttatcgtgcgcggggttgtaggagacgcgcgttcgcgcgtgagcggggttggtatagtaggggttgttttgcg

SEQ ID NO: 154 - DNA, 1100 bp, Artificial Sequence
  subsequence of ADCYAP1
gaggtaaaaagggaacgcgagttagggagtttgattcgttttgaatgaaaagaaagagaaattaaattaaattttttagttatttaaaatttttaggtttttagggaggttttgttataattttttttaagtatgattgtttttgggggaggggaaaggggtggttgtatttattgaaaatttaaatcgaaataataaatggttaaatgtggatatttatggatttaaatagttttgtttacgttagagaaattgagagtatagggtttgtgtgaagtttatttcggtagaaggtaatattttaataaagttcgtgggaaaatagattatattttcgttatgaataagttatgtagtgaaaaatattgtttatagtttgtcgatttatattattattacgttttttaattcggcgtgaggagggagaggagtgtttatatttgattaggaattgtaggatcgatgtaaattttagggtagtagttagattggtatatgtagggtttttcggttattttttttgtatgtcgcgggtgagaggaatagcgaggataatttagcgtaaatatacgaagggtcggattttaagggggtagcgttgggagaaaggttaggtttgaagcgcgcgtcgtttgttcggattttatttcgggtttttttcgtagggtttggtgttaggagattttgcgtggggaggggggtatcgaggggttgtcgtttcggttttttttacggttgtttttaggtagaggcgggcgacgcggtgggtagtgcgagtttcgggtttttttcgaaggttttcgcgtggggtggggttcgtttgtttttcgcggcgattgaatttgtgtttttcgtttcgttatttttttttcgatttttttgtttgtagtgggagtttcggcggcggcgcgggggacgacgcggagtcgttttttaagcgttattcggacgggatttttacggatagttatagtcgttatcggaaataaatggttgttaagaaatatttggcggtcgttttagggaagaggtataaataaagggttaaaaataaaggacgtcgaatagtttatttgtagcgatgggttattagttatttt

SEQ ID NO: 155 - DNA, 963 bp, Artificial Sequence
  subsequence of TBX5
gtagagaataattattgtattagggttcgtcgaggtacgaggtattttattttgttttgtaattacgacgattattatttttagtttgattaatgggtataatttttaagtagcgtagtggtggatgttcgtaaatttttgcgtatcgttggaaatttattaggttgagttgtaaaacgtatcgcgtagacgtttttggtggcgtcgagagaagagttaggtttgtttagtatagagtcggagagcgtcgggtttttcggaagggtaagtttttcgttaaggggtttcgagggagttggacgtttgaatttggatttgtttttagtttcggggttcgattttgggttttgcgcgtttttaatttttagggtttttcgaagtatggtttggttttaggttcggttttgtaaggattggaacggtagtaaaatgtgtagggaggtagtcggtcggtagagttgcggcgggagttaaggttaggttcgcggggagagcgggtagtttttagcgtcggttataagtttttaggttagttgggtcgtagatttttttgtttttagagagtataattcgcgtttttttttttagttaggttgtagtggttgtttcgagtttcgttttcgttttttaagttgttaataacgatatgtttttaaattcgaggttcgtgtttgtttttagatgttaagaacgtaattcgaaattttttttttaaattttaggtcgacgagatgagtttttatttgatttttgagtcgaggtgggtcggaaatcgaggtttaggtttcgtcggggttgtaaggaaaaggggaaatttcgagcgtagcgttttttttttgtggttttttttttcggtatttcggattgcgggttttgtagttatttggatcggtatttaaaggattttgtaagtttagttttatagattggtttttttagacgtttcgaagttcgtattacgaa

SEQ ID NO: 156 - DNA, 837 bp, Artificial Sequence
  subsequence
ttagtttttatttatatttttgttacgacgggtaattgggtatgtgtaggggaaaaatagtaacgttaaaacgtaattgtgtaaatgaggatagagagtgcgaaaggagggagaggcgaggagttgttttatttttagggaggttttggggagattgattagttttaaggatagatcgttgggaagggaaaaacggtttatatcgaattggatgtcggatggaaatttttttgcgttattagattgcgtttagtatagtagatggtacgagtacgtgcggcgtttagtttaggttttcggaggtagttgagttggaaatttcgacggaaagtatttataagtttttattttgcgttggtttattcgcgtgtacgtttattttttacgcgcgtttttggtttagaagcgtatagatgtttattgtttagagtcggtatcgttggggagatcgagcgatttgcgcggcgtatagtgcggcgttggtagggttttgggttttcggtcgggggttcgagcggttaagggatgggggtgggggcggggagagtggggggagggcgaaagatcgtcgagaggaggggggagtgggtggattaatgatgaaaaagttttttttattttagttttttaattaaatgtatggaaagaatcgaggcgagtatatttggttttaatttatagttttttgatggtattaaatgttttttttttagattagggttggaagttttgggttaattatggtcgtttggagtttagaaattatttatatatattcgtatttttttttttttttagtcgagttttttgattataggacgaaaaaaaaaaaaagtt

SEQ ID NO: 157 - DNA, 1012 bp, Artificial Sequence
  subsequence of NECAB1
tttgtgattttgggaaattttatatttgaatattatttaataatttttgttttatagtaaacgtttcgaagtttattttaggtagagtttatagtatcgtttttgttagtagtattgttataggtaagttttagaattttttggggtgagatcggtgtaattattttattgatgaggaaaagtgaggtttataggttaagtttttcgagcgtaagataatatcgaatggtttaatttttatattaaattagttgtttttcgattgttggtattcgtgaattttgttttcgtttttggggaaggtcgggtagataggttattgggattaaaagtagagtaggtagaatttttttgagtttttttttatttatggtatttatttaggtgaggttgggggcgtttttattttgcgttttggttgtttaggataaacgttttgttattcgttttttttttttgttcggacgtttttttttatttttgtatttggggtcgtcgtggggttggtaggggtttttaggttatttttagtcgtggtcgatggtcgtgtcgggggtagagttcgttttttttcgcgcgttgttacgtgcggggatgatatggatttagacgtcgttaattacgggaaggaggaggcgagagttggagcgcgtgggagcgtagaggtcggaggagggagggggggatatcgagcgcggagagcgcggagagcgcggagggaggcgcgcgcgggagcgaatattttttcggatttagagttcggcggcggcgaagtagtagttgcggtcgcgtttttgttagagtcggtgcgttcgtttagtttcgtttcgtttgaggtcgttagggttttcgaggatggaagatttttaggagatatcgtcgttttttaataatttttcggaggagtttagttttgttttgtatttgtttaagggtatgtcgatttttttcgacgtaagtatagatggtgggagttgggcggttgttttttagtatttttttttttttcgaa

SEQ ID NO: 158 - DNA, 1017 bp, Artificial Sequence
  subsequence of ADRB1
ttcgagtcgttgttttagtagtggatagcgggtatgggtttgttgatggcgtttatcgtgttgtttatcgtggcgggtaatgtgttggtgatcgtggttatcgttaagacgtcgcggttgtagacgtttattaatttttttattatgtttttggttagcgtcgatttggttatggggttgttggtggtgtcgttcggggttattatcgtggtgtggggtcgttgggagtacggtttttttttttgcgagttgtggattttagtggacgtgttgtgcgtgacggttagtatcgagattttgtgtgttattgttttggatcgttatttcgttattatttcgttttttcgttattagagtttgttgacgcgcgcgcgggcgcggggtttcgtgtgtatcgtgtgggttatttcggttttggtgttttttttgtttatttttatgtattggtggcgggcggagagcgacgaggcgcgtcgttgttataacgattttaagtgttgcgatttcgttattaatcgggtttacgttatcgtttcgttcgtagtttttttttacgtgtttttgtgtattatggttttcgtgtatttgcgggtgtttcgcgaggtttagaagtaggtgaagaagatcgatagttgcgagcgtcgttttttcggcggtttagcgcggtcgttttcgttttcgttttcgttcgttttcgcgttcgcgtcgtcgttcggattttcgcgtttcgtcgtcgtcgtcgttatcgtttcgttggttaacgggcgtgcgggtaagcggcggttttcgcgtttcgtggttttgcgcgagtagaaggcgtttaagacgttgggtattattatgggcgtttttacgttttgttggttgtttttttttttggttaacgtggtgaaggttttttatcgcgagttggtgttcgatcgttttttcgttttttttaattggttgggttacgttaattcggtttttaattttattatttattgtcgtagtttcgattttcgtaaggttttttag

SEQ ID NO: 159 - DNA, 1030 bp, Artificial Sequence
  subsequence of OTX2
ggcggttttcggtttaggtcgattcgtaagcgaatcgagttttcggcgcgcgggtttaaggaggcgtttggttttttattattgttgttttaatttatttatttagttatatttgtatttttttgtttcggattttaaaaaggtttttgggatttatttaaacgattttaattaaatttgggggttaaaacgtaaagatcgcgggagaagtttagaacggcgttgatataaaaataaaattataaataaaattttttaaaatattttagattatattcgtagcgtttcgacgacgttttgtagaagcgacgatttttaggagtacgttttttgttttttttttattatcgtttttatttttagattatatttttttttttgtaacgatcgttattatattttaaaatttgtaagagaaaaaatatattcgtttatagaattttacgttcgtagaggggtatcggtcggtttattggaggtattggggtgatggtcgatagatacggggatacgtagatatggatatagataagatagacggatatttattttatagttttatgggaggttagaaaaagttaaatattttttaaattttaaatagttagttattttaaaagaaattaagagtattgagttagaaattttgtagtttttatttttttatgaaaagttaaatataattaaaaaaaattttttttaaagaacgaaaatgaggaaggcggttagagttttaaatacgcgtgggtttttttgtaatatatataaagtagatgtggcgagtgagggttgttttagtaatttttatttttaattatagtggaggttgtgttggagttgaggtcggtttcgtttttagggagatttgttgagaaagcgtttttttggtaattttttgacgtaaattttttaattaatggtagggagagaatgattgatatatttaagttagagggaaaataataaaaatatataatagggggaggaaaataggtcgttgttgtacggggggacgagtaggtaataaatt

SEQ ID NO: 160 - DNA, 1076 bp, Artificial Sequence
  subsequence of NKX2-6
aagtgaatttttgagatttagggttttattttcgttaggggtgtgtgaagtatattgggtgttaggagaggatgggaatgggattcgagaggtttttttttggatttttcgagagaaaatggagagagtttcgaatttaggagataggaggcgtattttttttatgtatttatggattacgttttcgtttttatatttttttcgtaggaggtaagatttgagcgtttatttacgtggtttttttattcgtttcgcgtttatttttaagattgttttatagggatttttaggaggtttcgaattatttagttttttgttatcgtcgtcgttattagcgttgtgaatttttgattttcgcggttttgcgtttatttttaggtattgaaagtttttcgggttttttcgtattcgcggatgtggcgaagtcgcggggtagtttcgttcgcgttttagtcgtaggatgtttttgatcgagaagggggtggaggtgacggggtttagtagtatttcgaaggcggatggggcggggtcgaggaggttcgggtgaggagcggtattttgaatttttcgttttgtcgttgtaggtttcgtagatagatttaagttttgggatagacgtttagcgttttagatagcgtttttttttgggttatgttggtaggttcgggtttagggtcgggtgacgagatcgtagttttttattggttttcgtagaaattacgtgttagttttgtattttttttttttagcgtttttttttcgcgttcgtcgaattttttttagtttttagtcgtttttttgggaggtttggttcgtattgacggtttttaaagtaaagaaaacgtggagagatagtgttgcgcgcggtttggattttcgttaatacggtattagcgggagttttcgaggttaatttagggtttacggggatttttttagtggatatgcggggattggaggtggagtttttgttgtgtaattcgattcggtttatttagtttggttttagtttaattttgtatttttatggcggaggaaagttaagatagagatagttgggattcgcggaatttgag

SEQ ID NO: 161 - DNA, 927 bp, Artificial Sequence
  subsequence of SIM1
ttgatagagtttttttttcggaatgaatttaatatttttgataaaatatatattatagattcgatattattatcgtttttattttgataggaagaggaggaagataagcgtgtgttttgtttttttaaaatttttttttattttaataaataaacgttatattttaatagaaatgtattttttttgtagtttttttcgggaatttttatttttttaattaattgaggtgttttgtaggtaatgggggagggtggcggaggttttgttttatgatttgattacgatttggtgattgaggaggggaaagtttttttaggtcgaggttattgcggtttttgaatagtttgttttaattaattgtgtattttttgagagagtgtaggagagtttggtttagggggtaattttgaaaattttaaattttatgtattttgtcgggtttgtatattttcgttaaatgtgtattgtgtaagtttttttcgggttgaggcgtcgagtggttttcgtgtttagttttcgggcgttttcgtagtcgagttttttagagaaaaaaagagagggaaattggtgtaattagttcgaattaagtttttagagtagttattggtaggaggtttttttacgtattaaggcgtattcgattttatttttggtattgttgttcgttttgtttgcggtttttttcggttaaggagtttgtgtggttgatttgagggtatcggcgagcgcgtcgggttaggttttgttttacgtagtagtttggattttatagtgtgtgtttgtattcggtagtgttttgattttttttgtttgttgatttcgggttagagatatcgcggtcgtatttagggaatttattaatgttattgtaaatgtggggtggaggtcgaaggttatatcgttgtttgttttttttttttttttttt

SEQ ID NO: 162 - DNA, 927 bp, Artificial Sequence
  subsequence of DRD4
ataggtagatgtaggtttagttttttggttgtcgtgggatatatatatatatatattgttatagttattgtttattatatatatttagtgtagatgttggtatatttttagaaggaggtttatagttcgtaggggagatttgggttggataaaatttaggggaggggagggtgtgtggggattaggtttttgttgagaattttggggggaagtttgagggggaattgggggatggagtttatattttatattaggtttggttttcgagtgggtcggttttggtgttagtttttttgcggttagagaaaagtagtttagggttgagttggagacgcggtgttttcgattgtgggggagggggattcgaggtttttttttgatggatatagtgaatttaggcggttggggtagagattagtagtacgggatacgcgtgatttgtgtttttttcgagtcgtagacgttatagtgacgacgtttaagtttttaatttttttaaatcggcgggaaggattagaggggttgtttgtttttttgtttttggagagagttattttacgtggagttttacgttgggtattgggtacggtttttatatttttaattataatttatttttaagataattatgatgtggatattattattatttttgttttatagatgaagaaatagaaatgaattaacgtgttcgagttttttatagagaatttagttaatagagtagttagtttcgtttttaggtttagcggggattttgtttattttaggttggggaggggttttttttgagttcgatgatattaggttcgtttttagggaattttttaggtcgtttttatgtttgtaataaaagggagattaaggttagaagtcgtgatttacgtttgtaattttaggattttgggaggtaaaggtaggaggata

SEQ ID NO: 163 - DNA, 810 bp, Artificial Sequence
  subsequence of TBX15
gaaaaggtttggacggtcgaaataaatttttttttaattttttttttatcgattaataaaaataattttttagtattaaatttaaatatcgtaacgggttataaaaatacggagaatttataaaattttatttttgtaggttattcgttaatcgtattattattagtttcgggagtatggaaattgaattgttattgtttaaagagaaaatgtaagcgatagttgttttttttttgagttggatagttttgtggttgagatttttaagtttttgagttttagatcgtttttattttagtgtaggtcgttgtttttttttcgggtttgttagcgtgtgaagcggggtttattttttagttttggttgtttagtaggagtattttttagtatggttttagaagttcgggttggaaagtttttgaaatcgttaaattaagttgcgagcgttgtatgtgcgcgcgcgtatatttaagattttttcgataatagttgttttttcgggttgtttttgtatagttgaaattttggtatttaatataaaacgttaaagttggtttttttttttttagggttttgttaaaatatagatatgatattttttttgttttttatatgtttcgtgtatataatatatatgggttattgtaggatttgagatataaattaatcgtatttatattttaaatatatagagatgtgggttttgaagagtgatttaaggagtaaggggtttaatatttatttttgttttcgtaaacgttaaaggagtagaaatataattatgttttattatcgaaaagttggtgggag

SEQ ID NO: 164 - DNA, 1080 bp, Artificial Sequence
  subsequence of TRH
ttttttttttttttttttttgttttattttcgttcgtttgcgttttatattggttttgcggtcgtgtttttttcgtgtgtgtttgttttgtgttttttcgtcgttttcgtgtggatttcggtttttgtttcgttttttagttttttcgtgcgtttgtgtttaatcgtgcgttttttttaatttttttgtttttttttttgttttttatacgcgtgttttcgttaatagatttttagaggtggtgtagaaacgatttcgcgtcggcgttttattttgcggttagtgttttcgcgtttcggtttcggtttttatcgttttcgttttagattttcggaggagtaggcgggcggggtttcgcggggtcggttgtcgttagcgttttttttcggcggtcgcgattttttttcgttgattttattcgagtcgtcgtttggcgtagatataagcggcggtttatttgaagagggttcggtaggcgttcggggtttttagcgttgtagatttttgatttgtcgattgcggatttcgagttttcggatttcggatttattttgtggagtttatttttggtaggtaatcgttttaattttttttttttcgtagacggtgttcgggagtattggaaagggagttttttcggttcgtttttattttcggttttttgagagttttttggagaatagggtcggtgtataggcgggcgttgtgttcgtattttcgggtttttttcgagcgtaggtcggggattcgacgggaggtacggcgcgggtatatcggaggttttcgttgttgggtatttaggtcgttagagttcgtagcgcggggtgggagtttcgcggtattttttgtttgggtgtcgtcggatagagttgggtatttagggcgtcggtttgagaatttgggagttcgaattttaattttaacgttagaaatagaattttagcgttgaagttaggattttagcgttagaattagatttttggtttagttatgaaagtttagtattagaaatagaattttagttttgtaaatagattttgagttttagaatttgaattttagcgatagaaatgggatttt

SEQ ID NO: 165 - DNA, 1050 bp, Artificial Sequence
  subsequence of FBP1
gtaagaggattgtttgagtttaggagtttgaggttgtagtgagttagtgagaaatttgatttgggtttttaattgtagaaagagtgaaggaggataaagaagaaatggggaaggaaggtatttgagttagtatttttttgtttgaggttagggcgggtatgacgggtaggttaggtgtttatatttggtcggttgagaggggtacgaggtaggttgtttagggtagagaagaggaatgtaagatggaattaggtgtatatttgtgagacggatttttaggtgggtttttttaaggttaagggaggagatgaggatttgagtgaggttgagttagtttttggagagaggggttattagatagagagcgagagaggcgtttagatattagacggatagatagaggttgacggtaggaggtttagagggtttaacgttagttcgtcgggtaggttttttaggtagatagataggacggggtttatcgtttaaggttcgatttataggtgcgcgatgttcgttttgcgtatcgtcgaagagatggttttgattgttgtgtagagcgagttgagtagttgggttaattcgttcgtgtcgcgggtttttttgtttttttttatgacgaagcgggttagggtgttgacgttcgtgtcgaagggcgtttggttagttatgtttgaatcgggtagagcgcggggttgtaggtgtaagcggtaggtgcggggttgtaggtgcgggcggtaagagagggtagtaggtattggtcgtaggtgcggagttgtaggtgcgggcggtaggtgcgggtcgcgggatttggcgggaggattgatagatcgattgtcgtttcgagtgttcgtagcgttcgtggtgtaattgggttaggttaggcgtcggcgggtgaatcgcggaaatttttagacgcgggtcggtttttcgttttcgggaatatttttgcgtttcgtttatttcgcggattagatcgcggtttcgtttgtttggatttttagataaggtcggggattttttttgcggttttttaattttcgtttttat

SEQ ID NO: 166 - DNA, 968 bp, Artificial Sequence
  subsequence
tatttcgtggtgtttttttttttcgttttatagttaagtttagaggaatagggtatcgtttcgcgcggtttcggagttatattcggatttgggaatttcgtgtcgggtttagaggattttattgggcgggttggggtttatttttaataaatttagttgtttatatatatttttattattatttttacgcgcgcgcgcgtatatatatatatatatatatagagggatttgttaattattgagatagcgatttagaaaggtgtaaatttatttggtgtttatttaattgtaaagtttttagatttatataaaatattagcgagttttggaggtttgagacgtttcgcgttcgatttacggcgcgaatattagcgtttcggtcgggtcgtaggggtcggtgtttagcgggtcggggtttggcgagttaggtagcgggtcggttgagtttttgcgtttcgcggtcgcgtggtttattcgtttatttttttattattggttgggatttgtttttttttaaagtgtgatgttcggtgttttattttaggttacgcggagttttttttcggcgtgtcgggttttgcgtttttgtttagtggtttatttcggttcgttgcgttcgttttcgttttaagtgtttaggacggagcgaggggttgtgggtcggcgtagggacgttggttgtttatttttaggagtcgatagaaggtgttttcggcgttacgcgtttaattttggggttgatttaaataattaataagtttagagaaattttacgaggggaatttttttttttagtattaataaagtttagtaattgggtttgttggttatttaagttcgagttcgatttttttagttttttttttttttttttttttttatttagaggtaacgtttttaaaaatcggtaattgcgtgtgcgtttggggtgtgtaagtgtgagtgtagatgtgtgaaagttatttgtt

SEQ ID NO: 167 - DNA, 1080 bp, Artificial Sequence
  subsequence of BCAN
tagtttttttttacgttcgcgtagttttcgtcgtagttttagttgtagttgtaggattgagtcgtgtattcggaggagattttcggaggaggcgataaatttcgtagtgtcgcgatttaattttagttttgggtaggtgagtgttttcgtagtttcgtcgttcgtcgtggggtcggggatagggagaagggagtgtttgtttggtttgcgtttttcgtttgttagtttttgtttcgaggttttggggtatttaattcgtcgatttttgatatcgtagcggggtaggttgttggatagtttcgagcgtttgtagttgttgttgttatttttgatttatatgtttttagttttgttagtggtagtttttttgttgttcgtagtttgattagtaatttttcgggttttcgtattttttttgttgcgcgtttttgttttagcgcggtcgtcgagattttcgattttgttttaggtagggcggtagcgtttcggattagtttttgttttcgtgtttttacgtataggtagttttaggagtagcggttagtaatttttttggggatattttattgtagttcggtaggatagtcgattagagtcgttttagggggtggtcggagtgtttatttcggttggaattttaattcggttttttgttttgtgattttggggtagttagttgatttttttgaatttcgggttttttatcggtgtaatgagtaaaatataaataattttttttttatagttgaggttatttataggaagtatttaggagaattggtttaggtagatattagtaattattagttggaattcggttattattattgtatttttttttagtattgttaggggtttgggaatttttttttttaggtatttttatattttgttaggtatttttttatttattggaatagttttgtttatatggttttaataggattaagagattggcgttaagtttaaggggtattattattatttgtattatttagattgtagatgatgatagtaagattagggaatagtgttatttttagatttatttatagtattattagtgtttatgttgttatg

SEQ ID NO: 168 - DNA, 1016 bp, Artificial Sequence
  subsequence of TP73
ttttaggttagggtttaggtttcgtataggttaggagtgattttggtgggttttttttttttttcgttttttgtttattttggttgggggtgtaggggttagggtgtggtgtggttagatttttaggtttagggcgattttttttgttttttttgttttattgttttttgtttttaatgcgtcggtttttcgtaggatttgggggttttgaagattttcgagtagtatcgtatgattatttggcggggtttgtaggatttgaagtagggttacgattatagtatcgcgtagtagttgtttcgttttagtaacgcggttattatttttatcggcggtttaggggaattgtagcgttagcgggttatggaggtcgtgtattttcgcgtgcgttatattattattatttttaatcgcggcggtttaggcggcggttttgacgagtgggcggatttcggtttcgatttgttcgattgtaaggttcgtaagtagtttattaaggaggagtttacggaggtcgagatttattgagggtttcgtttggttgtagtttgcgttatcgtttagagatttaagttgtttttttttttttttttgtgtgtttaaaattgttttaggaggtaggattttcgggttgtgttcggggaaaggtaaggttcggtttatttttaggtattttataggttttaggaaaggtttagttatcgaagtcgtttgtggatagtttgagttatttgtagaattttttggagttgttttagtgttgggtttgtggggcgggggttggtttatttttagttttgttattgtttcggcgtgttttatggtaggcgtgggtggggatcgtagcgtcggtttcgatttttaggttttattttagagattgttattttttaattaggcgaggtttttttaaaggaaaggattttttttgttgatggattgttaaaaagtattttgcgatattttttggttttggatagtagtgagtagttaagtgattgtgtttgaaatattag

SEQ ID NO: 169 - DNA, 1058 bp, Artificial Sequence
  subsequence of MIIP
gtttttcgagtagttggattataggtacgtgtttggtttattttttgtagagacggggttttgttatgttgtttaggttgggtatttttttttttttttttttttttgagatggagttttgcgttttgttttgttatttaggttggagtgtagtggcgcgatttcggtttattgtaatttttgtttttttagtagttgggtttaagcgatttttttgttttagtttttttagtagttgggattataggcgtcggttatttcgttcggttaatttttgtatttttaggtttattggcgtgagtaatcgcggtcggttttaatattatatttttttgtttattgtgtagtttttattttttggcgtaaagcgggtattcgttaaaaatttgaatgaaagtataaagtaggtcgggcgtagtggtttatgtttgtaattttagtattttgggaggtcggggcgggcggattacgaggttaggagttcgagattagtttggttaatatagtgaaattttgtttttattaaaaatataaaaaaaaaaaaaaaaaaaaaaaaaaaaaaaaaaaaagtcgggtatggtggcgttcgtttgtagttttagttattcgggaggttgaggtaggagaattaatcgtttgaattcgggaggtagagattgtggtgagtcgagatcgcgttattgtattttagtttgggtaatagagtgagatttcgtttttaaaaaaaaaaaaaaaaagaaaagtatgaaacgatgagtataatgagtagttagtcgtttgttttatttatttcgtcgtttcggattgtcgtttgcgtcgagtttaggtcgtttagtttgattgaaattgtcgttgttgaatttagcgtatttagtttcgtagttgattaatcggagttcgttttttcggggttcgttttattttaggaatcgattttcgtatcggtttcgaaaattgattaatcggttgtgtagtttcgtttttagtttcgtttttacgttgaaattgatatttcggatcgtcgagtaacgtttattagacgtttcggttttgttttt

SEQ ID NO: 170 - DNA, 1166 bp, Artificial Sequence
  subsequenc of HOXC4
ttcggtttgggttcgaggtttcgaggcggttttataagtgtgaatttttgtttataaacggcgacgtatacgtaaacgtttatatatttaggtagatatattcggaggcgtgggggaatatattttagacgaggttcgagagaatttgggggttagatttattttaatttaagttaagatattttttttatttttatttttttttagaggcgcgattgggattttgcgttaagttttagtgggggaggggatcgttttacgattttttgtttaaattttgattcgtcgtttgtgggggggcggggatgggggaagaaatttgtttttattaaatttttaaaaatatagtttgtatttagattaaatcgtttgggttagagttgacggtgaattttattttttttttttttataattttttttttttttttttttgttttcgttaaatttttttttcgtagttattataaaggtttttgaggtattttttcgcgggaagaaatggtatttttttttttttttttttatttttttatttttagtaggatttgtgtgtcggtagaggcgtttgacgaggggttaatttcgttttttttgtttacgatcgagaaaagcgtttggttttttttaaatgggtttagttcgtcgtttgtttaggttgtcgcgcgttttttcgtcgtttaggtacggtttagtggttgatgtttcgcggatttagtttgcggtaggtcggaattcggagtttgtgggatttgaaaagggtaaagggagtgcggtgggatataagaggggttcgagaggttcgaaaaagggagttttttttttggagtaatgtgggaatcgtcgatcggtgaggtttttatttttttttttcgtttgtattttgttcgttttcgtttttgtggatggtcgttgatgggggggaatataagtgttttttgttcgttttcgaaagaaaattttttttagagaaggttatttaggttagtggagatttatttagaatattagaagggtttttttttattcgaggggcgggtttgggcgaggttgaggtattttttttaattttagaacgattttattgagtgtatttatagcgagatttggaggtgttagagttcgaggttggtcgtttaatagtattattttgaggtgtttttatat

SEQ ID NO: 171 - DNA, 1334 bp, Artificial Sequence
  subsequence of HOXA7
tcggtttcgcgtttcgcgtttcgcgttttttagcgttgcgtttttcgttttcggtttcgtttcgttagtttggttcgtttagcgattgcgtttatttgaagatcgtatttaggggtagatgcggaaattggttttagtcgcgttatgtagcgcgttttcgttcgttttgtcgtaggcgtttttggcgaggttattgtagagttcggggatgttttggtcgtaggaggcgtagggtaggttgtcgtaggcgtcggcgtttaggtcgtagtcggacgtaaaggggttttgataaagggggttgttgatattgtataagttcggaacggtcgaggcgaaggcgtcggcgttcgtttcgtagtcgtttttttgtgagttgggagtaaaggagtaagaagtcggttcggtattttggaatagagaagttttcgtcgtatatttgttaaaaagcgcgtttatataatacgaagaatttataattttgatttgtgatttgttgttcggtagtttttagtgtcggttttacgaggtagagtgatatatgataatattatatttttagatttatattaaattttatttttttttggacggagttcgtcgtagtacgtgatcgtttatatgatcgttttcgttaattttagtagtttttataggtggtttcgtttcgtagggttcgtagtcgtttagaatggaagggtaagaggtttaaatatgcggttaaagaattcgttcgcgttcggcgggtttggcgcgtttcgcggaaaaagatttggaggtttcgcgggagcgtttagttggcggttaattttcgtattggggtttgcggacgttaggcggttcggttttacgtagtattttttatttcgttttttcgtcgatttttgttagtgagttttggattaagtttgggattttttttattttttttttgttcgtttgtttagattttggaagggtttttgtttttcgtaatagtttgtttcgcggtggttttgtgggtaggatttagttatgagtagatcgattttgtttaagtttttttttatttaggtttagtgggcgataggtcggatttagattcggatttagacggggaaggcgtagtattttttgtagttgtagagagattgttatcgtaaattggagttatgtggttcgaataaagttaacgttttttagttttttttttttaatcggaggtatattgtttattcgttttaaaggaagtagtgaaatatttatttattaatgagatttatttgttaatagatttattaacgtggggttttttttttttttttcggacgttgtagtgttgtaggttttgtgttttt

SEQ ID NO: 172 - DNA, 1181 bp, Artificial Sequence
  subsequence of BST1
aaagagggtatttgttaaagttgtcgttttttggagttagaaaagtattttttttgatgatgattgatttttttttattttttttttaattttgcggtttttttggggtttttttttcgtggatagcggttaagattagtttgggttatagtgtattggttttgttttgggtgatgttttaagtttatttttttttaattttatttatttattaattttttttttagatagagttttattttgtcgtttagggttggagtgtagtggtgtaattattgttcgttgtagtttcgattttttggggttaagtttttttatattttatttcgtaggtagttgagattatagatgcgtattattaggattagttaagttttgtatttttttgtagagaggaggttttttatttgtatgttatttaggtttgtttcgaatttttatatttaagcgattcgttcgtttaggttttttaaagtgttgggattataggtatgagtcgtcgcgtttcgttttacgtttagttttgaaattgtttggaacgggaaacggtaaatagcgagatattcgagcgagagtttcgttttgtattagtttgcggaatcgttttggtagaaggagagaaggggagtggaggaagtacgggattggagggattaaagtttttcgatggcggtttaggggtgcgcggtatcgcggttgttttagttgttgttgtagtttttgtttttattgttgttgttggcggcgggcggggcgcgcgcgcggtggcgcggggagggtattagcgtatatttgcgggatatttttttgggtcgttgcgtcgagtatcgcgtattgttgagtttcgagtagcggtgaggtagtcggtcgggtggaaggggagtcggaaagaggtaacggtggggagggtttggggaggggaaaattggcgttaaagttcggggtgagggggtaatgagagaggttttgaggggagaggtgagtgtggagatagcgatggttttgaacgatgggggcgagtgaggagggggttgtgaagtgtgtttgtaggtgaggggtgcgttgtgcggggtttagagatgagtgtgtgtgtgtgcgcgtatatatatattgtagaggtgaggggtgtgtgcgtgtgttttagaggtgaggggggtgtgtgtgtgcgcgcgttttagagg

SEQ ID NO: 173 - DNA, 1039 bp, Artificial Sequence
  subsequence of C1orf114
aggtattattaacgaaatgaatattattgtttttttatggaagttataatttcgggagtgatttttttttttagggataaaattattattttttacgtttaagaattttgagaggggaaagaatatgataaaaatttagtttaagttatttttagacgagtattttttatatatagtgaagaaaggtgttattagatttttttattagtgttagattcggtggatttcggattttagaggataaggcgttattagaaagtttttttttttattatttatttttttttttagttatattagacgtttatatttttattttttattttattattaatattttcgtatcgttttttttttttttttttttatattttttttgtttgtgtaaaatgcggcggttgggattatagagatggtcgggggagtttttttttttttttttttttaagttttttatattgaggtaaaggagatttcggtatttgttttcgcggtagttaggattatattgttatggtaatagcgtgtttttgcgttttttattcgggtttttttaattacgagagcgataaaaatttgcgtaggcgtatgtaatatttttagattatcgatttttttcggtatttatttcggtgtttgcgaagggttagtgaagttgaggtttttaaggggacgattaaggaatttacgtattattaacgttatagagattcgcgaagtgtcgttgtgttggttgtgaaattttttttttgtagttgtttttcgttagatttagaattttttaggataatttttaaaattatatttttatatgttatgtgttttatagttaacgtagaaaagtagtttttagtttttattagtagataagtaaattgttaatgagttattatatttttgatttttagttttttttttttttaattaaaattaaaattttatttaagagagttgttaaagaaaataggatttttgttttagttttgaggtatgttaaaatggttaattagaatttttttaaattttgtttatttttatg

SEQ ID NO: 174 - DNA, 1028 bp, Artificial Sequence
  subsequence of FOXG1
ttgttttcgtcgtcgttatcgttattatcggtcgtcgttttggacggggttaaagcggacgggttgggcggtaagggcgagtcgggcggcgggtcgggggagttggcgttcgtcgggtcggacgagaaggagaagggcgtcggcgtcgggggggaggagaagaagggggcgggcgagggcggtaaggacggggaggggggtaaggagggcgagaagaagaacggtaagtacgagaagtcgtcgtttagttataacgcgtttattatgatggttattcggtagagtttcgagaagcggtttacgtttaacggtatttacgagtttattatgaagaattttttttattatcgcgagaataagtagggttggtagaattttattcgttataatttgttttttaataagtgtttcgtgaaggtgtcgcgttattacgacgattcgggtaagggtaattattggatgttggattcgtcgagcgacgacgtgtttatcggcggtattacgggtaagttgcggcgtcgttttattatttcgcgggttaagttggtttttaagcgcggtgcgcgttttatttttatcggttttatttttatggatcgcgtcggttttttttattggtttatgtcgttttttttgtttttgtattattttcgcgttagtagtattttgagttataacggtattacgtcggtttattttagttattttatgttttatagtttcgtgttgatttagaattcgttgggtaataattattttttttttatcgttaacggtttgagcgtggatcggttggttaacggggagatttcgtacgttacgtattattttacggtcgtcgcgttagtcgtttcggtgttttgcggtttgtcggtgttttgttttgggatttatttttttaatttttgtttcgttaatttgttcgcgggttagattagttatttttttttttacgtttcgtattcgttaatgatttcgtagagtagtacgtttatgagcgttagggtcgcgtttttttttacgtcgtr

SEQ ID NO: 175 - DNA, 1017 bp, Artificial Sequence
  subsequence of ATP4A
acgagggaacggggcggggttgaggagaggggcggggtcgagagttcggtgcgggttttgagagttgcggggaagggtgaaggtggaagatggaggttttgtgtggaggggtttttggtagaaggtaagcgttaaggcggggttaggtgtagatttggagttttggacgtagggaatgaatagaattagggtgcggagttgggttgggggcggatttggagagcgaggtgttttttatggatagtttcgtcgaggagaagttgtgggcggggttgggtggtgggcggggttttgtttttggtggacggggttataggcggagcgggagatggggtggggtttggttgcggagagaaggggtaaggagcgaagtttttcgtggttcgttgatgtgggtgtggtttggggcggggttcgaggtgggcgggtttaggtcgtgggcggggtcggttgcgtatttggaatttgttggtggagttgaagggtatttcgtagatttttgggaagcggtttcggtagtttatggcgttgtttagcgttagtttcgagaatttgagtagcgtcgttttcgatgcgtttttaattacgatgcgttgggagcggggatcggtgttaggggcgaagtcggttatattagtttttcgggattttttggaggttttttggtttttattttgggtataggtattgtattttggtcggatttgaaggcggcgcggttgtatagggtgagtattcggtatagcgttcgttacgttttcgaggattggttaaacgtttgttttgtagattaggcgtttaggttgggtttcgtacggcggttttttcggattagaatcgagttttttttttttaggtttatatcgcgggttttttttttagatttgggtggaattgggttttatttaattttgagggatttagttttcggatgatttttttttttagattcggtagcgagttttttttgagatttggagtcgagtcgtttcgttttcgtataaagttttttttatt

SEQ ID NO: 176 - DNA, 1161 bp, Artificial Sequence
  subsequence of NOTCH1
tttataaatatagaagaatttttttattttacgtaggaaaattttggtttttagaatttgtttgtttttttagaatagataaaagtttttatttggggttagataaaatagtatatataaataaaaaggtagtgtttttgtgtaaaataaaagtatataaataaatattaaaaaaaattaaaattttcgtttttattttgtataaaaatatgtgttttaaaaaggtttttttggtcggttttggtatttatagagcgtatatagacgttcgaaggtttgggaaaggaagtcggggtttcgtggggcgcgtcgtttatttgaaggttttcggaatgcgggcgatttgggattgtatgttggtgggagggttggagacgttttcggattagtcggagacgttggaatgcggggacgagttggattattggttaggggatttaggggacggggtgaggaaggggtgtttaggtatttgtagttggtggttgggggtgttgtttataggcgaggagtagttgtgttgcgaggggggcgttaggaattgggttgcggttacgggtgggattagcgaggatggtagcgacgtgggtagggcggggtttttttggggtagaatagtgtgtatcgttaggttgttggggtttagtggttgtacgtttgtttggttcggttttttatttaggaagtttcggtttaggtggtcgttggttgttgagtttacgttaaggtgcggttgtggtggtggtggtggcggttgtaggttttgttgttgttggatgtttgttggttgtaggttttgttgttgtatttgtaagttttgtggttgtatttgttgggtttgtattaggtgaggttgggtggttagtcgggtgttgggtaggttttggtagtttattatttgggatagggcgttggtagtaaggttattgtgtagcgggtttattatgttatgttgtagggagggggtttgtgtgtttagggggtttggtgttatattttttcgtagagggttgtattggttcggtattatgtcgttttgtagtcgggatagttattcgtattgattatttaaattggtggattcgtttatagtgaaatttagggttttttcgttgttggagtttaggacggtgttggtgttagaggttataggtaggtggg

SEQ ID NO: 177 - DNA, 981 bp, Artificial Sequence
  subsequence
ggtttcgtcgaatgcgtttttttggcggtgatggttttggatcgcgcggtcgtagtgtgtcgttcgttgcgttatgcggggttcgttttttcgcgtttatgtcgtacgttggttagcgttttttggttaagcggttttattaattcggttgcgtaaatcgcgtttttggttgagcggtcgttgtgcgcgtttcgtttgttggattattttatttgtgagttgtcggcgttgtttaagttggtttgcggaggcgacggagatattatcgagaattagatgttcgtcgttcgcgtggttattttgttgttgtcgtttgtcgttattttggttttttacggtgtcgtggttcgagttgtttgttgtatgcggtttagcggaggtcggaggagggcggtgggtacgtgtgggttttatttgatagtcgtttgtttgttttacggttcggttatttatatttatttgtagttcgcgtagcgttataattaggtacggggtaagttcgtatcgtttttttatatcgtggttatatttgtttttaattcgtttatttatatttttaggaataagaaagtgaagggggtagcgaggaggttgttgcggagtttggggagaggttaggttgggtagtgagtagttggggaggggagaaagtattaagttagaatttaaggatggaaatattttttagtgagttagtttagattttaggttgtttatttttgtatgataatttgtaagatttgttttaaggagtttaatgggggatatgtttttttttcgtgaggaaatgtttagtttttgagggaaaatttttaaattttttatatatttaggtttagggaaggaaaatttattttttataattttacgcgtagggaaaatgatggacgtgatgttcgtttttagttttttttttatttgatggaagattatggaagattttttggtttttgtaattagaagttttaagttgataagaaa

SEQ ID NO: 178 - DNA, 864 bp, Artificial Sequence
  subsequence
aatgtttttttttgaggtagttggaggttttttttttttgagagtttaattgtggatatagttttgagtagaggcgaaaaggaaagaaggttgggagataatcggggaaaaatatatatttttggtttggtttgaaagttggcgttcgaaaaggaataagaaaaaaaatacgtttcggaagtgtttgagattgttgcggttataaagtagagtattaattttggtattgatacgggaggggagtaagattttattttcgggtttgtgtttatgaatttaggtgaggaggggtattttttttttcgcgtttaaatgttgtattttttaagattattttggttcgttacgtttttattttgtgtttataaaaattttcgagattttagcgggtatagatataagcggttggatatgaagaggaatatatcggcgggagaatatagaatatttattttttttttagttattttggaggtttcggagaaggcggttttagtgattcgtgaagagattttgagttttttatatttcggagaatgataagagagtatttgggcgacgtaattttttgggtttttcggagatgcggttttttatacgttaggggttaagtttgagaaataggtggacggtaaggataggagtttttttcgcgttataaacgtttttgtttatatttgggttttttgatttttttgtttatataatcgagttatttatggtcgggtttcgagtttttattttgcggattgggataaaggggttaattgtgatgtgttttgtataattttaggattttgtatttgtttaagggcgaggtgtaaatttaaaattacgtacgattgaacgtcgagattagttgag

SEQ ID NO: 179 - DNA, 1004 bp, Artificial Sequence
  subsequence of HOXA7
tatttaggggtagatgcggaaattggttttagtcgcgttatgtagcgcgttttcgttcgttttgtcgtaggcgtttttggcgaggttattgtagagttcggggatgttttggtcgtaggaggcgtagggtaggttgtcgtaggcgtcggcgtttaggtcgtagtcggacgtaaaggggttttgataaagggggttgttgatattgtataagttcggaacggtcgaggcgaaggcgtcggcgttcgtttcgtagtcgtttttttgtgagttgggagtaaaggagtaagaagtcggttcggtattttggaatagagaagttttcgtcgtatatttgttaaaaagcgcgtttatataatacgaagaatttataattttgatttgtgatttgttgttcggtagtttttagtgtcggttttacgaggtagagtgatatatgataatattatatttttagatttatattaaattttatttttttttggacggagttcgtcgtagtacgtgatcgtttatatgatcgttttcgttaattttagtagtttttataggtggtttcgtttcgtagggttcgtagtcgtttagaatggaagggtaagaggtttaaatatgcggttaaagaattcgttcgcgttcggcgggtttggcgcgtttcgcggaaaaagatttggaggtttcgcgggagcgtttagttggcggttaattttcgtattggggtttgcggacgttaggcggttcggttttacgtagtattttttatttcgttttttcgtcgatttttgttagtgagttttggattaagtttgggattttttttattttttttttgttcgtttgtttagattttggaagggtttttgtttttcgtaatagtttgtttcgcggtggttttgtgggtaggatttagttatgagtagatcgattttgtttaagtttttttttatttaggtttagtgggcgataggtcggatttagattcggatttagacggggaaggcgtagtattt

SEQ ID NO: 180 - DNA, 963 bp, Artificial Sequence
  subsequence of ZNF529
tatttatattattatatacggacgtagttatagaacggtatatataaatataattatatagtttttttttttagtaggtgatttgtatataggtttggggtttttgtttttataaatttttttcgcgttttatgaatttaggttttttgtcgtgagtttttttcgtatttagattcgggttattttaatttattatatggaaaacgaatattaggttaacggaaaagggagtcggggttttggtagaagcgtagtgttagtcgtaatagggcggtcgtgggtgtaaacggaggggagcgtcggtagttagtatcgcgcggcgattaacgggtcgtttcggagatttttgggagtttaggtttacgcgcgagtgcgtaggcgtagacgatttattttgggtcgggggtgaggtttggtgggtgttaggggtgttgaggaggttaaggagggtattgggagtttcgtttcgggagagttgtttaaggacgcggaatcgggtggggaggttagggaggtaattaagagttcgagtcgggtttggaaattttgaggaggaaatcgggatcgcggtatttagacgtttcgatttgtacgagtcgggtttcgggcgtggtttatgggcgtgattttgagggtgattcggagcgagtttcgcgaagggggattttgttcgttttgatttcgcggaagcgttatcgttggcggcgggttttcgcgcggagcgggcgttgtgtgttcgcgcgcgcgggcgcgcgttgaataggggtggttttttgcgtttaatttgttgtattttaggtgtttgtttttttttgggatgttgtggtcgattgtgtgtgaaaagtgaacggagtagtgttgttgcgcgaggttttttttgcgtgtgtttatttttagattaggtgtgagtcgtatttgagattgtttttgagtgtggagaattgtaagtgatttgtaggtgtg

SEQ ID NO: 181 - DNA, 956 bp, Artificial Sequence
  subsequence of PRLHR
tttcgcgggagttgaacggatttaaatgttttttagtgggttagtagttttttagagggattgggagcgtttttttttagtttcgttttttattttagtttttatgtatggaaaataggggtggagcgcgttttgttatgttcggtgtttagagaattagtgaagaggatagtgtggggaggatggaattcgaaacgggaggaggggtcggtaaatttggttagagtagcgaagaggacgaatttttattgtaggagtttgtacggtttttggagggttagggttcggaggagcgtatagtggaggagggcggaggagaggcgcgaagcgttaggttatcgggaggagtcggtgtagttttaggagggaaggagcggggaaggaagtagcggtgggagattgtaatgtagttgggggtttgagagaggtacgattgattcgtttttaaaggttggattttgtttagcggttaggttgcggagggtagagacgttagagggttcgggttgggatttaatagtagagtttggagttggtcgcggatttgaggatttttattttttcgtggtttcgttatacgagttttttgtttggttgtagcgcgtttagcgggtagcgggttcggttaagttaaaggtaggagttagtattacggatagttttcgttggatttgtcgtttttcgggcggatgatgtggggaggagtaggggaaaatgattagggaatttttgtttttttttggattcgggtgtttggggaaggaatttggttcggtttaaagatttgtttcgttgtttgttttttgggttggggttgagaagagtagggtggagtggaggtagttgagtcgggggtttgggggtcggagatttatgatttttgttttttttggtggttatcgtatttagtgttaaggacggcgtcgttttttatttttcggggttagaaaatgtag

SEQ ID NO: 182 - DNA, 1037 bp, Artificial Sequence
  subsequence of ARL5C
gagggagcgaagagtagggaggtagtttgggatatttggtaggtttggagttgggtttggtagggttttcgggaagatggaggaaagtagtgggagttagggttgtttgtacggtgtaggatttgaatgttagatcgaggagtcgtagtattaggaaggtttaagtagcgtgtttaatcgttttttcggattatagaggagttcgggaatttagggaagagttttagtgattggtttttttgtttgttagtttggtgggaggtttagttttttatttttttcgttcgagagttatttataatcggtagagaatggtggttttttttttattgtttagttttacgatgatgatcgtgtgttttggaagcgtcggaggaagggtagcgttagggttaaattcgaagattaagggattgtgtgtttttattagattttttaggaaggagatagcgtttttcgtaggttggggatttttgtttatcgtatcgcgtttgttttttatttagtttcgatatttgttttatttcgggacggtggaaaagatagttgagtttttatttttttttatattttagaaaagtgtttgaaaggttcggggcgtttcggggtttgttaagagacggtgtttagagaaagagtataacgcgaagttataatcgtaggaaattcgtagtagttttttattttcgtcgttggtttcgtttagcggggagaaaggagggtcgtttagttttgcgttttggggcgtatcgaagcgtcgggatttaagaggagtaggtagggacgggggtaggggaggtcgcggggtagtcgaggagcgtttatatacgattttcggagttcgaggttttttcgtgcgttcgattatagattagaggagttttagaagagggcgagattaaagcgttcgtttggatgttttgtgcgttttttattttggttttcgaagatgtttattaatttggcgattagttgttttatggtatttttcgggtcggataggtgtaggagggtttagcggttttaggagcggagtt

SEQ ID NO: 183 - DNA, 1006 bp, Artificial Sequence
  subsequence of PAX9
tggagtttggttgatttgatgttggggtttaaagtttttttagttatatgtttgggttgagttgtttttagagtttttggtttttgttttttttgggtgggtgtatataaggatttggttagtgttgagtgtattggttttttttatttagtgtagtttttttttttatatttttggtttggtttttagttttttattgagtaaatatttatttagagagtgagttgttttttggaggaggttttgatgtggttagggaaaggttttttggtttttttttggtttgagttagttgtaggttttattggtgttttggttttggttttaaatttttttttttagttgaaatttttttgatttttttgagattttttgagtttagagtgagtagtgtaattaggtggtagattttagttgatttttgtttttgttttaggttttgtatttttatatttattgggattgattagattttagtgttttttttttttttttttttattttttttttttgttttagatttgttgttttttggttggttttagtgggttgttgattattttgttttagtatttggtttgtgttttgggaaggttttagtattatttttttttgttgggattttgttgattttgtttgtagttttggttttttttgtttttagagtggggtttttggtttgttgtggatatttagtggtttaaaatatttaaaattgattttttttgtgtttttgagaatgttaagagtatttagtatttgtaattgttggtatgagtggggtttgtggggagttgttagagttgtggataggttttttgtttattgagttgttatttttggtatgtttaggggatttgtagtagttgaggttatatggttatagttaagtttagtaggtggaaagggagagatggtattgaatttatgtgagaattgggaagatgtgtggtagttgaaggagttggtaggaataagagggagttgtatgttatttttatataat

SEQ ID NO: 184 - DNA, 1001 bp, Artificial Sequence
  subsequence of HOXD10
tggtttttttgagagttgaagttttgtgtagttttttggggtgtataggaatttggagttaggtaggaggattgagtgggaggataatgtagggattaatttatttatggggatttgggtttggttagttgtttggttttttggtttttgtggttttttttgtttttgtttttttagagatattttggttgttttttagttttaagggattttttttttggatttttggggtgggatgttttagggtttgtggaatttgatttatttttttgttgggttgtttgggattaaattaattagtttgtgtttttatttgtttgttttggatttggtttttttaagtgtgttttgtttggttgtgtgtggggggaatgtttttgtgtgttggtgttagggtattttggtttttttttttgtttgtgtgtgtttatttggaggtttttagagttgagattttttttttgttggttgggtttaggggttgaagtgggggatgtgagtggggtgggttggttgagtgagttttggagaggtggataggagggtggtggagagtgttgggttggttgtttttagtgtgtattattgtgggtgtgtagtagatgttgttgttgtttgtgtttatttggttggttggttaggttttggagtatgtgatttgagaggaggttgtggtttaaggttatttttaaattttattggtttggttgttatgtggttggtagaggtatttataattatatggggaatgtttttttagagatgttagtttataaaggatataattttttttttttaaatttttttttaaaatgtttttttttaatagtttttttgttgttaatatttttttagtagattttttgattagtgtttgtaggagtgatagtttttattttagtagtgttagtatgtatatgttattatttagtgtagatatggggatttatggaatgtaaatttgtggattgtttttgtttttggttaaaagagaagtgaat

SEQ ID NO: 185 - DNA, 468 bp, Artificial Sequence
  subsequence of TBX20
gtggtttttgttttttattagtgtgtttttagtttggggtttttattttttttagagggattttggaaaatgggatggttgttgaagagaaggtgaaggttagggtgtggagttttatggtaattatgtgatgtgtagtgggagagtgtgaattttatggtagtgtttggattaagtggatatagatttttttggttttataaaggtggttgtgatgaggattttttatggttttgttggagggtgttttgttagttttgtttagtttgaataatttaaattttttgaatttgtagggtaatttgttttgtttggagttgtgtaaatttaggttgatatatatatttaagttgtatatgtaaatatttgtttttttttttagttagttggtttggttattagaagtttttttgtgggttttaaaattaaaataataataataatttttaaaattttaattttttattg

SEQ ID NO: 186 - DNA, 1003 bp, Artificial Sequence
  subsequence of CACNA1B
ttgagggtatttaggggtggtgtggttggtagagtgggttttggggatggtttgggttggtgttgagtggttgttgaggatttataggtttgtttgtttttgggtttggtttagttttggggtgggaggtgtggggtgagggaggtgtagttggaggggttggggtggggtgggggtggttgtggggtggggttggtgtggtagggtgggtggggttggtgtggattggttgggttttgttatgtgattggttttttatagggtgtggtgtggggttgtggagttgggtgaggtggtggtggttgtggtggtggggttgggtgaggtttgttgtggttttggtggttttgtggttgttttgttttgagtgtttggtgtgttttgtgttttttttgttggggttgttgggttggggatgtatgtggggtttgggagttatggtttgttttggggatgagttgggtggttgttatgggggttttggtggtggagagtgggtttggggtggtggggttggtggggtggggggtttgggttttggggggttgtagtttggttagtgggttttttataagtaattgattgtgtagtgtgtgtggattatggtgttgtataattttattttggttaagtagaattgttttattgttaattgtttgttttttgtttttagtgaggataatgttgtttgtaaatatgtgaagtgtattattgagtggttatattttgttgggtggggttgggtggggttgggtggggattggggtgggggttggggttggggttatttttttggtggttgggagggtgtgatttggggaggtgttgggagatgggtgaggggggtatggagtgttttagggttttttggagtggtgggtgtgggagtatttttgtgagtgtggtgggtgtggggtggagtttttttgttttggatttgtttttttgtatgttgggttttggggattttggttggtgtatagtgtgtggttagtttggaggg

SEQ ID NO: 187 - DNA, 1058 bp, Artificial Sequence
  subsequence of ZIC1
aagtaatagggtaggagaataagttgtaaatgtgaaaattagaaattaggagttaggtggaagtaatttgaaattgtgtgtagttttgggtaatatgagtttttagatttgatgttaaaaattgattttttttattattaatttttttaaatataaaaataaaatgtagatttaattgtattagggattataatagagttaagatatttataattttattgtagatgtaagaatttattgatgttttgggtttttaagtttgtaaagtgttaattttgggttgttggttttttgttttattttttttttatttgtttagtttttgaaaaatggttgtggtatttttttttaattagattttttttattttattttggtattaggggagaagttttttaagtgtgagtttgagggttgtgattggtgttttgttaatagtagtgattgtaagaagtatatgtatgtgtatatgagtgataagttttatttttgtaagatgtgtgataagttttatatgtattttagtttgttgtgtaaatatatgaaggtaattgttgtatttttgttgttttttttgaggtaggagtttttttggtttttggtttggggttgggtggtgagtggtagataggtggtggtgggagttagaggaagtgggaaggtaaaggttttatttagtggaattgggtagagaaggtagggtgggatttggaaaaggggatgggagtgtttaaggttgttttaaatttttggtttaataataaaagttaaaagaggtgagtatgagtaaaggttgttattgaatttggtttagagttagggtttttgtagggggttgatgttgtggaaattgttgtttttgtagttgttagtgagatgtaagaattggatttttgtgtttaggtttgagttttggtttatttaaatatggataagtaaagtttagggaaagaaagtgtagtttttggttttatatttagtttttttttttttagatttattttttttttgtgagttttggggattttgatttttttaggagtatggtttttgtaggt

SEQ ID NO: 188 - DNA, 851 bp, Artificial Sequence
  subsequence of SIM1
tttttgttttatttatttttagtttttataagtggtagaggttttgggggtgtttattttttaattgtttttatgtttattgtttaatttagtgatattgttggtttttttgttttttattggtagagaggagtagagtatttttggtttttttttttggattatgaattggaggaggggtgtgtggtagaaagaggaggatgtaagttttgggatgagtgaggtgattttagaattttggttttttgtagttgttatgaagttagtttattattatttttaattggaagttgaaaattgttttttgtaatttttttatagtttaagggtttagttttaattttattttggggttgttttttttttgtttttttttaatgttatttataagtttttttgttttttattggtttggtgtggttaggggtgaggtgtttattggttaatagggttgagtgatatgagttggttttgagttgttttttgtgtgtttaggttttgggttttgaattttattatttgtgggattgttggatttttaatgagtttagggtgttgggttggtgttgtttggttgttgttgttgtttgtggttttttgggtttttttgatgttgtgtgtgatttgtgttttttgagttttttggggttgggtggttgagtgtttagtttagtgtggtggtttagtagaattgggaatgtttggaggtagtggaggttgggtttgtgggttaggtttattggtggaggaggtagggtttgtttaaaggtttattttgttggtagttgttggttgatggtgtgtgtgaggttggtttggggagttatttttttttttttgtttttttgaaa

SEQ ID NO: 189 - DNA, 1068 bp, Artificial Sequence
  subsequence of DLX1
tttgtaggtggtagttatggttggattgagtttttggtaggttaaggtttggattttggttttttttttattataatttttttttggttttttgagagttgtttttgtgggttgatggtggtgggaggtttggtttttgagtttttggtttttatgggggaagggaggaaggagggatgtttttgtttttttggtagggagttgttagttggtgtagggttgggaggttttatttttgttgttttgtggtttttttttttttttttgtgatttaggtaggtttagtggttttagtttgagttatgttgttgtttgtttttgtaggttaagatttggttttaaaataagtgatttaagtttaagaagttgatgaagtagggtggggtggttttggagggtagtgtgttggttaatggttgggttttgtttgttggttttttatttgtgttgtttggttggaattttaattttttatttgggaagggtttaggaggaaatgtgggtttttatatttttagttatatattgtggtattttttagtgtattaagaagttatgtagtaattttaatttatgtgaggttgtttgtttgttttttttttgtttttttggtttaggttttttttgtttttaggtttatttattttgtttggaaaagaaggatttagagggaagaaggaatagtggaggtgggatgttttttatttttttggagttttgtgaggtttggtttagtaattttttggtatttgtgttttagtttgaattttggtttgggttgagtagtggtagtagagagtggttttggagggaagttattgttatttgagatagtttaagtagtaagataaatttgttttatttgatttgttgatttttagttttgtgggattattaggaaaaaataaaataaaaataaaatgtagaaaaagtaaaagtttttttttgttttgttagttttttgtttttttttgttttgtttgtgtgttggtaaagtttaggtttttatttgtttgttgtttttattttgtggttttagtaaaaagttataaggtttgagtggtttgg

SEQ ID NO: 190 - DNA, 1008 bp, Artificial Sequence
  subsequence of LMX1A
ttaggttgtgagaagagggtggtatttatgagatgttgattagttttgagattaaaaatttagttttgggtatttttaattatttgttatttagatgtttatgaataagtttgtttgttttttgtggttttggggaatttggtgtttagtgtgtgaggtttggggtggtttgttggatttatttgggtagggatgatttataagtattgatggatagatagtgatggggtttaatttagtgtatgaagaggggtgttagtttttttattgtggattaggttttagagagtggggttttagagtttagtgttaagtggaaagagagtgtgtttaggatgtatggtttgaatatttatttagtagtgaggagaaggaggttgaggtgttgattgtgttttggaagtttttttttatttttaggttgtttagtatgtttgggttgggttgggaggatttgtagaggagaagaaatgatgtgtttgatgtttgtgtttgttgggatttggtgttagtagttattgtatttttgggaaagaattgagggagtgtttagggtgattagaattagttaggaggatagggtttagttaagagaatgtagggtgggaggagagattagttatagtgaattgttttggttgatttgattttatttgaagttaatatgttatgtatttaggtttttgttttttaattgtgttttttttttttttgttttttttatttttatttatattttttgttttaggttttttattttgaatttgattttgttttaatttatatgaaggtgggtttttgggatgtttttgtaggaatgtagttattggggtatattgggtatataaagagtgggtatttttttttgagtgattgggtttaggtatgtgggatgatggggtttgtaattttgtgttttagttgttttgttgtggtttttatttgttttaggttgagaaggggtattgtaagggatttggagggtgttttgtttgtttttggattttt

SEQ ID NO: 191 - DNA, 1007 bp, Artificial Sequence
  subsequence of DLX6AS1
ttgtggtgtgttattttggtatgttgtgtgtgggttatattatttttagttttttatttttgatattggtaggaaagtttgatagttaggtttgaagtttagattttattttgtaagtgtagagatattatattaagtgggattttttgtttgttttattttttagtttttgattgtttttgagtttagattgggttgtttagtaggttttagtaggatttttattatgtattataattattattttagtgtagttgttttattggaatagagtgtaaggattttagttattaattattaggggaaggttgagagttttgaagttataatttggataattttagtttttttggtttttttagtaattaaataaatgagaaaaaaaaatttttttgtaagtagaggtagttgtattttggatatagtgtttaattgtagggattttttgaggttttgttatgatatattttaattggggtgtagttagagttgtaggaagttggtgaggaaagtggtgtatttgtgagtataaagtgaaaaatatagataagtatagggtgagggtgtagggggtgaaatgtttttatggtgttaataataagttgtagggtataaagtaataaaattgttatgtttatttgttggtattgaggatattataaatagttttggtgtgtagtttgtgtgtattgagagtgtattagggttgggagtgggaaggtggggtgggaaattttttttttttttgatatttttttttgttttttattttttatattttttttttatttagtttatttttttttttttatgaagtttttttgttgttgttttaatttattgttgatttgtaaatgtgtagattgtgttattggtttgtgtgttaaagtgtattttttgttaaaaggtggggaatagggtatgttatttaaaaatgaatttagagttattgaattggttttttagatttaagaatttaagtgtaatgggttgggaaaaggaggggg

SEQ ID NO: 192 - DNA, 973 bp, Artificial Sequence
  subsequence of MIR196A1
ttatatttgtatttattgtaaaaatgtagttgtgtaggttgagggtggtggtggatttatttgggtggtggtggtgttggtagtgtgtggttgttggaaggtgtggagttagtggttgtggtttagtttaggtttttttttgtttttgtttagaagtgagggtttgagtggttatgtgtttggtagggaagtttgaggtagtgagggagtttatttggttgtttgtttttttttttgggtataaattttggggattggaaatataataaaattttattgtgttgatgaattttaaatggtttatatttttttttgttttgaaaagaaagatgtttgggggtggattaaaaggaaggggaaataaatttatgagtggtagaagtatttgttttggtttttttttttgtttgtatattttgtttgtgtggagagaagtagttttagtttttgggatttggtttttgttgaattggttgttaggtgtgttttttttttggaggagttggtgttgatttagtttgtgtttggtagagattggaagttgttgtttatatggaaaatttatagagttttgtgtagattttatgattggtttggtttgttgggtttgggatgaggttttttgttttttgttagagtagaattgggttttttggtgtttttttgtgaaagtttaggtttttttaattatgtttggtggtttttattttttgtatttttttgttgaaagtgggtttttttttttttttttttttttgatagagttttgttgtgttatttaggttggagtgtagtggtgtgattttggtttattgtaatttttgttttttggtttaagtgatttttttgttttagttttttgagtagttggaattataggtgtttgttattatgtttggttaatttttgtatttttagtagagatggggttttataatattggttaagttgattttgaatttttgattttgtg

SEQ ID NO: 193 - DNA, 1050 bp, Artificial Sequence
  subsequence of FEZF2
ttttaaaaggaggtaattggtgtttgtgttttttttgggaaagtgtgagtggtttgtgaatagggaaagagggaagagatgggagggggagggggaggaattgtgatggttttgttggtggaaggaaagggggggggggatttaaatttaaatttaggtagagttttgtgtgtgatttataattttggaggtttgtaggtttgggggatgtggggagggtggagggttttggatgtggtgtttttaaagggtttttgggtattagtttagtagttgaagtattttttagttttttgtagttgagttgggtattgtgttaataaattgttatttatttatggaattggtgttagttttgaatatgtgtaaatgataattattttattaggatgtggtgtatggatgtgggtgttgtgtttggaggggggaatttgttaatggggaaatattaatttatgtaaaagtaatgagtttgttttggttggtgttggaggttgggagaaagtttttattgattaaggatgattttgaagtgttatggagagtaaggttgtttgttggtattttgggggttttggtgttgtgtaggtgtgtttttagttttatggttagttttgggtttgaggttgggggagattaaattgagagttggaagatttttggagattttaatagattagaattgttgatttatgattgggtttttgaggtaaagttgagttttgtttttggtttagggttgtgtgtggggaggatttggagggtagtttttttagttgatgggtatttattgtttgtataattgagaaggttttatttttatttgtttaaggagtagattgaaatagtagaatttttttttggattttattaaaatgtttttttttttaaggttatttagttgaattaattttttgaagtgatttatagagttgaattttgttaaggtagtttttttatttttagttattaaagtattgtgtggaattgggttttgtgtttttttaaaataaagagaaggattattagagaggagagggagggggtttg

SEQ ID NO: 194 - DNA, 974 bp, Artificial Sequence
  subsequence of STAG3
tggatagggggtggggtttgaggtggggttttgttaataatggtttggagttggttttaggggtgggggtaaggaagaaattaagttaatgtagtgtggaagtttggtaggggggtgggatttggttggtatttaggaggttggtgaaataggggtgtggttttttttgggggtgtggtgatttggtttaaaaggtggggtttgggtggaatttagtttatggtaattgagaagttagattaaaggggttattagtagtttggtttaaaatttgtttaatggagtaggagattgagggtagtgggggtgggatttgggtgggggtggggttaaagtgggttgtttgtgtgtttaagtttatgtgagagggtaggatgtttgagagtttgaggttatatgaggttgtggagtggtgtgatttaaatgtggtgtgtattagtttgtatatttttaaattttgtgatagttattggttttgggtgagttgttgggattgtgtttgtgtatagtgtgttttgtatgtttttgtgtttttttggaattttttgtttttggaagggtagtggtgggtgtttgtgtggaaggtggggtggttagagatatttgagggatttgaggtggggattttttttgaattttgtttggttagaagttatttttttaggttttgataggtttttttttgatttaagaataggtttttttgtgatttttttggttttgatattaggagtttttttgggttgtgttttaatggtttttgttatagagttggagaattttttttttaggtttttatagattgagagtttatttttttaagtgtttggaaggttttttattttggagttgtttattttaggggtagttgtagatatttttattttttggaaaaataggaaatgtgtatttgttttttttttttttgtgtttttagttttatttttatggtgtttttatttttaaatttttaa

SEQ ID NO: 195 - DNA, 981 bp, Artificial Sequence
  subsequence of PTPRN2
taataatattgaaggatttgagggtggtttttttgtggttttgaggttaatgttgtagtgtatgtagtaaatatttgttaaggatttattgtgtgtttggtatattaaggtaggtaataaaggatttagtgtatgtttggtatgtagaggtaggtaataaaggatttattgtaggtttggtatgtagaggtaggtaataaatgattagttttagaagtagatgtgtttgttgtaaattatttttttatggtttagtagaggtataataagtagtgaattttttttagggttttttgtgaatatggtattttatgttgttatagtgatgttattttagttttgagttgtaataaagtggtagtgtttgtgttttatttttggttattttgttgagaattatgttgattaggatgtaggtgttgttttggtttgtattgttattgttaatagaaggagagaaatgaaagtgttgttgtttatatggaagtttgatttataataaagttagtgatagtttattttttttttgtttatgggggttggtgagaggaaaggatggtggatgtgagagggggaggaaggatgtgggttgggagaatttaagtgaggggagaagggaggtttttgggggttttgagtttttgagtagtttgtagtttgtgggatgagttgttgtgtttagatgtgatttttttttgtttgtttttttttttttggttaaagatgtggtaaattttgttagaataaaatgaattaagtgtttgattgtgttagagttgatggtatttgtattgaaaatatttgtaaggtgttttttttagtgttgttgggtaattttttgagtggagaggggagggtgttgggtggttgggttttgttggtttatgtatgtagggatattttaggtatatttttttaggttgtttgttattttttttaaatgtaggttttttgttttagaaggagaaattgatataatag

SEQ ID NO: 196 - DNA, 1004 bp, Artificial Sequence
  subsequence of BARHL1
ggggtattggatttgaatttgttttttaattttttttttgaatatatttattagatgtagatgtaaatgtataaatatagaggtatttatatatttaatttaaatagttatatattgatatatatattaatataatttgtagttatatatgtatgtatgtttagttttatagttatttgtatgtttttagtagaggtaggaatggtgttttttataaataagttttagaatatattgttttattaataataaatattgattattgttttgggtattaataattaaggtttgttatagtaattatataattatgatgatgatgaataatttagggagggaaatagggttggtgtggttgagtttattttagtgggattttggttggtttgtttagttttatttgtaggtgagtttagggtttaggtttgatttttttaaattttaggttgttggttggttaaggtttttggattttggggttagatagtgtgtagggtttgtagtgtgagttttggaggatggtaggtgtagtttgttttagttggtagggtgtgtgagttgggagtgggttttttttggttgttattttaggtttgtttgtttttgttagtttgtagtttggttagtttgtagaggaattaattgtatttttttttttgaagagtatttttttatttttttaggtttttttagggtgattttatttttataaagaggtatgtgtagggaggagtattttttatttagttttaagggtttgttttgtgattttttgggtagggtaaggtgtagttagagttgggttttggggttagatagtagggtttaaaatttaggtttttttttgaaaattggtttagattttagtttttttttttgtaaagtggggtaagagttatggaaggttggtggaagataaaaggagaggatgtatgtaaggtgtgtgatggtgtttggtatttggttatttattaataaatgagtatgattttttttggtttttt

SEQ ID NO: 197 - DNA, 1064 bp, Artificial Sequence
  subsequence of CCDC140
tgtttatgggtttataaattagttgttatttgttataaatatgtataaatggaggttataaggatgtgggggtgttggggatttaaagttttggaattaggaggtgatttatttttttttttttttggttttttttttttttgttgagtgttttgagatttatatgtatttagatgattagtttggttttttttattggttagtggttagaggtttttggatatttggagaggggtgggagggtatttttaggttttggatagttgggttatatttaaagatttaatgaatttaaattttttgtggtttgtgtttttgaagtttgatttgggatggttaggatagtaaagttggttgaggttgtttggtttagggtgtttgtatgttgttaaatttaatttggtttagagttgtgattttgtagaatagggtgtaataggttttaggaatgttgggtgattttagttattttttttttgtttttgagttttgggttttttttttatttttttttgaagtttttttggagtttaagttattttatatttaaattttgtagttggatgggagtttaggttatttttttatttgtagttggtgggttaaggagttttggtgttaaatttggttgtggtataggtgttaattggtaaagggatgatttagtggtggggtttggaaggtgagggtttgtgttttgtatttttgaattttggtttgggaggtagtgatttttatttgggttaataaattatttagaaagtattagtgggattttttataatggtgttgtgaatgagtgtagggtttatttatgttttgtgtatgtttgaaatgaaatgggagttttgaagatgatatttggataatttgataaaaaaaaaaaaaaggtgggtgggggagatagtttttattgttttttttgtgtttttgtttttagttttagagatattataggtgaaaataatagtgggttggttgtttaggtttgagtggagtgtgtttttgttagtttgaaagtttttttttgtagtttgtttggatgtgtgtgtttatagtttagt

SEQ ID NO: 198 - DNA, 1780 bp, Artificial Sequence
  subsequence
tgttttgttggggttttttttgttttgtaaagggagtggggagttgggggagttttgtatattagtttttttggagttgtagatgaggagttttgtgtttttgggagttttttggtggttttttttttaatgtgtgattgtgtagtttttttttgttgtttttatttgtggtttgtttttgttttttttttttagttttgttagttggagtgtgtatattgggattttggtatgtgggtgtgtgggaggtggtggttgttgttgttgttgttgttgttgttggagtttgaatttaagttttagttggagttggagttggagttggtgagattgttttttatgttgtgggagttgtggttgttttttgtttagtttttggttttaggtgagtttggtgagttggtgaagtattggtggggaggaggattagaataggaggaggggtatggtggattgaagtgagttgggttgtgagtaagggatatttatagtttggagaaatagttttgtttttttgtgtgttgtttgttttagttgttattgggggttttaagtagtgtgatgttgttttgttttttttaggtggtggttggtggaggttttttgtagttgtttggttggtgttggtttttattttgttggtaagttttttgtttattttggagggtgtatttggatgtttgagttggagtgagtgtgaagtttgaagtttgtttttagagttgttaatttttttgtgagtttttttttttgttgtagtttgtgttagatttgggagtgatgtgtttttatttgggtggtgtgttttttgttaatttgttatttatgggattgattgtttttagttgtttggtttggagtgtgtagtttttgttgtgtggtttaggagaggagtgagatattaaggtgttttgtggattttgtgtgtattagttggtttggtggttttgtgggatagtgtttatatttaggggtgagtaggttgttaatggaggttttttttatttttagttagtggtttgtatggatggtaaagagatgggagaaagttgggtttttttgtgtttaatttggtattggtagaggaatgtaatattgttttttttaatttgattgttgtgggggtttttttagttttttttatttttaagttaaggagggagtttttttttgttttttaaggagaaaaggggttttttagagtagattgttgatttttttattaatgtgttatttggggttttttagttgtttgtgtgttaagttagtttttagtataagtgtttagagatttgtagttgtttgggtgtgttaagagattgtgggtagatttagtttttagggtagtttaagtgtgttttattaaagaaaaaagattgttggtatattaaagaagtgtgtgtgtgagagagaaagagatagagaaagagatagagagatatgggtgggggtattaggaaaggtagtttgagtaggaggtgttagtgaaatttattttttgttgatggatttagtttttggaatgtttgattgttttgatttgtggtgtggtgtgggttttaggggtgtataatatagggtgtttagatagagtttaataggtggtttgtgtgggtattttgtggttaggtgtgggggaggggaatggttttttttttgagttttgggttgtttttgttgtttttaggggtgtatttgaatatggataaggaaatgtgttttttgtttttaggttttatttggggtgagtgtgtgaggtatttaaatgttttttgttgga

SEQ ID NO: 199 - DNA, 1038 bp, Artificial Sequence
  subsequence of GATA2
gttggtatataggaggggtaggtggggatggggtggtgtgtagtaggttgggtgtttatagtagttaggtttgggtgtaggggattgttattttttatttttatgttttttgttagtgatatttggtatttgatgttgtttttgttttttttttgggttgtattattttttgtggaagatgaggttggagatgtagtttttgtggtgttagggttaggagatatttttttgggtggtgtgggtgggaagttgaaaaggtgggagttagagtgggttgttgtaggggtgagggaggttattgagtttttgttgttttttttgtttttatttttagtttttgggtatatagagagtgggtttttagggtttttagtagttgaggggtgtagtggtgttttggagaaggggtttatggtttaggggttgtggtggtgggttgtagtggtagagagggttgttttgtttttgtttagttagggtaaatttgggttgtgtaataagtgtgggtggtatatttggtttttggttaggtgggttgtgggtaaagagagagaggattagggtgggtagaaagattagggtaggtagagttagggatgtttttgatagatattgagattatgatttttagaattagtagttattttttttttaaagaaagttagaaatataatattttattggtaataattaggaatgttagtttaagttgaaggataagtggtatagaaggaattttattggatagattttatagggaatttttataggttagttggaagtgggtagaaattttgtgggttttagattttttttaattggttgttgtttttattttttttgttttaattttttagtagtttgatttttgtggattttatatttgggaagtaagtagatgggtttttttttttttttttgtttggtgtgtggtgtttgggtttttattattatgggtttagtgtttattgtgtgtggggttgtaggagatgtgtgtttgtgtgtgagtggggttggtatagtaggggttgttttgtg

SEQ ID NO: 200 - DNA, 1100 bp, Artificial Sequence
  subsequence of ADCYAP1
gaggtaaaaagggaatgtgagttagggagtttgatttgttttgaatgaaaagaaagagaaattaaattaaattttttagttatttaaaatttttaggtttttagggaggttttgttataattttttttaagtatgattgtttttgggggaggggaaaggggtggttgtatttattgaaaatttaaattgaaataataaatggttaaatgtggatatttatggatttaaatagttttgtttatgttagagaaattgagagtatagggtttgtgtgaagtttattttggtagaaggtaatattttaataaagtttgtgggaaaatagattatatttttgttatgaataagttatgtagtgaaaaatattgtttatagtttgttgatttatattattattatgttttttaatttggtgtgaggagggagaggagtgtttatatttgattaggaattgtaggattgatgtaaattttagggtagtagttagattggtatatgtagggttttttggttattttttttgtatgttgtgggtgagaggaatagtgaggataatttagtgtaaatatatgaagggttggattttaagggggtagtgttgggagaaaggttaggtttgaagtgtgtgttgtttgtttggattttattttgggttttttttgtagggtttggtgttaggagattttgtgtggggaggggggtattgaggggttgttgttttggttttttttatggttgtttttaggtagaggtgggtgatgtggtgggtagtgtgagttttgggttttttttgaaggtttttgtgtggggtggggtttgtttgttttttgtggtgattgaatttgtgttttttgttttgttattttttttttgatttttttgtttgtagtgggagttttggtggtggtgtgggggatgatgtggagttgttttttaagtgttatttggatgggatttttatggatagttatagttgttattggaaataaatggttgttaagaaatatttggtggttgttttagggaagaggtataaataaagggttaaaaataaaggatgttgaatagtttatttgtagtgatgggttattagttatttt

SEQ ID NO: 201 - DNA, 963 bp, Artificial Sequence
  subsequence of TBX5
gtagagaataattattgtattagggtttgttgaggtatgaggtattttattttgttttgtaattatgatgattattatttttagtttgattaatgggtataatttttaagtagtgtagtggtggatgtttgtaaatttttgtgtattgttggaaatttattaggttgagttgtaaaatgtattgtgtagatgtttttggtggtgttgagagaagagttaggtttgtttagtatagagttggagagtgttgggttttttggaagggtaagttttttgttaaggggttttgagggagttggatgtttgaatttggatttgtttttagttttggggtttgattttgggttttgtgtgtttttaatttttagggttttttgaagtatggtttggttttaggtttggttttgtaaggattggaatggtagtaaaatgtgtagggaggtagttggttggtagagttgtggtgggagttaaggttaggtttgtggggagagtgggtagtttttagtgttggttataagtttttaggttagttgggttgtagatttttttgtttttagagagtataatttgtgtttttttttttagttaggttgtagtggttgttttgagttttgtttttgttttttaagttgttaataatgatatgtttttaaatttgaggtttgtgtttgtttttagatgttaagaatgtaatttgaaattttttttttaaattttaggttgatgagatgagtttttatttgatttttgagttgaggtgggttggaaattgaggtttaggttttgttggggttgtaaggaaaaggggaaattttgagtgtagtgttttttttttgtggtttttttttttggtattttggattgtgggttttgtagttatttggattggtatttaaaggattttgtaagtttagttttatagattggtttttttagatgttttgaagtttgtattatgaa

SEQ ID NO: 202 - DNA, 837 bp, Artificial Sequence
  subsequence
ttagtttttatttatatttttgttatgatgggtaattgggtatgtgtaggggaaaaatagtaatgttaaaatgtaattgtgtaaatgaggatagagagtgtgaaaggagggagaggtgaggagttgttttatttttagggaggttttggggagattgattagttttaaggatagattgttgggaagggaaaaatggtttatattgaattggatgttggatggaaatttttttgtgttattagattgtgtttagtatagtagatggtatgagtatgtgtggtgtttagtttaggtttttggaggtagttgagttggaaattttgatggaaagtatttataagtttttattttgtgttggtttatttgtgtgtatgtttattttttatgtgtgtttttggtttagaagtgtatagatgtttattgtttagagttggtattgttggggagattgagtgatttgtgtggtgtatagtgtggtgttggtagggttttgggtttttggttgggggtttgagtggttaagggatgggggtgggggtggggagagtggggggagggtgaaagattgttgagaggaggggggagtgggtggattaatgatgaaaaagttttttttattttagttttttaattaaatgtatggaaagaattgaggtgagtatatttggttttaatttatagttttttgatggtattaaatgttttttttttagattagggttggaagttttgggttaattatggttgtttggagtttagaaattatttatatatatttgtatttttttttttttttagttgagttttttgattataggatgaaaaaaaaaaaaagtt

SEQ ID NO: 203 - DNA, 1012 bp, Artificial Sequence
  subsequence of NECAB1
tttgtgattttgggaaattttatatttgaatattatttaataatttttgttttatagtaaatgttttgaagtttattttaggtagagtttatagtattgtttttgttagtagtattgttataggtaagttttagaattttttggggtgagattggtgtaattattttattgatgaggaaaagtgaggtttataggttaagttttttgagtgtaagataatattgaatggtttaatttttatattaaattagttgttttttgattgttggtatttgtgaattttgtttttgtttttggggaaggttgggtagataggttattgggattaaaagtagagtaggtagaatttttttgagtttttttttatttatggtatttatttaggtgaggttgggggtgtttttattttgtgttttggttgtttaggataaatgttttgttatttgttttttttttttgtttggatgtttttttttatttttgtatttggggttgttgtggggttggtaggggtttttaggttatttttagttgtggttgatggttgtgttgggggtagagtttgtttttttttgtgtgttgttatgtgtggggatgatatggatttagatgttgttaattatgggaaggaggaggtgagagttggagtgtgtgggagtgtagaggttggaggagggagggggggatattgagtgtggagagtgtggagagtgtggagggaggtgtgtgtgggagtgaatatttttttggatttagagtttggtggtggtgaagtagtagttgtggttgtgtttttgttagagttggtgtgtttgtttagttttgttttgtttgaggttgttagggtttttgaggatggaagatttttaggagatattgttgttttttaataattttttggaggagtttagttttgttttgtatttgtttaagggtatgttgattttttttgatgtaagtatagatggtgggagttgggtggttgttttttagtattttttttttttttgaa

SEQ ID NO: 204 - DNA, 1017 bp, Artificial Sequence
  subsequence of ADRB1
tttgagttgttgttttagtagtggatagtgggtatgggtttgttgatggtgtttattgtgttgtttattgtggtgggtaatgtgttggtgattgtggttattgttaagatgttgtggttgtagatgtttattaatttttttattatgtttttggttagtgttgatttggttatggggttgttggtggtgttgtttggggttattattgtggtgtggggttgttgggagtatggtttttttttttgtgagttgtggattttagtggatgtgttgtgtgtgatggttagtattgagattttgtgtgttattgttttggattgttattttgttattattttgtttttttgttattagagtttgttgatgtgtgtgtgggtgtggggttttgtgtgtattgtgtgggttattttggttttggtgttttttttgtttatttttatgtattggtggtgggtggagagtgatgaggtgtgttgttgttataatgattttaagtgttgtgattttgttattaattgggtttatgttattgttttgtttgtagtttttttttatgtgtttttgtgtattatggtttttgtgtatttgtgggtgttttgtgaggtttagaagtaggtgaagaagattgatagttgtgagtgttgtttttttggtggtttagtgtggttgtttttgtttttgtttttgtttgtttttgtgtttgtgttgttgtttggatttttgtgttttgttgttgttgttgttattgttttgttggttaatgggtgtgtgggtaagtggtggtttttgtgttttgtggttttgtgtgagtagaaggtgtttaagatgttgggtattattatgggtgtttttatgttttgttggttgtttttttttttggttaatgtggtgaaggttttttattgtgagttggtgtttgattgtttttttgttttttttaattggttgggttatgttaatttggtttttaattttattatttattgttgtagttttgatttttgtaaggttttttag

SEQ ID NO: 205 - DNA, 1030 bp, Artificial Sequence
  subsequence of OTX2
ggtggtttttggtttaggttgatttgtaagtgaattgagtttttggtgtgtgggtttaaggaggtgtttggttttttattattgttgttttaatttatttatttagttatatttgtatttttttgttttggattttaaaaaggtttttgggatttatttaaatgattttaattaaatttgggggttaaaatgtaaagattgtgggagaagtttagaatggtgttgatataaaaataaaattataaataaaattttttaaaatattttagattatatttgtagtgttttgatgatgttttgtagaagtgatgatttttaggagtatgttttttgttttttttttattattgtttttatttttagattatatttttttttttgtaatgattgttattatattttaaaatttgtaagagaaaaaatatatttgtttatagaattttatgtttgtagaggggtattggttggtttattggaggtattggggtgatggttgatagatatggggatatgtagatatggatatagataagatagatggatatttattttatagttttatgggaggttagaaaaagttaaatattttttaaattttaaatagttagttattttaaaagaaattaagagtattgagttagaaattttgtagtttttatttttttatgaaaagttaaatataattaaaaaaaattttttttaaagaatgaaaatgaggaaggtggttagagttttaaatatgtgtgggtttttttgtaatatatataaagtagatgtggtgagtgagggttgttttagtaatttttatttttaattatagtggaggttgtgttggagttgaggttggttttgtttttagggagatttgttgagaaagtgtttttttggtaattttttgatgtaaattttttaattaatggtagggagagaatgattgatatatttaagttagagggaaaataataaaaatatataatagggggaggaaaataggttgttgttgtatggggggatgagtaggtaataaatt

SEQ ID NO: 206 - DNA, 1076 bp, Artificial Sequence
  subsequence of NKX2-6
aagtgaatttttgagatttagggttttatttttgttaggggtgtgtgaagtatattgggtgttaggagaggatgggaatgggatttgagaggtttttttttggattttttgagagaaaatggagagagttttgaatttaggagataggaggtgtattttttttatgtatttatggattatgtttttgtttttatattttttttgtaggaggtaagatttgagtgtttatttatgtggtttttttatttgttttgtgtttatttttaagattgttttatagggatttttaggaggttttgaattatttagttttttgttattgttgttgttattagtgttgtgaatttttgatttttgtggttttgtgtttatttttaggtattgaaagttttttgggtttttttgtatttgtggatgtggtgaagttgtggggtagttttgtttgtgttttagttgtaggatgtttttgattgagaagggggtggaggtgatggggtttagtagtattttgaaggtggatggggtggggttgaggaggtttgggtgaggagtggtattttgaattttttgttttgttgttgtaggttttgtagatagatttaagttttgggatagatgtttagtgttttagatagtgtttttttttgggttatgttggtaggtttgggtttagggttgggtgatgagattgtagttttttattggtttttgtagaaattatgtgttagttttgtattttttttttttagtgttttttttttgtgtttgttgaattttttttagtttttagttgtttttttgggaggtttggtttgtattgatggtttttaaagtaaagaaaatgtggagagatagtgttgtgtgtggtttggatttttgttaatatggtattagtgggagtttttgaggttaatttagggtttatggggatttttttagtggatatgtggggattggaggtggagtttttgttgtgtaatttgatttggtttatttagtttggttttagtttaattttgtatttttatggtggaggaaagttaagatagagatagttgggatttgtggaatttgag

SEQ ID NO: 207 - DNA, 927 bp, Artificial Sequence
  subsequence of SIM1
ttgatagagttttttttttggaatgaatttaatatttttgataaaatatatattatagatttgatattattattgtttttattttgataggaagaggaggaagataagtgtgtgttttgtttttttaaaatttttttttattttaataaataaatgttatattttaatagaaatgtattttttttgtagttttttttgggaatttttatttttttaattaattgaggtgttttgtaggtaatgggggagggtggtggaggttttgttttatgatttgattatgatttggtgattgaggaggggaaagtttttttaggttgaggttattgtggtttttgaatagtttgttttaattaattgtgtattttttgagagagtgtaggagagtttggtttagggggtaattttgaaaattttaaattttatgtattttgttgggtttgtatatttttgttaaatgtgtattgtgtaagttttttttgggttgaggtgttgagtggtttttgtgtttagtttttgggtgtttttgtagttgagttttttagagaaaaaaagagagggaaattggtgtaattagtttgaattaagtttttagagtagttattggtaggaggtttttttatgtattaaggtgtatttgattttatttttggtattgttgtttgttttgtttgtggttttttttggttaaggagtttgtgtggttgatttgagggtattggtgagtgtgttgggttaggttttgttttatgtagtagtttggattttatagtgtgtgtttgtatttggtagtgttttgattttttttgtttgttgattttgggttagagatattgtggttgtatttagggaatttattaatgttattgtaaatgtggggtggaggttgaaggttatattgttgtttgttttttttttttttttttt

SEQ ID NO: 208 - DNA, 927 bp, Artificial Sequence
  subsequence of DRD4
ataggtagatgtaggtttagttttttggttgttgtgggatatatatatatatatattgttatagttattgtttattatatatatttagtgtagatgttggtatatttttagaaggaggtttatagtttgtaggggagatttgggttggataaaatttaggggaggggagggtgtgtggggattaggtttttgttgagaattttggggggaagtttgagggggaattgggggatggagtttatattttatattaggtttggtttttgagtgggttggttttggtgttagtttttttgtggttagagaaaagtagtttagggttgagttggagatgtggtgtttttgattgtgggggagggggatttgaggtttttttttgatggatatagtgaatttaggtggttggggtagagattagtagtatgggatatgtgtgatttgtgttttttttgagttgtagatgttatagtgatgatgtttaagtttttaatttttttaaattggtgggaaggattagaggggttgtttgtttttttgtttttggagagagttattttatgtggagttttatgttgggtattgggtatggtttttatatttttaattataatttatttttaagataattatgatgtggatattattattatttttgttttatagatgaagaaatagaaatgaattaatgtgtttgagttttttatagagaatttagttaatagagtagttagttttgtttttaggtttagtggggattttgtttattttaggttggggaggggttttttttgagtttgatgatattaggtttgtttttagggaattttttaggttgtttttatgtttgtaataaaagggagattaaggttagaagttgtgatttatgtttgtaattttaggattttgggaggtaaaggtaggaggata

SEQ ID NO: 209 - DNA, 810 bp, Artificial Sequence
  subsequence of TBX15
gaaaaggtttggatggttgaaataaatttttttttaattttttttttattgattaataaaaataattttttagtattaaatttaaatattgtaatgggttataaaaatatggagaatttataaaattttatttttgtaggttatttgttaattgtattattattagttttgggagtatggaaattgaattgttattgtttaaagagaaaatgtaagtgatagttgttttttttttgagttggatagttttgtggttgagatttttaagtttttgagttttagattgtttttattttagtgtaggttgttgttttttttttgggtttgttagtgtgtgaagtggggtttattttttagttttggttgtttagtaggagtattttttagtatggttttagaagtttgggttggaaagtttttgaaattgttaaattaagttgtgagtgttgtatgtgtgtgtgtgtatatttaagatttttttgataatagttgtttttttgggttgtttttgtatagttgaaattttggtatttaatataaaatgttaaagttggtttttttttttttagggttttgttaaaatatagatatgatattttttttgttttttatatgttttgtgtatataatatatatgggttattgtaggatttgagatataaattaattgtatttatattttaaatatatagagatgtgggttttgaagagtgatttaaggagtaaggggtttaatatttatttttgtttttgtaaatgttaaaggagtagaaatataattatgttttattattgaaaagttggtgggag

SEQ ID NO: 210 - DNA, 1080 bp, Artificial Sequence
  subsequence of TRH
ttttttttttttttttttttgttttatttttgtttgtttgtgttttatattggttttgtggttgtgttttttttgtgtgtgtttgttttgtgtttttttgttgtttttgtgtggattttggtttttgttttgttttttagtttttttgtgtgtttgtgtttaattgtgtgttttttttaatttttttgtttttttttttgttttttatatgtgtgtttttgttaatagatttttagaggtggtgtagaaatgattttgtgttggtgttttattttgtggttagtgtttttgtgttttggttttggtttttattgtttttgttttagatttttggaggagtaggtgggtggggttttgtggggttggttgttgttagtgtttttttttggtggttgtgatttttttttgttgattttatttgagttgttgtttggtgtagatataagtggtggtttatttgaagagggtttggtaggtgtttggggtttttagtgttgtagatttttgatttgttgattgtggattttgagtttttggattttggatttattttgtggagtttatttttggtaggtaattgttttaatttttttttttttgtagatggtgtttgggagtattggaaagggagtttttttggtttgtttttatttttggttttttgagagttttttggagaatagggttggtgtataggtgggtgttgtgtttgtatttttgggttttttttgagtgtaggttggggatttgatgggaggtatggtgtgggtatattggaggtttttgttgttgggtatttaggttgttagagtttgtagtgtggggtgggagttttgtggtattttttgtttgggtgttgttggatagagttgggtatttagggtgttggtttgagaatttgggagtttgaattttaattttaatgttagaaatagaattttagtgttgaagttaggattttagtgttagaattagatttttggtttagttatgaaagtttagtattagaaatagaattttagttttgtaaatagattttgagttttagaatttgaattttagtgatagaaatgggatttt

SEQ ID NO: 211 - DNA, 1050 bp, Artificial Sequence
  subsequence of FBP1
gtaagaggattgtttgagtttaggagtttgaggttgtagtgagttagtgagaaatttgatttgggtttttaattgtagaaagagtgaaggaggataaagaagaaatggggaaggaaggtatttgagttagtatttttttgtttgaggttagggtgggtatgatgggtaggttaggtgtttatatttggttggttgagaggggtatgaggtaggttgtttagggtagagaagaggaatgtaagatggaattaggtgtatatttgtgagatggatttttaggtgggtttttttaaggttaagggaggagatgaggatttgagtgaggttgagttagtttttggagagaggggttattagatagagagtgagagaggtgtttagatattagatggatagatagaggttgatggtaggaggtttagagggtttaatgttagtttgttgggtaggttttttaggtagatagataggatggggtttattgtttaaggtttgatttataggtgtgtgatgtttgttttgtgtattgttgaagagatggttttgattgttgtgtagagtgagttgagtagttgggttaatttgtttgtgttgtgggtttttttgtttttttttatgatgaagtgggttagggtgttgatgtttgtgttgaagggtgtttggttagttatgtttgaattgggtagagtgtggggttgtaggtgtaagtggtaggtgtggggttgtaggtgtgggtggtaagagagggtagtaggtattggttgtaggtgtggagttgtaggtgtgggtggtaggtgtgggttgtgggatttggtgggaggattgatagattgattgttgttttgagtgtttgtagtgtttgtggtgtaattgggttaggttaggtgttggtgggtgaattgtggaaatttttagatgtgggttggttttttgtttttgggaatatttttgtgttttgtttattttgtggattagattgtggttttgtttgtttggatttttagataaggttggggattttttttgtggttttttaatttttgtttttat

SEQ ID NO: 212 - DNA, 968 bp, Artificial Sequence
  subsequence
tattttgtggtgttttttttttttgttttatagttaagtttagaggaatagggtattgttttgtgtggttttggagttatatttggatttgggaattttgtgttgggtttagaggattttattgggtgggttggggtttatttttaataaatttagttgtttatatatatttttattattatttttatgtgtgtgtgtgtatatatatatatatatatatagagggatttgttaattattgagatagtgatttagaaaggtgtaaatttatttggtgtttatttaattgtaaagtttttagatttatataaaatattagtgagttttggaggtttgagatgttttgtgtttgatttatggtgtgaatattagtgttttggttgggttgtaggggttggtgtttagtgggttggggtttggtgagttaggtagtgggttggttgagtttttgtgttttgtggttgtgtggtttatttgtttatttttttattattggttgggatttgtttttttttaaagtgtgatgtttggtgttttattttaggttatgtggagtttttttttggtgtgttgggttttgtgtttttgtttagtggtttattttggtttgttgtgtttgtttttgttttaagtgtttaggatggagtgaggggttgtgggttggtgtagggatgttggttgtttatttttaggagttgatagaaggtgtttttggtgttatgtgtttaattttggggttgatttaaataattaataagtttagagaaattttatgaggggaatttttttttttagtattaataaagtttagtaattgggtttgttggttatttaagtttgagtttgatttttttagttttttttttttttttttttttttatttagaggtaatgtttttaaaaattggtaattgtgtgtgtgtttggggtgtgtaagtgtgagtgtagatgtgtgaaagttatttgtt

SEQ ID NO: 213 - DNA, 1080 bp, Artificial Sequence
  subsequence of BCAN
tagtttttttttatgtttgtgtagtttttgttgtagttttagttgtagttgtaggattgagttgtgtatttggaggagatttttggaggaggtgataaattttgtagtgttgtgatttaattttagttttgggtaggtgagtgtttttgtagttttgttgtttgttgtggggttggggatagggagaagggagtgtttgtttggtttgtgttttttgtttgttagtttttgttttgaggttttggggtatttaatttgttgatttttgatattgtagtggggtaggttgttggatagttttgagtgtttgtagttgttgttgttatttttgatttatatgtttttagttttgttagtggtagtttttttgttgtttgtagtttgattagtaattttttgggtttttgtattttttttgttgtgtgtttttgttttagtgtggttgttgagatttttgattttgttttaggtagggtggtagtgttttggattagtttttgtttttgtgtttttatgtataggtagttttaggagtagtggttagtaatttttttggggatattttattgtagtttggtaggatagttgattagagttgttttagggggtggttggagtgtttattttggttggaattttaatttggttttttgttttgtgattttggggtagttagttgatttttttgaattttgggttttttattggtgtaatgagtaaaatataaataattttttttttatagttgaggttatttataggaagtatttaggagaattggtttaggtagatattagtaattattagttggaatttggttattattattgtatttttttttagtattgttaggggtttgggaatttttttttttaggtatttttatattttgttaggtatttttttatttattggaatagttttgtttatatggttttaataggattaagagattggtgttaagtttaaggggtattattattatttgtattatttagattgtagatgatgatagtaagattagggaatagtgttatttttagatttatttatagtattattagtgtttatgttgttatg

SEQ ID NO: 214 - DNA, 1017 bp, Artificial Sequence
  subsequence of TP73
tttttaggttagggtttaggttttgtataggttaggagtgattttggtgggtttttttttttttttgttttttgtttattttggttgggggtgtaggggttagggtgtggtgtggttagatttttaggtttagggtgattttttttgttttttttgttttattgttttttgtttttaatgtgttggttttttgtaggatttgggggttttgaagatttttgagtagtattgtatgattatttggtggggtttgtaggatttgaagtagggttatgattatagtattgtgtagtagttgttttgttttagtaatgtggttattatttttattggtggtttaggggaattgtagtgttagtgggttatggaggttgtgtatttttgtgtgtgttatattattattatttttaattgtggtggtttaggtggtggttttgatgagtgggtggattttggttttgatttgtttgattgtaaggtttgtaagtagtttattaaggaggagtttatggaggttgagatttattgagggttttgtttggttgtagtttgtgttattgtttagagatttaagttgtttttttttttttttttgtgtgtttaaaattgttttaggaggtaggatttttgggttgtgtttggggaaaggtaaggtttggtttatttttaggtattttataggttttaggaaaggtttagttattgaagttgtttgtggatagtttgagttatttgtagaattttttggagttgttttagtgttgggtttgtggggtgggggttggtttatttttagttttgttattgttttggtgtgttttatggtaggtgtgggtggggattgtagtgttggttttgatttttaggttttattttagagattgttattttttaattaggtgaggtttttttaaaggaaaggattttttttgttgatggattgttaaaaagtattttgtgatattttttggttttggatagtagtgagtagttaagtgattgtgtttgaaatattag

SEQ ID NO: 215 - DNA, 1058 bp, Artificial Sequence
  subsequence of MIIP
gttttttgagtagttggattataggtatgtgtttggtttattttttgtagagatggggttttgttatgttgtttaggttgggtatttttttttttttttttttttttgagatggagttttgtgttttgttttgttatttaggttggagtgtagtggtgtgattttggtttattgtaatttttgtttttttagtagttgggtttaagtgatttttttgttttagtttttttagtagttgggattataggtgttggttattttgtttggttaatttttgtatttttaggtttattggtgtgagtaattgtggttggttttaatattatatttttttgtttattgtgtagtttttattttttggtgtaaagtgggtatttgttaaaaatttgaatgaaagtataaagtaggttgggtgtagtggtttatgtttgtaattttagtattttgggaggttggggtgggtggattatgaggttaggagtttgagattagtttggttaatatagtgaaattttgtttttattaaaaatataaaaaaaaaaaaaaaaaaaaaaaaaaaaaaaaaaaaagttgggtatggtggtgtttgtttgtagttttagttatttgggaggttgaggtaggagaattaattgtttgaatttgggaggtagagattgtggtgagttgagattgtgttattgtattttagtttgggtaatagagtgagattttgtttttaaaaaaaaaaaaaaaaagaaaagtatgaaatgatgagtataatgagtagttagttgtttgttttatttattttgttgttttggattgttgtttgtgttgagtttaggttgtttagtttgattgaaattgttgttgttgaatttagtgtatttagttttgtagttgattaattggagtttgtttttttggggtttgttttattttaggaattgatttttgtattggttttgaaaattgattaattggttgtgtagttttgtttttagttttgtttttatgttgaaattgatattttggattgttgagtaatgtttattagatgttttggttttgttttt

SEQ ID NO: 216 - DNA, 1166 bp, Artificial Sequence
  subsequence of HOXC4
tttggtttgggtttgaggttttgaggtggttttataagtgtgaatttttgtttataaatggtgatgtatatgtaaatgtttatatatttaggtagatatatttggaggtgtgggggaatatattttagatgaggtttgagagaatttgggggttagatttattttaatttaagttaagatattttttttatttttatttttttttagaggtgtgattgggattttgtgttaagttttagtgggggaggggattgttttatgattttttgtttaaattttgatttgttgtttgtgggggggtggggatgggggaagaaatttgtttttattaaatttttaaaaatatagtttgtatttagattaaattgtttgggttagagttgatggtgaattttattttttttttttttataattttttttttttttttttttgtttttgttaaattttttttttgtagttattataaaggtttttgaggtatttttttgtgggaagaaatggtatttttttttttttttttttatttttttatttttagtaggatttgtgtgttggtagaggtgtttgatgaggggttaattttgttttttttgtttatgattgagaaaagtgtttggttttttttaaatgggtttagtttgttgtttgtttaggttgttgtgtgtttttttgttgtttaggtatggtttagtggttgatgttttgtggatttagtttgtggtaggttggaatttggagtttgtgggatttgaaaagggtaaagggagtgtggtgggatataagaggggtttgagaggtttgaaaaagggagttttttttttggagtaatgtgggaattgttgattggtgaggtttttattttttttttttgtttgtattttgtttgtttttgtttttgtggatggttgttgatgggggggaatataagtgttttttgtttgtttttgaaagaaaattttttttagagaaggttatttaggttagtggagatttatttagaatattagaagggtttttttttatttgaggggtgggtttgggtgaggttgaggtattttttttaattttagaatgattttattgagtgtatttatagtgagatttggaggtgttagagtttgaggttggttgtttaatagtattattttgaggtgtttttatat

SEQ ID NO: 217 - DNA, 1334 bp, Artificial Sequence
  subsequence of HOXA7
ttggttttgtgttttgtgttttgtgttttttagtgttgtgttttttgtttttggttttgttttgttagtttggtttgtttagtgattgtgtttatttgaagattgtatttaggggtagatgtggaaattggttttagttgtgttatgtagtgtgtttttgtttgttttgttgtaggtgtttttggtgaggttattgtagagtttggggatgttttggttgtaggaggtgtagggtaggttgttgtaggtgttggtgtttaggttgtagttggatgtaaaggggttttgataaagggggttgttgatattgtataagtttggaatggttgaggtgaaggtgttggtgtttgttttgtagttgtttttttgtgagttgggagtaaaggagtaagaagttggtttggtattttggaatagagaagtttttgttgtatatttgttaaaaagtgtgtttatataatatgaagaatttataattttgatttgtgatttgttgtttggtagtttttagtgttggttttatgaggtagagtgatatatgataatattatatttttagatttatattaaattttatttttttttggatggagtttgttgtagtatgtgattgtttatatgattgtttttgttaattttagtagtttttataggtggttttgttttgtagggtttgtagttgtttagaatggaagggtaagaggtttaaatatgtggttaaagaatttgtttgtgtttggtgggtttggtgtgttttgtggaaaaagatttggaggttttgtgggagtgtttagttggtggttaatttttgtattggggtttgtggatgttaggtggtttggttttatgtagtattttttattttgtttttttgttgatttttgttagtgagttttggattaagtttgggattttttttattttttttttgtttgtttgtttagattttggaagggtttttgttttttgtaatagtttgttttgtggtggttttgtgggtaggatttagttatgagtagattgattttgtttaagtttttttttatttaggtttagtgggtgataggttggatttagatttggatttagatggggaaggtgtagtattttttgtagttgtagagagattgttattgtaaattggagttatgtggtttgaataaagttaatgttttttagttttttttttttaattggaggtatattgtttatttgttttaaaggaagtagtgaaatatttatttattaatgagatttatttgttaatagatttattaatgtggggtttttttttttttttttggatgttgtagtgttgtaggttttgtgttttt

SEQ ID NO: 218 - DNA, 1181 bp, Artificial Sequence
  subsequence of BST1
aaagagggtatttgttaaagttgttgttttttggagttagaaaagtattttttttgatgatgattgatttttttttattttttttttaattttgtggtttttttggggttttttttttgtggatagtggttaagattagtttgggttatagtgtattggttttgttttgggtgatgttttaagtttatttttttttaattttatttatttattaattttttttttagatagagttttattttgttgtttagggttggagtgtagtggtgtaattattgtttgttgtagttttgattttttggggttaagtttttttatattttattttgtaggtagttgagattatagatgtgtattattaggattagttaagttttgtatttttttgtagagaggaggttttttatttgtatgttatttaggtttgttttgaatttttatatttaagtgatttgtttgtttaggttttttaaagtgttgggattataggtatgagttgttgtgttttgttttatgtttagttttgaaattgtttggaatgggaaatggtaaatagtgagatatttgagtgagagttttgttttgtattagtttgtggaattgttttggtagaaggagagaaggggagtggaggaagtatgggattggagggattaaagttttttgatggtggtttaggggtgtgtggtattgtggttgttttagttgttgttgtagtttttgtttttattgttgttgttggtggtgggtggggtgtgtgtgtggtggtgtggggagggtattagtgtatatttgtgggatatttttttgggttgttgtgttgagtattgtgtattgttgagttttgagtagtggtgaggtagttggttgggtggaaggggagttggaaagaggtaatggtggggagggtttggggaggggaaaattggtgttaaagtttggggtgagggggtaatgagagaggttttgaggggagaggtgagtgtggagatagtgatggttttgaatgatgggggtgagtgaggagggggttgtgaagtgtgtttgtaggtgaggggtgtgttgtgtggggtttagagatgagtgtgtgtgtgtgtgtgtatatatatattgtagaggtgaggggtgtgtgtgtgtgttttagaggtgaggggggtgtgtgtgtgtgtgtgttttagagg

SEQ ID NO: 219 - DNA, 1039 bp, Artificial Sequence
  subsequence of C1orf114
aggtattattaatgaaatgaatattattgtttttttatggaagttataattttgggagtgatttttttttttagggataaaattattattttttatgtttaagaattttgagaggggaaagaatatgataaaaatttagtttaagttatttttagatgagtattttttatatatagtgaagaaaggtgttattagatttttttattagtgttagatttggtggattttggattttagaggataaggtgttattagaaagtttttttttttattatttatttttttttttagttatattagatgtttatatttttattttttattttattattaatatttttgtattgttttttttttttttttttttatattttttttgtttgtgtaaaatgtggtggttgggattatagagatggttgggggagtttttttttttttttttttttaagttttttatattgaggtaaaggagattttggtatttgtttttgtggtagttaggattatattgttatggtaatagtgtgtttttgtgttttttatttgggtttttttaattatgagagtgataaaaatttgtgtaggtgtatgtaatatttttagattattgattttttttggtatttattttggtgtttgtgaagggttagtgaagttgaggtttttaaggggatgattaaggaatttatgtattattaatgttatagagatttgtgaagtgttgttgtgttggttgtgaaattttttttttgtagttgttttttgttagatttagaattttttaggataatttttaaaattatatttttatatgttatgtgttttatagttaatgtagaaaagtagtttttagtttttattagtagataagtaaattgttaatgagttattatatttttgatttttagttttttttttttttaattaaaattaaaattttatttaagagagttgttaaagaaaataggatttttgttttagttttgaggtatgttaaaatggttaattagaatttttttaaattttgtttatttttatg

SEQ ID NO: 220 - DNA, 1027 bp, Artificial Sequence
  subsequence of FOXG1
ttgtttttgttgttgttattgttattattggttgttgttttggatggggttaaagtggatgggttgggtggtaagggtgagttgggtggtgggttgggggagttggtgtttgttgggttggatgagaaggagaagggtgttggtgttgggggggaggagaagaagggggtgggtgagggtggtaaggatggggaggggggtaaggagggtgagaagaagaatggtaagtatgagaagttgttgtttagttataatgtgtttattatgatggttatttggtagagttttgagaagtggtttatgtttaatggtatttatgagtttattatgaagaattttttttattattgtgagaataagtagggttggtagaattttatttgttataatttgttttttaataagtgttttgtgaaggtgttgtgttattatgatgatttgggtaagggtaattattggatgttggatttgttgagtgatgatgtgtttattggtggtattatgggtaagttgtggtgttgttttattattttgtgggttaagttggtttttaagtgtggtgtgtgttttatttttattggttttatttttatggattgtgttggttttttttattggtttatgttgttttttttgtttttgtattatttttgtgttagtagtattttgagttataatggtattatgttggtttattttagttattttatgttttatagttttgtgttgatttagaatttgttgggtaataattattttttttttattgttaatggtttgagtgtggattggttggttaatggggagattttgtatgttatgtattattttatggttgttgtgttagttgttttggtgttttgtggtttgttggtgttttgttttgggatttatttttttaatttttgttttgttaatttgtttgtgggttagattagttatttttttttttatgttttgtatttgttaatgattttgtagagtagtatgtttatgagtgttagggttgtgtttttttttatgttgt

SEQ ID NO: 221 - DNA, 1017 bp, Artificial Sequence
  subsequence of ATP4A
atgagggaatggggtggggttgaggagaggggtggggttgagagtttggtgtgggttttgagagttgtggggaagggtgaaggtggaagatggaggttttgtgtggaggggtttttggtagaaggtaagtgttaaggtggggttaggtgtagatttggagttttggatgtagggaatgaatagaattagggtgtggagttgggttgggggtggatttggagagtgaggtgttttttatggatagttttgttgaggagaagttgtgggtggggttgggtggtgggtggggttttgtttttggtggatggggttataggtggagtgggagatggggtggggtttggttgtggagagaaggggtaaggagtgaagttttttgtggtttgttgatgtgggtgtggtttggggtggggtttgaggtgggtgggtttaggttgtgggtggggttggttgtgtatttggaatttgttggtggagttgaagggtattttgtagatttttgggaagtggttttggtagtttatggtgttgtttagtgttagttttgagaatttgagtagtgttgtttttgatgtgtttttaattatgatgtgttgggagtggggattggtgttaggggtgaagttggttatattagttttttgggattttttggaggttttttggtttttattttgggtataggtattgtattttggttggatttgaaggtggtgtggttgtatagggtgagtatttggtatagtgtttgttatgtttttgaggattggttaaatgtttgttttgtagattaggtgtttaggttgggttttgtatggtggtttttttggattagaattgagttttttttttttaggtttatattgtgggttttttttttagatttgggtggaattgggttttatttaattttgagggatttagtttttggatgatttttttttttagatttggtagtgagttttttttgagatttggagttgagttgttttgtttttgtataaagttttttttatt

SEQ ID NO: 222 - DNA, 1161 bp, Artificial Sequence
  subsequence of NOTCH1
tttataaatatagaagaatttttttattttatgtaggaaaattttggtttttagaatttgtttgtttttttagaatagataaaagtttttatttggggttagataaaatagtatatataaataaaaaggtagtgtttttgtgtaaaataaaagtatataaataaatattaaaaaaaattaaaatttttgtttttattttgtataaaaatatgtgttttaaaaaggtttttttggttggttttggtatttatagagtgtatatagatgtttgaaggtttgggaaaggaagttggggttttgtggggtgtgttgtttatttgaaggtttttggaatgtgggtgatttgggattgtatgttggtgggagggttggagatgtttttggattagttggagatgttggaatgtggggatgagttggattattggttaggggatttaggggatggggtgaggaaggggtgtttaggtatttgtagttggtggttgggggtgttgtttataggtgaggagtagttgtgttgtgaggggggtgttaggaattgggttgtggttatgggtgggattagtgaggatggtagtgatgtgggtagggtggggtttttttggggtagaatagtgtgtattgttaggttgttggggtttagtggttgtatgtttgtttggtttggttttttatttaggaagttttggtttaggtggttgttggttgttgagtttatgttaaggtgtggttgtggtggtggtggtggtggttgtaggttttgttgttgttggatgtttgttggttgtaggttttgttgttgtatttgtaagttttgtggttgtatttgttgggtttgtattaggtgaggttgggtggttagttgggtgttgggtaggttttggtagtttattatttgggatagggtgttggtagtaaggttattgtgtagtgggtttattatgttatgttgtagggagggggtttgtgtgtttagggggtttggtgttatatttttttgtagagggttgtattggtttggtattatgttgttttgtagttgggatagttatttgtattgattatttaaattggtggatttgtttatagtgaaatttagggtttttttgttgttggagtttaggatggtgttggtgttagaggttataggtaggtggg

SEQ ID NO: 223 - DNA, 981 bp, Artificial Sequence
  subsequence
ggttttgttgaatgtgtttttttggtggtgatggttttggattgtgtggttgtagtgtgttgtttgttgtgttatgtggggtttgtttttttgtgtttatgttgtatgttggttagtgttttttggttaagtggttttattaatttggttgtgtaaattgtgtttttggttgagtggttgttgtgtgtgttttgtttgttggattattttatttgtgagttgttggtgttgtttaagttggtttgtggaggtgatggagatattattgagaattagatgtttgttgtttgtgtggttattttgttgttgttgtttgttgttattttggttttttatggtgttgtggtttgagttgtttgttgtatgtggtttagtggaggttggaggagggtggtgggtatgtgtgggttttatttgatagttgtttgtttgttttatggtttggttatttatatttatttgtagtttgtgtagtgttataattaggtatggggtaagtttgtattgtttttttatattgtggttatatttgtttttaatttgtttatttatatttttaggaataagaaagtgaagggggtagtgaggaggttgttgtggagtttggggagaggttaggttgggtagtgagtagttggggaggggagaaagtattaagttagaatttaaggatggaaatattttttagtgagttagtttagattttaggttgtttatttttgtatgataatttgtaagatttgttttaaggagtttaatgggggatatgttttttttttgtgaggaaatgtttagtttttgagggaaaatttttaaattttttatatatttaggtttagggaaggaaaatttattttttataattttatgtgtagggaaaatgatggatgtgatgtttgtttttagttttttttttatttgatggaagattatggaagattttttggtttttgtaattagaagttttaagttgataagaaa

SEQ ID NO: 224 - DNA, 864 bp, Artificial Sequence
  subsequence
aatgtttttttttgaggtagttggaggttttttttttttgagagtttaattgtggatatagttttgagtagaggtgaaaaggaaagaaggttgggagataattggggaaaaatatatatttttggtttggtttgaaagttggtgtttgaaaaggaataagaaaaaaaatatgttttggaagtgtttgagattgttgtggttataaagtagagtattaattttggtattgatatgggaggggagtaagattttatttttgggtttgtgtttatgaatttaggtgaggaggggtatttttttttttgtgtttaaatgttgtattttttaagattattttggtttgttatgtttttattttgtgtttataaaaatttttgagattttagtgggtatagatataagtggttggatatgaagaggaatatattggtgggagaatatagaatatttattttttttttagttattttggaggttttggagaaggtggttttagtgatttgtgaagagattttgagttttttatattttggagaatgataagagagtatttgggtgatgtaattttttgggttttttggagatgtggttttttatatgttaggggttaagtttgagaaataggtggatggtaaggataggagttttttttgtgttataaatgtttttgtttatatttgggttttttgatttttttgtttatataattgagttatttatggttgggttttgagtttttattttgtggattgggataaaggggttaattgtgatgtgttttgtataattttaggattttgtatttgtttaagggtgaggtgtaaatttaaaattatgtatgattgaatgttgagattagttgag

SEQ ID NO: 225 - DNA, 1004 bp, Artificial Sequence
  subsequence of HOXA7
tatttaggggtagatgtggaaattggttttagttgtgttatgtagtgtgtttttgtttgttttgttgtaggtgtttttggtgaggttattgtagagtttggggatgttttggttgtaggaggtgtagggtaggttgttgtaggtgttggtgtttaggttgtagttggatgtaaaggggttttgataaagggggttgttgatattgtataagtttggaatggttgaggtgaaggtgttggtgtttgttttgtagttgtttttttgtgagttgggagtaaaggagtaagaagttggtttggtattttggaatagagaagtttttgttgtatatttgttaaaaagtgtgtttatataatatgaagaatttataattttgatttgtgatttgttgtttggtagtttttagtgttggttttatgaggtagagtgatatatgataatattatatttttagatttatattaaattttatttttttttggatggagtttgttgtagtatgtgattgtttatatgattgtttttgttaattttagtagtttttataggtggttttgttttgtagggtttgtagttgtttagaatggaagggtaagaggtttaaatatgtggttaaagaatttgtttgtgtttggtgggtttggtgtgttttgtggaaaaagatttggaggttttgtgggagtgtttagttggtggttaatttttgtattggggtttgtggatgttaggtggtttggttttatgtagtattttttattttgtttttttgttgatttttgttagtgagttttggattaagtttgggattttttttattttttttttgtttgtttgtttagattttggaagggtttttgttttttgtaatagtttgttttgtggtggttttgtgggtaggatttagttatgagtagattgattttgtttaagtttttttttatttaggtttagtgggtgataggttggatttagatttggatttagatggggaaggtgtagtattt

SEQ ID NO: 226 - DNA, 963 bp, Artificial Sequence
  subsequence of ZNF529
tatttatattattatatatggatgtagttatagaatggtatatataaatataattatatagtttttttttttagtaggtgatttgtatataggtttggggtttttgtttttataaattttttttgtgttttatgaatttaggttttttgttgtgagttttttttgtatttagatttgggttattttaatttattatatggaaaatgaatattaggttaatggaaaagggagttggggttttggtagaagtgtagtgttagttgtaatagggtggttgtgggtgtaaatggaggggagtgttggtagttagtattgtgtggtgattaatgggttgttttggagatttttgggagtttaggtttatgtgtgagtgtgtaggtgtagatgatttattttgggttgggggtgaggtttggtgggtgttaggggtgttgaggaggttaaggagggtattgggagttttgttttgggagagttgtttaaggatgtggaattgggtggggaggttagggaggtaattaagagtttgagttgggtttggaaattttgaggaggaaattgggattgtggtatttagatgttttgatttgtatgagttgggttttgggtgtggtttatgggtgtgattttgagggtgatttggagtgagttttgtgaagggggattttgtttgttttgattttgtggaagtgttattgttggtggtgggtttttgtgtggagtgggtgttgtgtgtttgtgtgtgtgggtgtgtgttgaataggggtggttttttgtgtttaatttgttgtattttaggtgtttgtttttttttgggatgttgtggttgattgtgtgtgaaaagtgaatggagtagtgttgttgtgtgaggttttttttgtgtgtgtttatttttagattaggtgtgagttgtatttgagattgtttttgagtgtggagaattgtaagtgatttgtaggtgtg

SEQ ID NO: 227 - DNA, 956 bp, Artificial Sequence
  subsequence of PRLHR
ttttgtgggagttgaatggatttaaatgttttttagtgggttagtagttttttagagggattgggagtgtttttttttagttttgttttttattttagtttttatgtatggaaaataggggtggagtgtgttttgttatgtttggtgtttagagaattagtgaagaggatagtgtggggaggatggaatttgaaatgggaggaggggttggtaaatttggttagagtagtgaagaggatgaatttttattgtaggagtttgtatggtttttggagggttagggtttggaggagtgtatagtggaggagggtggaggagaggtgtgaagtgttaggttattgggaggagttggtgtagttttaggagggaaggagtggggaaggaagtagtggtgggagattgtaatgtagttgggggtttgagagaggtatgattgatttgtttttaaaggttggattttgtttagtggttaggttgtggagggtagagatgttagagggtttgggttgggatttaatagtagagtttggagttggttgtggatttgaggatttttatttttttgtggttttgttatatgagttttttgtttggttgtagtgtgtttagtgggtagtgggtttggttaagttaaaggtaggagttagtattatggatagtttttgttggatttgttgttttttgggtggatgatgtggggaggagtaggggaaaatgattagggaatttttgtttttttttggatttgggtgtttggggaaggaatttggtttggtttaaagatttgttttgttgtttgttttttgggttggggttgagaagagtagggtggagtggaggtagttgagttgggggtttgggggttggagatttatgatttttgttttttttggtggttattgtatttagtgttaaggatggtgttgttttttattttttggggttagaaaatgtag

SEQ ID NO: 228 - DNA, 1037 bp, Artificial Sequence
  subsequence of ARL5C
gagggagtgaagagtagggaggtagtttgggatatttggtaggtttggagttgggtttggtagggtttttgggaagatggaggaaagtagtgggagttagggttgtttgtatggtgtaggatttgaatgttagattgaggagttgtagtattaggaaggtttaagtagtgtgtttaattgtttttttggattatagaggagtttgggaatttagggaagagttttagtgattggtttttttgtttgttagtttggtgggaggtttagttttttattttttttgtttgagagttatttataattggtagagaatggtggttttttttttattgtttagttttatgatgatgattgtgtgttttggaagtgttggaggaagggtagtgttagggttaaatttgaagattaagggattgtgtgtttttattagattttttaggaaggagatagtgttttttgtaggttggggatttttgtttattgtattgtgtttgttttttatttagttttgatatttgttttattttgggatggtggaaaagatagttgagtttttatttttttttatattttagaaaagtgtttgaaaggtttggggtgttttggggtttgttaagagatggtgtttagagaaagagtataatgtgaagttataattgtaggaaatttgtagtagttttttatttttgttgttggttttgtttagtggggagaaaggagggttgtttagttttgtgttttggggtgtattgaagtgttgggatttaagaggagtaggtagggatgggggtaggggaggttgtggggtagttgaggagtgtttatatatgatttttggagtttgaggtttttttgtgtgtttgattatagattagaggagttttagaagagggtgagattaaagtgtttgtttggatgttttgtgtgttttttattttggtttttgaagatgtttattaatttggtgattagttgttttatggtattttttgggttggataggtgtaggagggtttagtggttttaggagtggagtt

SEQ ID NO: 229 - DNA, 20 bp, Artificial Sequence
  forward primer of PAX9
cagcgggtcgctgactacct

SEQ ID NO: 230 - DNA, 20 bp, Artificial Sequence
  reverse primer of PAX9
cgaagctgcagacagggtca

SEQ ID NO: 231 - DNA, 19 bp, Artificial Sequence
  forward primer of HOXD10
cctggagaggcggacagga

SEQ ID NO: 232 - DNA, 20 bp, Artificial Sequence
  reverse primer of HOXD10
gcacggacaacagcgacatc

SEQ ID NO: 233 - DNA, 20 bp, Artificial Sequence
  forward primer of TBX20
gcgacgcgtagtgggagagt

SEQ ID NO: 234 - DNA, 20 bp, Artificial Sequence
  reverse primer of TBX20
ccgtgggaagtcctcgtcac

SEQ ID NO: 235 - DNA, 19 bp, Artificial Sequence
  forward primer of CACNA1B
ggccagcgggtcctctaca

SEQ ID NO: 236 - DNA, 19 bp, Artificial Sequence
  reverse primer of CACNA1B
cgagcggttgacggtgaag

SEQ ID NO: 237 - DNA, 20 bp, Artificial Sequence
  forward primer of ZIC1
tctcttggctctcggcttgg

SEQ ID NO: 238 - DNA, 20 bp, Artificial Sequence
  reverse primer of ZIC1
aacctttgccttcccgcttc

SEQ ID NO: 239 - DNA, 20 bp, Artificial Sequence
  forward primer of SIM1
tggccaatagggctgagtga

SEQ ID NO: 240 - DNA, 19 bp, Artificial Sequence
  reverse primer of SIM1
cggtcccgcgggtagtaag

SEQ ID NO: 241 - DNA, 19 bp, Artificial Sequence
  forward primer of DLX1
gaggaaacgcgggctccta

SEQ ID NO: 242 - DNA, 19 bp, Artificial Sequence
  reverse primer of DLX1
ggcgggcaacctcacataa

SEQ ID NO: 243 - DNA, 19 bp, Artificial Sequence
  forward primer of LMX1A
gcttccctatcgcggacca

SEQ ID NO: 244 - DNA, 19 bp, Artificial Sequence
  reverse primer of LMX1A
ctcctcgctgctgggtgag

SEQ ID NO: 245 - DNA, 23 bp, Artificial Sequence
  forward primer of DLX6AS1
gccacgtctacctgctggtattg

SEQ ID NO: 246 - DNA, 19 bp, Artificial Sequence
  reverse primer of DLX6AS1
ccaccccaccttcccactc

SEQ ID NO: 247 - DNA, 20 bp, Artificial Sequence
  forward primer of MIR196A1
ccgcctacacggaaaatcca

SEQ ID NO: 248 - DNA, 20 bp, Artificial Sequence
  reverse primer of MIR196A1
cgagaagcagggagcctcat

SEQ ID NO: 249 - DNA, 20 bp, Artificial Sequence
  forward primer of FEZF2
aagcgtcacggagagcaagg

SEQ ID NO: 250 - DNA, 20 bp, Artificial Sequence
  reverse primer of FEZF2
gtctcccccagcctcagacc

SEQ ID NO: 251 - DNA, 19 bp, Artificial Sequence
  forward primer of STAG3
agggcaggacgcctgagag

SEQ ID NO: 252 - DNA, 20 bp, Artificial Sequence
  reverse primer of STAG3
tcgcgaggtttggaagtgtg

SEQ ID NO: 253 - DNA, 20 bp, Artificial Sequence
  forward primer of PTPRN2
gaagcccgacccacaacaaa

SEQ ID NO: 254 - DNA, 20 bp, Artificial Sequence
  reverse primer of PTPRN2
cctctcacatccgccatcct

SEQ ID NO: 255 - DNA, 19 bp, Artificial Sequence
  forward primer of BARHL1
tggaggatggcaggtgcag

SEQ ID NO: 256 - DNA, 19 bp, Artificial Sequence
  reverse primer of BARHL1
gaagcgagcaggcctgaaa

SEQ ID NO: 257 - DNA, 20 bp, Artificial Sequence
  forward primer of CCDC140
gagtcttgggcctccccttt

SEQ ID NO: 258 - DNA, 19 bp, Artificial Sequence
  reverse primer of CCDC140
gtggcctggactcccatcc

SEQ ID NO: 259 - DNA, 19 bp, Artificial Sequence
  forward primer
gaagcgagctgggctgtga

SEQ ID NO: 260 - DNA, 19 bp, Artificial Sequence
  reverse primer
cccagtagcggctggagca

SEQ ID NO: 261 - DNA, 18 bp, Artificial Sequence
  forward primer of GATA2
cgtccagccagggcaaac

SEQ ID NO: 262 - DNA, 20 bp, Artificial Sequence
  reverse primer of GATA2
ttctgcccaccctgatcctc

SEQ ID NO: 263 - DNA, 23 bp, Artificial Sequence
  forward primer of ADCYAP1
gggctctccggttactttctctg

SEQ ID NO: 264 - DNA, 19 bp, Artificial Sequence
  reverse primer of ADCYAP1
agcgctgcccccttgagat

SEQ ID NO: 265 - DNA, 20 bp, Artificial Sequence
  forward primer of TBX5
aatgtgcagggaggcagtcg

SEQ ID NO: 266 - DNA, 19 bp, Artificial Sequence
  reverse primer of TBX5
agctggcctgggagcttgt

SEQ ID NO: 267 - DNA, 20 bp, Artificial Sequence
  forward primer
acagcagatggcacgagcac

SEQ ID NO: 268 - DNA, 20 bp, Artificial Sequence
  reverse primer
tgggagcttgtgggtgcttt

SEQ ID NO: 269 - DNA, 22 bp, Artificial Sequence
  forward primer of NECAB1
aacaatccttgccccatagcaa

SEQ ID NO: 270 - DNA, 20 bp, Artificial Sequence
  reverse primer of NECAB1
ggcagtgctgctgacaaagg

SEQ ID NO: 271 - DNA, 19 bp, Artificial Sequence
  forward primer of ADRB1
cgtcaccaaccgggcctac

SEQ ID NO: 272 - DNA, 19 bp, Artificial Sequence
  reverse primer of ADRB1
cggaacacccgcaggtaca

SEQ ID NO: 273 - DNA, 21 bp, Artificial Sequence
  forward primer of OTX2
ccgcctacagaactccacgtt

SEQ ID NO: 274 - DNA, 22 bp, Artificial Sequence
  reverse primer of OTX2
tctacgtgtccccgtgtctgtc

SEQ ID NO: 275 - DNA, 20 bp, Artificial Sequence
  forward primer of NKX2-6
agaagggggtggaggtgacg

SEQ ID NO: 276 - DNA, 20 bp, Artificial Sequence
  reverse primer of NKX2-6
aagttcagggtgccgctcct

SEQ ID NO: 277 - DNA, 22 bp, Artificial Sequence
  forward primer of SIM1
accccaaatcccatgtatcctg

SEQ ID NO: 278 - DNA, 20 bp, Artificial Sequence
  reverse primer of SIM1
ggctgaacacgaaggccact

SEQ ID NO: 279 - DNA, 19 bp, Artificial Sequence
  forward primer of DRD4
gaccagcagcacgggacac

SEQ ID NO: 280 - DNA, 19 bp, Artificial Sequence
  reverse primer of DRD4
aatccttcccgccgatttg

SEQ ID NO: 281 - DNA, 19 bp, Artificial Sequence
  forward primer of TBX15
tggctgttcagcaggagca

SEQ ID NO: 282 - DNA, 21 bp, Artificial Sequence
  reverse primer of TBX15
acaacgctcgcaacttggttt

SEQ ID NO: 283 - DNA, 20 bp, Artificial Sequence
  forward primer of TRH
actcctgacctgccgactgc

SEQ ID NO: 284 - DNA, 20 bp, Artificial Sequence
  reverse primer of TRH
cggttacctgccaggagtgg

SEQ ID NO: 285 - DNA, 20 bp, Artificial Sequence
  forward primer of FBP1
accgccgaagagatggcttt

SEQ ID NO: 286 - DNA, 20 bp, Artificial Sequence
  reverse primer of FBP1
tcatggaggagggcaggaag

SEQ ID NO: 287 - DNA, 19 bp, Artificial Sequence
  forward primer
gtgtgatgcccggtgtcct

SEQ ID NO: 288 - DNA, 19 bp, Artificial Sequence
  reverse primer
gagccgaggtgagccactg

SEQ ID NO: 289 - DNA, 20 bp, Artificial Sequence
  forward primer of BCAN
gcgttccggatcagtccttg

SEQ ID NO: 290 - DNA, 19 bp, Artificial Sequence
  reverse primer of BCAN
agcggctctgatcggctgt

SEQ ID NO: 291 - DNA, 19 bp, Artificial Sequence
  forward primer of TP73
cgccacaccatcaccatcc

SEQ ID NO: 292 - DNA, 19 bp, Artificial Sequence
  reverse primer of TP73
tccttgatgggctgcttgc

SEQ ID NO: 293 - DNA, 23 bp, Artificial Sequence
  forward primer of MIIP
cagcctccctagtagctgggatt

SEQ ID NO: 294 - DNA, 20 bp, Artificial Sequence
  reverse primer of MIIP
cggttgctcacgccagtaaa

SEQ ID NO: 295 - DNA, 20 bp, Artificial Sequence
  forward primer of HOXC4
agaaaagcgcttggctctcc

SEQ ID NO: 296 - DNA, 18 bp, Artificial Sequence
  reverse primer of HOXC4
cactgggccgtgcctgag

SEQ ID NO: 297 - DNA, 20 bp, Artificial Sequence
  forward primer of HOXA7
cctccgccaatctcagcagt

SEQ ID NO: 298 - DNA, 20 bp, Artificial Sequence
  reverse primer of HOXA7
ttgagcctcttgcccttcca

SEQ ID NO: 299 - DNA, 20 bp, Artificial Sequence
  forward primer of BST1
gaacgggaaacggcaaacag

SEQ ID NO: 300 - DNA, 20 bp, Artificial Sequence
  reverse primer of BST1
gtcccgtgcttcctccactc

SEQ ID NO: 301 - DNA, 20 bp, Artificial Sequence
  forward primer of C1orf114
gtgcctctgcgtcctccatc

SEQ ID NO: 302 - DNA, 20 bp, Artificial Sequence
  reverse primer of C1orf114
ggggtcggtggtctgaggat

SEQ ID NO: 303 - DNA, 19 bp, Artificial Sequence
  forward primer of FOXG1
acaagcagggctggcagaa

SEQ ID NO: 304 - DNA, 18 bp, Artificial Sequence
  reverse primer of FOXG1
tgcccgggtcgtcgtagt

SEQ ID NO: 305 - DNA, 20 bp, Artificial Sequence
  forward primer of ATP4A
gcgcacctggaacttgttgg

SEQ ID NO: 306 - DNA, 19 bp, Artificial Sequence
  reverse primer of ATP4A
cggcgctgctcaagttctc

SEQ ID NO: 307 - DNA, 18 bp, Artificial Sequence
  forward primer of NOTCH1
ggaactgggctgcggtca

SEQ ID NO: 308 - DNA, 22 bp, Artificial Sequence
  reverse primer of NOTCH1
gcacactattctgccccaggag

SEQ ID NO: 309 - DNA, 19 bp, Artificial Sequence
  forward primer
acggctcggccatctacac

SEQ ID NO: 310 - DNA, 19 bp, Artificial Sequence
  reverse primer
agcgggttgagagcaggtg

SEQ ID NO: 311 - DNA, 19 bp, Artificial Sequence
  forward primer
agcgggcacagacacaagc

SEQ ID NO: 312 - DNA, 19 bp, Artificial Sequence
  reverse primer
cgaggcctccagggtgact

SEQ ID NO: 313 - DNA, 20 bp, Artificial Sequence
  forward primer of HOXA7
cctccgccaatctcagcagt

SEQ ID NO: 314 - DNA, 20 bp, Artificial Sequence
  reverse primer of HOXA7
ttgagcctcttgcccttcca

SEQ ID NO: 315 - DNA, 20 bp, Artificial Sequence
  forward primer of ZNF529
gtgctgaggaggccaaggag

SEQ ID NO: 316 - DNA, 20 bp, Artificial Sequence
  reverse primer of ZNF529
ccggctcggactcttggtta

SEQ ID NO: 317 - DNA, 18 bp, Artificial Sequence
  forward primer of PRLHR
acacgagccccctgcttg

SEQ ID NO: 318 - DNA, 19 bp, Artificial Sequence
  reverse primer of PRLHR
agcggaagctgtccgtggt

SEQ ID NO: 319 - DNA, 20 bp, Artificial Sequence
  forward primer of ARL5C
cgggacggtggaaaagacag

SEQ ID NO: 320 - DNA, 19 bp, Artificial Sequence
  reverse primer of ARL5C
ctcttggcaagccccgaag

SEQ ID NO: 321 - DNA, 900 bp, Artificial Sequence
  subsequence of SHOX2
gtaatgttaattagcttcatcttaaagaaaaaccaaacaccagagcaaataatgactcctttgcggagaaggagttgtaagggttggggagaggtaattagtgtcataaaagcctcactacaaagaagtttagaatttctctgttctgctgtgcagcagagtgaaacacagtagcagaataattgtgcaccattatcatgataatctaatttgcttctttagaaaaagccactgtttgcagttaggatagtaggaaaacatctagaaaataactaaaatgtaaataaaagtatgaaacaacaataaagttcacttcttaagagaaaaaaagaagagcactcagcgaaaggagaatgaagtatatataaagcaagtaactcttaggtactttgttctcctggatgttacctgcttaaacttgacaacttttacaggcagtatgacagattttttaaaattcaaataaagcttgcttttgtattccactttcaataataaagcatattgattgactcacaaattaaagtttttaaaaccccattaaagtaaaaatactgcttcagagctttcattggtatgtttttgaaagcaagtgtcatagtcaatgtaaatcttcaaaaatttctctgctatttagtacaacagagggtggattttgtgccagggtggcatcctttgtgtaattcacatggcctgaggcttcttgcctttttttcccctagaagagttggaattaagatactaataatcataactgtaataattatcatcatgtttttaaggggttgctgagcctctggagatctcagtgcacagagcgaagcaggagaggcttaaaaaggaaggctctgctgctgatgctgtgatgaccaaggcagcctattattacttttcctcttc